European Patent Application EP 4 803 149 A2, published September 9, 2026. Title: MULTI-SPECIFIC ANTIBODIES IN USES THEREOF IN AVIDITY RECEPTOR CROSSLINKING AND IMMUNE MODULATION. Applicant: Lyvgen Biopharma Holdings Limited. Application EP. The sequence listing filed with the application follows.

SEQUENCE LISTING (516 sequences)

SEQ ID NO: 1 - skipped

SEQ ID NO: 2 - protein, 4 aa, synthetic construct
GGGS

SEQ ID NO: 3 - protein, 5 aa, synthetic construct
GGGGS

SEQ ID NO: 4 - protein, 10 aa, synthetic construct
GGGGSGGGGS

SEQ ID NO: 5 - protein, 15 aa, synthetic construct
GGGGSGGGGSGGGGS

SEQ ID NO: 6 - protein, 20 aa, synthetic construct
GGGGSGGGGSGGGGSGGGGS

SEQ ID NO: 7 - protein, 25 aa, synthetic construct
GGGGSGGGGSGGGGSGGGGSGGGGS

SEQ ID NO: 8 - protein, 10 aa, synthetic construct
DKTHTCPPCP

SEQ ID NO: 9 - protein, 17 aa, synthetic construct
DKTHTCPPCPAPELLGP

SEQ ID NO: 10 - protein, 14 aa, synthetic construct
GGGGSDKTHTCPPC

SEQ ID NO: 11 - protein, 21 aa, synthetic construct
GGGSDKTHTCPPCPAPEAAGP

SEQ ID NO: 12 - protein, 25 aa, synthetic construct
GGGSGGGSDKTHTCPPCPAPEAAGP

SEQ ID NO: 13 - protein, 22 aa, synthetic construct
GGGGSDKTHTCPPCPAPEAAGP

SEQ ID NO: 14 - protein, 20 aa, synthetic construct
GGSDKTHTCPPCPAPEAAGP

SEQ ID NO: 15 - protein, 27 aa, synthetic construct
GGGGSGGGGSDKTHTCPPCPAPEAAGP

SEQ ID NO: 16 - protein, 32 aa, synthetic construct
GGGGSGGGGSGGGGSDKTHTCPPCPAPEAAGP

SEQ ID NO: 17 - protein, 25 aa, synthetic construct
DKTHTCPPCPGGGGSGGGGSGGGGS

SEQ ID NO: 18 - protein, 24 aa, synthetic construct
DKTHTCPPCGGGGSGGGGSGGGGS

SEQ ID NO: 19 - protein, 29 aa, synthetic construct
DKTHTCPPCGGGGSGGGGSGGGGSGGGGS

SEQ ID NO: 20 - protein, 19 aa, synthetic construct
DKTHTCPPCGGGGSGGGGS

SEQ ID NO: 21 - protein, 17 aa, synthetic construct
DKTHTCPPCPAPEAAGP

SEQ ID NO: 22 - protein, 14 aa, synthetic construct
DKTHTCPPCGGGGS

SEQ ID NO: 23 - protein, 23 aa, synthetic construct
GGGGSDKTHTCPPCPAPEAAGGP

SEQ ID NO: 24 - protein, 23 aa, synthetic construct
GGGGSDKTHTCPPCPAPELLGGP

SEQ ID NO: 25 - protein, 22 aa, synthetic construct
GGGGSDKTHTCPPCPAPELLGP

SEQ ID NO: 26 - protein, 9 aa, synthetic construct
DKTHTCPPC

SEQ ID NO: 27 - protein, 18 aa, synthetic construct
DKTHTCPPCPAPELLGGP

SEQ ID NO: 28 - protein, 8 aa, synthetic construct
PAPEAAGP

SEQ ID NO: 29 - protein, 20 aa, synthetic construct
  MOD_RES 3..20: note = may be absent
GSGSGSGSGSGSGSGSGSGS

SEQ ID NO: 30 - protein, 102 aa, synthetic construct
DVFLFPPKPKDTLMISRTPEVTCVVVDVSHEDPEVKFNWYVDGVEVHNAKTKPREEQYNSTYRVVSVLTVLHQDWLNGKEYKCKVSNKALPLPEEKTISKAK

SEQ ID NO: 31 - protein, 102 aa, synthetic construct
SVFLFPPKPKDTLMISRTPEVTCVVVAVSHEDPEVKFNWYVDGVEVHNAKTKPREEQYASTYRVVSVLTVLHQDWLNGKEYKCKVSNKALPAPIEKTISKAK

SEQ ID NO: 32 - protein, 102 aa, synthetic construct
SVFLFPPKPKDTLMISRTPEVTCVVVDVSHEDPEVKFNWYVDGVEVHNAKTKPREEQYNSTYRVVSVLTVLHQDWLNGKEYKCKVSNKALGAPIEKTISKAK

SEQ ID NO: 33 - protein, 102 aa, synthetic construct
SVFLFPPKPKDTLMISRTPEVTCVVVDVSHEDPEVKFNWYVDGVEVHNAKTKPREEQYNSTYRVVSVLTVLHQDWLNGKEYKCKVSNKALPAPIEKTISKAK

SEQ ID NO: 34 - protein, 106 aa, synthetic construct
GQPREPQVYTLPPSREEMTKNQVSLWCLVKGFYPSDIAVEWESNGQPENNYKTTPPVLDSDGSFFLYSKLTVDKSRWQQGNVFSCSVMHEALHNHYTQKSLSLSPG

SEQ ID NO: 35 - protein, 106 aa, synthetic construct
GQPREPQVYTLPPSREEMTKNQVSLSCAVKGFYPSDIAVEWESNGQPENNYKTTPPVLDSDGSFFLVSKLTVDKSRWQQGNVFSCSVMHEALHNRFTQKSLSLSPG

SEQ ID NO: 36 - protein, 106 aa, synthetic construct
GQPREPQVYTLPPSREEMTKNQVSLSCAVKGFYPSDIAVEWESNGQPENNYKTTPPVLDSDGSFFLVSKLTVDKSRWQQGNVFSCSVMHEALHNHYTQKSLSLSPG

SEQ ID NO: 37 - protein, 106 aa, synthetic construct
GQPREPQVYTLPPSREEMTKNQVSLTCLVKGFYPSDIAVEWESNGQPENNYKTTPPVLDSDGSFFLYSKLTVDKSRWQQGNVFSCSVMHEALHNHYTQKSLSLSPG

SEQ ID NO: 38 - protein, 125 aa, synthetic construct
EVQLVESGGGLVQPGGSLRLSCAASGFTFSTYAMNWVRQAPGKGLEWVGRIRSKYNNYATYYADSVKGRFTISRDDSKNSLYLQMNSLKTEDTAVYYCVRHGNFGNSYVSWFAYWGQGTLVTVSS

SEQ ID NO: 39 - protein, 109 aa, synthetic construct
QAVVTQEPSLTVSPGGTVTLTCRSSTGAVTTSNYANWVQQKPGQAPRGLIGGTNKRAPWTPARFSGSLLGGKAALTITGAQAEDEADYYCALWYSNLWVFGGGTKLTVL

SEQ ID NO: 40 - protein, 120 aa, synthetic construct
QVQLVQSGAEVKKPGASVKVSCKASGYTFTSYYIHWVRQAPGQGLEWIGCIYPGNVNTNYNEKFKDRATLTVDTSISTAYMELSRLRSDDTAVYFCTRSHYGLDWNFDVWGQGTTVTVSS

SEQ ID NO: 41 - protein, 107 aa, synthetic construct
DIQMTQSPSSLSASVGDRVTITCHASQNIYVWLNWYQQKPGKAPKLLIYKASNLHTGVPSRFSGSGSGTDFTLTISSLQPEDFATYYCQQGQTYPYTFGGGTKVEIK

SEQ ID NO: 42 - protein, 120 aa, synthetic construct
QVQLVQSGAEVVKPGASVKVSCKASGYTFTSYYIHWVRQAPGQGLEWIGSIYPGNVNTNYAQKFQGRATLTVDTSISTAYMELSRLRSDDTAVYYCTRSHYGLDWNFDVWGKGTTVTVSS

SEQ ID NO: 43 - protein, 107 aa, synthetic construct
DIQMTQSPSSLSASVGDRVTITCQASQNIYVWLNWYQQKPGKAPKLLIYKASNLHTGVPSRFSGSGSGTDFTLTISSLQPEDIATYYCQQGQTYPYTFGQGTKLEIK

SEQ ID NO: 44 - protein, 122 aa, synthetic construct
QVQLQESGPGLVKPSETLSLTCTVSGGSISSYYWSWIRQPPGKGLEWIGYIYYSGITHYNPSLKSRVTISVDTSKIQFSLKLSSVTAADTAVYYCARWGVRRDYYYYGMDVWGQGTTVTVSS

SEQ ID NO: 45 - protein, 108 aa, synthetic construct
EIVLTQSPGTLSLSPGERATLSCRASQSVSSSYLAWYQQKPGQAPRLLIYGASSRATGIPDRFSGSGSGTDFTLTISRLEPEDFAVYYCQQYGSSPWTFGQGTKVEIK

SEQ ID NO: 46 - protein, 121 aa, synthetic construct
QVQLVQSGAEVKKPGASVKVSCKASGYTFTSYVMHWVRQKPGQGLEWIGYINPYNEGTESTDKFKGRATMTSDKSTSTVYMELSSLRSEDTAVYYCASIYYGYEGTYFGVWGQGTLVTVSS

SEQ ID NO: 47 - protein, 106 aa, synthetic construct
EIVLTQSPATLSLSPGERATLSCRASSSVSYMHWYQQKPGQAPRPWIYATSNLASGIPARFSGSRSGTDYTLTISSLEPEDFAVYYCQQWSSNTLTFGGGTKVEIK

SEQ ID NO: 48 - protein, 124 aa, synthetic construct
QVQLQQSGAELVRPGSSVKISCKASGYAFSSYWMNWVKQRPGQGLEWIGQIWPGDGDTNYNGKFKGKATLTADESSSTAYMQLSSLASEDSAVYFCARRETTTVGRYYYAMDYWGQGTTVTVSS

SEQ ID NO: 49 - protein, 111 aa, synthetic construct
DIQLTQSPASLAVSLGQRATISCKASQSVDYDGDSYLNWYQQIPGQPPKLLIYDASNLVSGIPPRFSGSGSGTDFTLNIHPVEKVDAATYHCQQSTEDPWTFGGGTKLEIK

SEQ ID NO: 50 - protein, 115 aa, synthetic construct
EVQLVQSGPEVKKPGATVKISCKTSGYTFTEYTIHWVKQAPGKGLEWIGNINPNNGGTTYNQKFEDKATLTVDKSTDTAYMELSSLRSEDTAVYYCAAGWNFDYWGQGTLLTVSS

SEQ ID NO: 51 - protein, 107 aa, synthetic construct
DIQMTQSPSSLSTSVGDRVTLTCKASQDVGTAVDWYQQKPGPSPKLLIYWASTRHTGIPSRFSGSGSGTDFTLTISSLQPEDFADYYCQQYNSYPLTFGPGTKVDIK

SEQ ID NO: 52 - protein, 121 aa, synthetic construct
QVQLVESGGGLVKPGESLRLSCAASGFTFSDYYMYWVRQAPGKGLEWVAIISDGGYYTYYSDIIKGRFTISRDNAKNSLYLQMNSLKAEDTAVYYCARGFPLLRHGAMDYWGQGTLVTVSS

SEQ ID NO: 53 - protein, 107 aa, synthetic construct
DIQMTQSPSSLSASVGDRVTITCKASQNVDTNVAWYQQKPGQAPKSLIYSASYVYWDVPSRFSGSASGTDFTLTISSVQSEDFATYYCQQYDQQLITFGGGTKLEIK

SEQ ID NO: 54 - protein, 116 aa, synthetic construct
QVQLVQSGAEVKKPGASVKVSCKASGYTFAGFEMHWVRQAPGQGLEWMGAIDPKTGGTDYNQKFKDRVTMTRDTSISTAYMELSRLRSDDTAVYYCARDLGYFDVWGQGTLVTVSS

SEQ ID NO: 55 - protein, 107 aa, synthetic construct
DIQMTQSPSSLSASVGDRVTITCRASQDIRSNLNWYQQKPGGAVKLLIYYTSRLHSGVPSRFSGSGSGTDYTLTISSLQPEDFATYFCQQSEKLPRTFGGGTKVEIR

SEQ ID NO: 56 - protein, 121 aa, synthetic construct [sequence omitted]

SEQ ID NO: 57 - protein, 109 aa, synthetic construct [sequence omitted]

SEQ ID NO: 58 - protein, 121 aa, synthetic construct
QVTLKESGPALVKPTQTLTLTCTFSGFSLSTSGTCVSWIRQPPGKALEWLATICWEDSKGYNPSLKSRLTISKDTSKNQAVLTMTNMDPVDTATYYCARREDSGYFWFPYWGQGTLVTVSS

SEQ ID NO: 59 - protein, 106 aa, synthetic construct
NIQMTQSPSSLSASVGDRVTITCKAGQNVNNYLAWYQQKPGKAPKVLIFNANSLQTGVPSRFSGSGSGTDFTLTISSLQPEDFATYYCQQYNSWPTFGGGTKVEIK

SEQ ID NO: 60 - protein, 122 aa, synthetic construct
QVQLVQSGAEVKKPGASVKVSCKASGYTFTDFWMSWVRQAPGQGLEWMGQIYPNTGTTHSNEKFKGRVTMTRDTSTSTVYMELSSLRSEDTAVYYCARSYHISTTPNWFAYWGQGTLVTVSS

SEQ ID NO: 61 - protein, 106 aa, synthetic construct
DIQMTQSPSSLSASVGDRVTITCKASQNVYKKLEWYQQKPGKVPKVLIYHTNILQTGVPSRFSGSGSGTDYTLTISSLQPEDVATYYCYQWNSGPTFGGGTKVEIK

SEQ ID NO: 62 - protein, 126 aa, synthetic construct
QVQLVQSGAEVKKPGASVKVSCKASGYTFTGYYMHWVRQAPGQGLEWMGWINPDSGGTNYAQKFQGRVTMTRDTSISTAYMELNRLRSDDTAVYYCARDQPLGYCTNGVCSYFDYWGQGTLVTVSS

SEQ ID NO: 63 - protein, 107 aa, synthetic construct
DIQMTQSPSSVSASVGDRVTITCRASQGIYSWLAWYQQKPGKAPNLLIYTASTLQSGVPSRFSGSGSGTDFTLTISSLQPEDFATYYCQQANIFPLTFGGGTKVEIK

SEQ ID NO: 64 - protein, 122 aa, synthetic construct
EVQLVESGGGLVQPGGSLRLSCAASGFTFTNYGLHWVRQAPGKGLEWVSSISPSGGVTYYRDSVKGRFTISRDNSKNTLYLQMNSLRAEDTAVYYCAKPFLGWGGANWIAHWGQGTLVTVSS

SEQ ID NO: 65 - protein, 107 aa, synthetic construct
DIQMTQSPSSLSASVGDRVTITCLASEDISNDLAWYQQKPGKAPKLLIYFVDRLLDGVPSRFSGSGSGTDFTLTISSLQPEDFATYYCQQSYKYPPTFGQGTKLEIK

SEQ ID NO: 66 - protein, 121 aa, synthetic construct [sequence omitted]

SEQ ID NO: 67 - protein, 106 aa, synthetic construct [sequence omitted]

SEQ ID NO: 68 - protein, 121 aa, synthetic construct
QVQLQESGPGLVKPSETLSLTCTVSGFSLTSYNVHWIRQPPGKGLEWIGVIWSGVRTDYNSVLKPRVTISVDTSKNQFSLKLSSVTAADTAVYYCARGTYDDNYHDVMDAWGQGTLVTVSS

SEQ ID NO: 69 - protein, 106 aa, synthetic construct
EIVLTQSPATLSLSPGERATLSCRASKSVRTGMHWYQQKPGQAPRLLIYGASNLESGIPARFSGSGSGTDFTLTISSLEPEDFAVYYCQQSWNHFTFGQGTKLEIK

SEQ ID NO: 70 - protein, 119 aa, synthetic construct [sequence omitted]

SEQ ID NO: 71 - protein, 107 aa, synthetic construct [sequence omitted]

SEQ ID NO: 72 - protein, 120 aa, synthetic construct [sequence omitted]

SEQ ID NO: 73 - protein, 107 aa, synthetic construct [sequence omitted]

SEQ ID NO: 74 - protein, 121 aa, synthetic construct
EVQLVESGGGLVQPGGSLRLSCAASGFNVYASGMHWVRQAPGKGLEWVAKIYPDSDYTYYADSVKGRFTISADTSKNTAYLQMNSLRAEDTAVYYCSRDSSFYYVYAMDYWGQGTLVTVSS

SEQ ID NO: 75 - protein, 108 aa, synthetic construct
DIQMTQSPSSLSASVGDRVTITCRASQDVNTAVAWYQQKPGKAPKLLIYSAYFLYSGVPSRFSGSRSGTDFTLTISSLQPEDFATYYCQQYSRYSPVTFGQGTKVEIK

SEQ ID NO: 76 - protein, 121 aa, synthetic construct
QVQLVQSGAEVKKPGASVKVSCKASGYTFTEFGMNWVRQAPGQGLEWMGWINTKTGEATYVEEFKGRVTFTTDTSTSTAYMELRSLRSDDTAVYYCARWDFAYYVEAMDYWGQGTTVTVSS

SEQ ID NO: 77 - protein, 108 aa, synthetic construct
DIQMTQSPSSLSASVGDRVTITCKASAAVGTYVAWYQQKPGKAPKLLIYSASYRKRGVPSRFSGSGSGTDFTLTISSLQPEDFATYYCHQYYTYPLFTFGQGTKLEIK

SEQ ID NO: 78 - protein, 119 aa, synthetic construct
EVQLVESGGGVVQPGRSLRLSCSASGFDFTTYWMSWVRQAPGKGLEWIGEIHPDSSTINYAPSLKDRFTISRDNAKNTLFLQMDSLRPEDTGVYFCASLYFGFPWFAYWGQGTPVTVSS

SEQ ID NO: 79 - protein, 106 aa, synthetic construct
DIQLTQSPSSLSASVGDRVTITCKASQDVGTSVAWYQQKPGKAPKLLIYWTSTRHTGVPSRFSGSGSGTDFTFTISSLQPEDIATYYCQQYSLYRSFGQGTKVEIK

SEQ ID NO: 80 - protein, 121 aa, synthetic construct
EVQLVESGGGLVQPGGSLRLSCAASGFNIKDTYMHWVRQAPGKGLEWVARIDPANGNSKYADSVKGRFTISADTSKNTAYLQMNSLRAEDTAVYYCAPFGYYVSDYAMAYWGQGTLVTVSS

SEQ ID NO: 81 - protein, 111 aa, synthetic construct
DIQLTQSPSSLSASVGDRVTITCRAGESVDIFGVGFLHWYQQKPGKAPKLLIYRASNLESGVPSRFSGSGSRTDFTLTISSLQPEDFATYYCQQTNEDPYTFGQGTKVEIK

SEQ ID NO: 82 - protein, 121 aa, synthetic construct
QLQLQESGPGLVKPSETLSLTCTVSGGSISSGSYFWGWIRQPPGKGLEWIGSIYYSGITYYNPSLKSRVTISVDTSKNQFSLKLSSVTAADTAVYYCARHDGAVAGLFDYWGQGTLVTVSS

SEQ ID NO: 83 - protein, 108 aa, synthetic construct
SYVLTQPPSVSVAPGQTARITCGGNNIGSKSVHWYQQPPGQAPVVVVYDDSDRPSGIPERFSGSNSGNTATLTISRVEAGDEAVYYCQVWDSSSDHVVFGGGTKLTVL

SEQ ID NO: 84 - protein, 121 aa, synthetic construct
QVQLVQSGAEVKKPGASVKVSCKASGYTFTNHIIHWVRQAPGQGLEWMGYINPYPGYHAYNEKFQGRATMTSDTSTSTVYMELSSLRSEDTAVYYCARDGYYRDTDVLDYWGQGTLVTVSS

SEQ ID NO: 85 - protein, 107 aa, synthetic construct
DIQMTQSPSSLSASVGDRVTITCQASQDISNYLNWYQQKPGKAPKLLIYYTSRLHTGVPSRFSGSGSGTDFTFTISSLEPEDIATYYCQQGNTLPWTFGQGTKVEIK

SEQ ID NO: 86 - protein, 119 aa, synthetic construct
EVQLLESGGGLVQPGGSLRLSCAASGFTFSNFAMSWVRQAPGKGLEWVSTISASGGRTFYADSVKGRITISRDNSKNTLFLQMNGLRAEDTAVYYCAKEGSFGEGVDPWGQGTLVTVSS

SEQ ID NO: 87 - protein, 108 aa, synthetic construct
SYEMTQPPSVSVSPGQTARITCSGDALPKKYAYWYQQKSGQAPVLVIYEDNKRPSGIPERFSGSSSGTMATLTISGAQVEDEADYYCYSTDISGNHWVFGGGTELTVL

SEQ ID NO: 88 - protein, 119 aa, synthetic construct [sequence omitted]

SEQ ID NO: 89 - protein, 113 aa, synthetic construct [sequence omitted]

SEQ ID NO: 90 - protein, 119 aa, synthetic construct [sequence omitted]

SEQ ID NO: 91 - protein, 107 aa, synthetic construct [sequence omitted]

SEQ ID NO: 92 - protein, 119 aa, synthetic construct [sequence omitted]

SEQ ID NO: 93 - protein, 106 aa, synthetic construct [sequence omitted]

SEQ ID NO: 94 - protein, 117 aa, synthetic construct
EVQLVESGGGLVKPGGSLKLSCEASRFTFSSYAMSWVRQTPEKRLEWVAAISGGGRYTYYPDSMKGRFTISRDNAKNFLYLQMSSLRSEDTAMYYCARHYDGYLDYWGQGTTLTVSS

SEQ ID NO: 95 - protein, 108 aa, synthetic construct
DIVMTQSHKFMSTSIGARVSITCKASQDVRTAVAWYQQKPGQSPKLLIYSASYRYTGVPDRFTGSGSGTDFTFTISSVQAEDLAVYYCQQHYGTPPWTFGGGTKLEIK

SEQ ID NO: 96 - protein, 120 aa, synthetic construct [sequence omitted]

SEQ ID NO: 97 - protein, 111 aa, synthetic construct [sequence omitted]

SEQ ID NO: 98 - protein, 118 aa, synthetic construct [sequence omitted]

SEQ ID NO: 99 - protein, 107 aa, synthetic construct [sequence omitted]

SEQ ID NO: 100 - protein, 118 aa, synthetic construct
QVQLVESGGGVVQPGRSLRLSCAASGFTFSSYTMHWVRQAPGKGLEWVTFISYDGNNKYYADSVKGRFTISRDNSKNTLYLQMNSLRAEDTAIYYCARTGWLGPFDYWGQGTLVTVSS

SEQ ID NO: 101 - protein, 108 aa, synthetic construct
EIVLTQSPGTLSLSPGERATLSCRASQSVGSSYLAWYQQKPGQAPRLLIYGAFSRATGIPDRFSGSGSGTDFTLTISRLEPEDFAVYYCQQYGSSPWTFGQGTKVEIK

SEQ ID NO: 102 - protein, 125 aa, synthetic construct
QVQLVESGGGVVQPGRSLRLSCAASGFTFSSYGMHWVRQAPGKGLEWVAVIWYDGSNKYYADSVKGRFTISRDNSKNTLYLQMNSLRAEDTAVYYCARDPRGATLYYYYYGMDVWGQGTTVTVSS

SEQ ID NO: 103 - protein, 107 aa, synthetic construct
DIQMTQSPSSLSASVGDRVTITCRASQSINSYLDWYQQKPGKAPKLLIYAASSLQSGVPSRFSGSGSGTDFTLTISSLQPEDFATYYCQQYYSTPFTFGPGTKVEIK

SEQ ID NO: 104 - protein, 115 aa, synthetic construct
QVQLVESGAEVKKPGASVKVSCKASGYSFTGYTMNWVRQAPGQCLEWIGLINPYNNITNYAQKFQGRVTFTVDTSISTAYMELSRLRSDDTGVYFCARLDYRSYWGQGTLVTVSA

SEQ ID NO: 105 - protein, 109 aa, synthetic construct
QAVVTQEPSLTVSPGGTVTLTCGSSTGAVTTSNFPNWVQQKPGQAPRSLIGGTNNKASWTPARFSGSLLGGKAALTISGAQPEDEAEYYCALWYSNHWVFGCGTKLTVL

SEQ ID NO: 106 - skipped

SEQ ID NO: 107 - protein, 218 aa, synthetic construct
DIQLTQSPASLAVSLGQRATISCKASQSVDYDGDSYLNWYQQIPGQPPKLLIYDASNLVSGIPPRFSGSGSGTDFTLNIHPVEKVDAATYHCQQSTEDPWTFGGGTKLEIKRTVAAPSVFIFPPSDEQLKSGTASVVCLLNNFYPREAKVQWKVDNALQSGNSQESVTEQDSKDSTYSLSSTLTLSKADYEKHKVYACEVTHQGLSSPVTKSFNRGEC

SEQ ID NO: 108 - protein, 216 aa, synthetic construct
DIQLTQSPASLAVSLGQRATISCKASQSVDYDGDSYLNWYQQIPGQPPKLLIYDASNLVSGIPPRFSGSGSGTDFTLNIHPVEKVDAATYHCQQSTEDPWTFGGGTKLEIKSSASTKGPSVFPLAPSSKSTSGGTAALGCLVKDYFPEPVTVSWNSGALTSGVHTFPAVLQSSGLYSLSSVVTVPSSSLGTQTYICNVNHKPSNTKVDKKVEPKSC

SEQ ID NO: 109 - protein, 213 aa, synthetic construct
DIQLTQSPSSLSASVGDRVTITCKASQDVGTSVAWYQQKPGKAPKLLIYWTSTRHTGVPSRFSGSGSGTDFTFTISSLQPEDIATYYCQQYSLYRSFGQGTKVEIKRTVAAPSVFIFPPSDEQLKSGTASVVCLLNNFYPREAKVQWKVDNALQSGNSQESVTEQDSKDSTYSLSSTLTLSKADYEKHKVYACEVTHQGLSSPVTKSFNRGEC

SEQ ID NO: 110 - protein, 218 aa, synthetic construct
DIQLTQSPSSLSASVGDRVTITCRAGESVDIFGVGFLHWYQQKPGKAPKLLIYRASNLESGVPSRFSGSGSRTDFTLTISSLQPEDFATYYCQQTNEDPYTFGQGTKVEIKRTVAAPSVFIFPPSDEQLKSGTASVVCLLNNFYPREAKVQWKVDNALQSGNSQESVTEQDSKDSTYSLSSTLTLSKADYEKHKVYACEVTHQGLSSPVTKSFNRGEC

SEQ ID NO: 111 - protein, 215 aa, synthetic construct
DIQMTQSPSSLSASVGDRVTITCKASAAVGTYVAWYQQKPGKAPKLLIYSASYRKRGVPSRFSGSGSGTDFTLTISSLQPEDFATYYCHQYYTYPLFTFGQGTKLEIKRTVAAPSVFIFPPSDEQLKSGTASVVCLLNNFYPREAKVQWKVDNALQSGNSQESVTEQDSKDSTYSLSSTLTLSKADYEKHKVYACEVTHQGLSSPVTKSFNRGEC

SEQ ID NO: 112 - protein, 214 aa, synthetic construct
DIQMTQSPSSLSASVGDRVTITCKASQDVSIGVAWYQQKPGKAPKLLIYSASYRYTGVPSRFSGSGSGTDFTLTISSLQPEDFATYYCQQYYIYPYTFGQGTKVEIKRTVAAPSVFIFPPSDEQLKSGTASVVCLLNNFYPREAKVQWKVDNALQSGNSQESVTEQDSKDSTYSLSSTLTLSKADYEKHKVYACEVTHQGLSSPVTKSFNRGEC

SEQ ID NO: 113 - protein, 212 aa, synthetic construct
DIQMTQSPSSLSASVGDRVTITCKASQDVSIGVAWYQQKPGKAPKLLIYSASYRYTGVPSRFSGSGSGTDFTLTISSLQPEDFATYYCQQYYIYPYTFGQGTKVEIKSSASTKGPSVFPLAPSSKSTSGGTAALGCLVKDYFPEPVTVSWNSGALTSGVHTFPAVLQSSGLYSLSSVVTVPSSSLGTQTYICNVNHKPSNTKVDKKVEPKSC

SEQ ID NO: 114 - protein, 214 aa, synthetic construct
DIQMTQSPSSLSASVGDRVTITCKASQNVDTNVAWYQQKPGQAPKSLIYSASYVYWDVPSRFSGSASGTDFTLTISSVQSEDFATYYCQQYDQQLITFGGGTKLEIKRTVAAPSVFIFPPSDEQLKSGTASVVCLLNNFYPREAKVQWKVDNALQSGNSQESVTEQDSKDSTYSLSSTLTLSKADYEKHKVYACEVTHQGLSSPVTKSFNRGEC

SEQ ID NO: 115 - protein, 213 aa, synthetic construct
DIQMTQSPSSLSASVGDRVTITCKASQNVYKKLEWYQQKPGKVPKVLIYHTNILQTGVPSRFSGSGSGTDYTLTISSLQPEDVATYYCYQWNSGPTFGGGTKVEIKRTVAAPSVFIFPPSDEQLKSGTASVVCLLNNFYPREAKVQWKVDNALQSGNSQESVTEQDSKDSTYSLSSTLTLSKADYEKHKVYACEVTHQGLSSPVTKSFNRGEC

SEQ ID NO: 116 - protein, 218 aa, synthetic construct
DIQMTQSPSSLSASVGDRVTITCKSSQSLLYTSSQKNYLAWYQQKPGKAPKLLIYWASTRESGVPSRFSGSGSGTDFTLTISSLQPEDFATYYCQQYYAYPWTFGQGTKVEIKSSASTKGPSVFPLAPSSKSTSGGTAALGCLVKDYFPEPVTVSWNSGALTSGVHTFPAVLQSSGLYSLSSVVTVPSSSLGTQTYICNVNHKPSNTKVDKKVEPKSC

SEQ ID NO: 117 - protein, 214 aa, synthetic construct
DIQMTQSPSSLSASVGDRVTITCQASQDISNYLNWYQQKPGKAPKLLIYDASNLETGVPSRFSGSGSGTDFTFTISSLQPEDIATYFCQHFDHLPLAFGGGTKVEIKRTVAAPSVFIFPPSDEQLKSGTASVVCLLNNFYPREAKVQWKVDNALQSGNSQESVTEQDSKDSTYSLSSTLTLSKADYEKHKVYACEVTHQGLSSPVTKSFNRGEC

SEQ ID NO: 118 - protein, 214 aa, synthetic construct
DIQMTQSPSSLSASVGDRVTITCQASQDISNYLNWYQQKPGKAPKLLIYYTSRLHTGVPSRFSGSGSGTDFTFTISSLEPEDIATYYCQQGNTLPWTFGQGTKVEIKRTVAAPSVFIFPPSDEQLKSGTASVVCLLNNFYPREAKVQWKVDNALQSGNSQESVTEQDSKDSTYSLSSTLTLSKADYEKHKVYACEVTHQGLSSPVTKSFNRGEC

SEQ ID NO: 119 - protein, 608 aa, synthetic construct
DIQMTQSPSSLSASVGDRVTITCRASQDVNTAVAWYQQKPGKAPKLLIYSASFLYSGVPSRFSGSRSGTDFTLTISSLQPEDFATYYCQQHYTTPPTFGQGTKVEIKGGGGSGGGGSGGGGSGGGGSEVQLVESGGGLVQPGGSLRLSCAASGFNIKDTYIHWVRQAPGKGLEWVARIYPTNGYTRYADSVKGRFTISADTSKNTAYLQMNSLRAEDTAVYYCSRWGGDGFYAMDYWGQGTLVTVSSDKTHTCPPCPAPEAAGPSVFLFPPKPKDTLMISRTPEVTCVVVDVSHEDPEVKFNWYVDGVEVHNAKTKPREEQYNSTYRVVSVLTVLHQDWLNGKEYKCKVSNKALPAPIEKTISKAKGQPREPQVYTLPPSREEMTKNQVSLWCLVKGFYPSDIAVEWESNGQPENNYKTTPPVLDSDGSFFLYSKLTVDKSRWQQGNVFSCSVMHEALHNHYTQKSLSLSPGGGGGSGGGGSGGGGSGGGGSQVQLVQSGAEVKKPGASVKVSCKASGYTFAGFEMHWVRQAPGQGLEWMGAIDPKTGGTDYNQKFKDRVTMTRDTSISTAYMELSRLRSDDTAVYYCARDLGYFDVWGQGTLVTVSS

SEQ ID NO: 120 - protein, 758 aa, synthetic construct
DIQMTQSPSSLSASVGDRVTITCRASQDVNTAVAWYQQKPGKAPKLLIYSASFLYSGVPSRFSGSRSGTDFTLTISSLQPEDFATYYCQQHYTTPPTFGQGTKVEIKGGGGSGGGGSGGGGSGGGGSEVQLVESGGGLVQPGGSLRLSCAASGFNIKDTYIHWVRQAPGKGLEWVARIYPTNGYTRYADSVKGRFTISADTSKNTAYLQMNSLRAEDTAVYYCSRWGGDGFYAMDYWGQGTLVTVSSGGGGSGGGGSGGGGSGGGGSEVQLVESGGGLVQPGGSLRLSCAASGFTFSTYAMNWVRQAPGKGLEWVGRIRSKYNNYATYYADSVKGRFTISRDDSKNSLYLQMNSLKTEDTAVYYCVRHGNFGNSYVSWFAYWGQGTLVTVSSGGGGSDKTHTCPPCPAPEAAGPSVFLFPPKPKDTLMISRTPEVTCVVVDVSHEDPEVKFNWYVDGVEVHNAKTKPREEQYNSTYRVVSVLTVLHQDWLNGKEYKCKVSNKALPAPIEKTISKAKGQPREPQVYTLPPSREEMTKNQVSLWCLVKGFYPSDIAVEWESNGQPENNYKTTPPVLDSDGSFFLYSKLTVDKSRWQQGNVFSCSVMHEALHNHYTQKSLSLSPGGGGGSGGGGSGGGGSGGGGSQVQLVQSGAEVKKPGASVKVSCKASGYTFAGFEMHWVRQAPGQGLEWMGAIDPKTGGTDYNQKFKDRVTMTRDTSISTAYMELSRLRSDDTAVYYCARDLGYFDVWGQGTLVTVSS

SEQ ID NO: 121 - protein, 622 aa, synthetic construct
DIQMTQSPSSLSASVGDRVTITCRASQDVNTAVAWYQQKPGKAPKLLIYSASFLYSGVPSRFSGSRSGTDFTLTISSLQPEDFATYYCQQHYTTPPTFGQGTKVEIKGGGGSGGGGSGGGGSGGGGSEVQLVESGGGLVQPGGSLRLSCAASGFNIKDTYIHWVRQAPGKGLEWVARIYPTNGYTRYADSVKGRFTISADTSKNTAYLQMNSLRAEDTAVYYCSRWGGDGFYAMDYWGQGTLVTVSSGGGGSGGGGSGGGGSGGGGSEVQLVESGGGLVQPGGSLRLSCAASGFTFSTYAMNWVRQAPGKGLEWVGRIRSKYNNYATYYADSVKGRFTISRDDSKNSLYLQMNSLKTEDTAVYYCVRHGNFGNSYVSWFAYWGQGTLVTVSSGGGGSDKTHTCPPCPAPEAAGPSVFLFPPKPKDTLMISRTPEVTCVVVDVSHEDPEVKFNWYVDGVEVHNAKTKPREEQYNSTYRVVSVLTVLHQDWLNGKEYKCKVSNKALPAPIEKTISKAKGQPREPQVYTLPPSREEMTKNQVSLWCLVKGFYPSDIAVEWESNGQPENNYKTTPPVLDSDGSFFLYSKLTVDKSRWQQGNVFSCSVMHEALHNHYTQKSLSLSPG

SEQ ID NO: 122 - protein, 214 aa, synthetic construct
DIQMTQSPSSLSASVGDRVTITCRASQDVNTAVAWYQQKPGKAPKLLIYSASFLYSGVPSRFSGSRSGTDFTLTISSLQPEDFATYYCQQHYTTPPTFGQGTKVEIKRTVAAPSVFIFPPSDEQLKSGTASVVCLLNNFYPREAKVQWKVDNALQSGNSQESVTEQDSKDSTYSLSSTLTLSKADYEKHKVYACEVTHQGLSSPVTKSFNRGEC

SEQ ID NO: 123 - protein, 212 aa, synthetic construct
DIQMTQSPSSLSASVGDRVTITCRASQDVNTAVAWYQQKPGKAPKLLIYSASFLYSGVPSRFSGSRSGTDFTLTISSLQPEDFATYYCQQHYTTPPTFGQGTKVEIKSSASTKGPSVFPLAPSSKSTSGGTAALGCLVKDYFPEPVTVSWNSGALTSGVHTFPAVLQSSGLYSLSSVVTVPSSSLGTQTYICNVNHKPSNTKVDKKVEPKSC

SEQ ID NO: 124 - protein, 215 aa, synthetic construct
DIQMTQSPSSLSASVGDRVTITCRASQDVNTAVAWYQQKPGKAPKLLIYSAYFLYSGVPSRFSGSRSGTDFTLTISSLQPEDFATYYCQQYSRYSPVTFGQGTKVEIKRTVAAPSVFIFPPSDEQLKSGTASVVCLLNNFYPREAKVQWKVDNALQSGNSQESVTEQDSKDSTYSLSSTLTLSKADYEKHKVYACEVTHQGLSSPVTKSFNRGEC

SEQ ID NO: 125 - protein, 214 aa, synthetic construct
DIQMTQSPSSLSASVGDRVTITCRASQDVSTAVAWYQQKPGKAPKLLIYSASFLYSGVPSRFSGSGSGTDFTLTISSLQPEDFATYYCQQYLYHPATFGQGTKVEIKRTVAAPSVFIFPPSDEQLKSGTASVVCLLNNFYPREAKVQWKVDNALQSGNSQESVTEQDSKDSTYSLSSTLTLSKADYEKHKVYACEVTHQGLSSPVTKSFNRGEC

SEQ ID NO: 126 - protein, 213 aa, synthetic construct
DIQMTQSPSSLSASVGDRVTITCRASSSVSYMHWYQQKPGKAPKPLIYAPSNLASGVPSRFSGSGSGTDFTLTISSLQPEDFATYYCQQWSFNPPTFGQGTKVEIKRTVAAPSVFIFPPSDEQLKSGTASVVCLLNNFYPREAKVQWKVDNALQSGNSQESVTEQDSKDSTYSLSSTLTLSKADYEKHKVYACEVTHQGLSSPVTKSFNRGEC

SEQ ID NO: 127 - protein, 214 aa, synthetic construct
DIQMTQSPSSLSTSVGDRVTLTCKASQDVGTAVDWYQQKPGPSPKLLIYWASTRHTGIPSRFSGSGSGTDFTLTISSLQPEDFADYYCQQYNSYPLTFGPGTKVDIKRTVAAPSVFIFPPSDEQLKSGTASVVCLLNNFYPREAKVQWKVDNALQSGNSQESVTEQDSKDSTYSLSSTLTLSKADYEKHKVYACEVTHQGLSSPVTKSFNRGEC

SEQ ID NO: 128 - protein, 215 aa, synthetic construct
DIVMTQSHKFMSTSIGARVSITCKASQDVRTAVAWYQQKPGQSPKLLIYSASYRYTGVPDRFTGSGSGTDFTFTISSVQAEDLAVYYCQQHYGTPPWTFGGGTKLEIKRTVAAPSVFIFPPSDEQLKSGTASVVCLLNNFYPREAKVQWKVDNALQSGNSQESVTEQDSKDSTYSLSSTLTLSKADYEKHKVYACEVTHQGLSSPVTKSFNRGEC

SEQ ID NO: 129 - protein, 219 aa, synthetic construct
DIVMTQSPDSLAVSLGERATINCKSSQSLLNSRTRKNYLAWYQQKPGQPPKLLIYWASTRESGVPDRFSGSGSGTDFTLTISSLQAEDVAVYYCTQSFILRTFGQGTKVEIKRTVAAPSVFIFPPSDEQLKSGTASVVCLLNNFYPREAKVQWKVDNALQSGNSQESVTEQDSKDSTYSLSSTLTLSKADYEKHKVYACEVTHQGLSSPVTKSFNRGEC

SEQ ID NO: 130 - protein, 219 aa, synthetic construct
DIVMTQTPLSLPVTPGEPASISCRSSKSLLHSNGITYLYWYLQKPGQSPQLLIYQMSNLVSGVPDRFSGSGSGTDFTLKISRVEAEDVGVYYCAQNLELPYTFGGGTKVEIKRTVAAPSVFIFPPSDRKLKSGTASVVCLLNNFYPREAKVQWKVDNALQSGNSQESVTEQDSKDSTYSLSSTLTLSKADYEKHKVYACEVTHQGLSSPVTKSFNRGEC

SEQ ID NO: 131 - protein, 213 aa, synthetic construct
EIVLTQSPATLSLSPGERATLSCRASSSVSYMHWYQQKPGQAPRPWIYATSNLASGIPARFSGSRSGTDYTLTISSLEPEDFAVYYCQQWSSNTLTFGGGTKVEIKRTVAAPSVFIFPPSDEQLKSGTASVVCLLNNFYPREAKVQWKVDNALQSGNSQESVTEQDSKDSTYSLSSTLTLSKADYEKHKVYACEVTHQGLSSPVTKSFNRGEC

SEQ ID NO: 132 - protein, 232 aa, synthetic construct
EVQLLESGGGLVQPGGSLRLSCAASGFTFSTYAMNWVRQAPGKGLEWVSRIRSKYNNYATYYADSVKGRFTISRDDSKNTLYLQMNSLRAEDTAVYYCVRHGNFGNSYVSWFAYWGQGTLVTVSSASVAAPSVFIFPPSDEQLKSGTASVVCLLNNFYPREAKVQWKVDNALQSGNSQESVTEQDSKDSTYSLSSTLTLSKADYEKHKVYACEVTHQGLSSPVTKSFNRGEC

SEQ ID NO: 133 - protein, 732 aa, synthetic construct
EVQLVESGGGLVKPGGSLKLSCEASRFTFSSYAMSWVRQTPEKRLEWVAAISGGGRYTYYPDSMKGRFTISRDNAKNFLYLQMSSLRSEDTAMYYCARHYDGYLDYWGQGTTLTVSSASTKGPSVFPLAPSSKSTSGGTAALGCLVKDYFPEPVTVSWNSGALTSGVHTFPAVLQSSGLYSLSSVVTVPSSSLGTQTYICNVNHKPSNTKVDKKVEPKSCGGGGSGGGGSGGGGSGGGGSEVQLVESGGGLVQPGGSLRLSCAASGFTFSTYAMNWVRQAPGKGLEWVGRIRSKYNNYATYYADSVKGRFTISRDDSKNSLYLQMNSLKTEDTAVYYCVRHGNFGNSYVSWFAYWGQGTLVTVSSGGGGSDKTHTCPPCPAPELLGPSVFLFPPKPKDTLMISRTPEVTCVVVDVSHEDPEVKFNWYVDGVEVHNAKTKPREEQYNSTYRVVSVLTVLHQDWLNGKEYKCKVSNKALGAPIEKTISKAKGQPREPQVYTLPPSREEMTKNQVSLWCLVKGFYPSDIAVEWESNGQPENNYKTTPPVLDSDGSFFLYSKLTVDKSRWQQGNVFSCSVMHEALHNHYTQKSLSLSPGKGGGGSGGGGSGGGGSGGGGSQVQLVQSGAEVKKPGASVKVSCKASGYTFAGFEMHWVRQAPGQGLEWMGAIDPKTGGTDYNQKFKDRVTMTRDTSISTAYMELSRLRSDDTAVYYCARDLGYFDVWGQGTLVTVSS

SEQ ID NO: 134 - protein, 707 aa, synthetic construct
EVQLVESGGGLVKPGGSLKLSCEASRFTFSSYAMSWVRQTPEKRLEWVAAISGGGRYTYYPDSMKGRFTISRDNAKNFLYLQMSSLRSEDTAMYYCARHYDGYLDYWGQGTTLTVSSASTKGPSVFPLAPSSKSTSGGTAALGCLVKDYFPEPVTVSWNSGALTSGVHTFPAVLQSSGLYSLSSVVTVPSSSLGTQTYICNVNHKPSNTKVDKKVEPKSCGGGGSGGGGSGGGGSGGGGSQAVVTQEPSLTVSPGGTVTLTCRSSTGAVTTSNYANWVQQKPGQAPRGLIGGTNKRAPWTPARFSGSLLGGKAALTITGAQAEDEADYYCALWYSNLWVFGGGTKLTVLGGGGSDKTHTCPPCPAPELLGPSVFLFPPKPKDTLMISRTPEVTCVVVDVSHEDPEVKFNWYVDGVEVHNAKTKPREEQYNSTYRVVSVLTVLHQDWLNGKEYKCKVSNKALGAPIEKTISKAKGQPREPQVYTLPPSREEMTKNQVSLSCAVKGFYPSDIAVEWESNGQPENNYKTTPPVLDSDGSFFLVSKLTVDKSRWQQGNVFSCSVMHEALHNHYTQKSLSLSPGKGGGGSGGGGSGGGGSGGGGSDIQMTQSPSSLSASVGDRVTITCRASQDIRSNLNWYQQKPGGAVKLLIYYTSRLHSGVPSRFSGSGSGTDYTLTISSLQPEDFATYFCQQSEKLPRTFGGGTKVEIR

SEQ ID NO: 135 - protein, 584 aa, synthetic construct
EVQLVESGGGLVQPGGSLRLSCAASGFNIKDTYIHWVRQAPGKGLEWVARIYPTNGYTRYADSVKGRFTISADTSKNTAYLQMNSLRAEDTAVYYCSRWGGDGFYAMDYWGQGTLVTVSSASTKGPSVFPLAPSSKSTSGGTAALGCLVKDYFPEPVTVSWNSGALTSGVHTFPAVLQSSGLYSLSSVVTVPSSSLGTQTYICNVNHKPSNTKVDKKVEPKSCDKTHTCPPCPAPEAAGPSVFLFPPKPKDTLMISRTPEVTCVVVDVSHEDPEVKFNWYVDGVEVHNAKTKPREEQYNSTYRVVSVLTVLHQDWLNGKEYKCKVSNKALPAPIEKTISKAKGQPREPQVYTLPPSREEMTKNQVSLWCLVKGFYPSDIAVEWESNGQPENNYKTTPPVLDSDGSFFLYSKLTVDKSRWQQGNVFSCSVMHEALHNHYTQKSLSLSPGGGGGSGGGGSGGGGSGGGGSQVQLVQSGAEVKKPGASVKVSCKASGYTFAGFEMHWVRQAPGQGLEWMGAIDPKTGGTDYNQKFKDRVTMTRDTSISTAYMELSRLRSDDTAVYYCARDLGYFDVWGQGTLVTVSS

SEQ ID NO: 136 - protein, 575 aa, synthetic construct
EVQLVESGGGLVQPGGSLRLSCAASGFNIKDTYIHWVRQAPGKGLEWVARIYPTNGYTRYADSVKGRFTISADTSKNTAYLQMNSLRAEDTAVYYCSRWGGDGFYAMDYWGQGTLVTVSSASTKGPSVFPLAPSSKSTSGGTAALGCLVKDYFPEPVTVSWNSGALTSGVHTFPAVLQSSGLYSLSSVVTVPSSSLGTQTYICNVNHKPSNTKVDKKVEPKSCDKTHTCPPCPAPEAAGPSVFLFPPKPKDTLMISRTPEVTCVVVDVSHEDPEVKFNWYVDGVEVHNAKTKPREEQYNSTYRVVSVLTVLHQDWLNGKEYKCKVSNKALPAPIEKTISKAKGQPREPQVYTLPPSREEMTKNQVSLSCAVKGFYPSDIAVEWESNGQPENNYKTTPPVLDSDGSFFLVSKLTVDKSRWQQGNVFSCSVMHEALHNRFTQKSLSLSPGGGGGSGGGGSGGGGSGGGGSDIQMTQSPSSLSASVGDRVTITCRASQDIRSNLNWYQQKPGGAVKLLIYYTSRLHSGVPSRFSGSGSGTDYTLTISSLQPEDFATYFCQQSEKLPRTFGGGTKVEIR

SEQ ID NO: 137 - protein, 734 aa, synthetic construct
EVQLVESGGGLVQPGGSLRLSCAASGFNIKDTYIHWVRQAPGKGLEWVARIYPTNGYTRYADSVKGRFTISADTSKNTAYLQMNSLRAEDTAVYYCSRWGGDGFYAMDYWGQGTLVTVSSASTKGPSVFPLAPSSKSTSGGTAALGCLVKDYFPEPVTVSWNSGALTSGVHTFPAVLQSSGLYSLSSVVTVPSSSLGTQTYICNVNHKPSNTKVDKKVEPKSCGGGGSGGGGSGGGGSGGGGSEVQLVESGGGLVQPGGSLRLSCAASGFTFSTYAMNWVRQAPGKGLEWVGRIRSKYNNYATYYADSVKGRFTISRDDSKNSLYLQMNSLKTEDTAVYYCVRHGNFGNSYVSWFAYWGQGTLVTVSSGGGGSDKTHTCPPCPAPEAAGPSVFLFPPKPKDTLMISRTPEVTCVVVDVSHEDPEVKFNWYVDGVEVHNAKTKPREEQYNSTYRVVSVLTVLHQDWLNGKEYKCKVSNKALPAPIEKTISKAKGQPREPQVYTLPPSREEMTKNQVSLWCLVKGFYPSDIAVEWESNGQPENNYKTTPPVLDSDGSFFLYSKLTVDKSRWQQGNVFSCSVMHEALHNHYTQKSLSLSPGGGGGSGGGGSGGGGSGGGGSQVQLVQSGAEVKKPGASVKVSCKASGYTFAGFEMHWVRQAPGQGLEWMGAIDPKTGGTDYNQKFKDRVTMTRDTSISTAYMELSRLRSDDTAVYYCARDLGYFDVWGQGTLVTVSS

SEQ ID NO: 138 - protein, 598 aa, synthetic construct
EVQLVESGGGLVQPGGSLRLSCAASGFNIKDTYIHWVRQAPGKGLEWVARIYPTNGYTRYADSVKGRFTISADTSKNTAYLQMNSLRAEDTAVYYCSRWGGDGFYAMDYWGQGTLVTVSSASTKGPSVFPLAPSSKSTSGGTAALGCLVKDYFPEPVTVSWNSGALTSGVHTFPAVLQSSGLYSLSSVVTVPSSSLGTQTYICNVNHKPSNTKVDKKVEPKSCGGGGSGGGGSGGGGSGGGGSEVQLVESGGGLVQPGGSLRLSCAASGFTFSTYAMNWVRQAPGKGLEWVGRIRSKYNNYATYYADSVKGRFTISRDDSKNSLYLQMNSLKTEDTAVYYCVRHGNFGNSYVSWFAYWGQGTLVTVSSGGGGSDKTHTCPPCPAPEAAGPSVFLFPPKPKDTLMISRTPEVTCVVVDVSHEDPEVKFNWYVDGVEVHNAKTKPREEQYNSTYRVVSVLTVLHQDWLNGKEYKCKVSNKALPAPIEKTISKAKGQPREPQVYTLPPSREEMTKNQVSLWCLVKGFYPSDIAVEWESNGQPENNYKTTPPVLDSDGSFFLYSKLTVDKSRWQQGNVFSCSVMHEALHNHYTQKSLSLSPG

SEQ ID NO: 139 - protein, 709 aa, synthetic construct
EVQLVESGGGLVQPGGSLRLSCAASGFNIKDTYIHWVRQAPGKGLEWVARIYPTNGYTRYADSVKGRFTISADTSKNTAYLQMNSLRAEDTAVYYCSRWGGDGFYAMDYWGQGTLVTVSSASTKGPSVFPLAPSSKSTSGGTAALGCLVKDYFPEPVTVSWNSGALTSGVHTFPAVLQSSGLYSLSSVVTVPSSSLGTQTYICNVNHKPSNTKVDKKVEPKSCGGGGSGGGGSGGGGSGGGGSQAVVTQEPSLTVSPGGTVTLTCRSSTGAVTTSNYANWVQQKPGQAPRGLIGGTNKRAPWTPARFSGSLLGGKAALTITGAQAEDEADYYCALWYSNLWVFGGGTKLTVLGGGGSDKTHTCPPCPAPEAAGPSVFLFPPKPKDTLMISRTPEVTCVVVDVSHEDPEVKFNWYVDGVEVHNAKTKPREEQYNSTYRVVSVLTVLHQDWLNGKEYKCKVSNKALPAPIEKTISKAKGQPREPQVYTLPPSREEMTKNQVSLSCAVKGFYPSDIAVEWESNGQPENNYKTTPPVLDSDGSFFLVSKLTVDKSRWQQGNVFSCSVMHEALHNRFTQKSLSLSPGGGGGSGGGGSGGGGSGGGGSDIQMTQSPSSLSASVGDRVTITCRASQDIRSNLNWYQQKPGGAVKLLIYYTSRLHSGVPSRFSGSGSGTDYTLTISSLQPEDFATYFCQQSEKLPRTFGGGTKVEIR

SEQ ID NO: 140 - protein, 582 aa, synthetic construct
EVQLVESGGGLVQPGGSLRLSCAASGFNIKDTYIHWVRQAPGKGLEWVARIYPTNGYTRYADSVKGRFTISADTSKNTAYLQMNSLRAEDTAVYYCSRWGGDGFYAMDYWGQGTLVTVSSASTKGPSVFPLAPSSKSTSGGTAALGCLVKDYFPEPVTVSWNSGALTSGVHTFPAVLQSSGLYSLSSVVTVPSSSLGTQTYICNVNHKPSNTKVDKKVEPKSCGGGGSGGGGSGGGGSGGGGSQAVVTQEPSLTVSPGGTVTLTCRSSTGAVTTSNYANWVQQKPGQAPRGLIGGTNKRAPWTPARFSGSLLGGKAALTITGAQAEDEADYYCALWYSNLWVFGGGTKLTVLGGGGSDKTHTCPPCPAPEAAGPSVFLFPPKPKDTLMISRTPEVTCVVVDVSHEDPEVKFNWYVDGVEVHNAKTKPREEQYNSTYRVVSVLTVLHQDWLNGKEYKCKVSNKALPAPIEKTISKAKGQPREPQVYTLPPSREEMTKNQVSLSCAVKGFYPSDIAVEWESNGQPENNYKTTPPVLDSDGSFFLVSKLTVDKSRWQQGNVFSCSVMHEALHNRFTQKSLSLSPG

SEQ ID NO: 141 - protein, 710 aa, synthetic construct
EVQLVESGGGLVQPGGSLRLSCAASGFNIKDTYIHWVRQAPGKGLEWVARIYPTNGYTRYADSVKGRFTISADTSKNTAYLQMNSLRAEDTAVYYCSRWGGDGFYAMDYWGQGTLVTVSSASTKGPSVFPLAPSSKSTSGGTAALGCLVKDYFPEPVTVSWNSGALTSGVHTFPAVLQSSGLYSLSSVVTVPSSSLGTQTYICNVNHKPSNTKVDKKVEPKSCGGGGSGGGGSGGGGSGGGGSQAVVTQEPSLTVSPGGTVTLTCRSSTGAVTTSNYANWVQQKPGQAPRGLIGGTNKRAPWTPARFSGSLLGGKAALTITGAQAEDEADYYCALWYSNLWVFGGGTKLTVLGGGGSDKTHTCPPCPAPELLGPSVFLFPPKPKDTLMISRTPEVTCVVVDVSHEDPEVKFNWYVDGVEVHNAKTKPREEQYNSTYRVVSVLTVLHQDWLNGKEYKCKVSNKALGAPIEKTISKAKGQPREPQVYTLPPSREEMTKNQVSLSCAVKGFYPSDIAVEWESNGQPENNYKTTPPVLDSDGSFFLVSKLTVDKSRWQQGNVFSCSVMHEALHNRFTQKSLSLSPGKGGGGSGGGGSGGGGSGGGGSDIQMTQSPSSLSASVGDRVTITCHASQNIYVWLNWYQQKPGKAPKLLIYKASNLHTGVPSRFSGSGSGTDFTLTISSLQPEDFATYYCQQGQTYPYTFGGGTKVEIK

SEQ ID NO: 142 - protein, 583 aa, synthetic construct
EVQLVESGGGLVQPGGSLRLSCAASGFNIKDTYIHWVRQAPGKGLEWVARIYPTNGYTRYADSVKGRFTISADTSKNTAYLQMNSLRAEDTAVYYCSRWGGDGFYAMDYWGQGTLVTVSSASTKGPSVFPLAPSSKSTSGGTAALGCLVKDYFPEPVTVSWNSGALTSGVHTFPAVLQSSGLYSLSSVVTVPSSSLGTQTYICNVNHKPSNTKVDKKVEPKSCGGGGSGGGGSGGGGSGGGGSQAVVTQEPSLTVSPGGTVTLTCRSSTGAVTTSNYANWVQQKPGQAPRGLIGGTNKRAPWTPARFSGSLLGGKAALTITGAQAEDEADYYCALWYSNLWVFGGGTKLTVLGGGGSDKTHTCPPCPAPELLGPSVFLFPPKPKDTLMISRTPEVTCVVVDVSHEDPEVKFNWYVDGVEVHNAKTKPREEQYNSTYRVVSVLTVLHQDWLNGKEYKCKVSNKALGAPIEKTISKAKGQPREPQVYTLPPSREEMTKNQVSLSCAVKGFYPSDIAVEWESNGQPENNYKTTPPVLDSDGSFFLVSKLTVDKSRWQQGNVFSCSVMHEALHNRFTQKSLSLSPGK

SEQ ID NO: 143 - protein, 743 aa, synthetic construct
EVQLVESGGGLVQPGGSLRLSCAASGFNIKDTYIHWVRQAPGKGLEWVARIYPTNGYTRYADSVKGRFTISADTSKNTAYLQMNSLRAEDTAVYYCSRWGGDGFYAMDYWGQGTLVTVSSASVAAPSVFIFPPSDEQLKSGTASVVCLLNNFYPREAKVQWKVDNALQSGNSQESVTEQDSKDSTYSLSSTLTLSKADYEKHKVYACEVTHQGLSSPVTKSFNRGECGGGGSGGGGSGGGGSGGGGSEVQLVESGGGLVQPGGSLRLSCAASGFTFSTYAMNWVRQAPGKGLEWVGRIRSKYNNYATYYADSVKGRFTISRDDSKNSLYLQMNSLKTEDTAVYYCVRHGNFGNSYVSWFAYWGQGTLVTVSSGGGGSDKTHTCPPCPAPELLGPSVFLFPPKPKDTLMISRTPEVTCVVVDVSHEDPEVKFNWYVDGVEVHNAKTKPREEQYNSTYRVVSVLTVLHQDWLNGKEYKCKVSNKALGAPIEKTISKAKGQPREPQVYTLPPSREEMTKNQVSLWCLVKGFYPSDIAVEWESNGQPENNYKTTPPVLDSDGSFFLYSKLTVDKSRWQQGNVFSCSVMHEALHNHYTQKSLSLSPGKGGGGSGGGGSGGGGSGGGGSQVQLVQSGAEVKKPGASVKVSCKASGYTFTSYYIHWVRQAPGQGLEWIGCIYPGNVNTNYNEKFKDRATLTVDTSISTAYMELSRLRSDDTAVYFCTRSHYGLDWNFDVWGQGTTVTVSS

SEQ ID NO: 144 - protein, 585 aa, synthetic construct
EVQLVESGGGLVQPGGSLRLSCAASGFNIKDTYMHWVRQAPGKGLEWVARIDPANGNSKYADSVKGRFTISADTSKNTAYLQMNSLRAEDTAVYYCAPFGYYVSDYAMAYWGQGTLVTVSSASTKGPSVFPLAPSSKSTSGGTAALGCLVKDYFPEPVTVSWNSGALTSGVHTFPAVLQSSGLYSLSSVVTVPSSSLGTQTYICNVNHKPSNTKVDKKVEPKSCDKTHTCPPCPAPEAAGPSVFLFPPKPKDTLMISRTPEVTCVVVDVSHEDPEVKFNWYVDGVEVHNAKTKPREEQYNSTYRVVSVLTVLHQDWLNGKEYKCKVSNKALPAPIEKTISKAKGQPREPQVYTLPPSREEMTKNQVSLWCLVKGFYPSDIAVEWESNGQPENNYKTTPPVLDSDGSFFLYSKLTVDKSRWQQGNVFSCSVMHEALHNHYTQKSLSLSPGGGGGSGGGGSGGGGSGGGGSQVQLVQSGAEVKKPGASVKVSCKASGYTFAGFEMHWVRQAPGQGLEWMGAIDPKTGGTDYNQKFKDRVTMTRDTSISTAYMELSRLRSDDTAVYYCARDLGYFDVWGQGTLVTVSS

SEQ ID NO: 145 - protein, 576 aa, synthetic construct
EVQLVESGGGLVQPGGSLRLSCAASGFNIKDTYMHWVRQAPGKGLEWVARIDPANGNSKYADSVKGRFTISADTSKNTAYLQMNSLRAEDTAVYYCAPFGYYVSDYAMAYWGQGTLVTVSSASTKGPSVFPLAPSSKSTSGGTAALGCLVKDYFPEPVTVSWNSGALTSGVHTFPAVLQSSGLYSLSSVVTVPSSSLGTQTYICNVNHKPSNTKVDKKVEPKSCDKTHTCPPCPAPEAAGPSVFLFPPKPKDTLMISRTPEVTCVVVDVSHEDPEVKFNWYVDGVEVHNAKTKPREEQYNSTYRVVSVLTVLHQDWLNGKEYKCKVSNKALPAPIEKTISKAKGQPREPQVYTLPPSREEMTKNQVSLSCAVKGFYPSDIAVEWESNGQPENNYKTTPPVLDSDGSFFLVSKLTVDKSRWQQGNVFSCSVMHEALHNRFTQKSLSLSPGGGGGSGGGGSGGGGSGGGGSDIQMTQSPSSLSASVGDRVTITCRASQDIRSNLNWYQQKPGGAVKLLIYYTSRLHSGVPSRFSGSGSGTDYTLTISSLQPEDFATYFCQQSEKLPRTFGGGTKVEIR

SEQ ID NO: 146 - protein, 735 aa, synthetic construct
EVQLVESGGGLVQPGGSLRLSCAASGFNIKDTYMHWVRQAPGKGLEWVARIDPANGNSKYADSVKGRFTISADTSKNTAYLQMNSLRAEDTAVYYCAPFGYYVSDYAMAYWGQGTLVTVSSASTKGPSVFPLAPSSKSTSGGTAALGCLVKDYFPEPVTVSWNSGALTSGVHTFPAVLQSSGLYSLSSVVTVPSSSLGTQTYICNVNHKPSNTKVDKKVEPKSCGGGGSGGGGSGGGGSGGGGSEVQLVESGGGLVQPGGSLRLSCAASGFTFSTYAMNWVRQAPGKGLEWVGRIRSKYNNYATYYADSVKGRFTISRDDSKNSLYLQMNSLKTEDTAVYYCVRHGNFGNSYVSWFAYWGQGTLVTVSSGGGGSDKTHTCPPCPAPEAAGPSVFLFPPKPKDTLMISRTPEVTCVVVDVSHEDPEVKFNWYVDGVEVHNAKTKPREEQYNSTYRVVSVLTVLHQDWLNGKEYKCKVSNKALPAPIEKTISKAKGQPREPQVYTLPPSREEMTKNQVSLWCLVKGFYPSDIAVEWESNGQPENNYKTTPPVLDSDGSFFLYSKLTVDKSRWQQGNVFSCSVMHEALHNHYTQKSLSLSPGGGGGSGGGGSGGGGSGGGGSQVQLVQSGAEVKKPGASVKVSCKASGYTFAGFEMHWVRQAPGQGLEWMGAIDPKTGGTDYNQKFKDRVTMTRDTSISTAYMELSRLRSDDTAVYYCARDLGYFDVWGQGTLVTVSS

SEQ ID NO: 147 - protein, 599 aa, synthetic construct
EVQLVESGGGLVQPGGSLRLSCAASGFNIKDTYMHWVRQAPGKGLEWVARIDPANGNSKYADSVKGRFTISADTSKNTAYLQMNSLRAEDTAVYYCAPFGYYVSDYAMAYWGQGTLVTVSSASTKGPSVFPLAPSSKSTSGGTAALGCLVKDYFPEPVTVSWNSGALTSGVHTFPAVLQSSGLYSLSSVVTVPSSSLGTQTYICNVNHKPSNTKVDKKVEPKSCGGGGSGGGGSGGGGSGGGGSEVQLVESGGGLVQPGGSLRLSCAASGFTFSTYAMNWVRQAPGKGLEWVGRIRSKYNNYATYYADSVKGRFTISRDDSKNSLYLQMNSLKTEDTAVYYCVRHGNFGNSYVSWFAYWGQGTLVTVSSGGGGSDKTHTCPPCPAPEAAGPSVFLFPPKPKDTLMISRTPEVTCVVVDVSHEDPEVKFNWYVDGVEVHNAKTKPREEQYNSTYRVVSVLTVLHQDWLNGKEYKCKVSNKALPAPIEKTISKAKGQPREPQVYTLPPSREEMTKNQVSLWCLVKGFYPSDIAVEWESNGQPENNYKTTPPVLDSDGSFFLYSKLTVDKSRWQQGNVFSCSVMHEALHNHYTQKSLSLSPG

SEQ ID NO: 148 - protein, 740 aa, synthetic construct
EVQLVESGGGLVQPGGSLRLSCAASGFNIKDTYMHWVRQAPGKGLEWVARIDPANGNSKYADSVKGRFTISADTSKNTAYLQMNSLRAEDTAVYYCAPFGYYVSDYAMAYWGQGTLVTVSSASTKGPSVFPLAPSSKSTSGGTAALGCLVKDYFPEPVTVSWNSGALTSGVHTFPAVLQSSGLYSLSSVVTVPSSSLGTQTYICNVNHKPSNTKVDKKVEPKSCGGGGSGGGGSGGGGSGGGGSEVQLVESGGGLVQPGGSLRLSCAASGFTFSTYAMNWVRQAPGKGLEWVGRIRSKYNNYATYYADSVKGRFTISRDDSKNSLYLQMNSLKTEDTAVYYCVRHGNFGNSYVSWFAYWGQGTLVTVSSGGGGSDKTHTCPPCPAPELLGPSVFLFPPKPKDTLMISRTPEVTCVVVDVSHEDPEVKFNWYVDGVEVHNAKTKPREEQYNSTYRVVSVLTVLHQDWLNGKEYKCKVSNKALGAPIEKTISKAKGQPREPQVYTLPPSREEMTKNQVSLWCLVKGFYPSDIAVEWESNGQPENNYKTTPPVLDSDGSFFLYSKLTVDKSRWQQGNVFSCSVMHEALHNHYTQKSLSLSPGKGGGGSGGGGSGGGGSGGGGSQVQLVQSGAEVKKPGASVKVSCKASGYTFTSYYIHWVRQAPGQGLEWIGCIYPGNVNTNYNEKFKDRATLTVDTSISTAYMELSRLRSDDTAVYFCTRSHYGLDWNFDVWGQGTTVTVSS

SEQ ID NO: 149 - protein, 600 aa, synthetic construct
EVQLVESGGGLVQPGGSLRLSCAASGFNIKDTYMHWVRQAPGKGLEWVARIDPANGNSKYADSVKGRFTISADTSKNTAYLQMNSLRAEDTAVYYCAPFGYYVSDYAMAYWGQGTLVTVSSASTKGPSVFPLAPSSKSTSGGTAALGCLVKDYFPEPVTVSWNSGALTSGVHTFPAVLQSSGLYSLSSVVTVPSSSLGTQTYICNVNHKPSNTKVDKKVEPKSCGGGGSGGGGSGGGGSGGGGSEVQLVESGGGLVQPGGSLRLSCAASGFTFSTYAMNWVRQAPGKGLEWVGRIRSKYNNYATYYADSVKGRFTISRDDSKNSLYLQMNSLKTEDTAVYYCVRHGNFGNSYVSWFAYWGQGTLVTVSSGGGGSDKTHTCPPCPAPELLGPSVFLFPPKPKDTLMISRTPEVTCVVVDVSHEDPEVKFNWYVDGVEVHNAKTKPREEQYNSTYRVVSVLTVLHQDWLNGKEYKCKVSNKALGAPIEKTISKAKGQPREPQVYTLPPSREEMTKNQVSLWCLVKGFYPSDIAVEWESNGQPENNYKTTPPVLDSDGSFFLYSKLTVDKSRWQQGNVFSCSVMHEALHNHYTQKSLSLSPGK

SEQ ID NO: 150 - protein, 710 aa, synthetic construct
EVQLVESGGGLVQPGGSLRLSCAASGFNIKDTYMHWVRQAPGKGLEWVARIDPANGNSKYADSVKGRFTISADTSKNTAYLQMNSLRAEDTAVYYCAPFGYYVSDYAMAYWGQGTLVTVSSASTKGPSVFPLAPSSKSTSGGTAALGCLVKDYFPEPVTVSWNSGALTSGVHTFPAVLQSSGLYSLSSVVTVPSSSLGTQTYICNVNHKPSNTKVDKKVEPKSCGGGGSGGGGSGGGGSGGGGSQAVVTQEPSLTVSPGGTVTLTCRSSTGAVTTSNYANWVQQKPGQAPRGLIGGTNKRAPWTPARFSGSLLGGKAALTITGAQAEDEADYYCALWYSNLWVFGGGTKLTVLGGGGSDKTHTCPPCPAPEAAGPSVFLFPPKPKDTLMISRTPEVTCVVVDVSHEDPEVKFNWYVDGVEVHNAKTKPREEQYNSTYRVVSVLTVLHQDWLNGKEYKCKVSNKALPAPIEKTISKAKGQPREPQVYTLPPSREEMTKNQVSLSCAVKGFYPSDIAVEWESNGQPENNYKTTPPVLDSDGSFFLVSKLTVDKSRWQQGNVFSCSVMHEALHNRFTQKSLSLSPGGGGGSGGGGSGGGGSGGGGSDIQMTQSPSSLSASVGDRVTITCRASQDIRSNLNWYQQKPGGAVKLLIYYTSRLHSGVPSRFSGSGSGTDYTLTISSLQPEDFATYFCQQSEKLPRTFGGGTKVEIR

SEQ ID NO: 151 - protein, 583 aa, synthetic construct
EVQLVESGGGLVQPGGSLRLSCAASGFNIKDTYMHWVRQAPGKGLEWVARIDPANGNSKYADSVKGRFTISADTSKNTAYLQMNSLRAEDTAVYYCAPFGYYVSDYAMAYWGQGTLVTVSSASTKGPSVFPLAPSSKSTSGGTAALGCLVKDYFPEPVTVSWNSGALTSGVHTFPAVLQSSGLYSLSSVVTVPSSSLGTQTYICNVNHKPSNTKVDKKVEPKSCGGGGSGGGGSGGGGSGGGGSQAVVTQEPSLTVSPGGTVTLTCRSSTGAVTTSNYANWVQQKPGQAPRGLIGGTNKRAPWTPARFSGSLLGGKAALTITGAQAEDEADYYCALWYSNLWVFGGGTKLTVLGGGGSDKTHTCPPCPAPEAAGPSVFLFPPKPKDTLMISRTPEVTCVVVDVSHEDPEVKFNWYVDGVEVHNAKTKPREEQYNSTYRVVSVLTVLHQDWLNGKEYKCKVSNKALPAPIEKTISKAKGQPREPQVYTLPPSREEMTKNQVSLSCAVKGFYPSDIAVEWESNGQPENNYKTTPPVLDSDGSFFLVSKLTVDKSRWQQGNVFSCSVMHEALHNRFTQKSLSLSPG

SEQ ID NO: 152 - protein, 711 aa, synthetic construct
EVQLVESGGGLVQPGGSLRLSCAASGFNIKDTYMHWVRQAPGKGLEWVARIDPANGNSKYADSVKGRFTISADTSKNTAYLQMNSLRAEDTAVYYCAPFGYYVSDYAMAYWGQGTLVTVSSASTKGPSVFPLAPSSKSTSGGTAALGCLVKDYFPEPVTVSWNSGALTSGVHTFPAVLQSSGLYSLSSVVTVPSSSLGTQTYICNVNHKPSNTKVDKKVEPKSCGGGGSGGGGSGGGGSGGGGSQAVVTQEPSLTVSPGGTVTLTCRSSTGAVTTSNYANWVQQKPGQAPRGLIGGTNKRAPWTPARFSGSLLGGKAALTITGAQAEDEADYYCALWYSNLWVFGGGTKLTVLGGGGSDKTHTCPPCPAPELLGPSVFLFPPKPKDTLMISRTPEVTCVVVDVSHEDPEVKFNWYVDGVEVHNAKTKPREEQYNSTYRVVSVLTVLHQDWLNGKEYKCKVSNKALGAPIEKTISKAKGQPREPQVYTLPPSREEMTKNQVSLSCAVKGFYPSDIAVEWESNGQPENNYKTTPPVLDSDGSFFLVSKLTVDKSRWQQGNVFSCSVMHEALHNRFTQKSLSLSPGKGGGGSGGGGSGGGGSGGGGSDIQMTQSPSSLSASVGDRVTITCHASQNIYVWLNWYQQKPGKAPKLLIYKASNLHTGVPSRFSGSGSGTDFTLTISSLQPEDFATYYCQQGQTYPYTFGGGTKVEIK

SEQ ID NO: 153 - protein, 584 aa, synthetic construct
EVQLVESGGGLVQPGGSLRLSCAASGFNIKDTYMHWVRQAPGKGLEWVARIDPANGNSKYADSVKGRFTISADTSKNTAYLQMNSLRAEDTAVYYCAPFGYYVSDYAMAYWGQGTLVTVSSASTKGPSVFPLAPSSKSTSGGTAALGCLVKDYFPEPVTVSWNSGALTSGVHTFPAVLQSSGLYSLSSVVTVPSSSLGTQTYICNVNHKPSNTKVDKKVEPKSCGGGGSGGGGSGGGGSGGGGSQAVVTQEPSLTVSPGGTVTLTCRSSTGAVTTSNYANWVQQKPGQAPRGLIGGTNKRAPWTPARFSGSLLGGKAALTITGAQAEDEADYYCALWYSNLWVFGGGTKLTVLGGGGSDKTHTCPPCPAPELLGPSVFLFPPKPKDTLMISRTPEVTCVVVDVSHEDPEVKFNWYVDGVEVHNAKTKPREEQYNSTYRVVSVLTVLHQDWLNGKEYKCKVSNKALGAPIEKTISKAKGQPREPQVYTLPPSREEMTKNQVSLSCAVKGFYPSDIAVEWESNGQPENNYKTTPPVLDSDGSFFLVSKLTVDKSRWQQGNVFSCSVMHEALHNRFTQKSLSLSPGK

SEQ ID NO: 154 - protein, 585 aa, synthetic construct
EVQLVESGGGLVQPGGSLRLSCAASGFNVYASGMHWVRQAPGKGLEWVAKIYPDSDYTYYADSVKGRFTISADTSKNTAYLQMNSLRAEDTAVYYCSRDSSFYYVYAMDYWGQGTLVTVSSASTKGPSVFPLAPSSKSTSGGTAALGCLVKDYFPEPVTVSWNSGALTSGVHTFPAVLQSSGLYSLSSVVTVPSSSLGTQTYICNVNHKPSNTKVDKKVEPKSCDKTHTCPPCPAPEAAGPSVFLFPPKPKDTLMISRTPEVTCVVVDVSHEDPEVKFNWYVDGVEVHNAKTKPREEQYNSTYRVVSVLTVLHQDWLNGKEYKCKVSNKALPAPIEKTISKAKGQPREPQVYTLPPSREEMTKNQVSLWCLVKGFYPSDIAVEWESNGQPENNYKTTPPVLDSDGSFFLYSKLTVDKSRWQQGNVFSCSVMHEALHNHYTQKSLSLSPGGGGGSGGGGSGGGGSGGGGSQVQLVQSGAEVKKPGASVKVSCKASGYTFAGFEMHWVRQAPGQGLEWMGAIDPKTGGTDYNQKFKDRVTMTRDTSISTAYMELSRLRSDDTAVYYCARDLGYFDVWGQGTLVTVSS

SEQ ID NO: 155 - protein, 576 aa, synthetic construct
EVQLVESGGGLVQPGGSLRLSCAASGFNVYASGMHWVRQAPGKGLEWVAKIYPDSDYTYYADSVKGRFTISADTSKNTAYLQMNSLRAEDTAVYYCSRDSSFYYVYAMDYWGQGTLVTVSSASTKGPSVFPLAPSSKSTSGGTAALGCLVKDYFPEPVTVSWNSGALTSGVHTFPAVLQSSGLYSLSSVVTVPSSSLGTQTYICNVNHKPSNTKVDKKVEPKSCDKTHTCPPCPAPEAAGPSVFLFPPKPKDTLMISRTPEVTCVVVDVSHEDPEVKFNWYVDGVEVHNAKTKPREEQYNSTYRVVSVLTVLHQDWLNGKEYKCKVSNKALPAPIEKTISKAKGQPREPQVYTLPPSREEMTKNQVSLSCAVKGFYPSDIAVEWESNGQPENNYKTTPPVLDSDGSFFLVSKLTVDKSRWQQGNVFSCSVMHEALHNRFTQKSLSLSPGGGGGSGGGGSGGGGSGGGGSDIQMTQSPSSLSASVGDRVTITCRASQDIRSNLNWYQQKPGGAVKLLIYYTSRLHSGVPSRFSGSGSGTDYTLTISSLQPEDFATYFCQQSEKLPRTFGGGTKVEIR

SEQ ID NO: 156 - protein, 735 aa, synthetic construct
EVQLVESGGGLVQPGGSLRLSCAASGFNVYASGMHWVRQAPGKGLEWVAKIYPDSDYTYYADSVKGRFTISADTSKNTAYLQMNSLRAEDTAVYYCSRDSSFYYVYAMDYWGQGTLVTVSSASTKGPSVFPLAPSSKSTSGGTAALGCLVKDYFPEPVTVSWNSGALTSGVHTFPAVLQSSGLYSLSSVVTVPSSSLGTQTYICNVNHKPSNTKVDKKVEPKSCGGGGSGGGGSGGGGSGGGGSEVQLVESGGGLVQPGGSLRLSCAASGFTFSTYAMNWVRQAPGKGLEWVGRIRSKYNNYATYYADSVKGRFTISRDDSKNSLYLQMNSLKTEDTAVYYCVRHGNFGNSYVSWFAYWGQGTLVTVSSGGGGSDKTHTCPPCPAPEAAGPSVFLFPPKPKDTLMISRTPEVTCVVVDVSHEDPEVKFNWYVDGVEVHNAKTKPREEQYNSTYRVVSVLTVLHQDWLNGKEYKCKVSNKALPAPIEKTISKAKGQPREPQVYTLPPSREEMTKNQVSLWCLVKGFYPSDIAVEWESNGQPENNYKTTPPVLDSDGSFFLYSKLTVDKSRWQQGNVFSCSVMHEALHNHYTQKSLSLSPGGGGGSGGGGSGGGGSGGGGSQVQLVQSGAEVKKPGASVKVSCKASGYTFAGFEMHWVRQAPGQGLEWMGAIDPKTGGTDYNQKFKDRVTMTRDTSISTAYMELSRLRSDDTAVYYCARDLGYFDVWGQGTLVTVSS

SEQ ID NO: 157 - protein, 599 aa, synthetic construct
EVQLVESGGGLVQPGGSLRLSCAASGFNVYASGMHWVRQAPGKGLEWVAKIYPDSDYTYYADSVKGRFTISADTSKNTAYLQMNSLRAEDTAVYYCSRDSSFYYVYAMDYWGQGTLVTVSSASTKGPSVFPLAPSSKSTSGGTAALGCLVKDYFPEPVTVSWNSGALTSGVHTFPAVLQSSGLYSLSSVVTVPSSSLGTQTYICNVNHKPSNTKVDKKVEPKSCGGGGSGGGGSGGGGSGGGGSEVQLVESGGGLVQPGGSLRLSCAASGFTFSTYAMNWVRQAPGKGLEWVGRIRSKYNNYATYYADSVKGRFTISRDDSKNSLYLQMNSLKTEDTAVYYCVRHGNFGNSYVSWFAYWGQGTLVTVSSGGGGSDKTHTCPPCPAPEAAGPSVFLFPPKPKDTLMISRTPEVTCVVVDVSHEDPEVKFNWYVDGVEVHNAKTKPREEQYNSTYRVVSVLTVLHQDWLNGKEYKCKVSNKALPAPIEKTISKAKGQPREPQVYTLPPSREEMTKNQVSLWCLVKGFYPSDIAVEWESNGQPENNYKTTPPVLDSDGSFFLYSKLTVDKSRWQQGNVFSCSVMHEALHNHYTQKSLSLSPG

SEQ ID NO: 158 - protein, 710 aa, synthetic construct
EVQLVESGGGLVQPGGSLRLSCAASGFNVYASGMHWVRQAPGKGLEWVAKIYPDSDYTYYADSVKGRFTISADTSKNTAYLQMNSLRAEDTAVYYCSRDSSFYYVYAMDYWGQGTLVTVSSASTKGPSVFPLAPSSKSTSGGTAALGCLVKDYFPEPVTVSWNSGALTSGVHTFPAVLQSSGLYSLSSVVTVPSSSLGTQTYICNVNHKPSNTKVDKKVEPKSCGGGGSGGGGSGGGGSGGGGSQAVVTQEPSLTVSPGGTVTLTCRSSTGAVTTSNYANWVQQKPGQAPRGLIGGTNKRAPWTPARFSGSLLGGKAALTITGAQAEDEADYYCALWYSNLWVFGGGTKLTVLGGGGSDKTHTCPPCPAPEAAGPSVFLFPPKPKDTLMISRTPEVTCVVVDVSHEDPEVKFNWYVDGVEVHNAKTKPREEQYNSTYRVVSVLTVLHQDWLNGKEYKCKVSNKALPAPIEKTISKAKGQPREPQVYTLPPSREEMTKNQVSLSCAVKGFYPSDIAVEWESNGQPENNYKTTPPVLDSDGSFFLVSKLTVDKSRWQQGNVFSCSVMHEALHNRFTQKSLSLSPGGGGGSGGGGSGGGGSGGGGSDIQMTQSPSSLSASVGDRVTITCRASQDIRSNLNWYQQKPGGAVKLLIYYTSRLHSGVPSRFSGSGSGTDYTLTISSLQPEDFATYFCQQSEKLPRTFGGGTKVEIR

SEQ ID NO: 159 - protein, 583 aa, synthetic construct
EVQLVESGGGLVQPGGSLRLSCAASGFNVYASGMHWVRQAPGKGLEWVAKIYPDSDYTYYADSVKGRFTISADTSKNTAYLQMNSLRAEDTAVYYCSRDSSFYYVYAMDYWGQGTLVTVSSASTKGPSVFPLAPSSKSTSGGTAALGCLVKDYFPEPVTVSWNSGALTSGVHTFPAVLQSSGLYSLSSVVTVPSSSLGTQTYICNVNHKPSNTKVDKKVEPKSCGGGGSGGGGSGGGGSGGGGSQAVVTQEPSLTVSPGGTVTLTCRSSTGAVTTSNYANWVQQKPGQAPRGLIGGTNKRAPWTPARFSGSLLGGKAALTITGAQAEDEADYYCALWYSNLWVFGGGTKLTVLGGGGSDKTHTCPPCPAPEAAGPSVFLFPPKPKDTLMISRTPEVTCVVVDVSHEDPEVKFNWYVDGVEVHNAKTKPREEQYNSTYRVVSVLTVLHQDWLNGKEYKCKVSNKALPAPIEKTISKAKGQPREPQVYTLPPSREEMTKNQVSLSCAVKGFYPSDIAVEWESNGQPENNYKTTPPVLDSDGSFFLVSKLTVDKSRWQQGNVFSCSVMHEALHNRFTQKSLSLSPG

SEQ ID NO: 160 - protein, 582 aa, synthetic construct
EVQLVESGGGLVQPGGSLRLSCAASGFTFSDSWIHWVRQAPGKGLEWVAWISPYGGSTYYADSVKGRFTISADTSKNTAYLQMNSLRAEDTAVYYCARRHWPGGFDYWGQGTLVTVSSASTKGPSVFPLAPSSKSTSGGTAALGCLVKDYFPEPVTVSWNSGALTSGVHTFPAVLQSSGLYSLSSVVTVPSSSLGTQTYICNVNHKPSNTKVDKKVEPKSCDKTHTCPPCPAPEAAGPSVFLFPPKPKDTLMISRTPEVTCVVVDVSHEDPEVKFNWYVDGVEVHNAKTKPREEQYNSTYRVVSVLTVLHQDWLNGKEYKCKVSNKALPAPIEKTISKAKGQPREPQVYTLPPSREEMTKNQVSLWCLVKGFYPSDIAVEWESNGQPENNYKTTPPVLDSDGSFFLYSKLTVDKSRWQQGNVFSCSVMHEALHNHYTQKSLSLSPGGGGGSGGGGSGGGGSGGGGSQVQLVQSGAEVKKPGASVKVSCKASGYTFAGFEMHWVRQAPGQGLEWMGAIDPKTGGTDYNQKFKDRVTMTRDTSISTAYMELSRLRSDDTAVYYCARDLGYFDVWGQGTLVTVSS

SEQ ID NO: 161 - protein, 573 aa, synthetic construct
EVQLVESGGGLVQPGGSLRLSCAASGFTFSDSWIHWVRQAPGKGLEWVAWISPYGGSTYYADSVKGRFTISADTSKNTAYLQMNSLRAEDTAVYYCARRHWPGGFDYWGQGTLVTVSSASTKGPSVFPLAPSSKSTSGGTAALGCLVKDYFPEPVTVSWNSGALTSGVHTFPAVLQSSGLYSLSSVVTVPSSSLGTQTYICNVNHKPSNTKVDKKVEPKSCDKTHTCPPCPAPEAAGPSVFLFPPKPKDTLMISRTPEVTCVVVDVSHEDPEVKFNWYVDGVEVHNAKTKPREEQYNSTYRVVSVLTVLHQDWLNGKEYKCKVSNKALPAPIEKTISKAKGQPREPQVYTLPPSREEMTKNQVSLSCAVKGFYPSDIAVEWESNGQPENNYKTTPPVLDSDGSFFLVSKLTVDKSRWQQGNVFSCSVMHEALHNRFTQKSLSLSPGGGGGSGGGGSGGGGSGGGGSDIQMTQSPSSLSASVGDRVTITCRASQDIRSNLNWYQQKPGGAVKLLIYYTSRLHSGVPSRFSGSGSGTDYTLTISSLQPEDFATYFCQQSEKLPRTFGGGTKVEIR

SEQ ID NO: 162 - protein, 705 aa, synthetic construct
EVQLVESGGGLVQPGGSLRLSCAASGFTFSDSWIHWVRQAPGKGLEWVAWISPYGGSTYYADSVKGRFTISADTSKNTAYLQMNSLRAEDTAVYYCARRHWPGGFDYWGQGTLVTVSSASTKGPSVFPLAPSSKSTSGGTAALGCLVKDYFPEPVTVSWNSGALTSGVHTFPAVLQSSGLYSLSSVVTVPSSSLGTQTYICNVNHKPSNTKVDKKVEPKSCGGGGSGGGGSGGGGSGGGGSDIQMTQSPSSLSASVGDRVTITCLASEDISNDLAWYQQKPGKAPKLLIYFVDRLLDGVPSRFSGSGSGTDFTLTISSLQPEDFATYYCQQSYKYPPTFGQGTKLEIKGGGGSDKTHTCPPCPAPEAAGPSVFLFPPKPKDTLMISRTPEVTCVVVDVSHEDPEVKFNWYVDGVEVHNAKTKPREEQYNSTYRVVSVLTVLHQDWLNGKEYKCKVSNKALPAPIEKTISKAKGQPREPQVYTLPPSREEMTKNQVSLSCAVKGFYPSDIAVEWESNGQPENNYKTTPPVLDSDGSFFLVSKLTVDKSRWQQGNVFSCSVMHEALHNRFTQKSLSLSPGGGGGSGGGGSGGGGSGGGGSDIQMTQSPSSLSASVGDRVTITCRASQDIRSNLNWYQQKPGGAVKLLIYYTSRLHSGVPSRFSGSGSGTDYTLTISSLQPEDFATYFCQQSEKLPRTFGGGTKVEIR

SEQ ID NO: 163 - protein, 705 aa, synthetic construct
EVQLVESGGGLVQPGGSLRLSCAASGFTFSDSWIHWVRQAPGKGLEWVAWISPYGGSTYYADSVKGRFTISADTSKNTAYLQMNSLRAEDTAVYYCARRHWPGGFDYWGQGTLVTVSSASTKGPSVFPLAPSSKSTSGGTAALGCLVKDYFPEPVTVSWNSGALTSGVHTFPAVLQSSGLYSLSSVVTVPSSSLGTQTYICNVNHKPSNTKVDKKVEPKSCGGGGSGGGGSGGGGSGGGGSDIQMTQSPSSLSASVGDRVTITCRASQDIRSNLNWYQQKPGGAVKLLIYYTSRLHSGVPSRFSGSGSGTDYTLTISSLQPEDFATYFCQQSEKLPRTFGGGTKVEIRGGGGSDKTHTCPPCPAPEAAGPSVFLFPPKPKDTLMISRTPEVTCVVVDVSHEDPEVKFNWYVDGVEVHNAKTKPREEQYNSTYRVVSVLTVLHQDWLNGKEYKCKVSNKALPAPIEKTISKAKGQPREPQVYTLPPSREEMTKNQVSLSCAVKGFYPSDIAVEWESNGQPENNYKTTPPVLDSDGSFFLVSKLTVDKSRWQQGNVFSCSVMHEALHNRFTQKSLSLSPGGGGGSGGGGSGGGGSGGGGSDIQMTQSPSSVSASVGDRVTITCRASQGIYSWLAWYQQKPGKAPNLLIYTASTLQSGVPSRFSGSGSGTDFTLTISSLQPEDFATYYCQQANIFPLTFGGGTKVEIK

SEQ ID NO: 164 - protein, 705 aa, synthetic construct
EVQLVESGGGLVQPGGSLRLSCAASGFTFSDSWIHWVRQAPGKGLEWVAWISPYGGSTYYADSVKGRFTISADTSKNTAYLQMNSLRAEDTAVYYCARRHWPGGFDYWGQGTLVTVSSASTKGPSVFPLAPSSKSTSGGTAALGCLVKDYFPEPVTVSWNSGALTSGVHTFPAVLQSSGLYSLSSVVTVPSSSLGTQTYICNVNHKPSNTKVDKKVEPKSCGGGGSGGGGSGGGGSGGGGSDIQMTQSPSSLSASVGDRVTITCRASQDIRSNLNWYQQKPGGAVKLLIYYTSRLHSGVPSRFSGSGSGTDYTLTISSLQPEDFATYFCQQSEKLPRTFGGGTKVEIRGGGGSDKTHTCPPCPAPEAAGPSVFLFPPKPKDTLMISRTPEVTCVVVDVSHEDPEVKFNWYVDGVEVHNAKTKPREEQYNSTYRVVSVLTVLHQDWLNGKEYKCKVSNKALPAPIEKTISKAKGQPREPQVYTLPPSREEMTKNQVSLSCAVKGFYPSDIAVEWESNGQPENNYKTTPPVLDSDGSFFLVSKLTVDKSRWQQGNVFSCSVMHEALHNRFTQKSLSLSPGGGGGSGGGGSGGGGSGGGGSDIQMTQSPSSLSASVGDRVTITCLASEDISNDLAWYQQKPGKAPKLLIYFVDRLLDGVPSRFSGSGSGTDFTLTISSLQPEDFATYYCQQSYKYPPTFGQGTKLEIK

SEQ ID NO: 165 - protein, 578 aa, synthetic construct
EVQLVESGGGLVQPGGSLRLSCAASGFTFSDSWIHWVRQAPGKGLEWVAWISPYGGSTYYADSVKGRFTISADTSKNTAYLQMNSLRAEDTAVYYCARRHWPGGFDYWGQGTLVTVSSASTKGPSVFPLAPSSKSTSGGTAALGCLVKDYFPEPVTVSWNSGALTSGVHTFPAVLQSSGLYSLSSVVTVPSSSLGTQTYICNVNHKPSNTKVDKKVEPKSCGGGGSGGGGSGGGGSGGGGSDIQMTQSPSSLSASVGDRVTITCRASQDIRSNLNWYQQKPGGAVKLLIYYTSRLHSGVPSRFSGSGSGTDYTLTISSLQPEDFATYFCQQSEKLPRTFGGGTKVEIRGGGGSDKTHTCPPCPAPEAAGPSVFLFPPKPKDTLMISRTPEVTCVVVDVSHEDPEVKFNWYVDGVEVHNAKTKPREEQYNSTYRVVSVLTVLHQDWLNGKEYKCKVSNKALPAPIEKTISKAKGQPREPQVYTLPPSREEMTKNQVSLSCAVKGFYPSDIAVEWESNGQPENNYKTTPPVLDSDGSFFLVSKLTVDKSRWQQGNVFSCSVMHEALHNRFTQKSLSLSPG

SEQ ID NO: 166 - protein, 705 aa, synthetic construct
EVQLVESGGGLVQPGGSLRLSCAASGFTFSDSWIHWVRQAPGKGLEWVAWISPYGGSTYYADSVKGRFTISADTSKNTAYLQMNSLRAEDTAVYYCARRHWPGGFDYWGQGTLVTVSSASTKGPSVFPLAPSSKSTSGGTAALGCLVKDYFPEPVTVSWNSGALTSGVHTFPAVLQSSGLYSLSSVVTVPSSSLGTQTYICNVNHKPSNTKVDKKVEPKSCGGGGSGGGGSGGGGSGGGGSDIQMTQSPSSVSASVGDRVTITCRASQGIYSWLAWYQQKPGKAPNLLIYTASTLQSGVPSRFSGSGSGTDFTLTISSLQPEDFATYYCQQANIFPLTFGGGTKVEIKGGGGSDKTHTCPPCPAPEAAGPSVFLFPPKPKDTLMISRTPEVTCVVVDVSHEDPEVKFNWYVDGVEVHNAKTKPREEQYNSTYRVVSVLTVLHQDWLNGKEYKCKVSNKALPAPIEKTISKAKGQPREPQVYTLPPSREEMTKNQVSLSCAVKGFYPSDIAVEWESNGQPENNYKTTPPVLDSDGSFFLVSKLTVDKSRWQQGNVFSCSVMHEALHNRFTQKSLSLSPGGGGGSGGGGSGGGGSGGGGSDIQMTQSPSSLSASVGDRVTITCRASQDIRSNLNWYQQKPGGAVKLLIYYTSRLHSGVPSRFSGSGSGTDYTLTISSLQPEDFATYFCQQSEKLPRTFGGGTKVEIR

SEQ ID NO: 167 - protein, 596 aa, synthetic construct
EVQLVESGGGLVQPGGSLRLSCAASGFTFSDSWIHWVRQAPGKGLEWVAWISPYGGSTYYADSVKGRFTISADTSKNTAYLQMNSLRAEDTAVYYCARRHWPGGFDYWGQGTLVTVSSASTKGPSVFPLAPSSKSTSGGTAALGCLVKDYFPEPVTVSWNSGALTSGVHTFPAVLQSSGLYSLSSVVTVPSSSLGTQTYICNVNHKPSNTKVDKKVEPKSCGGGGSGGGGSGGGGSGGGGSEVQLVESGGGLVQPGGSLRLSCAASGFTFSTYAMNWVRQAPGKGLEWVGRIRSKYNNYATYYADSVKGRFTISRDDSKNSLYLQMNSLKTEDTAVYYCVRHGNFGNSYVSWFAYWGQGTLVTVSSGGGGSDKTHTCPPCPAPEAAGPSVFLFPPKPKDTLMISRTPEVTCVVVDVSHEDPEVKFNWYVDGVEVHNAKTKPREEQYNSTYRVVSVLTVLHQDWLNGKEYKCKVSNKALPAPIEKTISKAKGQPREPQVYTLPPSREEMTKNQVSLWCLVKGFYPSDIAVEWESNGQPENNYKTTPPVLDSDGSFFLYSKLTVDKSRWQQGNVFSCSVMHEALHNHYTQKSLSLSPG

SEQ ID NO: 168 - protein, 732 aa, synthetic construct
EVQLVESGGGLVQPGGSLRLSCAASGFTFSDSWIHWVRQAPGKGLEWVAWISPYGGSTYYADSVKGRFTISADTSKNTAYLQMNSLRAEDTAVYYCARRHWPGGFDYWGQGTLVTVSSASTKGPSVFPLAPSSKSTSGGTAALGCLVKDYFPEPVTVSWNSGALTSGVHTFPAVLQSSGLYSLSSVVTVPSSSLGTQTYICNVNHKPSNTKVDKKVEPKSCGGGGSGGGGSGGGGSGGGGSEVQLVESGGGLVQPGGSLRLSCAASGFTFSTYAMNWVRQAPGKGLEWVGRIRSKYNNYATYYADSVKGRFTISRDDSKNSLYLQMNSLKTEDTAVYYCVRHGNFGNSYVSWFAYWGQGTLVTVSSGGGGSDKTHTCPPCPAPEAAGPSVFLFPPKPKDTLMISRTPEVTCVVVDVSHEDPEVKFNWYVDGVEVHNAKTKPREEQYNSTYRVVSVLTVLHQDWLNGKEYKCKVSNKALPAPIEKTISKAKGQPREPQVYTLPPSREEMTKNQVSLWCLVKGFYPSDIAVEWESNGQPENNYKTTPPVLDSDGSFFLYSKLTVDKSRWQQGNVFSCSVMHEALHNHYTQKSLSLSPGGGGGSGGGGSGGGGSGGGGSQVQLVQSGAEVKKPGASVKVSCKASGYTFAGFEMHWVRQAPGQGLEWMGAIDPKTGGTDYNQKFKDRVTMTRDTSISTAYMELSRLRSDDTAVYYCARDLGYFDVWGQGTLVTVSS

SEQ ID NO: 169 - protein, 736 aa, synthetic construct
EVQLVESGGGLVQPGGSLRLSCAASGFTFSDSWIHWVRQAPGKGLEWVAWISPYGGSTYYADSVKGRFTISADTSKNTAYLQMNSLRAEDTAVYYCARRHWPGGFDYWGQGTLVTVSSASTKGPSVFPLAPSSKSTSGGTAALGCLVKDYFPEPVTVSWNSGALTSGVHTFPAVLQSSGLYSLSSVVTVPSSSLGTQTYICNVNHKPSNTKVDKKVEPKSCGGGGSGGGGSGGGGSGGGGSEVQLVESGGGLVQPGGSLRLSCAASGFTFSTYAMNWVRQAPGKGLEWVGRIRSKYNNYATYYADSVKGRFTISRDDSKNSLYLQMNSLKTEDTAVYYCVRHGNFGNSYVSWFAYWGQGTLVTVSSGGGGSDKTHTCPPCPAPEAAGPSVFLFPPKPKDTLMISRTPEVTCVVVDVSHEDPEVKFNWYVDGVEVHNAKTKPREEQYNSTYRVVSVLTVLHQDWLNGKEYKCKVSNKALPAPIEKTISKAKGQPREPQVYTLPPSREEMTKNQVSLWCLVKGFYPSDIAVEWESNGQPENNYKTTPPVLDSDGSFFLYSKLTVDKSRWQQGNVFSCSVMHEALHNHYTQKSLSLSPGGGGGSGGGGSGGGGSGGGGSQVQLVQSGAEVKKPGASVKVSCKASGYTFTSYYIHWVRQAPGQGLEWIGCIYPGNVNTNYNEKFKDRATLTVDTSISTAYMELSRLRSDDTAVYFCTRSHYGLDWNFDVWGQGTTVTVSS

SEQ ID NO: 170 - protein, 729 aa, synthetic construct
EVQLVESGGGLVQPGGSLRLSCAASGFTFSDSWIHWVRQAPGKGLEWVAWISPYGGSTYYADSVKGRFTISADTSKNTAYLQMNSLRAEDTAVYYCARRHWPGGFDYWGQGTLVTVSSASTKGPSVFPLAPSSKSTSGGTAALGCLVKDYFPEPVTVSWNSGALTSGVHTFPAVLQSSGLYSLSSVVTVPSSSLGTQTYICNVNHKPSNTKVDKKVEPKSCGGGGSGGGGSGGGGSGGGGSEVQLVESGGGLVQPGGSLRLSCAASGFTFTNYGLHWVRQAPGKGLEWVSSISPSGGVTYYRDSVKGRFTISRDNSKNTLYLQMNSLRAEDTAVYYCAKPFLGWGGANWIAHWGQGTLVTVSSGGGGSDKTHTCPPCPAPEAAGPSVFLFPPKPKDTLMISRTPEVTCVVVDVSHEDPEVKFNWYVDGVEVHNAKTKPREEQYNSTYRVVSVLTVLHQDWLNGKEYKCKVSNKALPAPIEKTISKAKGQPREPQVYTLPPSREEMTKNQVSLWCLVKGFYPSDIAVEWESNGQPENNYKTTPPVLDSDGSFFLYSKLTVDKSRWQQGNVFSCSVMHEALHNHYTQKSLSLSPGGGGGSGGGGSGGGGSGGGGSQVQLVQSGAEVKKPGASVKVSCKASGYTFAGFEMHWVRQAPGQGLEWMGAIDPKTGGTDYNQKFKDRVTMTRDTSISTAYMELSRLRSDDTAVYYCARDLGYFDVWGQGTLVTVSS

SEQ ID NO: 171 - protein, 580 aa, synthetic construct
EVQLVESGGGLVQPGGSLRLSCAASGFTFSDSWIHWVRQAPGKGLEWVAWISPYGGSTYYADSVKGRFTISADTSKNTAYLQMNSLRAEDTAVYYCARRHWPGGFDYWGQGTLVTVSSASTKGPSVFPLAPSSKSTSGGTAALGCLVKDYFPEPVTVSWNSGALTSGVHTFPAVLQSSGLYSLSSVVTVPSSSLGTQTYICNVNHKPSNTKVDKKVEPKSCGGGGSGGGGSGGGGSGGGGSQAVVTQEPSLTVSPGGTVTLTCRSSTGAVTTSNYANWVQQKPGQAPRGLIGGTNKRAPWTPARFSGSLLGGKAALTITGAQAEDEADYYCALWYSNLWVFGGGTKLTVLGGGGSDKTHTCPPCPAPEAAGPSVFLFPPKPKDTLMISRTPEVTCVVVDVSHEDPEVKFNWYVDGVEVHNAKTKPREEQYNSTYRVVSVLTVLHQDWLNGKEYKCKVSNKALPAPIEKTISKAKGQPREPQVYTLPPSREEMTKNQVSLSCAVKGFYPSDIAVEWESNGQPENNYKTTPPVLDSDGSFFLVSKLTVDKSRWQQGNVFSCSVMHEALHNRFTQKSLSLSPG

SEQ ID NO: 172 - protein, 707 aa, synthetic construct
EVQLVESGGGLVQPGGSLRLSCAASGFTFSDSWIHWVRQAPGKGLEWVAWISPYGGSTYYADSVKGRFTISADTSKNTAYLQMNSLRAEDTAVYYCARRHWPGGFDYWGQGTLVTVSSASTKGPSVFPLAPSSKSTSGGTAALGCLVKDYFPEPVTVSWNSGALTSGVHTFPAVLQSSGLYSLSSVVTVPSSSLGTQTYICNVNHKPSNTKVDKKVEPKSCGGGGSGGGGSGGGGSGGGGSQAVVTQEPSLTVSPGGTVTLTCRSSTGAVTTSNYANWVQQKPGQAPRGLIGGTNKRAPWTPARFSGSLLGGKAALTITGAQAEDEADYYCALWYSNLWVFGGGTKLTVLGGGGSDKTHTCPPCPAPEAAGPSVFLFPPKPKDTLMISRTPEVTCVVVDVSHEDPEVKFNWYVDGVEVHNAKTKPREEQYNSTYRVVSVLTVLHQDWLNGKEYKCKVSNKALPAPIEKTISKAKGQPREPQVYTLPPSREEMTKNQVSLSCAVKGFYPSDIAVEWESNGQPENNYKTTPPVLDSDGSFFLVSKLTVDKSRWQQGNVFSCSVMHEALHNRFTQKSLSLSPGGGGGSGGGGSGGGGSGGGGSDIQMTQSPSSLSASVGDRVTITCRASQDIRSNLNWYQQKPGGAVKLLIYYTSRLHSGVPSRFSGSGSGTDYTLTISSLQPEDFATYFCQQSEKLPRTFGGGTKVEIR

SEQ ID NO: 173 - protein, 707 aa, synthetic construct
EVQLVESGGGLVQPGGSLRLSCAASGFTFSDSWIHWVRQAPGKGLEWVAWISPYGGSTYYADSVKGRFTISADTSKNTAYLQMNSLRAEDTAVYYCARRHWPGGFDYWGQGTLVTVSSASTKGPSVFPLAPSSKSTSGGTAALGCLVKDYFPEPVTVSWNSGALTSGVHTFPAVLQSSGLYSLSSVVTVPSSSLGTQTYICNVNHKPSNTKVDKKVEPKSCGGGGSGGGGSGGGGSGGGGSQAVVTQEPSLTVSPGGTVTLTCRSSTGAVTTSNYANWVQQKPGQAPRGLIGGTNKRAPWTPARFSGSLLGGKAALTITGAQAEDEADYYCALWYSNLWVFGGGTKLTVLGGGGSDKTHTCPPCPAPEAAGPSVFLFPPKPKDTLMISRTPEVTCVVVDVSHEDPEVKFNWYVDGVEVHNAKTKPREEQYNSTYRVVSVLTVLHQDWLNGKEYKCKVSNKALPAPIEKTISKAKGQPREPQVYTLPPSREEMTKNQVSLSCAVKGFYPSDIAVEWESNGQPENNYKTTPPVLDSDGSFFLVSKLTVDKSRWQQGNVFSCSVMHEALHNRFTQKSLSLSPGGGGGSGGGGSGGGGSGGGGSDIQMTQSPSSLSASVGDRVTITCHASQNIYVWLNWYQQKPGKAPKLLIYKASNLHTGVPSRFSGSGSGTDFTLTISSLQPEDFATYYCQQGQTYPYTFGGGTKVEIK

SEQ ID NO: 174 - protein, 733 aa, synthetic construct
EVQLVESGGGLVQPGGSLRLSCAASGFTFSDSWIHWVRQAPGKGLEWVAWISPYGGSTYYADSVKGRFTISADTSKNTAYLQMNSLRAEDTAVYYCARRHWPGGFDYWGQGTLVTVSSASTKGPSVFPLAPSSKSTSGGTAALGCLVKDYFPEPVTVSWNSGALTSGVHTFPAVLQSSGLYSLSSVVTVPSSSLGTQTYICNVNHKPSNTKVDKKVEPKSCGGGGSGGGGSGGGGSGGGGSQVQLVQSGAEVKKPGASVKVSCKASGYTFTGYYMHWVRQAPGQGLEWMGWINPDSGGTNYAQKFQGRVTMTRDTSISTAYMELNRLRSDDTAVYYCARDQPLGYCTNGVCSYFDYWGQGTLVTVSSGGGGSDKTHTCPPCPAPEAAGPSVFLFPPKPKDTLMISRTPEVTCVVVDVSHEDPEVKFNWYVDGVEVHNAKTKPREEQYNSTYRVVSVLTVLHQDWLNGKEYKCKVSNKALPAPIEKTISKAKGQPREPQVYTLPPSREEMTKNQVSLWCLVKGFYPSDIAVEWESNGQPENNYKTTPPVLDSDGSFFLYSKLTVDKSRWQQGNVFSCSVMHEALHNHYTQKSLSLSPGGGGGSGGGGSGGGGSGGGGSQVQLVQSGAEVKKPGASVKVSCKASGYTFAGFEMHWVRQAPGQGLEWMGAIDPKTGGTDYNQKFKDRVTMTRDTSISTAYMELSRLRSDDTAVYYCARDLGYFDVWGQGTLVTVSS

SEQ ID NO: 175 - protein, 733 aa, synthetic construct
EVQLVESGGGLVQPGGSLRLSCAASGFTFSDSWIHWVRQAPGKGLEWVAWISPYGGSTYYADSVKGRFTISADTSKNTAYLQMNSLRAEDTAVYYCARRHWPGGFDYWGQGTLVTVSSASTKGPSVFPLAPSSKSTSGGTAALGCLVKDYFPEPVTVSWNSGALTSGVHTFPAVLQSSGLYSLSSVVTVPSSSLGTQTYICNVNHKPSNTKVDKKVEPKSCGGGGSGGGGSGGGGSGGGGSQVQLVQSGAEVKKPGASVKVSCKASGYTFAGFEMHWVRQAPGQGLEWMGAIDPKTGGTDYNQKFKDRVTMTRDTSISTAYMELSRLRSDDTAVYYCARDLGYFDVWGQGTLVTVSSGGGGSDKTHTCPPCPAPEAAGPSVFLFPPKPKDTLMISRTPEVTCVVVDVSHEDPEVKFNWYVDGVEVHNAKTKPREEQYNSTYRVVSVLTVLHQDWLNGKEYKCKVSNKALPAPIEKTISKAKGQPREPQVYTLPPSREEMTKNQVSLWCLVKGFYPSDIAVEWESNGQPENNYKTTPPVLDSDGSFFLYSKLTVDKSRWQQGNVFSCSVMHEALHNHYTQKSLSLSPGGGGGSGGGGSGGGGSGGGGSQVQLVQSGAEVKKPGASVKVSCKASGYTFTGYYMHWVRQAPGQGLEWMGWINPDSGGTNYAQKFQGRVTMTRDTSISTAYMELNRLRSDDTAVYYCARDQPLGYCTNGVCSYFDYWGQGTLVTVSS

SEQ ID NO: 176 - protein, 729 aa, synthetic construct
EVQLVESGGGLVQPGGSLRLSCAASGFTFSDSWIHWVRQAPGKGLEWVAWISPYGGSTYYADSVKGRFTISADTSKNTAYLQMNSLRAEDTAVYYCARRHWPGGFDYWGQGTLVTVSSASTKGPSVFPLAPSSKSTSGGTAALGCLVKDYFPEPVTVSWNSGALTSGVHTFPAVLQSSGLYSLSSVVTVPSSSLGTQTYICNVNHKPSNTKVDKKVEPKSCGGGGSGGGGSGGGGSGGGGSQVQLVQSGAEVKKPGASVKVSCKASGYTFAGFEMHWVRQAPGQGLEWMGAIDPKTGGTDYNQKFKDRVTMTRDTSISTAYMELSRLRSDDTAVYYCARDLGYFDVWGQGTLVTVSSGGGGSDKTHTCPPCPAPEAAGPSVFLFPPKPKDTLMISRTPEVTCVVVDVSHEDPEVKFNWYVDGVEVHNAKTKPREEQYNSTYRVVSVLTVLHQDWLNGKEYKCKVSNKALPAPIEKTISKAKGQPREPQVYTLPPSREEMTKNQVSLWCLVKGFYPSDIAVEWESNGQPENNYKTTPPVLDSDGSFFLYSKLTVDKSRWQQGNVFSCSVMHEALHNHYTQKSLSLSPGGGGGSGGGGSGGGGSGGGGSEVQLVESGGGLVQPGGSLRLSCAASGFTFTNYGLHWVRQAPGKGLEWVSSISPSGGVTYYRDSVKGRFTISRDNSKNTLYLQMNSLRAEDTAVYYCAKPFLGWGGANWIAHWGQGTLVTVSS

SEQ ID NO: 177 - protein, 587 aa, synthetic construct
EVQLVESGGGLVQPGGSLRLSCAASGFTFSDSWIHWVRQAPGKGLEWVAWISPYGGSTYYADSVKGRFTISADTSKNTAYLQMNSLRAEDTAVYYCARRHWPGGFDYWGQGTLVTVSSASTKGPSVFPLAPSSKSTSGGTAALGCLVKDYFPEPVTVSWNSGALTSGVHTFPAVLQSSGLYSLSSVVTVPSSSLGTQTYICNVNHKPSNTKVDKKVEPKSCGGGGSGGGGSGGGGSGGGGSQVQLVQSGAEVKKPGASVKVSCKASGYTFAGFEMHWVRQAPGQGLEWMGAIDPKTGGTDYNQKFKDRVTMTRDTSISTAYMELSRLRSDDTAVYYCARDLGYFDVWGQGTLVTVSSGGGGSDKTHTCPPCPAPEAAGPSVFLFPPKPKDTLMISRTPEVTCVVVDVSHEDPEVKFNWYVDGVEVHNAKTKPREEQYNSTYRVVSVLTVLHQDWLNGKEYKCKVSNKALPAPIEKTISKAKGQPREPQVYTLPPSREEMTKNQVSLWCLVKGFYPSDIAVEWESNGQPENNYKTTPPVLDSDGSFFLYSKLTVDKSRWQQGNVFSCSVMHEALHNHYTQKSLSLSPG

SEQ ID NO: 178 - protein, 583 aa, synthetic construct
EVQLVESGGGLVQPGGSLRLSCAASGFTFTDYTMDWVRQAPGKGLEWVADVNPNSGGSIYNQRFKGRFTLSVDRSKNTLYLQMNSLRAEDTAVYYCARNLGPSFYFDYWGQGTLVTVSSASTKGPSVFPLAPSSKSTSGGTAALGCLVKDYFPEPVTVSWNSGALTSGVHTFPAVLQSSGLYSLSSVVTVPSSSLGTQTYICNVNHKPSNTKVDKKVEPKSCDKTHTCPPCPAPEAAGPSVFLFPPKPKDTLMISRTPEVTCVVVDVSHEDPEVKFNWYVDGVEVHNAKTKPREEQYNSTYRVVSVLTVLHQDWLNGKEYKCKVSNKALPAPIEKTISKAKGQPREPQVYTLPPSREEMTKNQVSLWCLVKGFYPSDIAVEWESNGQPENNYKTTPPVLDSDGSFFLYSKLTVDKSRWQQGNVFSCSVMHEALHNHYTQKSLSLSPGGGGGSGGGGSGGGGSGGGGSQVQLVQSGAEVKKPGASVKVSCKASGYTFAGFEMHWVRQAPGQGLEWMGAIDPKTGGTDYNQKFKDRVTMTRDTSISTAYMELSRLRSDDTAVYYCARDLGYFDVWGQGTLVTVSS

SEQ ID NO: 179 - protein, 574 aa, synthetic construct
EVQLVESGGGLVQPGGSLRLSCAASGFTFTDYTMDWVRQAPGKGLEWVADVNPNSGGSIYNQRFKGRFTLSVDRSKNTLYLQMNSLRAEDTAVYYCARNLGPSFYFDYWGQGTLVTVSSASTKGPSVFPLAPSSKSTSGGTAALGCLVKDYFPEPVTVSWNSGALTSGVHTFPAVLQSSGLYSLSSVVTVPSSSLGTQTYICNVNHKPSNTKVDKKVEPKSCDKTHTCPPCPAPEAAGPSVFLFPPKPKDTLMISRTPEVTCVVVDVSHEDPEVKFNWYVDGVEVHNAKTKPREEQYNSTYRVVSVLTVLHQDWLNGKEYKCKVSNKALPAPIEKTISKAKGQPREPQVYTLPPSREEMTKNQVSLSCAVKGFYPSDIAVEWESNGQPENNYKTTPPVLDSDGSFFLVSKLTVDKSRWQQGNVFSCSVMHEALHNRFTQKSLSLSPGGGGGSGGGGSGGGGSGGGGSDIQMTQSPSSLSASVGDRVTITCRASQDIRSNLNWYQQKPGGAVKLLIYYTSRLHSGVPSRFSGSGSGTDYTLTISSLQPEDFATYFCQQSEKLPRTFGGGTKVEIR

SEQ ID NO: 180 - protein, 733 aa, synthetic construct
EVQLVESGGGLVQPGGSLRLSCAASGFTFTDYTMDWVRQAPGKGLEWVADVNPNSGGSIYNQRFKGRFTLSVDRSKNTLYLQMNSLRAEDTAVYYCARNLGPSFYFDYWGQGTLVTVSSASTKGPSVFPLAPSSKSTSGGTAALGCLVKDYFPEPVTVSWNSGALTSGVHTFPAVLQSSGLYSLSSVVTVPSSSLGTQTYICNVNHKPSNTKVDKKVEPKSCGGGGSGGGGSGGGGSGGGGSEVQLVESGGGLVQPGGSLRLSCAASGFTFSTYAMNWVRQAPGKGLEWVGRIRSKYNNYATYYADSVKGRFTISRDDSKNSLYLQMNSLKTEDTAVYYCVRHGNFGNSYVSWFAYWGQGTLVTVSSGGGGSDKTHTCPPCPAPEAAGPSVFLFPPKPKDTLMISRTPEVTCVVVDVSHEDPEVKFNWYVDGVEVHNAKTKPREEQYNSTYRVVSVLTVLHQDWLNGKEYKCKVSNKALPAPIEKTISKAKGQPREPQVYTLPPSREEMTKNQVSLWCLVKGFYPSDIAVEWESNGQPENNYKTTPPVLDSDGSFFLYSKLTVDKSRWQQGNVFSCSVMHEALHNHYTQKSLSLSPGGGGGSGGGGSGGGGSGGGGSQVQLVQSGAEVKKPGASVKVSCKASGYTFAGFEMHWVRQAPGQGLEWMGAIDPKTGGTDYNQKFKDRVTMTRDTSISTAYMELSRLRSDDTAVYYCARDLGYFDVWGQGTLVTVSS

SEQ ID NO: 181 - protein, 597 aa, synthetic construct
EVQLVESGGGLVQPGGSLRLSCAASGFTFTDYTMDWVRQAPGKGLEWVADVNPNSGGSIYNQRFKGRFTLSVDRSKNTLYLQMNSLRAEDTAVYYCARNLGPSFYFDYWGQGTLVTVSSASTKGPSVFPLAPSSKSTSGGTAALGCLVKDYFPEPVTVSWNSGALTSGVHTFPAVLQSSGLYSLSSVVTVPSSSLGTQTYICNVNHKPSNTKVDKKVEPKSCGGGGSGGGGSGGGGSGGGGSEVQLVESGGGLVQPGGSLRLSCAASGFTFSTYAMNWVRQAPGKGLEWVGRIRSKYNNYATYYADSVKGRFTISRDDSKNSLYLQMNSLKTEDTAVYYCVRHGNFGNSYVSWFAYWGQGTLVTVSSGGGGSDKTHTCPPCPAPEAAGPSVFLFPPKPKDTLMISRTPEVTCVVVDVSHEDPEVKFNWYVDGVEVHNAKTKPREEQYNSTYRVVSVLTVLHQDWLNGKEYKCKVSNKALPAPIEKTISKAKGQPREPQVYTLPPSREEMTKNQVSLWCLVKGFYPSDIAVEWESNGQPENNYKTTPPVLDSDGSFFLYSKLTVDKSRWQQGNVFSCSVMHEALHNHYTQKSLSLSPG

SEQ ID NO: 182 - protein, 708 aa, synthetic construct
EVQLVESGGGLVQPGGSLRLSCAASGFTFTDYTMDWVRQAPGKGLEWVADVNPNSGGSIYNQRFKGRFTLSVDRSKNTLYLQMNSLRAEDTAVYYCARNLGPSFYFDYWGQGTLVTVSSASTKGPSVFPLAPSSKSTSGGTAALGCLVKDYFPEPVTVSWNSGALTSGVHTFPAVLQSSGLYSLSSVVTVPSSSLGTQTYICNVNHKPSNTKVDKKVEPKSCGGGGSGGGGSGGGGSGGGGSQAVVTQEPSLTVSPGGTVTLTCRSSTGAVTTSNYANWVQQKPGQAPRGLIGGTNKRAPWTPARFSGSLLGGKAALTITGAQAEDEADYYCALWYSNLWVFGGGTKLTVLGGGGSDKTHTCPPCPAPEAAGPSVFLFPPKPKDTLMISRTPEVTCVVVDVSHEDPEVKFNWYVDGVEVHNAKTKPREEQYNSTYRVVSVLTVLHQDWLNGKEYKCKVSNKALPAPIEKTISKAKGQPREPQVYTLPPSREEMTKNQVSLSCAVKGFYPSDIAVEWESNGQPENNYKTTPPVLDSDGSFFLVSKLTVDKSRWQQGNVFSCSVMHEALHNRFTQKSLSLSPGGGGGSGGGGSGGGGSGGGGSDIQMTQSPSSLSASVGDRVTITCRASQDIRSNLNWYQQKPGGAVKLLIYYTSRLHSGVPSRFSGSGSGTDYTLTISSLQPEDFATYFCQQSEKLPRTFGGGTKVEIR

SEQ ID NO: 183 - protein, 581 aa, synthetic construct
EVQLVESGGGLVQPGGSLRLSCAASGFTFTDYTMDWVRQAPGKGLEWVADVNPNSGGSIYNQRFKGRFTLSVDRSKNTLYLQMNSLRAEDTAVYYCARNLGPSFYFDYWGQGTLVTVSSASTKGPSVFPLAPSSKSTSGGTAALGCLVKDYFPEPVTVSWNSGALTSGVHTFPAVLQSSGLYSLSSVVTVPSSSLGTQTYICNVNHKPSNTKVDKKVEPKSCGGGGSGGGGSGGGGSGGGGSQAVVTQEPSLTVSPGGTVTLTCRSSTGAVTTSNYANWVQQKPGQAPRGLIGGTNKRAPWTPARFSGSLLGGKAALTITGAQAEDEADYYCALWYSNLWVFGGGTKLTVLGGGGSDKTHTCPPCPAPEAAGPSVFLFPPKPKDTLMISRTPEVTCVVVDVSHEDPEVKFNWYVDGVEVHNAKTKPREEQYNSTYRVVSVLTVLHQDWLNGKEYKCKVSNKALPAPIEKTISKAKGQPREPQVYTLPPSREEMTKNQVSLSCAVKGFYPSDIAVEWESNGQPENNYKTTPPVLDSDGSFFLVSKLTVDKSRWQQGNVFSCSVMHEALHNRFTQKSLSLSPG

SEQ ID NO: 184 - protein, 709 aa, synthetic construct
EVQLVESGGGLVQPGGSLRLSCAASGFTFTDYTMDWVRQAPGKGLEWVADVNPNSGGSIYNQRFKGRFTLSVDRSKNTLYLQMNSLRAEDTAVYYCARNLGPSFYFDYWGQGTLVTVSSASTKGPSVFPLAPSSKSTSGGTAALGCLVKDYFPEPVTVSWNSGALTSGVHTFPAVLQSSGLYSLSSVVTVPSSSLGTQTYICNVNHKPSNTKVDKKVEPKSCGGGGSGGGGSGGGGSGGGGSQAVVTQEPSLTVSPGGTVTLTCRSSTGAVTTSNYANWVQQKPGQAPRGLIGGTNKRAPWTPARFSGSLLGGKAALTITGAQAEDEADYYCALWYSNLWVFGGGTKLTVLGGGGSDKTHTCPPCPAPELLGPSVFLFPPKPKDTLMISRTPEVTCVVVDVSHEDPEVKFNWYVDGVEVHNAKTKPREEQYNSTYRVVSVLTVLHQDWLNGKEYKCKVSNKALGAPIEKTISKAKGQPREPQVYTLPPSREEMTKNQVSLSCAVKGFYPSDIAVEWESNGQPENNYKTTPPVLDSDGSFFLVSKLTVDKSRWQQGNVFSCSVMHEALHNRFTQKSLSLSPGKGGGGSGGGGSGGGGSGGGGSDIQMTQSPSSLSASVGDRVTITCHASQNIYVWLNWYQQKPGKAPKLLIYKASNLHTGVPSRFSGSGSGTDFTLTISSLQPEDFATYYCQQGQTYPYTFGGGTKVEIK

SEQ ID NO: 185 - protein, 587 aa, synthetic construct
EVQLVESGGGLVQPGGSLRLSCAASGFTFTDYTMDWVRQAPGKGLEWVADVNPNSGGSIYNQRFKGRFTLSVDRSKNTLYLQMNSLRAEDTAVYYCARNLGPSFYFDYWGQGTLVTVSSASVAAPSVFIFPPSDEQLKSGTASVVCLLNNFYPREAKVQWKVDNALQSGNSQESVTEQDSKDSTYSLSSTLTLSKADYEKHKVYACEVTHQGLSSPVTKSFNRGECDKTHTCPPCPAPEAAGPSVFLFPPKPKDTLMISRTPEVTCVVVDVSHEDPEVKFNWYVDGVEVHNAKTKPREEQYNSTYRVVSVLTVLHQDWLNGKEYKCKVSNKALPAPIEKTISKAKGQPREPQVYTLPPSREEMTKNQVSLWCLVKGFYPSDIAVEWESNGQPENNYKTTPPVLDSDGSFFLYSKLTVDKSRWQQGNVFSCSVMHEALHNHYTQKSLSLSPGGGGGSGGGGSGGGGSGGGGSQVQLVQSGAEVKKPGASVKVSCKASGYTFAGFEMHWVRQAPGQGLEWMGAIDPKTGGTDYNQKFKDRVTMTRDTSISTAYMELSRLRSDDTAVYYCARDLGYFDVWGQGTLVTVSS

SEQ ID NO: 186 - protein, 737 aa, synthetic construct
EVQLVESGGGLVQPGGSLRLSCAASGFTFTDYTMDWVRQAPGKGLEWVADVNPNSGGSIYNQRFKGRFTLSVDRSKNTLYLQMNSLRAEDTAVYYCARNLGPSFYFDYWGQGTLVTVSSASVAAPSVFIFPPSDEQLKSGTASVVCLLNNFYPREAKVQWKVDNALQSGNSQESVTEQDSKDSTYSLSSTLTLSKADYEKHKVYACEVTHQGLSSPVTKSFNRGECGGGGSGGGGSGGGGSGGGGSEVQLVESGGGLVQPGGSLRLSCAASGFTFSTYAMNWVRQAPGKGLEWVGRIRSKYNNYATYYADSVKGRFTISRDDSKNSLYLQMNSLKTEDTAVYYCVRHGNFGNSYVSWFAYWGQGTLVTVSSGGGGSDKTHTCPPCPAPEAAGPSVFLFPPKPKDTLMISRTPEVTCVVVDVSHEDPEVKFNWYVDGVEVHNAKTKPREEQYNSTYRVVSVLTVLHQDWLNGKEYKCKVSNKALPAPIEKTISKAKGQPREPQVYTLPPSREEMTKNQVSLWCLVKGFYPSDIAVEWESNGQPENNYKTTPPVLDSDGSFFLYSKLTVDKSRWQQGNVFSCSVMHEALHNHYTQKSLSLSPGGGGGSGGGGSGGGGSGGGGSQVQLVQSGAEVKKPGASVKVSCKASGYTFAGFEMHWVRQAPGQGLEWMGAIDPKTGGTDYNQKFKDRVTMTRDTSISTAYMELSRLRSDDTAVYYCARDLGYFDVWGQGTLVTVSS

SEQ ID NO: 187 - protein, 601 aa, synthetic construct
EVQLVESGGGLVQPGGSLRLSCAASGFTFTDYTMDWVRQAPGKGLEWVADVNPNSGGSIYNQRFKGRFTLSVDRSKNTLYLQMNSLRAEDTAVYYCARNLGPSFYFDYWGQGTLVTVSSASVAAPSVFIFPPSDEQLKSGTASVVCLLNNFYPREAKVQWKVDNALQSGNSQESVTEQDSKDSTYSLSSTLTLSKADYEKHKVYACEVTHQGLSSPVTKSFNRGECGGGGSGGGGSGGGGSGGGGSEVQLVESGGGLVQPGGSLRLSCAASGFTFSTYAMNWVRQAPGKGLEWVGRIRSKYNNYATYYADSVKGRFTISRDDSKNSLYLQMNSLKTEDTAVYYCVRHGNFGNSYVSWFAYWGQGTLVTVSSGGGGSDKTHTCPPCPAPEAAGPSVFLFPPKPKDTLMISRTPEVTCVVVDVSHEDPEVKFNWYVDGVEVHNAKTKPREEQYNSTYRVVSVLTVLHQDWLNGKEYKCKVSNKALPAPIEKTISKAKGQPREPQVYTLPPSREEMTKNQVSLWCLVKGFYPSDIAVEWESNGQPENNYKTTPPVLDSDGSFFLYSKLTVDKSRWQQGNVFSCSVMHEALHNHYTQKSLSLSPG

SEQ ID NO: 188 - protein, 742 aa, synthetic construct
EVQLVESGGGLVQPGGSLRLSCAASGFTFTDYTMDWVRQAPGKGLEWVADVNPNSGGSIYNQRFKGRFTLSVDRSKNTLYLQMNSLRAEDTAVYYCARNLGPSFYFDYWGQGTLVTVSSASVAAPSVFIFPPSDEQLKSGTASVVCLLNNFYPREAKVQWKVDNALQSGNSQESVTEQDSKDSTYSLSSTLTLSKADYEKHKVYACEVTHQGLSSPVTKSFNRGECGGGGSGGGGSGGGGSGGGGSEVQLVESGGGLVQPGGSLRLSCAASGFTFSTYAMNWVRQAPGKGLEWVGRIRSKYNNYATYYADSVKGRFTISRDDSKNSLYLQMNSLKTEDTAVYYCVRHGNFGNSYVSWFAYWGQGTLVTVSSGGGGSDKTHTCPPCPAPELLGPSVFLFPPKPKDTLMISRTPEVTCVVVDVSHEDPEVKFNWYVDGVEVHNAKTKPREEQYNSTYRVVSVLTVLHQDWLNGKEYKCKVSNKALGAPIEKTISKAKGQPREPQVYTLPPSREEMTKNQVSLWCLVKGFYPSDIAVEWESNGQPENNYKTTPPVLDSDGSFFLYSKLTVDKSRWQQGNVFSCSVMHEALHNHYTQKSLSLSPGKGGGGSGGGGSGGGGSGGGGSQVQLVQSGAEVKKPGASVKVSCKASGYTFTSYYIHWVRQAPGQGLEWIGCIYPGNVNTNYNEKFKDRATLTVDTSISTAYMELSRLRSDDTAVYFCTRSHYGLDWNFDVWGQGTTVTVSS

SEQ ID NO: 189 - protein, 602 aa, synthetic construct
EVQLVESGGGLVQPGGSLRLSCAASGFTFTDYTMDWVRQAPGKGLEWVADVNPNSGGSIYNQRFKGRFTLSVDRSKNTLYLQMNSLRAEDTAVYYCARNLGPSFYFDYWGQGTLVTVSSASVAAPSVFIFPPSDEQLKSGTASVVCLLNNFYPREAKVQWKVDNALQSGNSQESVTEQDSKDSTYSLSSTLTLSKADYEKHKVYACEVTHQGLSSPVTKSFNRGECGGGGSGGGGSGGGGSGGGGSEVQLVESGGGLVQPGGSLRLSCAASGFTFSTYAMNWVRQAPGKGLEWVGRIRSKYNNYATYYADSVKGRFTISRDDSKNSLYLQMNSLKTEDTAVYYCVRHGNFGNSYVSWFAYWGQGTLVTVSSGGGGSDKTHTCPPCPAPELLGPSVFLFPPKPKDTLMISRTPEVTCVVVDVSHEDPEVKFNWYVDGVEVHNAKTKPREEQYNSTYRVVSVLTVLHQDWLNGKEYKCKVSNKALGAPIEKTISKAKGQPREPQVYTLPPSREEMTKNQVSLWCLVKGFYPSDIAVEWESNGQPENNYKTTPPVLDSDGSFFLYSKLTVDKSRWQQGNVFSCSVMHEALHNHYTQKSLSLSPGK

SEQ ID NO: 190 - protein, 452 aa, synthetic construct
EVQLVESGGGLVQPGGSLRLSCAASGYTFTSYNMHWVRQAPGKGLEWVGAIYPGNGDTSYNQKFKGRFTISVDKSKNTLYLQMNSLRAEDTAVYYCARVVYYSNSYWYFDVWGQGTLVTVSSASTKGPSVFPLAPSSKSTSGGTAALGCLVKDYFPEPVTVSWNSGALTSGVHTFPAVLQSSGLYSLSSVVTVPSSSLGTQTYICNVNHKPSNTKVDKKVEPKSCDKTHTCPPCPAPELLGGPSVFLFPPKPKDTLMISRTPEVTCVVVDVSHEDPEVKFNWYVDGVEVHNAKTKPREEQYGSTYRVVSVLTVLHQDWLNGKEYKCKVSNKALPAPIEKTISKAKGQPREPQVYTLPPSREEMTKNQVSLWCLVKGFYPSDIAVEWESNGQPENNYKTTPPVLDSDGSFFLYSKLTVDKSRWQQGNVFSCSVMHEALHNHYTQKSLSLSPGK

SEQ ID NO: 191 - protein, 592 aa, synthetic construct
EVQLVESGGGLVQPGGSLRLSCAASGYTFTSYWLHWVRQAPGKGLEWVGMIDPSNSDTRFNPNFKDRFTISADTSKNTAYLQMNSLRAEDTAVYYCATYRSYVTPLDYWGQGTLVTVSSASVAAPSVFIFPPSDEQLKSGTASVVCLLNNFYPREAKVQWKVDNALQSGNSQESVTEQDSKDSTYSLSSTLTLSKADYEKHKVYACEVTHQGLSSPVTKSFNRGECDKTHTCPPCPAPELLGGPDVFLFPPKPKDTLMISRTPEVTCVVVDVSHEDPEVKFNWYVDGVEVHNAKTKPREEQYNSTYRVVSVLTVLHQDWLNGKEYKCKVSNKALPLPEEKTISKAKGQPREPQVYTLPPSRDELTKNQVSLWCLVKGFYPSDIAVEWESNGQPENNYKTTPPVLDSDGSFFLYSKLTVDKSRWQQGNVFSCSVMHEALHNHYTQKSLSLSPGKGGGGSGGGGSGGGGSGGGGSEVQLLESGGGLVQPGGSLRLSCAASGFTFSNFAMSWVRQAPGKGLEWVSTISASGGRTFYADSVKGRITISRDNSKNTLFLQMNGLRAEDTAVYYCAKEGSFGEGVDPWGQGTLVTVSS

SEQ ID NO: 192 - protein, 597 aa, synthetic construct
EVQLVESGGGLVQPGGSLRLSCAASGYTFTSYWLHWVRQAPGKGLEWVGMIDPSNSDTRFNPNFKDRFTISADTSKNTAYLQMNSLRAEDTAVYYCATYRSYVTPLDYWGQGTLVTVSSASVAAPSVFIFPPSDEQLKSGTASVVCLLNNFYPREAKVQWKVDNALQSGNSQESVTEQDSKDSTYSLSSTLTLSKADYEKHKVYACEVTHQGLSSPVTKSFNRGECGGGGSGGGGSGGGGSGGGGSEVQLLESGGGLVQPGGSLRLSCAASGFTFSNFAMSWVRQAPGKGLEWVSTISASGGRTFYADSVKGRITISRDNSKNTLFLQMNGLRAEDTAVYYCAKEGSFGEGVDPWGQGTLVTVSSGGGGSDKTHTCPPCPAPELLGGPDVFLFPPKPKDTLMISRTPEVTCVVVDVSHEDPEVKFNWYVDGVEVHNAKTKPREEQYNSTYRVVSVLTVLHQDWLNGKEYKCKVSNKALPLPEEKTISKAKGQPREPQVYTLPPSRDELTKNQVSLWCLVKGFYPSDIAVEWESNGQPENNYKTTPPVLDSDGSFFLYSKLTVDKSRWQQGNVFSCSVMHEALHNHYTQKSLSLSPGK

SEQ ID NO: 193 - protein, 583 aa, synthetic construct
EVQLVESGGGVVQPGRSLRLSCSASGFDFTTYWMSWVRQAPGKGLEWIGEIHPDSSTINYAPSLKDRFTISRDNAKNTLFLQMDSLRPEDTGVYFCASLYFGFPWFAYWGQGTPVTVSSASTKGPSVFPLAPSSKSTSGGTAALGCLVKDYFPEPVTVSWNSGALTSGVHTFPAVLQSSGLYSLSSVVTVPSSSLGTQTYICNVNHKPSNTKVDKKVEPKSCDKTHTCPPCPAPEAAGPSVFLFPPKPKDTLMISRTPEVTCVVVDVSHEDPEVKFNWYVDGVEVHNAKTKPREEQYNSTYRVVSVLTVLHQDWLNGKEYKCKVSNKALPAPIEKTISKAKGQPREPQVYTLPPSREEMTKNQVSLWCLVKGFYPSDIAVEWESNGQPENNYKTTPPVLDSDGSFFLYSKLTVDKSRWQQGNVFSCSVMHEALHNHYTQKSLSLSPGGGGGSGGGGSGGGGSGGGGSQVQLVQSGAEVKKPGASVKVSCKASGYTFAGFEMHWVRQAPGQGLEWMGAIDPKTGGTDYNQKFKDRVTMTRDTSISTAYMELSRLRSDDTAVYYCARDLGYFDVWGQGTLVTVSS

SEQ ID NO: 194 - protein, 574 aa, synthetic construct
EVQLVESGGGVVQPGRSLRLSCSASGFDFTTYWMSWVRQAPGKGLEWIGEIHPDSSTINYAPSLKDRFTISRDNAKNTLFLQMDSLRPEDTGVYFCASLYFGFPWFAYWGQGTPVTVSSASTKGPSVFPLAPSSKSTSGGTAALGCLVKDYFPEPVTVSWNSGALTSGVHTFPAVLQSSGLYSLSSVVTVPSSSLGTQTYICNVNHKPSNTKVDKKVEPKSCDKTHTCPPCPAPEAAGPSVFLFPPKPKDTLMISRTPEVTCVVVDVSHEDPEVKFNWYVDGVEVHNAKTKPREEQYNSTYRVVSVLTVLHQDWLNGKEYKCKVSNKALPAPIEKTISKAKGQPREPQVYTLPPSREEMTKNQVSLSCAVKGFYPSDIAVEWESNGQPENNYKTTPPVLDSDGSFFLVSKLTVDKSRWQQGNVFSCSVMHEALHNRFTQKSLSLSPGGGGGSGGGGSGGGGSGGGGSDIQMTQSPSSLSASVGDRVTITCRASQDIRSNLNWYQQKPGGAVKLLIYYTSRLHSGVPSRFSGSGSGTDYTLTISSLQPEDFATYFCQQSEKLPRTFGGGTKVEIR

SEQ ID NO: 195 - protein, 733 aa, synthetic construct
EVQLVESGGGVVQPGRSLRLSCSASGFDFTTYWMSWVRQAPGKGLEWIGEIHPDSSTINYAPSLKDRFTISRDNAKNTLFLQMDSLRPEDTGVYFCASLYFGFPWFAYWGQGTPVTVSSASTKGPSVFPLAPSSKSTSGGTAALGCLVKDYFPEPVTVSWNSGALTSGVHTFPAVLQSSGLYSLSSVVTVPSSSLGTQTYICNVNHKPSNTKVDKKVEPKSCGGGGSGGGGSGGGGSGGGGSEVQLVESGGGLVQPGGSLRLSCAASGFTFSTYAMNWVRQAPGKGLEWVGRIRSKYNNYATYYADSVKGRFTISRDDSKNSLYLQMNSLKTEDTAVYYCVRHGNFGNSYVSWFAYWGQGTLVTVSSGGGGSDKTHTCPPCPAPEAAGPSVFLFPPKPKDTLMISRTPEVTCVVVDVSHEDPEVKFNWYVDGVEVHNAKTKPREEQYNSTYRVVSVLTVLHQDWLNGKEYKCKVSNKALPAPIEKTISKAKGQPREPQVYTLPPSREEMTKNQVSLWCLVKGFYPSDIAVEWESNGQPENNYKTTPPVLDSDGSFFLYSKLTVDKSRWQQGNVFSCSVMHEALHNHYTQKSLSLSPGGGGGSGGGGSGGGGSGGGGSQVQLVQSGAEVKKPGASVKVSCKASGYTFAGFEMHWVRQAPGQGLEWMGAIDPKTGGTDYNQKFKDRVTMTRDTSISTAYMELSRLRSDDTAVYYCARDLGYFDVWGQGTLVTVSS

SEQ ID NO: 196 - protein, 597 aa, synthetic construct
EVQLVESGGGVVQPGRSLRLSCSASGFDFTTYWMSWVRQAPGKGLEWIGEIHPDSSTINYAPSLKDRFTISRDNAKNTLFLQMDSLRPEDTGVYFCASLYFGFPWFAYWGQGTPVTVSSASTKGPSVFPLAPSSKSTSGGTAALGCLVKDYFPEPVTVSWNSGALTSGVHTFPAVLQSSGLYSLSSVVTVPSSSLGTQTYICNVNHKPSNTKVDKKVEPKSCGGGGSGGGGSGGGGSGGGGSEVQLVESGGGLVQPGGSLRLSCAASGFTFSTYAMNWVRQAPGKGLEWVGRIRSKYNNYATYYADSVKGRFTISRDDSKNSLYLQMNSLKTEDTAVYYCVRHGNFGNSYVSWFAYWGQGTLVTVSSGGGGSDKTHTCPPCPAPEAAGPSVFLFPPKPKDTLMISRTPEVTCVVVDVSHEDPEVKFNWYVDGVEVHNAKTKPREEQYNSTYRVVSVLTVLHQDWLNGKEYKCKVSNKALPAPIEKTISKAKGQPREPQVYTLPPSREEMTKNQVSLWCLVKGFYPSDIAVEWESNGQPENNYKTTPPVLDSDGSFFLYSKLTVDKSRWQQGNVFSCSVMHEALHNHYTQKSLSLSPG

SEQ ID NO: 197 - protein, 708 aa, synthetic construct
EVQLVESGGGVVQPGRSLRLSCSASGFDFTTYWMSWVRQAPGKGLEWIGEIHPDSSTINYAPSLKDRFTISRDNAKNTLFLQMDSLRPEDTGVYFCASLYFGFPWFAYWGQGTPVTVSSASTKGPSVFPLAPSSKSTSGGTAALGCLVKDYFPEPVTVSWNSGALTSGVHTFPAVLQSSGLYSLSSVVTVPSSSLGTQTYICNVNHKPSNTKVDKKVEPKSCGGGGSGGGGSGGGGSGGGGSQAVVTQEPSLTVSPGGTVTLTCRSSTGAVTTSNYANWVQQKPGQAPRGLIGGTNKRAPWTPARFSGSLLGGKAALTITGAQAEDEADYYCALWYSNLWVFGGGTKLTVLGGGGSDKTHTCPPCPAPEAAGPSVFLFPPKPKDTLMISRTPEVTCVVVDVSHEDPEVKFNWYVDGVEVHNAKTKPREEQYNSTYRVVSVLTVLHQDWLNGKEYKCKVSNKALPAPIEKTISKAKGQPREPQVYTLPPSREEMTKNQVSLSCAVKGFYPSDIAVEWESNGQPENNYKTTPPVLDSDGSFFLVSKLTVDKSRWQQGNVFSCSVMHEALHNRFTQKSLSLSPGGGGGSGGGGSGGGGSGGGGSDIQMTQSPSSLSASVGDRVTITCRASQDIRSNLNWYQQKPGGAVKLLIYYTSRLHSGVPSRFSGSGSGTDYTLTISSLQPEDFATYFCQQSEKLPRTFGGGTKVEIR

SEQ ID NO: 198 - protein, 581 aa, synthetic construct
EVQLVESGGGVVQPGRSLRLSCSASGFDFTTYWMSWVRQAPGKGLEWIGEIHPDSSTINYAPSLKDRFTISRDNAKNTLFLQMDSLRPEDTGVYFCASLYFGFPWFAYWGQGTPVTVSSASTKGPSVFPLAPSSKSTSGGTAALGCLVKDYFPEPVTVSWNSGALTSGVHTFPAVLQSSGLYSLSSVVTVPSSSLGTQTYICNVNHKPSNTKVDKKVEPKSCGGGGSGGGGSGGGGSGGGGSQAVVTQEPSLTVSPGGTVTLTCRSSTGAVTTSNYANWVQQKPGQAPRGLIGGTNKRAPWTPARFSGSLLGGKAALTITGAQAEDEADYYCALWYSNLWVFGGGTKLTVLGGGGSDKTHTCPPCPAPEAAGPSVFLFPPKPKDTLMISRTPEVTCVVVDVSHEDPEVKFNWYVDGVEVHNAKTKPREEQYNSTYRVVSVLTVLHQDWLNGKEYKCKVSNKALPAPIEKTISKAKGQPREPQVYTLPPSREEMTKNQVSLSCAVKGFYPSDIAVEWESNGQPENNYKTTPPVLDSDGSFFLVSKLTVDKSRWQQGNVFSCSVMHEALHNRFTQKSLSLSPG

SEQ ID NO: 199 - protein, 449 aa, synthetic construct
EVQLVQSGAEVKKPGASVKVSCKASGYTFTNYYIHWVRQAPGQGLEWIGWIYPGDGNTKYNEKFKGRATLTADTSTSTAYLELSSLRSEDTAVYYCARDSYSNYYFDYWGQGTLVTVSSASTKGPSVFPLAPSSKSTSGGTAALGCLVKDYFPEPVTVSWNSGALTSGVHTFPAVLQSSGLYSLSSVVTVPSSSLGTQTYICNVNHKPSNTKVDKKVEPKSCDKTHTCPPCPAPELLGGPSVFLFPPKPKDTLMISRTPEVTCVVVDVSHEDPEVKFNWYVDGVEVHNAKTKPREEQYGSTYRVVSVLTVLHQDWLNGKEYKCKVSNKALPAPIEKTISKAKGQPREPQVYTLPPSREEMTKNQVSLSCAVKGFYPSDIAVEWESNGQPENNYKTTPPVLDSDGSFFLVSKLTVDKSRWQQGNVFSCSVMHEALHNHYTQKSLSLSPGK

SEQ ID NO: 200 - protein, 579 aa, synthetic construct
EVQLVQSGPEVKKPGATVKISCKTSGYTFTEYTIHWVKQAPGKGLEWIGNINPNNGGTTYNQKFEDKATLTVDKSTDTAYMELSSLRSEDTAVYYCAAGWNFDYWGQGTLLTVSSASTKGPSVFPLAPSSKSTSGGTAALGCLVKDYFPEPVTVSWNSGALTSGVHTFPAVLQSSGLYSLSSVVTVPSSSLGTQTYICNVNHKPSNTKVDKKVEPKSCDKTHTCPPCPAPEAAGPSVFLFPPKPKDTLMISRTPEVTCVVVDVSHEDPEVKFNWYVDGVEVHNAKTKPREEQYNSTYRVVSVLTVLHQDWLNGKEYKCKVSNKALPAPIEKTISKAKGQPREPQVYTLPPSREEMTKNQVSLWCLVKGFYPSDIAVEWESNGQPENNYKTTPPVLDSDGSFFLYSKLTVDKSRWQQGNVFSCSVMHEALHNHYTQKSLSLSPGGGGGSGGGGSGGGGSGGGGSQVQLVQSGAEVKKPGASVKVSCKASGYTFAGFEMHWVRQAPGQGLEWMGAIDPKTGGTDYNQKFKDRVTMTRDTSISTAYMELSRLRSDDTAVYYCARDLGYFDVWGQGTLVTVSS

SEQ ID NO: 201 - protein, 570 aa, synthetic construct
EVQLVQSGPEVKKPGATVKISCKTSGYTFTEYTIHWVKQAPGKGLEWIGNINPNNGGTTYNQKFEDKATLTVDKSTDTAYMELSSLRSEDTAVYYCAAGWNFDYWGQGTLLTVSSASTKGPSVFPLAPSSKSTSGGTAALGCLVKDYFPEPVTVSWNSGALTSGVHTFPAVLQSSGLYSLSSVVTVPSSSLGTQTYICNVNHKPSNTKVDKKVEPKSCDKTHTCPPCPAPEAAGPSVFLFPPKPKDTLMISRTPEVTCVVVDVSHEDPEVKFNWYVDGVEVHNAKTKPREEQYNSTYRVVSVLTVLHQDWLNGKEYKCKVSNKALPAPIEKTISKAKGQPREPQVYTLPPSREEMTKNQVSLSCAVKGFYPSDIAVEWESNGQPENNYKTTPPVLDSDGSFFLVSKLTVDKSRWQQGNVFSCSVMHEALHNRFTQKSLSLSPGGGGGSGGGGSGGGGSGGGGSDIQMTQSPSSLSASVGDRVTITCRASQDIRSNLNWYQQKPGGAVKLLIYYTSRLHSGVPSRFSGSGSGTDYTLTISSLQPEDFATYFCQQSEKLPRTFGGGTKVEIR

SEQ ID NO: 202 - protein, 729 aa, synthetic construct
EVQLVQSGPEVKKPGATVKISCKTSGYTFTEYTIHWVKQAPGKGLEWIGNINPNNGGTTYNQKFEDKATLTVDKSTDTAYMELSSLRSEDTAVYYCAAGWNFDYWGQGTLLTVSSASTKGPSVFPLAPSSKSTSGGTAALGCLVKDYFPEPVTVSWNSGALTSGVHTFPAVLQSSGLYSLSSVVTVPSSSLGTQTYICNVNHKPSNTKVDKKVEPKSCGGGGSGGGGSGGGGSGGGGSEVQLVESGGGLVQPGGSLRLSCAASGFTFSTYAMNWVRQAPGKGLEWVGRIRSKYNNYATYYADSVKGRFTISRDDSKNSLYLQMNSLKTEDTAVYYCVRHGNFGNSYVSWFAYWGQGTLVTVSSGGGGSDKTHTCPPCPAPEAAGPSVFLFPPKPKDTLMISRTPEVTCVVVDVSHEDPEVKFNWYVDGVEVHNAKTKPREEQYNSTYRVVSVLTVLHQDWLNGKEYKCKVSNKALPAPIEKTISKAKGQPREPQVYTLPPSREEMTKNQVSLWCLVKGFYPSDIAVEWESNGQPENNYKTTPPVLDSDGSFFLYSKLTVDKSRWQQGNVFSCSVMHEALHNHYTQKSLSLSPGGGGGSGGGGSGGGGSGGGGSQVQLVQSGAEVKKPGASVKVSCKASGYTFAGFEMHWVRQAPGQGLEWMGAIDPKTGGTDYNQKFKDRVTMTRDTSISTAYMELSRLRSDDTAVYYCARDLGYFDVWGQGTLVTVSS

SEQ ID NO: 203 - protein, 593 aa, synthetic construct
EVQLVQSGPEVKKPGATVKISCKTSGYTFTEYTIHWVKQAPGKGLEWIGNINPNNGGTTYNQKFEDKATLTVDKSTDTAYMELSSLRSEDTAVYYCAAGWNFDYWGQGTLLTVSSASTKGPSVFPLAPSSKSTSGGTAALGCLVKDYFPEPVTVSWNSGALTSGVHTFPAVLQSSGLYSLSSVVTVPSSSLGTQTYICNVNHKPSNTKVDKKVEPKSCGGGGSGGGGSGGGGSGGGGSEVQLVESGGGLVQPGGSLRLSCAASGFTFSTYAMNWVRQAPGKGLEWVGRIRSKYNNYATYYADSVKGRFTISRDDSKNSLYLQMNSLKTEDTAVYYCVRHGNFGNSYVSWFAYWGQGTLVTVSSGGGGSDKTHTCPPCPAPEAAGPSVFLFPPKPKDTLMISRTPEVTCVVVDVSHEDPEVKFNWYVDGVEVHNAKTKPREEQYNSTYRVVSVLTVLHQDWLNGKEYKCKVSNKALPAPIEKTISKAKGQPREPQVYTLPPSREEMTKNQVSLWCLVKGFYPSDIAVEWESNGQPENNYKTTPPVLDSDGSFFLYSKLTVDKSRWQQGNVFSCSVMHEALHNHYTQKSLSLSPG

SEQ ID NO: 204 - protein, 704 aa, synthetic construct
EVQLVQSGPEVKKPGATVKISCKTSGYTFTEYTIHWVKQAPGKGLEWIGNINPNNGGTTYNQKFEDKATLTVDKSTDTAYMELSSLRSEDTAVYYCAAGWNFDYWGQGTLLTVSSASTKGPSVFPLAPSSKSTSGGTAALGCLVKDYFPEPVTVSWNSGALTSGVHTFPAVLQSSGLYSLSSVVTVPSSSLGTQTYICNVNHKPSNTKVDKKVEPKSCGGGGSGGGGSGGGGSGGGGSQAVVTQEPSLTVSPGGTVTLTCRSSTGAVTTSNYANWVQQKPGQAPRGLIGGTNKRAPWTPARFSGSLLGGKAALTITGAQAEDEADYYCALWYSNLWVFGGGTKLTVLGGGGSDKTHTCPPCPAPEAAGPSVFLFPPKPKDTLMISRTPEVTCVVVDVSHEDPEVKFNWYVDGVEVHNAKTKPREEQYNSTYRVVSVLTVLHQDWLNGKEYKCKVSNKALPAPIEKTISKAKGQPREPQVYTLPPSREEMTKNQVSLSCAVKGFYPSDIAVEWESNGQPENNYKTTPPVLDSDGSFFLVSKLTVDKSRWQQGNVFSCSVMHEALHNRFTQKSLSLSPGGGGGSGGGGSGGGGSGGGGSDIQMTQSPSSLSASVGDRVTITCRASQDIRSNLNWYQQKPGGAVKLLIYYTSRLHSGVPSRFSGSGSGTDYTLTISSLQPEDFATYFCQQSEKLPRTFGGGTKVEIR

SEQ ID NO: 205 - protein, 704 aa, synthetic construct
EVQLVQSGPEVKKPGATVKISCKTSGYTFTEYTIHWVKQAPGKGLEWIGNINPNNGGTTYNQKFEDKATLTVDKSTDTAYMELSSLRSEDTAVYYCAAGWNFDYWGQGTLLTVSSASTKGPSVFPLAPSSKSTSGGTAALGCLVKDYFPEPVTVSWNSGALTSGVHTFPAVLQSSGLYSLSSVVTVPSSSLGTQTYICNVNHKPSNTKVDKKVEPKSCGGGGSGGGGSGGGGSGGGGSQAVVTQEPSLTVSPGGTVTLTCRSSTGAVTTSNYANWVQQKPGQAPRGLIGGTNKRAPWTPARFSGSLLGGKAALTITGAQAEDEADYYCALWYSNLWVFGGGTKLTVLGGGGSDKTHTCPPCPAPEAAGPSVFLFPPKPKDTLMISRTPEVTCVVVDVSHEDPEVKFNWYVDGVEVHNAKTKPREEQYNSTYRVVSVLTVLHQDWLNGKEYKCKVSNKALPAPIEKTISKAKGQPREPQVYTLPPSREEMTKNQVSLSCAVKGFYPSDIAVEWESNGQPENNYKTTPPVLDSDGSFFLVSKLTVDKSRWQQGNVFSCSVMHEALHNHYTQKSLSLSPGGGGGSGGGGSGGGGSGGGGSDIQMTQSPSSLSASVGDRVTITCRASQDIRSNLNWYQQKPGGAVKLLIYYTSRLHSGVPSRFSGSGSGTDYTLTISSLQPEDFATYFCQQSEKLPRTFGGGTKVEIR

SEQ ID NO: 206 - protein, 577 aa, synthetic construct
EVQLVQSGPEVKKPGATVKISCKTSGYTFTEYTIHWVKQAPGKGLEWIGNINPNNGGTTYNQKFEDKATLTVDKSTDTAYMELSSLRSEDTAVYYCAAGWNFDYWGQGTLLTVSSASTKGPSVFPLAPSSKSTSGGTAALGCLVKDYFPEPVTVSWNSGALTSGVHTFPAVLQSSGLYSLSSVVTVPSSSLGTQTYICNVNHKPSNTKVDKKVEPKSCGGGGSGGGGSGGGGSGGGGSQAVVTQEPSLTVSPGGTVTLTCRSSTGAVTTSNYANWVQQKPGQAPRGLIGGTNKRAPWTPARFSGSLLGGKAALTITGAQAEDEADYYCALWYSNLWVFGGGTKLTVLGGGGSDKTHTCPPCPAPEAAGPSVFLFPPKPKDTLMISRTPEVTCVVVDVSHEDPEVKFNWYVDGVEVHNAKTKPREEQYNSTYRVVSVLTVLHQDWLNGKEYKCKVSNKALPAPIEKTISKAKGQPREPQVYTLPPSREEMTKNQVSLSCAVKGFYPSDIAVEWESNGQPENNYKTTPPVLDSDGSFFLVSKLTVDKSRWQQGNVFSCSVMHEALHNRFTQKSLSLSPG

SEQ ID NO: 207 - protein, 213 aa, synthetic construct
NIQMTQSPSSLSASVGDRVTITCKAGQNVNNYLAWYQQKPGKAPKVLIFNANSLQTGVPSRFSGSGSGTDFTLTISSLQPEDFATYYCQQYNSWPTFGGGTKVEIKRTVAAPSVFIFPPSDEQLKSGTASVVCLLNNFYPREAKVQWKVDNALQSGNSQESVTEQDSKDSTYSLSSTLTLSKADYEKHKVYACEVTHQGLSSPVTKSFNRGEC

SEQ ID NO: 208 - protein, 213 aa, synthetic construct
QIVLSQSPAILSASPGEKVTMTCRASSSVSYIHWFQQKPGSSPKPWIYATSNLASGVPVRFSGSGSGTSYSLTISRVEAEDAATYYCQQWTSNPPTFGGGTKLEIKRTVAAPSVFIFPPSDEQLKSGTASVVCLLNNFYPREAKVQWKVDNALQSGNSQESVTEQDSKDSTYSLSSTLTLSKADYEKHKVYACEVTHQGLSSPVTKSFNRGEC

SEQ ID NO: 209 - protein, 211 aa, synthetic construct
QIVLSQSPAILSASPGEKVTMTCRASSSVSYIHWFQQKPGSSPKPWIYATSNLASGVPVRFSGSGSGTSYSLTISRVEAEDAATYYCQQWTSNPPTFGGGTKLEIKSSASTKGPSVFPLAPSSKSTSGGTAALGCLVKDYFPEPVTVSWNSGALTSGVHTFPAVLQSSGLYSLSSVVTVPSSSLGTQTYICNVNHKPSNTKVDKKVEPKSC

SEQ ID NO: 210 - protein, 585 aa, synthetic construct
QLQLQESGPGLVKPSETLSLTCTVSGGSISSGSYFWGWIRQPPGKGLEWIGSIYYSGITYYNPSLKSRVTISVDTSKNQFSLKLSSVTAADTAVYYCARHDGAVAGLFDYWGQGTLVTVSSASTKGPSVFPLAPSSKSTSGGTAALGCLVKDYFPEPVTVSWNSGALTSGVHTFPAVLQSSGLYSLSSVVTVPSSSLGTQTYICNVNHKPSNTKVDKKVEPKSCDKTHTCPPCPAPEAAGPSVFLFPPKPKDTLMISRTPEVTCVVVDVSHEDPEVKFNWYVDGVEVHNAKTKPREEQYNSTYRVVSVLTVLHQDWLNGKEYKCKVSNKALPAPIEKTISKAKGQPREPQVYTLPPSREEMTKNQVSLWCLVKGFYPSDIAVEWESNGQPENNYKTTPPVLDSDGSFFLYSKLTVDKSRWQQGNVFSCSVMHEALHNHYTQKSLSLSPGGGGGSGGGGSGGGGSGGGGSQVQLVQSGAEVKKPGASVKVSCKASGYTFAGFEMHWVRQAPGQGLEWMGAIDPKTGGTDYNQKFKDRVTMTRDTSISTAYMELSRLRSDDTAVYYCARDLGYFDVWGQGTLVTVSS

SEQ ID NO: 211 - protein, 576 aa, synthetic construct
QLQLQESGPGLVKPSETLSLTCTVSGGSISSGSYFWGWIRQPPGKGLEWIGSIYYSGITYYNPSLKSRVTISVDTSKNQFSLKLSSVTAADTAVYYCARHDGAVAGLFDYWGQGTLVTVSSASTKGPSVFPLAPSSKSTSGGTAALGCLVKDYFPEPVTVSWNSGALTSGVHTFPAVLQSSGLYSLSSVVTVPSSSLGTQTYICNVNHKPSNTKVDKKVEPKSCDKTHTCPPCPAPEAAGPSVFLFPPKPKDTLMISRTPEVTCVVVDVSHEDPEVKFNWYVDGVEVHNAKTKPREEQYNSTYRVVSVLTVLHQDWLNGKEYKCKVSNKALPAPIEKTISKAKGQPREPQVYTLPPSREEMTKNQVSLSCAVKGFYPSDIAVEWESNGQPENNYKTTPPVLDSDGSFFLVSKLTVDKSRWQQGNVFSCSVMHEALHNRFTQKSLSLSPGGGGGSGGGGSGGGGSGGGGSDIQMTQSPSSLSASVGDRVTITCRASQDIRSNLNWYQQKPGGAVKLLIYYTSRLHSGVPSRFSGSGSGTDYTLTISSLQPEDFATYFCQQSEKLPRTFGGGTKVEIR

SEQ ID NO: 212 - protein, 735 aa, synthetic construct
QLQLQESGPGLVKPSETLSLTCTVSGGSISSGSYFWGWIRQPPGKGLEWIGSIYYSGITYYNPSLKSRVTISVDTSKNQFSLKLSSVTAADTAVYYCARHDGAVAGLFDYWGQGTLVTVSSASTKGPSVFPLAPSSKSTSGGTAALGCLVKDYFPEPVTVSWNSGALTSGVHTFPAVLQSSGLYSLSSVVTVPSSSLGTQTYICNVNHKPSNTKVDKKVEPKSCGGGGSGGGGSGGGGSGGGGSEVQLVESGGGLVQPGGSLRLSCAASGFTFSTYAMNWVRQAPGKGLEWVGRIRSKYNNYATYYADSVKGRFTISRDDSKNSLYLQMNSLKTEDTAVYYCVRHGNFGNSYVSWFAYWGQGTLVTVSSGGGGSDKTHTCPPCPAPEAAGPSVFLFPPKPKDTLMISRTPEVTCVVVDVSHEDPEVKFNWYVDGVEVHNAKTKPREEQYNSTYRVVSVLTVLHQDWLNGKEYKCKVSNKALPAPIEKTISKAKGQPREPQVYTLPPSREEMTKNQVSLWCLVKGFYPSDIAVEWESNGQPENNYKTTPPVLDSDGSFFLYSKLTVDKSRWQQGNVFSCSVMHEALHNHYTQKSLSLSPGGGGGSGGGGSGGGGSGGGGSQVQLVQSGAEVKKPGASVKVSCKASGYTFAGFEMHWVRQAPGQGLEWMGAIDPKTGGTDYNQKFKDRVTMTRDTSISTAYMELSRLRSDDTAVYYCARDLGYFDVWGQGTLVTVSS

SEQ ID NO: 213 - protein, 599 aa, synthetic construct
QLQLQESGPGLVKPSETLSLTCTVSGGSISSGSYFWGWIRQPPGKGLEWIGSIYYSGITYYNPSLKSRVTISVDTSKNQFSLKLSSVTAADTAVYYCARHDGAVAGLFDYWGQGTLVTVSSASTKGPSVFPLAPSSKSTSGGTAALGCLVKDYFPEPVTVSWNSGALTSGVHTFPAVLQSSGLYSLSSVVTVPSSSLGTQTYICNVNHKPSNTKVDKKVEPKSCGGGGSGGGGSGGGGSGGGGSEVQLVESGGGLVQPGGSLRLSCAASGFTFSTYAMNWVRQAPGKGLEWVGRIRSKYNNYATYYADSVKGRFTISRDDSKNSLYLQMNSLKTEDTAVYYCVRHGNFGNSYVSWFAYWGQGTLVTVSSGGGGSDKTHTCPPCPAPEAAGPSVFLFPPKPKDTLMISRTPEVTCVVVDVSHEDPEVKFNWYVDGVEVHNAKTKPREEQYNSTYRVVSVLTVLHQDWLNGKEYKCKVSNKALPAPIEKTISKAKGQPREPQVYTLPPSREEMTKNQVSLWCLVKGFYPSDIAVEWESNGQPENNYKTTPPVLDSDGSFFLYSKLTVDKSRWQQGNVFSCSVMHEALHNHYTQKSLSLSPG

SEQ ID NO: 214 - protein, 740 aa, synthetic construct
QLQLQESGPGLVKPSETLSLTCTVSGGSISSGSYFWGWIRQPPGKGLEWIGSIYYSGITYYNPSLKSRVTISVDTSKNQFSLKLSSVTAADTAVYYCARHDGAVAGLFDYWGQGTLVTVSSASTKGPSVFPLAPSSKSTSGGTAALGCLVKDYFPEPVTVSWNSGALTSGVHTFPAVLQSSGLYSLSSVVTVPSSSLGTQTYICNVNHKPSNTKVDKKVEPKSCGGGGSGGGGSGGGGSGGGGSEVQLVESGGGLVQPGGSLRLSCAASGFTFSTYAMNWVRQAPGKGLEWVGRIRSKYNNYATYYADSVKGRFTISRDDSKNSLYLQMNSLKTEDTAVYYCVRHGNFGNSYVSWFAYWGQGTLVTVSSGGGGSDKTHTCPPCPAPELLGPSVFLFPPKPKDTLMISRTPEVTCVVVDVSHEDPEVKFNWYVDGVEVHNAKTKPREEQYNSTYRVVSVLTVLHQDWLNGKEYKCKVSNKALGAPIEKTISKAKGQPREPQVYTLPPSREEMTKNQVSLWCLVKGFYPSDIAVEWESNGQPENNYKTTPPVLDSDGSFFLYSKLTVDKSRWQQGNVFSCSVMHEALHNHYTQKSLSLSPGKGGGGSGGGGSGGGGSGGGGSQVQLVQSGAEVKKPGASVKVSCKASGYTFTSYYIHWVRQAPGQGLEWIGCIYPGNVNTNYNEKFKDRATLTVDTSISTAYMELSRLRSDDTAVYFCTRSHYGLDWNFDVWGQGTTVTVSS

SEQ ID NO: 215 - protein, 600 aa, synthetic construct
QLQLQESGPGLVKPSETLSLTCTVSGGSISSGSYFWGWIRQPPGKGLEWIGSIYYSGITYYNPSLKSRVTISVDTSKNQFSLKLSSVTAADTAVYYCARHDGAVAGLFDYWGQGTLVTVSSASTKGPSVFPLAPSSKSTSGGTAALGCLVKDYFPEPVTVSWNSGALTSGVHTFPAVLQSSGLYSLSSVVTVPSSSLGTQTYICNVNHKPSNTKVDKKVEPKSCGGGGSGGGGSGGGGSGGGGSEVQLVESGGGLVQPGGSLRLSCAASGFTFSTYAMNWVRQAPGKGLEWVGRIRSKYNNYATYYADSVKGRFTISRDDSKNSLYLQMNSLKTEDTAVYYCVRHGNFGNSYVSWFAYWGQGTLVTVSSGGGGSDKTHTCPPCPAPELLGPSVFLFPPKPKDTLMISRTPEVTCVVVDVSHEDPEVKFNWYVDGVEVHNAKTKPREEQYNSTYRVVSVLTVLHQDWLNGKEYKCKVSNKALGAPIEKTISKAKGQPREPQVYTLPPSREEMTKNQVSLWCLVKGFYPSDIAVEWESNGQPENNYKTTPPVLDSDGSFFLYSKLTVDKSRWQQGNVFSCSVMHEALHNHYTQKSLSLSPGK

SEQ ID NO: 216 - protein, 710 aa, synthetic construct
QLQLQESGPGLVKPSETLSLTCTVSGGSISSGSYFWGWIRQPPGKGLEWIGSIYYSGITYYNPSLKSRVTISVDTSKNQFSLKLSSVTAADTAVYYCARHDGAVAGLFDYWGQGTLVTVSSASTKGPSVFPLAPSSKSTSGGTAALGCLVKDYFPEPVTVSWNSGALTSGVHTFPAVLQSSGLYSLSSVVTVPSSSLGTQTYICNVNHKPSNTKVDKKVEPKSCGGGGSGGGGSGGGGSGGGGSQAVVTQEPSLTVSPGGTVTLTCRSSTGAVTTSNYANWVQQKPGQAPRGLIGGTNKRAPWTPARFSGSLLGGKAALTITGAQAEDEADYYCALWYSNLWVFGGGTKLTVLGGGGSDKTHTCPPCPAPEAAGPSVFLFPPKPKDTLMISRTPEVTCVVVDVSHEDPEVKFNWYVDGVEVHNAKTKPREEQYNSTYRVVSVLTVLHQDWLNGKEYKCKVSNKALPAPIEKTISKAKGQPREPQVYTLPPSREEMTKNQVSLSCAVKGFYPSDIAVEWESNGQPENNYKTTPPVLDSDGSFFLVSKLTVDKSRWQQGNVFSCSVMHEALHNRFTQKSLSLSPGGGGGSGGGGSGGGGSGGGGSDIQMTQSPSSLSASVGDRVTITCRASQDIRSNLNWYQQKPGGAVKLLIYYTSRLHSGVPSRFSGSGSGTDYTLTISSLQPEDFATYFCQQSEKLPRTFGGGTKVEIR

SEQ ID NO: 217 - protein, 583 aa, synthetic construct
QLQLQESGPGLVKPSETLSLTCTVSGGSISSGSYFWGWIRQPPGKGLEWIGSIYYSGITYYNPSLKSRVTISVDTSKNQFSLKLSSVTAADTAVYYCARHDGAVAGLFDYWGQGTLVTVSSASTKGPSVFPLAPSSKSTSGGTAALGCLVKDYFPEPVTVSWNSGALTSGVHTFPAVLQSSGLYSLSSVVTVPSSSLGTQTYICNVNHKPSNTKVDKKVEPKSCGGGGSGGGGSGGGGSGGGGSQAVVTQEPSLTVSPGGTVTLTCRSSTGAVTTSNYANWVQQKPGQAPRGLIGGTNKRAPWTPARFSGSLLGGKAALTITGAQAEDEADYYCALWYSNLWVFGGGTKLTVLGGGGSDKTHTCPPCPAPEAAGPSVFLFPPKPKDTLMISRTPEVTCVVVDVSHEDPEVKFNWYVDGVEVHNAKTKPREEQYNSTYRVVSVLTVLHQDWLNGKEYKCKVSNKALPAPIEKTISKAKGQPREPQVYTLPPSREEMTKNQVSLSCAVKGFYPSDIAVEWESNGQPENNYKTTPPVLDSDGSFFLVSKLTVDKSRWQQGNVFSCSVMHEALHNRFTQKSLSLSPG

SEQ ID NO: 218 - protein, 711 aa, synthetic construct
QLQLQESGPGLVKPSETLSLTCTVSGGSISSGSYFWGWIRQPPGKGLEWIGSIYYSGITYYNPSLKSRVTISVDTSKNQFSLKLSSVTAADTAVYYCARHDGAVAGLFDYWGQGTLVTVSSASTKGPSVFPLAPSSKSTSGGTAALGCLVKDYFPEPVTVSWNSGALTSGVHTFPAVLQSSGLYSLSSVVTVPSSSLGTQTYICNVNHKPSNTKVDKKVEPKSCGGGGSGGGGSGGGGSGGGGSQAVVTQEPSLTVSPGGTVTLTCRSSTGAVTTSNYANWVQQKPGQAPRGLIGGTNKRAPWTPARFSGSLLGGKAALTITGAQAEDEADYYCALWYSNLWVFGGGTKLTVLGGGGSDKTHTCPPCPAPELLGPSVFLFPPKPKDTLMISRTPEVTCVVVDVSHEDPEVKFNWYVDGVEVHNAKTKPREEQYNSTYRVVSVLTVLHQDWLNGKEYKCKVSNKALGAPIEKTISKAKGQPREPQVYTLPPSREEMTKNQVSLSCAVKGFYPSDIAVEWESNGQPENNYKTTPPVLDSDGSFFLVSKLTVDKSRWQQGNVFSCSVMHEALHNRFTQKSLSLSPGKGGGGSGGGGSGGGGSGGGGSDIQMTQSPSSLSASVGDRVTITCHASQNIYVWLNWYQQKPGKAPKLLIYKASNLHTGVPSRFSGSGSGTDFTLTISSLQPEDFATYYCQQGQTYPYTFGGGTKVEIK

SEQ ID NO: 219 - protein, 584 aa, synthetic construct
QLQLQESGPGLVKPSETLSLTCTVSGGSISSGSYFWGWIRQPPGKGLEWIGSIYYSGITYYNPSLKSRVTISVDTSKNQFSLKLSSVTAADTAVYYCARHDGAVAGLFDYWGQGTLVTVSSASTKGPSVFPLAPSSKSTSGGTAALGCLVKDYFPEPVTVSWNSGALTSGVHTFPAVLQSSGLYSLSSVVTVPSSSLGTQTYICNVNHKPSNTKVDKKVEPKSCGGGGSGGGGSGGGGSGGGGSQAVVTQEPSLTVSPGGTVTLTCRSSTGAVTTSNYANWVQQKPGQAPRGLIGGTNKRAPWTPARFSGSLLGGKAALTITGAQAEDEADYYCALWYSNLWVFGGGTKLTVLGGGGSDKTHTCPPCPAPELLGPSVFLFPPKPKDTLMISRTPEVTCVVVDVSHEDPEVKFNWYVDGVEVHNAKTKPREEQYNSTYRVVSVLTVLHQDWLNGKEYKCKVSNKALGAPIEKTISKAKGQPREPQVYTLPPSREEMTKNQVSLSCAVKGFYPSDIAVEWESNGQPENNYKTTPPVLDSDGSFFLVSKLTVDKSRWQQGNVFSCSVMHEALHNRFTQKSLSLSPGK

SEQ ID NO: 220 - protein, 577 aa, synthetic construct
QVQLQESGPGLVKPSETLSLTCTVSGGSVSSGDYYWTWIRQSPGKGLEWIGHIYYSGNTNYNPSLKSRLTISIDTSKTQFSLKLSSVTAADTAIYYCVRDRVTGAFDIWGQGTMVTVSSASTKGPSVFPLAPSSKSTSGGTAALGCLVKDYFPEPVTVSWNSGALTSGVHTFPAVLQSSGLYSLSSVVTVPSSSLGTQTYICNVNHKPSNTKVDKKVEPKSCDKTHTCPPCPAPELLGGPDVFLFPPKPKDTLMISRTPEVTCVVVDVSHEDPEVKFNWYVDGVEVHNAKTKPREEQYNSTYRVVSVLTVLHQDWLNGKEYKCKVSNKALPLPEEKTISKAKGQPREPQVYTLPPSRDELTKNQVSLSCAVKGFYPSDIAVEWESNGQPENNYKTTPPVLDSDGSFFLVSKLTVDKSRWQQGNVFSCSVMHEALHNRFTQKSLSLSPGKGGGGSGGGGSGGGGSGGGGSSYEMTQPPSVSVSPGQTARITCSGDALPKKYAYWYQQKSGQAPVLVIYEDNKRPSGIPERFSGSSSGTMATLTISGAQVEDEADYYCYSTDISGNHWVFGGGTELTVL

SEQ ID NO: 221 - protein, 582 aa, synthetic construct
QVQLQESGPGLVKPSETLSLTCTVSGGSVSSGDYYWTWIRQSPGKGLEWIGHIYYSGNTNYNPSLKSRLTISIDTSKTQFSLKLSSVTAADTAIYYCVRDRVTGAFDIWGQGTMVTVSSASTKGPSVFPLAPSSKSTSGGTAALGCLVKDYFPEPVTVSWNSGALTSGVHTFPAVLQSSGLYSLSSVVTVPSSSLGTQTYICNVNHKPSNTKVDKKVEPKSCGGGGSGGGGSGGGGSGGGGSSYEMTQPPSVSVSPGQTARITCSGDALPKKYAYWYQQKSGQAPVLVIYEDNKRPSGIPERFSGSSSGTMATLTISGAQVEDEADYYCYSTDISGNHWVFGGGTELTVLGGGGSDKTHTCPPCPAPELLGGPDVFLFPPKPKDTLMISRTPEVTCVVVDVSHEDPEVKFNWYVDGVEVHNAKTKPREEQYNSTYRVVSVLTVLHQDWLNGKEYKCKVSNKALPLPEEKTISKAKGQPREPQVYTLPPSRDELTKNQVSLSCAVKGFYPSDIAVEWESNGQPENNYKTTPPVLDSDGSFFLVSKLTVDKSRWQQGNVFSCSVMHEALHNRFTQKSLSLSPGK

SEQ ID NO: 222 - protein, 577 aa, synthetic construct
QVQLQQPGAELVKPGASVKMSCKASGYTFTSYNMHWVKQTPGRGLEWIGAIYPGNGDTSYNQKFKGKATLTADKSSSTAYMQLSSLTSEDSAVYYCARSTYYGGDWYFNVWGAGTTVTVSAASTKGPSVFPLAPSSKSTSGGTAALGCLVKDYFPEPVTVSWNSGALTSGVHTFPAVLQSSGLYSLSSVVTVPSSSLGTQTYICNVNHKPSNTKVDKKVEPKSCDKTHTCPPCPAPELLGPSVFLFPPKPKDTLMISRTPEVTCVVVDVSHEDPEVKFNWYVDGVEVHNAKTKPREEQYNSTYRVVSVLTVLHQDWLNGKEYKCKVSNKALGAPIEKTISKAKGQPREPQVYTLPPSREEMTKNQVSLSCAVKGFYPSDIAVEWESNGQPENNYKTTPPVLDSDGSFFLVSKLTVDKSRWQQGNVFSCSVMHEALHNRFTQKSLSLSPGKGGGGSGGGGSGGGGSGGGGSDIQMTQSPSSLSASVGDRVTITCRASQDIRSNLNWYQQKPGGAVKLLIYYTSRLHSGVPSRFSGSGSGTDYTLTISSLQPEDFATYFCQQSEKLPRTFGGGTKVEIR

SEQ ID NO: 223 - protein, 711 aa, synthetic construct
QVQLQQPGAELVKPGASVKMSCKASGYTFTSYNMHWVKQTPGRGLEWIGAIYPGNGDTSYNQKFKGKATLTADKSSSTAYMQLSSLTSEDSAVYYCARSTYYGGDWYFNVWGAGTTVTVSAASTKGPSVFPLAPSSKSTSGGTAALGCLVKDYFPEPVTVSWNSGALTSGVHTFPAVLQSSGLYSLSSVVTVPSSSLGTQTYICNVNHKPSNTKVDKKVEPKSCGGGGSGGGGSGGGGSGGGGSQAVVTQEPSLTVSPGGTVTLTCRSSTGAVTTSNYANWVQQKPGQAPRGLIGGTNKRAPWTPARFSGSLLGGKAALTITGAQAEDEADYYCALWYSNLWVFGGGTKLTVLGGGGSDKTHTCPPCPAPEAAGPSVFLFPPKPKDTLMISRTPEVTCVVVDVSHEDPEVKFNWYVDGVEVHNAKTKPREEQYNSTYRVVSVLTVLHQDWLNGKEYKCKVSNKALGAPIEKTISKAKGQPREPQVYTLPPSREEMTKNQVSLSCAVKGFYPSDIAVEWESNGQPENNYKTTPPVLDSDGSFFLVSKLTVDKSRWQQGNVFSCSVMHEALHNHYTQKSLSLSPGKGGGGSGGGGSGGGGSGGGGSDIQMTQSPSSLSASVGDRVTITCRASQDIRSNLNWYQQKPGGAVKLLIYYTSRLHSGVPSRFSGSGSGTDYTLTISSLQPEDFATYFCQQSEKLPRTFGGGTKVEIR

SEQ ID NO: 224 - protein, 711 aa, synthetic construct
QVQLQQPGAELVKPGASVKMSCKASGYTFTSYNMHWVKQTPGRGLEWIGAIYPGNGDTSYNQKFKGKATLTADKSSSTAYMQLSSLTSEDSAVYYCARSTYYGGDWYFNVWGAGTTVTVSAASTKGPSVFPLAPSSKSTSGGTAALGCLVKDYFPEPVTVSWNSGALTSGVHTFPAVLQSSGLYSLSSVVTVPSSSLGTQTYICNVNHKPSNTKVDKKVEPKSCGGGGSGGGGSGGGGSGGGGSQAVVTQEPSLTVSPGGTVTLTCRSSTGAVTTSNYANWVQQKPGQAPRGLIGGTNKRAPWTPARFSGSLLGGKAALTITGAQAEDEADYYCALWYSNLWVFGGGTKLTVLGGGGSDKTHTCPPCPAPELLGPSVFLFPPKPKDTLMISRTPEVTCVVVDVSHEDPEVKFNWYVDGVEVHNAKTKPREEQYNSTYRVVSVLTVLHQDWLNGKEYKCKVSNKALGAPIEKTISKAKGQPREPQVYTLPPSREEMTKNQVSLSCAVKGFYPSDIAVEWESNGQPENNYKTTPPVLDSDGSFFLVSKLTVDKSRWQQGNVFSCSVMHEALHNRFTQKSLSLSPGKGGGGSGGGGSGGGGSGGGGSDIQMTQSPSSLSASVGDRVTITCRASQDIRSNLNWYQQKPGGAVKLLIYYTSRLHSGVPSRFSGSGSGTDYTLTISSLQPEDFATYFCQQSEKLPRTFGGGTKVEIR

SEQ ID NO: 225 - protein, 711 aa, synthetic construct
QVQLQQPGAELVKPGASVKMSCKASGYTFTSYNMHWVKQTPGRGLEWIGAIYPGNGDTSYNQKFKGKATLTADKSSSTAYMQLSSLTSEDSAVYYCARSTYYGGDWYFNVWGAGTTVTVSAASTKGPSVFPLAPSSKSTSGGTAALGCLVKDYFPEPVTVSWNSGALTSGVHTFPAVLQSSGLYSLSSVVTVPSSSLGTQTYICNVNHKPSNTKVDKKVEPKSCGGGGSGGGGSGGGGSGGGGSQAVVTQEPSLTVSPGGTVTLTCRSSTGAVTTSNYANWVQQKPGQAPRGLIGGTNKRAPWTPARFSGSLLGGKAALTITGAQAEDEADYYCALWYSNLWVFGGGTKLTVLGGGGSDKTHTCPPCPAPELLGPSVFLFPPKPKDTLMISRTPEVTCVVVDVSHEDPEVKFNWYVDGVEVHNAKTKPREEQYNSTYRVVSVLTVLHQDWLNGKEYKCKVSNKALGAPIEKTISKAKGQPREPQVYTLPPSREEMTKNQVSLSCAVKGFYPSDIAVEWESNGQPENNYKTTPPVLDSDGSFFLVSKLTVDKSRWQQGNVFSCSVMHEALHNHYTQKSLSLSPGKGGGGSGGGGSGGGGSGGGGSDIQMTQSPSSLSASVGDRVTITCRASQDIRSNLNWYQQKPGGAVKLLIYYTSRLHSGVPSRFSGSGSGTDYTLTISSLQPEDFATYFCQQSEKLPRTFGGGTKVEIR

SEQ ID NO: 226 - protein, 584 aa, synthetic construct
QVQLQQPGAELVKPGASVKMSCKASGYTFTSYNMHWVKQTPGRGLEWIGAIYPGNGDTSYNQKFKGKATLTADKSSSTAYMQLSSLTSEDSAVYYCARSTYYGGDWYFNVWGAGTTVTVSAASTKGPSVFPLAPSSKSTSGGTAALGCLVKDYFPEPVTVSWNSGALTSGVHTFPAVLQSSGLYSLSSVVTVPSSSLGTQTYICNVNHKPSNTKVDKKVEPKSCGGGGSGGGGSGGGGSGGGGSQAVVTQEPSLTVSPGGTVTLTCRSSTGAVTTSNYANWVQQKPGQAPRGLIGGTNKRAPWTPARFSGSLLGGKAALTITGAQAEDEADYYCALWYSNLWVFGGGTKLTVLGGGGSDKTHTCPPCPAPELLGPSVFLFPPKPKDTLMISRTPEVTCVVVDVSHEDPEVKFNWYVDGVEVHNAKTKPREEQYNSTYRVVSVLTVLHQDWLNGKEYKCKVSNKALGAPIEKTISKAKGQPREPQVYTLPPSREEMTKNQVSLSCAVKGFYPSDIAVEWESNGQPENNYKTTPPVLDSDGSFFLVSKLTVDKSRWQQGNVFSCSVMHEALHNRFTQKSLSLSPGK

SEQ ID NO: 227 - protein, 590 aa, synthetic construct
QVQLQQPGAELVKPGASVKMSCKASGYTFTSYNMHWVKQTPGRGLEWIGAIYPGNGDTSYNQKFKGKATLTADKSSSTAYMQLSSLTSEDSAVYYCARSTYYGGDWYFNVWGAGTTVTVSAASVAAPSVFIFPPSDEQLKSGTASVVCLLNNFYPREAKVQWKVDNALQSGNSQESVTEQDSKDSTYSLSSTLTLSKADYEKHKVYACEVTHQGLSSPVTKSFNRGECDKTHTCPPCPAPELLGPSVFLFPPKPKDTLMISRTPEVTCVVVDVSHEDPEVKFNWYVDGVEVHNAKTKPREEQYNSTYRVVSVLTVLHQDWLNGKEYKCKVSNKALGAPIEKTISKAKGQPREPQVYTLPPSREEMTKNQVSLWCLVKGFYPSDIAVEWESNGQPENNYKTTPPVLDSDGSFFLYSKLTVDKSRWQQGNVFSCSVMHEALHNHYTQKSLSLSPGKGGGGSGGGGSGGGGSGGGGSQVQLVQSGAEVKKPGASVKVSCKASGYTFAGFEMHWVRQAPGQGLEWMGAIDPKTGGTDYNQKFKDRVTMTRDTSISTAYMELSRLRSDDTAVYYCARDLGYFDVWGQGTLVTVSS

SEQ ID NO: 228 - protein, 740 aa, synthetic construct
QVQLQQPGAELVKPGASVKMSCKASGYTFTSYNMHWVKQTPGRGLEWIGAIYPGNGDTSYNQKFKGKATLTADKSSSTAYMQLSSLTSEDSAVYYCARSTYYGGDWYFNVWGAGTTVTVSAASVAAPSVFIFPPSDEQLKSGTASVVCLLNNFYPREAKVQWKVDNALQSGNSQESVTEQDSKDSTYSLSSTLTLSKADYEKHKVYACEVTHQGLSSPVTKSFNRGECGGGGSGGGGSGGGGSGGGGSEVQLVESGGGLVQPGGSLRLSCAASGFTFSTYAMNWVRQAPGKGLEWVGRIRSKYNNYATYYADSVKGRFTISRDDSKNSLYLQMNSLKTEDTAVYYCVRHGNFGNSYVSWFAYWGQGTLVTVSSGGGGSDKTHTCPPCPAPEAAGPSVFLFPPKPKDTLMISRTPEVTCVVVDVSHEDPEVKFNWYVDGVEVHNAKTKPREEQYNSTYRVVSVLTVLHQDWLNGKEYKCKVSNKALGAPIEKTISKAKGQPREPQVYTLPPSREEMTKNQVSLWCLVKGFYPSDIAVEWESNGQPENNYKTTPPVLDSDGSFFLYSKLTVDKSRWQQGNVFSCSVMHEALHNHYTQKSLSLSPGKGGGGSGGGGSGGGGSGGGGSQVQLVQSGAEVKKPGASVKVSCKASGYTFAGFEMHWVRQAPGQGLEWMGAIDPKTGGTDYNQKFKDRVTMTRDTSISTAYMELSRLRSDDTAVYYCARDLGYFDVWGQGTLVTVSS

SEQ ID NO: 229 - protein, 740 aa, synthetic construct
QVQLQQPGAELVKPGASVKMSCKASGYTFTSYNMHWVKQTPGRGLEWIGAIYPGNGDTSYNQKFKGKATLTADKSSSTAYMQLSSLTSEDSAVYYCARSTYYGGDWYFNVWGAGTTVTVSAASVAAPSVFIFPPSDEQLKSGTASVVCLLNNFYPREAKVQWKVDNALQSGNSQESVTEQDSKDSTYSLSSTLTLSKADYEKHKVYACEVTHQGLSSPVTKSFNRGECGGGGSGGGGSGGGGSGGGGSEVQLVESGGGLVQPGGSLRLSCAASGFTFSTYAMNWVRQAPGKGLEWVGRIRSKYNNYATYYADSVKGRFTISRDDSKNSLYLQMNSLKTEDTAVYYCVRHGNFGNSYVSWFAYWGQGTLVTVSSGGGGSDKTHTCPPCPAPELLGPSVFLFPPKPKDTLMISRTPEVTCVVVDVSHEDPEVKFNWYVDGVEVHNAKTKPREEQYNSTYRVVSVLTVLHQDWLNGKEYKCKVSNKALGAPIEKTISKAKGQPREPQVYTLPPSREEMTKNQVSLWCLVKGFYPSDIAVEWESNGQPENNYKTTPPVLDSDGSFFLYSKLTVDKSRWQQGNVFSCSVMHEALHNHYTQKSLSLSPGKGGGGSGGGGSGGGGSGGGGSQVQLVQSGAEVKKPGASVKVSCKASGYTFAGFEMHWVRQAPGQGLEWMGAIDPKTGGTDYNQKFKDRVTMTRDTSISTAYMELSRLRSDDTAVYYCARDLGYFDVWGQGTLVTVSS

SEQ ID NO: 230 - protein, 604 aa, synthetic construct
QVQLQQPGAELVKPGASVKMSCKASGYTFTSYNMHWVKQTPGRGLEWIGAIYPGNGDTSYNQKFKGKATLTADKSSSTAYMQLSSLTSEDSAVYYCARSTYYGGDWYFNVWGAGTTVTVSAASVAAPSVFIFPPSDEQLKSGTASVVCLLNNFYPREAKVQWKVDNALQSGNSQESVTEQDSKDSTYSLSSTLTLSKADYEKHKVYACEVTHQGLSSPVTKSFNRGECGGGGSGGGGSGGGGSGGGGSEVQLVESGGGLVQPGGSLRLSCAASGFTFSTYAMNWVRQAPGKGLEWVGRIRSKYNNYATYYADSVKGRFTISRDDSKNSLYLQMNSLKTEDTAVYYCVRHGNFGNSYVSWFAYWGQGTLVTVSSGGGGSDKTHTCPPCPAPELLGPSVFLFPPKPKDTLMISRTPEVTCVVVDVSHEDPEVKFNWYVDGVEVHNAKTKPREEQYNSTYRVVSVLTVLHQDWLNGKEYKCKVSNKALGAPIEKTISKAKGQPREPQVYTLPPSREEMTKNQVSLWCLVKGFYPSDIAVEWESNGQPENNYKTTPPVLDSDGSFFLYSKLTVDKSRWQQGNVFSCSVMHEALHNHYTQKSLSLSPGK

SEQ ID NO: 231 - protein, 588 aa, synthetic construct
QVQLQQSGAELVRPGSSVKISCKASGYAFSSYWMNWVKQRPGQGLEWIGQIWPGDGDTNYNGKFKGKATLTADESSSTAYMQLSSLASEDSAVYFCARRETTTVGRYYYAMDYWGQGTTVTVSSASTKGPSVFPLAPSSKSTSGGTAALGCLVKDYFPEPVTVSWNSGALTSGVHTFPAVLQSSGLYSLSSVVTVPSSSLGTQTYICNVNHKPSNTKVDKKVEPKSCDKTHTCPPCPAPEAAGPSVFLFPPKPKDTLMISRTPEVTCVVVDVSHEDPEVKFNWYVDGVEVHNAKTKPREEQYNSTYRVVSVLTVLHQDWLNGKEYKCKVSNKALPAPIEKTISKAKGQPREPQVYTLPPSREEMTKNQVSLWCLVKGFYPSDIAVEWESNGQPENNYKTTPPVLDSDGSFFLYSKLTVDKSRWQQGNVFSCSVMHEALHNHYTQKSLSLSPGGGGGSGGGGSGGGGSGGGGSQVQLVQSGAEVKKPGASVKVSCKASGYTFAGFEMHWVRQAPGQGLEWMGAIDPKTGGTDYNQKFKDRVTMTRDTSISTAYMELSRLRSDDTAVYYCARDLGYFDVWGQGTLVTVSS

SEQ ID NO: 232 - protein, 579 aa, synthetic construct
QVQLQQSGAELVRPGSSVKISCKASGYAFSSYWMNWVKQRPGQGLEWIGQIWPGDGDTNYNGKFKGKATLTADESSSTAYMQLSSLASEDSAVYFCARRETTTVGRYYYAMDYWGQGTTVTVSSASTKGPSVFPLAPSSKSTSGGTAALGCLVKDYFPEPVTVSWNSGALTSGVHTFPAVLQSSGLYSLSSVVTVPSSSLGTQTYICNVNHKPSNTKVDKKVEPKSCDKTHTCPPCPAPEAAGPSVFLFPPKPKDTLMISRTPEVTCVVVDVSHEDPEVKFNWYVDGVEVHNAKTKPREEQYNSTYRVVSVLTVLHQDWLNGKEYKCKVSNKALPAPIEKTISKAKGQPREPQVYTLPPSREEMTKNQVSLSCAVKGFYPSDIAVEWESNGQPENNYKTTPPVLDSDGSFFLVSKLTVDKSRWQQGNVFSCSVMHEALHNRFTQKSLSLSPGGGGGSGGGGSGGGGSGGGGSDIQMTQSPSSLSASVGDRVTITCRASQDIRSNLNWYQQKPGGAVKLLIYYTSRLHSGVPSRFSGSGSGTDYTLTISSLQPEDFATYFCQQSEKLPRTFGGGTKVEIR

SEQ ID NO: 233 - protein, 580 aa, synthetic construct
QVQLQQSGAELVRPGSSVKISCKASGYAFSSYWMNWVKQRPGQGLEWIGQIWPGDGDTNYNGKFKGKATLTADESSSTAYMQLSSLASEDSAVYFCARRETTTVGRYYYAMDYWGQGTTVTVSSASTKGPSVFPLAPSSKSTSGGTAALGCLVKDYFPEPVTVSWNSGALTSGVHTFPAVLQSSGLYSLSSVVTVPSSSLGTQTYICNVNHKPSNTKVDKKVEPKSCDKTHTCPPCPAPELLGPSVFLFPPKPKDTLMISRTPEVTCVVVDVSHEDPEVKFNWYVDGVEVHNAKTKPREEQYNSTYRVVSVLTVLHQDWLNGKEYKCKVSNKALGAPIEKTISKAKGQPREPQVYTLPPSREEMTKNQVSLSCAVKGFYPSDIAVEWESNGQPENNYKTTPPVLDSDGSFFLVSKLTVDKSRWQQGNVFSCSVMHEALHNRFTQKSLSLSPGKGGGGSGGGGSGGGGSGGGGSDIQMTQSPSSLSASVGDRVTITCRASQDIRSNLNWYQQKPGGAVKLLIYYTSRLHSGVPSRFSGSGSGTDYTLTISSLQPEDFATYFCQQSEKLPRTFGGGTKVEIR

SEQ ID NO: 234 - protein, 602 aa, synthetic construct
QVQLQQSGAELVRPGSSVKISCKASGYAFSSYWMNWVKQRPGQGLEWIGQIWPGDGDTNYNGKFKGKATLTADESSSTAYMQLSSLASEDSAVYFCARRETTTVGRYYYAMDYWGQGTTVTVSSASTKGPSVFPLAPSSKSTSGGTAALGCLVKDYFPEPVTVSWNSGALTSGVHTFPAVLQSSGLYSLSSVVTVPSSSLGTQTYICNVNHKPSNTKVDKKVEPKSCGGGGSGGGGSGGGGSGGGGSEVQLVESGGGLVQPGGSLRLSCAASGFTFSTYAMNWVRQAPGKGLEWVGRIRSKYNNYATYYADSVKGRFTISRDDSKNSLYLQMNSLKTEDTAVYYCVRHGNFGNSYVSWFAYWGQGTLVTVSSGGGGSDKTHTCPPCPAPEAAGPSVFLFPPKPKDTLMISRTPEVTCVVVDVSHEDPEVKFNWYVDGVEVHNAKTKPREEQYNSTYRVVSVLTVLHQDWLNGKEYKCKVSNKALPAPIEKTISKAKGQPREPQVYTLPPSREEMTKNQVSLWCLVKGFYPSDIAVEWESNGQPENNYKTTPPVLDSDGSFFLYSKLTVDKSRWQQGNVFSCSVMHEALHNHYTQKSLSLSPG

SEQ ID NO: 235 - protein, 738 aa, synthetic construct
QVQLQQSGAELVRPGSSVKISCKASGYAFSSYWMNWVKQRPGQGLEWIGQIWPGDGDTNYNGKFKGKATLTADESSSTAYMQLSSLASEDSAVYFCARRETTTVGRYYYAMDYWGQGTTVTVSSASTKGPSVFPLAPSSKSTSGGTAALGCLVKDYFPEPVTVSWNSGALTSGVHTFPAVLQSSGLYSLSSVVTVPSSSLGTQTYICNVNHKPSNTKVDKKVEPKSCGGGGSGGGGSGGGGSGGGGSEVQLVESGGGLVQPGGSLRLSCAASGFTFSTYAMNWVRQAPGKGLEWVGRIRSKYNNYATYYADSVKGRFTISRDDSKNSLYLQMNSLKTEDTAVYYCVRHGNFGNSYVSWFAYWGQGTLVTVSSGGGGSDKTHTCPPCPAPEAAGPSVFLFPPKPKDTLMISRTPEVTCVVVDVSHEDPEVKFNWYVDGVEVHNAKTKPREEQYNSTYRVVSVLTVLHQDWLNGKEYKCKVSNKALPAPIEKTISKAKGQPREPQVYTLPPSREEMTKNQVSLWCLVKGFYPSDIAVEWESNGQPENNYKTTPPVLDSDGSFFLYSKLTVDKSRWQQGNVFSCSVMHEALHNHYTQKSLSLSPGGGGGSGGGGSGGGGSGGGGSQVQLVQSGAEVKKPGASVKVSCKASGYTFAGFEMHWVRQAPGQGLEWMGAIDPKTGGTDYNQKFKDRVTMTRDTSISTAYMELSRLRSDDTAVYYCARDLGYFDVWGQGTLVTVSS

SEQ ID NO: 236 - protein, 738 aa, synthetic construct
QVQLQQSGAELVRPGSSVKISCKASGYAFSSYWMNWVKQRPGQGLEWIGQIWPGDGDTNYNGKFKGKATLTADESSSTAYMQLSSLASEDSAVYFCARRETTTVGRYYYAMDYWGQGTTVTVSSASTKGPSVFPLAPSSKSTSGGTAALGCLVKDYFPEPVTVSWNSGALTSGVHTFPAVLQSSGLYSLSSVVTVPSSSLGTQTYICNVNHKPSNTKVDKKVEPKSCGGGGSGGGGSGGGGSGGGGSEVQLVESGGGLVQPGGSLRLSCAASGFTFSTYAMNWVRQAPGKGLEWVGRIRSKYNNYATYYADSVKGRFTISRDDSKNSLYLQMNSLKTEDTAVYYCVRHGNFGNSYVSWFAYWGQGTLVTVSSGGGGSDKTHTCPPCPAPELLGPSVFLFPPKPKDTLMISRTPEVTCVVVAVSHEDPEVKFNWYVDGVEVHNAKTKPREEQYASTYRVVSVLTVLHQDWLNGKEYKCKVSNKALPAPIEKTISKAKGQPREPQVYTLPPSREEMTKNQVSLWCLVKGFYPSDIAVEWESNGQPENNYKTTPPVLDSDGSFFLYSKLTVDKSRWQQGNVFSCSVMHEALHNHYTQKSLSLSPGGGGGSGGGGSGGGGSGGGGSQVQLVQSGAEVKKPGASVKVSCKASGYTFAGFEMHWVRQAPGQGLEWMGAIDPKTGGTDYNQKFKDRVTMTRDTSISTAYMELSRLRSDDTAVYYCARDLGYFDVWGQGTLVTVSS

SEQ ID NO: 237 - protein, 740 aa, synthetic construct
QVQLQQSGAELVRPGSSVKISCKASGYAFSSYWMNWVKQRPGQGLEWIGQIWPGDGDTNYNGKFKGKATLTADESSSTAYMQLSSLASEDSAVYFCARRETTTVGRYYYAMDYWGQGTTVTVSSASTKGPSVFPLAPSSKSTSGGTAALGCLVKDYFPEPVTVSWNSGALTSGVHTFPAVLQSSGLYSLSSVVTVPSSSLGTQTYICNVNHKPSNTKVDKKVEPKSCGGGGSGGGGSGGGGSGGGGSEVQLVESGGGLVQPGGSLRLSCAASGFTFSTYAMNWVRQAPGKGLEWVGRIRSKYNNYATYYADSVKGRFTISRDDSKNSLYLQMNSLKTEDTAVYYCVRHGNFGNSYVSWFAYWGQGTLVTVSSGGGGSDKTHTCPPCPAPEAAGGPSVFLFPPKPKDTLMISRTPEVTCVVVDVSHEDPEVKFNWYVDGVEVHNAKTKPREEQYNSTYRVVSVLTVLHQDWLNGKEYKCKVSNKALGAPIEKTISKAKGQPREPQVYTLPPSREEMTKNQVSLWCLVKGFYPSDIAVEWESNGQPENNYKTTPPVLDSDGSFFLYSKLTVDKSRWQQGNVFSCSVMHEALHNHYTQKSLSLSPGKGGGGSGGGGSGGGGSGGGGSQVQLVQSGAEVKKPGASVKVSCKASGYTFAGFEMHWVRQAPGQGLEWMGAIDPKTGGTDYNQKFKDRVTMTRDTSISTAYMELSRLRSDDTAVYYCARDLGYFDVWGQGTLVTVSS

SEQ ID NO: 238 - protein, 739 aa, synthetic construct
QVQLQQSGAELVRPGSSVKISCKASGYAFSSYWMNWVKQRPGQGLEWIGQIWPGDGDTNYNGKFKGKATLTADESSSTAYMQLSSLASEDSAVYFCARRETTTVGRYYYAMDYWGQGTTVTVSSASTKGPSVFPLAPSSKSTSGGTAALGCLVKDYFPEPVTVSWNSGALTSGVHTFPAVLQSSGLYSLSSVVTVPSSSLGTQTYICNVNHKPSNTKVDKKVEPKSCGGGGSGGGGSGGGGSGGGGSEVQLVESGGGLVQPGGSLRLSCAASGFTFSTYAMNWVRQAPGKGLEWVGRIRSKYNNYATYYADSVKGRFTISRDDSKNSLYLQMNSLKTEDTAVYYCVRHGNFGNSYVSWFAYWGQGTLVTVSSGGGGSDKTHTCPPCPAPEAAGPSVFLFPPKPKDTLMISRTPEVTCVVVDVSHEDPEVKFNWYVDGVEVHNAKTKPREEQYNSTYRVVSVLTVLHQDWLNGKEYKCKVSNKALGAPIEKTISKAKGQPREPQVYTLPPSREEMTKNQVSLWCLVKGFYPSDIAVEWESNGQPENNYKTTPPVLDSDGSFFLYSKLTVDKSRWQQGNVFSCSVMHEALHNHYTQKSLSLSPGKGGGGSGGGGSGGGGSGGGGSQVQLVQSGAEVKKPGASVKVSCKASGYTFAGFEMHWVRQAPGQGLEWMGAIDPKTGGTDYNQKFKDRVTMTRDTSISTAYMELSRLRSDDTAVYYCARDLGYFDVWGQGTLVTVSS

SEQ ID NO: 239 - protein, 738 aa, synthetic construct
QVQLQQSGAELVRPGSSVKISCKASGYAFSSYWMNWVKQRPGQGLEWIGQIWPGDGDTNYNGKFKGKATLTADESSSTAYMQLSSLASEDSAVYFCARRETTTVGRYYYAMDYWGQGTTVTVSSASTKGPSVFPLAPSSKSTSGGTAALGCLVKDYFPEPVTVSWNSGALTSGVHTFPAVLQSSGLYSLSSVVTVPSSSLGTQTYICNVNHKPSNTKVDKKVEPKSCGGGGSGGGGSGGGGSGGGGSEVQLVESGGGLVQPGGSLRLSCAASGFTFSTYAMNWVRQAPGKGLEWVGRIRSKYNNYATYYADSVKGRFTISRDDSKNSLYLQMNSLKTEDTAVYYCVRHGNFGNSYVSWFAYWGQGTLVTVSSGGGGSDKTHTCPPCPAPELLGPSVFLFPPKPKDTLMISRTPEVTCVVVDVSHEDPEVKFNWYVDGVEVHNAKTKPREEQYNSTYRVVSVLTVLHQDWLNGKEYKCKVSNKALGAPIEKTISKAKGQPREPQVYTLPPSREEMTKNQVSLWCLVKGFYPSDIAVEWESNGQPENNYKTTPPVLDSDGSFFLYSKLTVDKSRWQQGNVFSCSVMHEALHNHYTQKSLSLSPGGGGGSGGGGSGGGGSGGGGSQVQLVQSGAEVKKPGASVKVSCKASGYTFAGFEMHWVRQAPGQGLEWMGAIDPKTGGTDYNQKFKDRVTMTRDTSISTAYMELSRLRSDDTAVYYCARDLGYFDVWGQGTLVTVSS

SEQ ID NO: 240 - protein, 733 aa, synthetic construct
QVQLQQSGAELVRPGSSVKISCKASGYAFSSYWMNWVKQRPGQGLEWIGQIWPGDGDTNYNGKFKGKATLTADESSSTAYMQLSSLASEDSAVYFCARRETTTVGRYYYAMDYWGQGTTVTVSSASTKGPSVFPLAPSSKSTSGGTAALGCLVKDYFPEPVTVSWNSGALTSGVHTFPAVLQSSGLYSLSSVVTVPSSSLGTQTYICNVNHKPSNTKVDKKVEPKSCGGGGSGGGGSGGGGSGGGGSEVQLVESGGGLVQPGGSLRLSCAASGFTFSTYAMNWVRQAPGKGLEWVGRIRSKYNNYATYYADSVKGRFTISRDDSKNSLYLQMNSLKTEDTAVYYCVRHGNFGNSYVSWFAYWGQGTLVTVSSDKTHTCPPCPAPEAAGPSVFLFPPKPKDTLMISRTPEVTCVVVDVSHEDPEVKFNWYVDGVEVHNAKTKPREEQYNSTYRVVSVLTVLHQDWLNGKEYKCKVSNKALPAPIEKTISKAKGQPREPQVYTLPPSREEMTKNQVSLWCLVKGFYPSDIAVEWESNGQPENNYKTTPPVLDSDGSFFLYSKLTVDKSRWQQGNVFSCSVMHEALHNHYTQKSLSLSPGGGGGSGGGGSGGGGSGGGGSQVQLVQSGAEVKKPGASVKVSCKASGYTFAGFEMHWVRQAPGQGLEWMGAIDPKTGGTDYNQKFKDRVTMTRDTSISTAYMELSRLRSDDTAVYYCARDLGYFDVWGQGTLVTVSS

SEQ ID NO: 241 - protein, 736 aa, synthetic construct
QVQLQQSGAELVRPGSSVKISCKASGYAFSSYWMNWVKQRPGQGLEWIGQIWPGDGDTNYNGKFKGKATLTADESSSTAYMQLSSLASEDSAVYFCARRETTTVGRYYYAMDYWGQGTTVTVSSASTKGPSVFPLAPSSKSTSGGTAALGCLVKDYFPEPVTVSWNSGALTSGVHTFPAVLQSSGLYSLSSVVTVPSSSLGTQTYICNVNHKPSNTKVDKKVEPKSCGGGGSGGGGSGGGGSGGGGSEVQLVESGGGLVQPGGSLRLSCAASGFTFSTYAMNWVRQAPGKGLEWVGRIRSKYNNYATYYADSVKGRFTISRDDSKNSLYLQMNSLKTEDTAVYYCVRHGNFGNSYVSWFAYWGQGTLVTVSSGGSDKTHTCPPCPAPEAAGPSVFLFPPKPKDTLMISRTPEVTCVVVDVSHEDPEVKFNWYVDGVEVHNAKTKPREEQYNSTYRVVSVLTVLHQDWLNGKEYKCKVSNKALPAPIEKTISKAKGQPREPQVYTLPPSREEMTKNQVSLWCLVKGFYPSDIAVEWESNGQPENNYKTTPPVLDSDGSFFLYSKLTVDKSRWQQGNVFSCSVMHEALHNHYTQKSLSLSPGGGGGSGGGGSGGGGSGGGGSQVQLVQSGAEVKKPGASVKVSCKASGYTFAGFEMHWVRQAPGQGLEWMGAIDPKTGGTDYNQKFKDRVTMTRDTSISTAYMELSRLRSDDTAVYYCARDLGYFDVWGQGTLVTVSS

SEQ ID NO: 242 - protein, 737 aa, synthetic construct
QVQLQQSGAELVRPGSSVKISCKASGYAFSSYWMNWVKQRPGQGLEWIGQIWPGDGDTNYNGKFKGKATLTADESSSTAYMQLSSLASEDSAVYFCARRETTTVGRYYYAMDYWGQGTTVTVSSASTKGPSVFPLAPSSKSTSGGTAALGCLVKDYFPEPVTVSWNSGALTSGVHTFPAVLQSSGLYSLSSVVTVPSSSLGTQTYICNVNHKPSNTKVDKKVEPKSCGGGGSGGGGSGGGGSGGGGSEVQLVESGGGLVQPGGSLRLSCAASGFTFSTYAMNWVRQAPGKGLEWVGRIRSKYNNYATYYADSVKGRFTISRDDSKNSLYLQMNSLKTEDTAVYYCVRHGNFGNSYVSWFAYWGQGTLVTVSSGGGSDKTHTCPPCPAPEAAGPSVFLFPPKPKDTLMISRTPEVTCVVVDVSHEDPEVKFNWYVDGVEVHNAKTKPREEQYNSTYRVVSVLTVLHQDWLNGKEYKCKVSNKALPAPIEKTISKAKGQPREPQVYTLPPSREEMTKNQVSLWCLVKGFYPSDIAVEWESNGQPENNYKTTPPVLDSDGSFFLYSKLTVDKSRWQQGNVFSCSVMHEALHNHYTQKSLSLSPGGGGGSGGGGSGGGGSGGGGSQVQLVQSGAEVKKPGASVKVSCKASGYTFAGFEMHWVRQAPGQGLEWMGAIDPKTGGTDYNQKFKDRVTMTRDTSISTAYMELSRLRSDDTAVYYCARDLGYFDVWGQGTLVTVSS

SEQ ID NO: 243 - protein, 741 aa, synthetic construct
QVQLQQSGAELVRPGSSVKISCKASGYAFSSYWMNWVKQRPGQGLEWIGQIWPGDGDTNYNGKFKGKATLTADESSSTAYMQLSSLASEDSAVYFCARRETTTVGRYYYAMDYWGQGTTVTVSSASTKGPSVFPLAPSSKSTSGGTAALGCLVKDYFPEPVTVSWNSGALTSGVHTFPAVLQSSGLYSLSSVVTVPSSSLGTQTYICNVNHKPSNTKVDKKVEPKSCGGGGSGGGGSGGGGSGGGGSEVQLVESGGGLVQPGGSLRLSCAASGFTFSTYAMNWVRQAPGKGLEWVGRIRSKYNNYATYYADSVKGRFTISRDDSKNSLYLQMNSLKTEDTAVYYCVRHGNFGNSYVSWFAYWGQGTLVTVSSGGGSGGGSDKTHTCPPCPAPEAAGPSVFLFPPKPKDTLMISRTPEVTCVVVDVSHEDPEVKFNWYVDGVEVHNAKTKPREEQYNSTYRVVSVLTVLHQDWLNGKEYKCKVSNKALPAPIEKTISKAKGQPREPQVYTLPPSREEMTKNQVSLWCLVKGFYPSDIAVEWESNGQPENNYKTTPPVLDSDGSFFLYSKLTVDKSRWQQGNVFSCSVMHEALHNHYTQKSLSLSPGGGGGSGGGGSGGGGSGGGGSQVQLVQSGAEVKKPGASVKVSCKASGYTFAGFEMHWVRQAPGQGLEWMGAIDPKTGGTDYNQKFKDRVTMTRDTSISTAYMELSRLRSDDTAVYYCARDLGYFDVWGQGTLVTVSS

SEQ ID NO: 244 - protein, 743 aa, synthetic construct
QVQLQQSGAELVRPGSSVKISCKASGYAFSSYWMNWVKQRPGQGLEWIGQIWPGDGDTNYNGKFKGKATLTADESSSTAYMQLSSLASEDSAVYFCARRETTTVGRYYYAMDYWGQGTTVTVSSASTKGPSVFPLAPSSKSTSGGTAALGCLVKDYFPEPVTVSWNSGALTSGVHTFPAVLQSSGLYSLSSVVTVPSSSLGTQTYICNVNHKPSNTKVDKKVEPKSCGGGGSGGGGSGGGGSGGGGSEVQLVESGGGLVQPGGSLRLSCAASGFTFSTYAMNWVRQAPGKGLEWVGRIRSKYNNYATYYADSVKGRFTISRDDSKNSLYLQMNSLKTEDTAVYYCVRHGNFGNSYVSWFAYWGQGTLVTVSSGGGGSGGGGSDKTHTCPPCPAPEAAGPSVFLFPPKPKDTLMISRTPEVTCVVVDVSHEDPEVKFNWYVDGVEVHNAKTKPREEQYNSTYRVVSVLTVLHQDWLNGKEYKCKVSNKALPAPIEKTISKAKGQPREPQVYTLPPSREEMTKNQVSLWCLVKGFYPSDIAVEWESNGQPENNYKTTPPVLDSDGSFFLYSKLTVDKSRWQQGNVFSCSVMHEALHNHYTQKSLSLSPGGGGGSGGGGSGGGGSGGGGSQVQLVQSGAEVKKPGASVKVSCKASGYTFAGFEMHWVRQAPGQGLEWMGAIDPKTGGTDYNQKFKDRVTMTRDTSISTAYMELSRLRSDDTAVYYCARDLGYFDVWGQGTLVTVSS

SEQ ID NO: 245 - protein, 748 aa, synthetic construct
QVQLQQSGAELVRPGSSVKISCKASGYAFSSYWMNWVKQRPGQGLEWIGQIWPGDGDTNYNGKFKGKATLTADESSSTAYMQLSSLASEDSAVYFCARRETTTVGRYYYAMDYWGQGTTVTVSSASTKGPSVFPLAPSSKSTSGGTAALGCLVKDYFPEPVTVSWNSGALTSGVHTFPAVLQSSGLYSLSSVVTVPSSSLGTQTYICNVNHKPSNTKVDKKVEPKSCGGGGSGGGGSGGGGSGGGGSEVQLVESGGGLVQPGGSLRLSCAASGFTFSTYAMNWVRQAPGKGLEWVGRIRSKYNNYATYYADSVKGRFTISRDDSKNSLYLQMNSLKTEDTAVYYCVRHGNFGNSYVSWFAYWGQGTLVTVSSGGGGSGGGGSGGGGSDKTHTCPPCPAPEAAGPSVFLFPPKPKDTLMISRTPEVTCVVVDVSHEDPEVKFNWYVDGVEVHNAKTKPREEQYNSTYRVVSVLTVLHQDWLNGKEYKCKVSNKALPAPIEKTISKAKGQPREPQVYTLPPSREEMTKNQVSLWCLVKGFYPSDIAVEWESNGQPENNYKTTPPVLDSDGSFFLYSKLTVDKSRWQQGNVFSCSVMHEALHNHYTQKSLSLSPGGGGGSGGGGSGGGGSGGGGSQVQLVQSGAEVKKPGASVKVSCKASGYTFAGFEMHWVRQAPGQGLEWMGAIDPKTGGTDYNQKFKDRVTMTRDTSISTAYMELSRLRSDDTAVYYCARDLGYFDVWGQGTLVTVSS

SEQ ID NO: 246 - protein, 586 aa, synthetic construct
QVQLQQSGAELVRPGSSVKISCKASGYAFSSYWMNWVKQRPGQGLEWIGQIWPGDGDTNYNGKFKGKATLTADESSSTAYMQLSSLASEDSAVYFCARRETTTVGRYYYAMDYWGQGTTVTVSSASTKGPSVFPLAPSSKSTSGGTAALGCLVKDYFPEPVTVSWNSGALTSGVHTFPAVLQSSGLYSLSSVVTVPSSSLGTQTYICNVNHKPSNTKVDKKVEPKSCGGGGSGGGGSGGGGSGGGGSQAVVTQEPSLTVSPGGTVTLTCRSSTGAVTTSNYANWVQQKPGQAPRGLIGGTNKRAPWTPARFSGSLLGGKAALTITGAQAEDEADYYCALWYSNLWVFGGGTKLTVLGGGGSDKTHTCPPCPAPEAAGPSVFLFPPKPKDTLMISRTPEVTCVVVDVSHEDPEVKFNWYVDGVEVHNAKTKPREEQYNSTYRVVSVLTVLHQDWLNGKEYKCKVSNKALPAPIEKTISKAKGQPREPQVYTLPPSREEMTKNQVSLSCAVKGFYPSDIAVEWESNGQPENNYKTTPPVLDSDGSFFLVSKLTVDKSRWQQGNVFSCSVMHEALHNRFTQKSLSLSPG

SEQ ID NO: 247 - protein, 713 aa, synthetic construct
QVQLQQSGAELVRPGSSVKISCKASGYAFSSYWMNWVKQRPGQGLEWIGQIWPGDGDTNYNGKFKGKATLTADESSSTAYMQLSSLASEDSAVYFCARRETTTVGRYYYAMDYWGQGTTVTVSSASTKGPSVFPLAPSSKSTSGGTAALGCLVKDYFPEPVTVSWNSGALTSGVHTFPAVLQSSGLYSLSSVVTVPSSSLGTQTYICNVNHKPSNTKVDKKVEPKSCGGGGSGGGGSGGGGSGGGGSQAVVTQEPSLTVSPGGTVTLTCRSSTGAVTTSNYANWVQQKPGQAPRGLIGGTNKRAPWTPARFSGSLLGGKAALTITGAQAEDEADYYCALWYSNLWVFGGGTKLTVLGGGGSDKTHTCPPCPAPEAAGPSVFLFPPKPKDTLMISRTPEVTCVVVDVSHEDPEVKFNWYVDGVEVHNAKTKPREEQYNSTYRVVSVLTVLHQDWLNGKEYKCKVSNKALPAPIEKTISKAKGQPREPQVYTLPPSREEMTKNQVSLSCAVKGFYPSDIAVEWESNGQPENNYKTTPPVLDSDGSFFLVSKLTVDKSRWQQGNVFSCSVMHEALHNRFTQKSLSLSPGGGGGSGGGGSGGGGSGGGGSDIQMTQSPSSLSASVGDRVTITCRASQDIRSNLNWYQQKPGGAVKLLIYYTSRLHSGVPSRFSGSGSGTDYTLTISSLQPEDFATYFCQQSEKLPRTFGGGTKVEIR

SEQ ID NO: 248 - protein, 713 aa, synthetic construct
QVQLQQSGAELVRPGSSVKISCKASGYAFSSYWMNWVKQRPGQGLEWIGQIWPGDGDTNYNGKFKGKATLTADESSSTAYMQLSSLASEDSAVYFCARRETTTVGRYYYAMDYWGQGTTVTVSSASTKGPSVFPLAPSSKSTSGGTAALGCLVKDYFPEPVTVSWNSGALTSGVHTFPAVLQSSGLYSLSSVVTVPSSSLGTQTYICNVNHKPSNTKVDKKVEPKSCGGGGSGGGGSGGGGSGGGGSQAVVTQEPSLTVSPGGTVTLTCRSSTGAVTTSNYANWVQQKPGQAPRGLIGGTNKRAPWTPARFSGSLLGGKAALTITGAQAEDEADYYCALWYSNLWVFGGGTKLTVLGGGGSDKTHTCPPCPAPEAAGPSVFLFPPKPKDTLMISRTPEVTCVVVDVSHEDPEVKFNWYVDGVEVHNAKTKPREEQYNSTYRVVSVLTVLHQDWLNGKEYKCKVSNKALPAPIEKTISKAKGQPREPQVYTLPPSREEMTKNQVSLSCAVKGFYPSDIAVEWESNGQPENNYKTTPPVLDSDGSFFLVSKLTVDKSRWQQGNVFSCSVMHEALHNHYTQKSLSLSPGGGGGSGGGGSGGGGSGGGGSDIQMTQSPSSLSASVGDRVTITCRASQDIRSNLNWYQQKPGGAVKLLIYYTSRLHSGVPSRFSGSGSGTDYTLTISSLQPEDFATYFCQQSEKLPRTFGGGTKVEIR

SEQ ID NO: 249 - protein, 713 aa, synthetic construct
QVQLQQSGAELVRPGSSVKISCKASGYAFSSYWMNWVKQRPGQGLEWIGQIWPGDGDTNYNGKFKGKATLTADESSSTAYMQLSSLASEDSAVYFCARRETTTVGRYYYAMDYWGQGTTVTVSSASTKGPSVFPLAPSSKSTSGGTAALGCLVKDYFPEPVTVSWNSGALTSGVHTFPAVLQSSGLYSLSSVVTVPSSSLGTQTYICNVNHKPSNTKVDKKVEPKSCGGGGSGGGGSGGGGSGGGGSQAVVTQEPSLTVSPGGTVTLTCRSSTGAVTTSNYANWVQQKPGQAPRGLIGGTNKRAPWTPARFSGSLLGGKAALTITGAQAEDEADYYCALWYSNLWVFGGGTKLTVLGGGGSDKTHTCPPCPAPELLGPSVFLFPPKPKDTLMISRTPEVTCVVVAVSHEDPEVKFNWYVDGVEVHNAKTKPREEQYASTYRVVSVLTVLHQDWLNGKEYKCKVSNKALPAPIEKTISKAKGQPREPQVYTLPPSREEMTKNQVSLSCAVKGFYPSDIAVEWESNGQPENNYKTTPPVLDSDGSFFLVSKLTVDKSRWQQGNVFSCSVMHEALHNHYTQKSLSLSPGGGGGSGGGGSGGGGSGGGGSDIQMTQSPSSLSASVGDRVTITCRASQDIRSNLNWYQQKPGGAVKLLIYYTSRLHSGVPSRFSGSGSGTDYTLTISSLQPEDFATYFCQQSEKLPRTFGGGTKVEIR

SEQ ID NO: 250 - protein, 715 aa, synthetic construct
QVQLQQSGAELVRPGSSVKISCKASGYAFSSYWMNWVKQRPGQGLEWIGQIWPGDGDTNYNGKFKGKATLTADESSSTAYMQLSSLASEDSAVYFCARRETTTVGRYYYAMDYWGQGTTVTVSSASTKGPSVFPLAPSSKSTSGGTAALGCLVKDYFPEPVTVSWNSGALTSGVHTFPAVLQSSGLYSLSSVVTVPSSSLGTQTYICNVNHKPSNTKVDKKVEPKSCGGGGSGGGGSGGGGSGGGGSQAVVTQEPSLTVSPGGTVTLTCRSSTGAVTTSNYANWVQQKPGQAPRGLIGGTNKRAPWTPARFSGSLLGGKAALTITGAQAEDEADYYCALWYSNLWVFGGGTKLTVLGGGGSDKTHTCPPCPAPEAAGGPSVFLFPPKPKDTLMISRTPEVTCVVVDVSHEDPEVKFNWYVDGVEVHNAKTKPREEQYNSTYRVVSVLTVLHQDWLNGKEYKCKVSNKALGAPIEKTISKAKGQPREPQVYTLPPSREEMTKNQVSLSCAVKGFYPSDIAVEWESNGQPENNYKTTPPVLDSDGSFFLVSKLTVDKSRWQQGNVFSCSVMHEALHNHYTQKSLSLSPGKGGGGSGGGGSGGGGSGGGGSDIQMTQSPSSLSASVGDRVTITCRASQDIRSNLNWYQQKPGGAVKLLIYYTSRLHSGVPSRFSGSGSGTDYTLTISSLQPEDFATYFCQQSEKLPRTFGGGTKVEIR

SEQ ID NO: 251 - protein, 714 aa, synthetic construct
QVQLQQSGAELVRPGSSVKISCKASGYAFSSYWMNWVKQRPGQGLEWIGQIWPGDGDTNYNGKFKGKATLTADESSSTAYMQLSSLASEDSAVYFCARRETTTVGRYYYAMDYWGQGTTVTVSSASTKGPSVFPLAPSSKSTSGGTAALGCLVKDYFPEPVTVSWNSGALTSGVHTFPAVLQSSGLYSLSSVVTVPSSSLGTQTYICNVNHKPSNTKVDKKVEPKSCGGGGSGGGGSGGGGSGGGGSQAVVTQEPSLTVSPGGTVTLTCRSSTGAVTTSNYANWVQQKPGQAPRGLIGGTNKRAPWTPARFSGSLLGGKAALTITGAQAEDEADYYCALWYSNLWVFGGGTKLTVLGGGGSDKTHTCPPCPAPEAAGPSVFLFPPKPKDTLMISRTPEVTCVVVDVSHEDPEVKFNWYVDGVEVHNAKTKPREEQYNSTYRVVSVLTVLHQDWLNGKEYKCKVSNKALGAPIEKTISKAKGQPREPQVYTLPPSREEMTKNQVSLSCAVKGFYPSDIAVEWESNGQPENNYKTTPPVLDSDGSFFLVSKLTVDKSRWQQGNVFSCSVMHEALHNHYTQKSLSLSPGKGGGGSGGGGSGGGGSGGGGSDIQMTQSPSSLSASVGDRVTITCRASQDIRSNLNWYQQKPGGAVKLLIYYTSRLHSGVPSRFSGSGSGTDYTLTISSLQPEDFATYFCQQSEKLPRTFGGGTKVEIR

SEQ ID NO: 252 - protein, 713 aa, synthetic construct
QVQLQQSGAELVRPGSSVKISCKASGYAFSSYWMNWVKQRPGQGLEWIGQIWPGDGDTNYNGKFKGKATLTADESSSTAYMQLSSLASEDSAVYFCARRETTTVGRYYYAMDYWGQGTTVTVSSASTKGPSVFPLAPSSKSTSGGTAALGCLVKDYFPEPVTVSWNSGALTSGVHTFPAVLQSSGLYSLSSVVTVPSSSLGTQTYICNVNHKPSNTKVDKKVEPKSCGGGGSGGGGSGGGGSGGGGSQAVVTQEPSLTVSPGGTVTLTCRSSTGAVTTSNYANWVQQKPGQAPRGLIGGTNKRAPWTPARFSGSLLGGKAALTITGAQAEDEADYYCALWYSNLWVFGGGTKLTVLGGGGSDKTHTCPPCPAPELLGPSVFLFPPKPKDTLMISRTPEVTCVVVDVSHEDPEVKFNWYVDGVEVHNAKTKPREEQYNSTYRVVSVLTVLHQDWLNGKEYKCKVSNKALGAPIEKTISKAKGQPREPQVYTLPPSREEMTKNQVSLSCAVKGFYPSDIAVEWESNGQPENNYKTTPPVLDSDGSFFLVSKLTVDKSRWQQGNVFSCSVMHEALHNHYTQKSLSLSPGGGGGSGGGGSGGGGSGGGGSDIQMTQSPSSLSASVGDRVTITCRASQDIRSNLNWYQQKPGGAVKLLIYYTSRLHSGVPSRFSGSGSGTDYTLTISSLQPEDFATYFCQQSEKLPRTFGGGTKVEIR

SEQ ID NO: 253 - protein, 708 aa, synthetic construct
QVQLQQSGAELVRPGSSVKISCKASGYAFSSYWMNWVKQRPGQGLEWIGQIWPGDGDTNYNGKFKGKATLTADESSSTAYMQLSSLASEDSAVYFCARRETTTVGRYYYAMDYWGQGTTVTVSSASTKGPSVFPLAPSSKSTSGGTAALGCLVKDYFPEPVTVSWNSGALTSGVHTFPAVLQSSGLYSLSSVVTVPSSSLGTQTYICNVNHKPSNTKVDKKVEPKSCGGGGSGGGGSGGGGSGGGGSQAVVTQEPSLTVSPGGTVTLTCRSSTGAVTTSNYANWVQQKPGQAPRGLIGGTNKRAPWTPARFSGSLLGGKAALTITGAQAEDEADYYCALWYSNLWVFGGGTKLTVLDKTHTCPPCPAPEAAGPSVFLFPPKPKDTLMISRTPEVTCVVVDVSHEDPEVKFNWYVDGVEVHNAKTKPREEQYNSTYRVVSVLTVLHQDWLNGKEYKCKVSNKALPAPIEKTISKAKGQPREPQVYTLPPSREEMTKNQVSLSCAVKGFYPSDIAVEWESNGQPENNYKTTPPVLDSDGSFFLVSKLTVDKSRWQQGNVFSCSVMHEALHNRFTQKSLSLSPGGGGGSGGGGSGGGGSGGGGSDIQMTQSPSSLSASVGDRVTITCRASQDIRSNLNWYQQKPGGAVKLLIYYTSRLHSGVPSRFSGSGSGTDYTLTISSLQPEDFATYFCQQSEKLPRTFGGGTKVEIR

SEQ ID NO: 254 - protein, 711 aa, synthetic construct
QVQLQQSGAELVRPGSSVKISCKASGYAFSSYWMNWVKQRPGQGLEWIGQIWPGDGDTNYNGKFKGKATLTADESSSTAYMQLSSLASEDSAVYFCARRETTTVGRYYYAMDYWGQGTTVTVSSASTKGPSVFPLAPSSKSTSGGTAALGCLVKDYFPEPVTVSWNSGALTSGVHTFPAVLQSSGLYSLSSVVTVPSSSLGTQTYICNVNHKPSNTKVDKKVEPKSCGGGGSGGGGSGGGGSGGGGSQAVVTQEPSLTVSPGGTVTLTCRSSTGAVTTSNYANWVQQKPGQAPRGLIGGTNKRAPWTPARFSGSLLGGKAALTITGAQAEDEADYYCALWYSNLWVFGGGTKLTVLGGSDKTHTCPPCPAPEAAGPSVFLFPPKPKDTLMISRTPEVTCVVVDVSHEDPEVKFNWYVDGVEVHNAKTKPREEQYNSTYRVVSVLTVLHQDWLNGKEYKCKVSNKALPAPIEKTISKAKGQPREPQVYTLPPSREEMTKNQVSLSCAVKGFYPSDIAVEWESNGQPENNYKTTPPVLDSDGSFFLVSKLTVDKSRWQQGNVFSCSVMHEALHNRFTQKSLSLSPGGGGGSGGGGSGGGGSGGGGSDIQMTQSPSSLSASVGDRVTITCRASQDIRSNLNWYQQKPGGAVKLLIYYTSRLHSGVPSRFSGSGSGTDYTLTISSLQPEDFATYFCQQSEKLPRTFGGGTKVEIR

SEQ ID NO: 255 - protein, 712 aa, synthetic construct
QVQLQQSGAELVRPGSSVKISCKASGYAFSSYWMNWVKQRPGQGLEWIGQIWPGDGDTNYNGKFKGKATLTADESSSTAYMQLSSLASEDSAVYFCARRETTTVGRYYYAMDYWGQGTTVTVSSASTKGPSVFPLAPSSKSTSGGTAALGCLVKDYFPEPVTVSWNSGALTSGVHTFPAVLQSSGLYSLSSVVTVPSSSLGTQTYICNVNHKPSNTKVDKKVEPKSCGGGGSGGGGSGGGGSGGGGSQAVVTQEPSLTVSPGGTVTLTCRSSTGAVTTSNYANWVQQKPGQAPRGLIGGTNKRAPWTPARFSGSLLGGKAALTITGAQAEDEADYYCALWYSNLWVFGGGTKLTVLGGGSDKTHTCPPCPAPEAAGPSVFLFPPKPKDTLMISRTPEVTCVVVDVSHEDPEVKFNWYVDGVEVHNAKTKPREEQYNSTYRVVSVLTVLHQDWLNGKEYKCKVSNKALPAPIEKTISKAKGQPREPQVYTLPPSREEMTKNQVSLSCAVKGFYPSDIAVEWESNGQPENNYKTTPPVLDSDGSFFLVSKLTVDKSRWQQGNVFSCSVMHEALHNRFTQKSLSLSPGGGGGSGGGGSGGGGSGGGGSDIQMTQSPSSLSASVGDRVTITCRASQDIRSNLNWYQQKPGGAVKLLIYYTSRLHSGVPSRFSGSGSGTDYTLTISSLQPEDFATYFCQQSEKLPRTFGGGTKVEIR

SEQ ID NO: 256 - protein, 716 aa, synthetic construct
QVQLQQSGAELVRPGSSVKISCKASGYAFSSYWMNWVKQRPGQGLEWIGQIWPGDGDTNYNGKFKGKATLTADESSSTAYMQLSSLASEDSAVYFCARRETTTVGRYYYAMDYWGQGTTVTVSSASTKGPSVFPLAPSSKSTSGGTAALGCLVKDYFPEPVTVSWNSGALTSGVHTFPAVLQSSGLYSLSSVVTVPSSSLGTQTYICNVNHKPSNTKVDKKVEPKSCGGGGSGGGGSGGGGSGGGGSQAVVTQEPSLTVSPGGTVTLTCRSSTGAVTTSNYANWVQQKPGQAPRGLIGGTNKRAPWTPARFSGSLLGGKAALTITGAQAEDEADYYCALWYSNLWVFGGGTKLTVLGGGSGGGSDKTHTCPPCPAPEAAGPSVFLFPPKPKDTLMISRTPEVTCVVVDVSHEDPEVKFNWYVDGVEVHNAKTKPREEQYNSTYRVVSVLTVLHQDWLNGKEYKCKVSNKALPAPIEKTISKAKGQPREPQVYTLPPSREEMTKNQVSLSCAVKGFYPSDIAVEWESNGQPENNYKTTPPVLDSDGSFFLVSKLTVDKSRWQQGNVFSCSVMHEALHNRFTQKSLSLSPGGGGGSGGGGSGGGGSGGGGSDIQMTQSPSSLSASVGDRVTITCRASQDIRSNLNWYQQKPGGAVKLLIYYTSRLHSGVPSRFSGSGSGTDYTLTISSLQPEDFATYFCQQSEKLPRTFGGGTKVEIR

SEQ ID NO: 257 - protein, 718 aa, synthetic construct
QVQLQQSGAELVRPGSSVKISCKASGYAFSSYWMNWVKQRPGQGLEWIGQIWPGDGDTNYNGKFKGKATLTADESSSTAYMQLSSLASEDSAVYFCARRETTTVGRYYYAMDYWGQGTTVTVSSASTKGPSVFPLAPSSKSTSGGTAALGCLVKDYFPEPVTVSWNSGALTSGVHTFPAVLQSSGLYSLSSVVTVPSSSLGTQTYICNVNHKPSNTKVDKKVEPKSCGGGGSGGGGSGGGGSGGGGSQAVVTQEPSLTVSPGGTVTLTCRSSTGAVTTSNYANWVQQKPGQAPRGLIGGTNKRAPWTPARFSGSLLGGKAALTITGAQAEDEADYYCALWYSNLWVFGGGTKLTVLGGGGSGGGGSDKTHTCPPCPAPEAAGPSVFLFPPKPKDTLMISRTPEVTCVVVDVSHEDPEVKFNWYVDGVEVHNAKTKPREEQYNSTYRVVSVLTVLHQDWLNGKEYKCKVSNKALPAPIEKTISKAKGQPREPQVYTLPPSREEMTKNQVSLSCAVKGFYPSDIAVEWESNGQPENNYKTTPPVLDSDGSFFLVSKLTVDKSRWQQGNVFSCSVMHEALHNRFTQKSLSLSPGGGGGSGGGGSGGGGSGGGGSDIQMTQSPSSLSASVGDRVTITCRASQDIRSNLNWYQQKPGGAVKLLIYYTSRLHSGVPSRFSGSGSGTDYTLTISSLQPEDFATYFCQQSEKLPRTFGGGTKVEIR

SEQ ID NO: 258 - protein, 723 aa, synthetic construct
QVQLQQSGAELVRPGSSVKISCKASGYAFSSYWMNWVKQRPGQGLEWIGQIWPGDGDTNYNGKFKGKATLTADESSSTAYMQLSSLASEDSAVYFCARRETTTVGRYYYAMDYWGQGTTVTVSSASTKGPSVFPLAPSSKSTSGGTAALGCLVKDYFPEPVTVSWNSGALTSGVHTFPAVLQSSGLYSLSSVVTVPSSSLGTQTYICNVNHKPSNTKVDKKVEPKSCGGGGSGGGGSGGGGSGGGGSQAVVTQEPSLTVSPGGTVTLTCRSSTGAVTTSNYANWVQQKPGQAPRGLIGGTNKRAPWTPARFSGSLLGGKAALTITGAQAEDEADYYCALWYSNLWVFGGGTKLTVLGGGGSGGGGSGGGGSDKTHTCPPCPAPEAAGPSVFLFPPKPKDTLMISRTPEVTCVVVDVSHEDPEVKFNWYVDGVEVHNAKTKPREEQYNSTYRVVSVLTVLHQDWLNGKEYKCKVSNKALPAPIEKTISKAKGQPREPQVYTLPPSREEMTKNQVSLSCAVKGFYPSDIAVEWESNGQPENNYKTTPPVLDSDGSFFLVSKLTVDKSRWQQGNVFSCSVMHEALHNRFTQKSLSLSPGGGGGSGGGGSGGGGSGGGGSDIQMTQSPSSLSASVGDRVTITCRASQDIRSNLNWYQQKPGGAVKLLIYYTSRLHSGVPSRFSGSGSGTDYTLTISSLQPEDFATYFCQQSEKLPRTFGGGTKVEIR

SEQ ID NO: 259 - protein, 714 aa, synthetic construct; identical to SEQ ID NO: 251

SEQ ID NO: 260 - protein, 714 aa, synthetic construct
QVQLQQSGAELVRPGSSVKISCKASGYAFSSYWMNWVKQRPGQGLEWIGQIWPGDGDTNYNGKFKGKATLTADESSSTAYMQLSSLASEDSAVYFCARRETTTVGRYYYAMDYWGQGTTVTVSSASTKGPSVFPLAPSSKSTSGGTAALGCLVKDYFPEPVTVSWNSGALTSGVHTFPAVLQSSGLYSLSSVVTVPSSSLGTQTYICNVNHKPSNTKVDKKVEPKSCGGGGSGGGGSGGGGSGGGGSQAVVTQEPSLTVSPGGTVTLTCRSSTGAVTTSNYANWVQQKPGQAPRGLIGGTNKRAPWTPARFSGSLLGGKAALTITGAQAEDEADYYCALWYSNLWVFGGGTKLTVLGGGGSDKTHTCPPCPAPELLGPSVFLFPPKPKDTLMISRTPEVTCVVVDVSHEDPEVKFNWYVDGVEVHNAKTKPREEQYNSTYRVVSVLTVLHQDWLNGKEYKCKVSNKALGAPIEKTISKAKGQPREPQVYTLPPSREEMTKNQVSLSCAVKGFYPSDIAVEWESNGQPENNYKTTPPVLDSDGSFFLVSKLTVDKSRWQQGNVFSCSVMHEALHNRFTQKSLSLSPGKGGGGSGGGGSGGGGSGGGGSDIQMTQSPSSLSASVGDRVTITCRASQDIRSNLNWYQQKPGGAVKLLIYYTSRLHSGVPSRFSGSGSGTDYTLTISSLQPEDFATYFCQQSEKLPRTFGGGTKVEIR

SEQ ID NO: 261 - protein, 714 aa, synthetic construct
QVQLQQSGAELVRPGSSVKISCKASGYAFSSYWMNWVKQRPGQGLEWIGQIWPGDGDTNYNGKFKGKATLTADESSSTAYMQLSSLASEDSAVYFCARRETTTVGRYYYAMDYWGQGTTVTVSSASTKGPSVFPLAPSSKSTSGGTAALGCLVKDYFPEPVTVSWNSGALTSGVHTFPAVLQSSGLYSLSSVVTVPSSSLGTQTYICNVNHKPSNTKVDKKVEPKSCGGGGSGGGGSGGGGSGGGGSQAVVTQEPSLTVSPGGTVTLTCRSSTGAVTTSNYANWVQQKPGQAPRGLIGGTNKRAPWTPARFSGSLLGGKAALTITGAQAEDEADYYCALWYSNLWVFGGGTKLTVLGGGGSDKTHTCPPCPAPELLGPSVFLFPPKPKDTLMISRTPEVTCVVVDVSHEDPEVKFNWYVDGVEVHNAKTKPREEQYNSTYRVVSVLTVLHQDWLNGKEYKCKVSNKALGAPIEKTISKAKGQPREPQVYTLPPSREEMTKNQVSLSCAVKGFYPSDIAVEWESNGQPENNYKTTPPVLDSDGSFFLVSKLTVDKSRWQQGNVFSCSVMHEALHNHYTQKSLSLSPGKGGGGSGGGGSGGGGSGGGGSDIQMTQSPSSLSASVGDRVTITCRASQDIRSNLNWYQQKPGGAVKLLIYYTSRLHSGVPSRFSGSGSGTDYTLTISSLQPEDFATYFCQQSEKLPRTFGGGTKVEIR

SEQ ID NO: 262 - protein, 587 aa, synthetic construct
QVQLQQSGAELVRPGSSVKISCKASGYAFSSYWMNWVKQRPGQGLEWIGQIWPGDGDTNYNGKFKGKATLTADESSSTAYMQLSSLASEDSAVYFCARRETTTVGRYYYAMDYWGQGTTVTVSSASTKGPSVFPLAPSSKSTSGGTAALGCLVKDYFPEPVTVSWNSGALTSGVHTFPAVLQSSGLYSLSSVVTVPSSSLGTQTYICNVNHKPSNTKVDKKVEPKSCGGGGSGGGGSGGGGSGGGGSQAVVTQEPSLTVSPGGTVTLTCRSSTGAVTTSNYANWVQQKPGQAPRGLIGGTNKRAPWTPARFSGSLLGGKAALTITGAQAEDEADYYCALWYSNLWVFGGGTKLTVLGGGGSDKTHTCPPCPAPELLGPSVFLFPPKPKDTLMISRTPEVTCVVVDVSHEDPEVKFNWYVDGVEVHNAKTKPREEQYNSTYRVVSVLTVLHQDWLNGKEYKCKVSNKALGAPIEKTISKAKGQPREPQVYTLPPSREEMTKNQVSLSCAVKGFYPSDIAVEWESNGQPENNYKTTPPVLDSDGSFFLVSKLTVDKSRWQQGNVFSCSVMHEALHNRFTQKSLSLSPGK

SEQ ID NO: 263 - protein, 593 aa, synthetic construct
QVQLQQSGAELVRPGSSVKISCKASGYAFSSYWMNWVKQRPGQGLEWIGQIWPGDGDTNYNGKFKGKATLTADESSSTAYMQLSSLASEDSAVYFCARRETTTVGRYYYAMDYWGQGTTVTVSSASVAAPSVFIFPPSDEQLKSGTASVVCLLNNFYPREAKVQWKVDNALQSGNSQESVTEQDSKDSTYSLSSTLTLSKADYEKHKVYACEVTHQGLSSPVTKSFNRGECDKTHTCPPCPAPELLGPSVFLFPPKPKDTLMISRTPEVTCVVVDVSHEDPEVKFNWYVDGVEVHNAKTKPREEQYNSTYRVVSVLTVLHQDWLNGKEYKCKVSNKALGAPIEKTISKAKGQPREPQVYTLPPSREEMTKNQVSLWCLVKGFYPSDIAVEWESNGQPENNYKTTPPVLDSDGSFFLYSKLTVDKSRWQQGNVFSCSVMHEALHNHYTQKSLSLSPGKGGGGSGGGGSGGGGSGGGGSQVQLVQSGAEVKKPGASVKVSCKASGYTFAGFEMHWVRQAPGQGLEWMGAIDPKTGGTDYNQKFKDRVTMTRDTSISTAYMELSRLRSDDTAVYYCARDLGYFDVWGQGTLVTVSS

SEQ ID NO: 264 - protein, 743 aa, synthetic construct
QVQLQQSGAELVRPGSSVKISCKASGYAFSSYWMNWVKQRPGQGLEWIGQIWPGDGDTNYNGKFKGKATLTADESSSTAYMQLSSLASEDSAVYFCARRETTTVGRYYYAMDYWGQGTTVTVSSASVAAPSVFIFPPSDEQLKSGTASVVCLLNNFYPREAKVQWKVDNALQSGNSQESVTEQDSKDSTYSLSSTLTLSKADYEKHKVYACEVTHQGLSSPVTKSFNRGECGGGGSGGGGSGGGGSGGGGSEVQLVESGGGLVQPGGSLRLSCAASGFTFSTYAMNWVRQAPGKGLEWVGRIRSKYNNYATYYADSVKGRFTISRDDSKNSLYLQMNSLKTEDTAVYYCVRHGNFGNSYVSWFAYWGQGTLVTVSSGGGGSDKTHTCPPCPAPEAAGPSVFLFPPKPKDTLMISRTPEVTCVVVDVSHEDPEVKFNWYVDGVEVHNAKTKPREEQYNSTYRVVSVLTVLHQDWLNGKEYKCKVSNKALGAPIEKTISKAKGQPREPQVYTLPPSREEMTKNQVSLWCLVKGFYPSDIAVEWESNGQPENNYKTTPPVLDSDGSFFLYSKLTVDKSRWQQGNVFSCSVMHEALHNHYTQKSLSLSPGKGGGGSGGGGSGGGGSGGGGSQVQLVQSGAEVKKPGASVKVSCKASGYTFAGFEMHWVRQAPGQGLEWMGAIDPKTGGTDYNQKFKDRVTMTRDTSISTAYMELSRLRSDDTAVYYCARDLGYFDVWGQGTLVTVSS

SEQ ID NO: 265 - protein, 743 aa, synthetic construct
QVQLQQSGAELVRPGSSVKISCKASGYAFSSYWMNWVKQRPGQGLEWIGQIWPGDGDTNYNGKFKGKATLTADESSSTAYMQLSSLASEDSAVYFCARRETTTVGRYYYAMDYWGQGTTVTVSSASVAAPSVFIFPPSDEQLKSGTASVVCLLNNFYPREAKVQWKVDNALQSGNSQESVTEQDSKDSTYSLSSTLTLSKADYEKHKVYACEVTHQGLSSPVTKSFNRGECGGGGSGGGGSGGGGSGGGGSEVQLVESGGGLVQPGGSLRLSCAASGFTFSTYAMNWVRQAPGKGLEWVGRIRSKYNNYATYYADSVKGRFTISRDDSKNSLYLQMNSLKTEDTAVYYCVRHGNFGNSYVSWFAYWGQGTLVTVSSGGGGSDKTHTCPPCPAPELLGPSVFLFPPKPKDTLMISRTPEVTCVVVDVSHEDPEVKFNWYVDGVEVHNAKTKPREEQYNSTYRVVSVLTVLHQDWLNGKEYKCKVSNKALGAPIEKTISKAKGQPREPQVYTLPPSREEMTKNQVSLWCLVKGFYPSDIAVEWESNGQPENNYKTTPPVLDSDGSFFLYSKLTVDKSRWQQGNVFSCSVMHEALHNHYTQKSLSLSPGKGGGGSGGGGSGGGGSGGGGSQVQLVQSGAEVKKPGASVKVSCKASGYTFAGFEMHWVRQAPGQGLEWMGAIDPKTGGTDYNQKFKDRVTMTRDTSISTAYMELSRLRSDDTAVYYCARDLGYFDVWGQGTLVTVSS

SEQ ID NO: 266 - protein, 607 aa, synthetic construct
QVQLQQSGAELVRPGSSVKISCKASGYAFSSYWMNWVKQRPGQGLEWIGQIWPGDGDTNYNGKFKGKATLTADESSSTAYMQLSSLASEDSAVYFCARRETTTVGRYYYAMDYWGQGTTVTVSSASVAAPSVFIFPPSDEQLKSGTASVVCLLNNFYPREAKVQWKVDNALQSGNSQESVTEQDSKDSTYSLSSTLTLSKADYEKHKVYACEVTHQGLSSPVTKSFNRGECGGGGSGGGGSGGGGSGGGGSEVQLVESGGGLVQPGGSLRLSCAASGFTFSTYAMNWVRQAPGKGLEWVGRIRSKYNNYATYYADSVKGRFTISRDDSKNSLYLQMNSLKTEDTAVYYCVRHGNFGNSYVSWFAYWGQGTLVTVSSGGGGSDKTHTCPPCPAPELLGPSVFLFPPKPKDTLMISRTPEVTCVVVDVSHEDPEVKFNWYVDGVEVHNAKTKPREEQYNSTYRVVSVLTVLHQDWLNGKEYKCKVSNKALGAPIEKTISKAKGQPREPQVYTLPPSREEMTKNQVSLWCLVKGFYPSDIAVEWESNGQPENNYKTTPPVLDSDGSFFLYSKLTVDKSRWQQGNVFSCSVMHEALHNHYTQKSLSLSPGK

SEQ ID NO: 267 - protein, 585 aa, synthetic construct
QVQLVESGGGLVKPGESLRLSCAASGFTFSDYYMYWVRQAPGKGLEWVAIISDGGYYTYYSDIIKGRFTISRDNAKNSLYLQMNSLKAEDTAVYYCARGFPLLRHGAMDYWGQGTLVTVSSASTKGPSVFPLAPSSKSTSGGTAALGCLVKDYFPEPVTVSWNSGALTSGVHTFPAVLQSSGLYSLSSVVTVPSSSLGTQTYICNVNHKPSNTKVDKKVEPKSCDKTHTCPPCPAPEAAGPSVFLFPPKPKDTLMISRTPEVTCVVVDVSHEDPEVKFNWYVDGVEVHNAKTKPREEQYNSTYRVVSVLTVLHQDWLNGKEYKCKVSNKALPAPIEKTISKAKGQPREPQVYTLPPSREEMTKNQVSLWCLVKGFYPSDIAVEWESNGQPENNYKTTPPVLDSDGSFFLYSKLTVDKSRWQQGNVFSCSVMHEALHNHYTQKSLSLSPGGGGGSGGGGSGGGGSGGGGSQVQLVQSGAEVKKPGASVKVSCKASGYTFAGFEMHWVRQAPGQGLEWMGAIDPKTGGTDYNQKFKDRVTMTRDTSISTAYMELSRLRSDDTAVYYCARDLGYFDVWGQGTLVTVSS

SEQ ID NO: 268 - protein, 576 aa, synthetic construct
QVQLVESGGGLVKPGESLRLSCAASGFTFSDYYMYWVRQAPGKGLEWVAIISDGGYYTYYSDIIKGRFTISRDNAKNSLYLQMNSLKAEDTAVYYCARGFPLLRHGAMDYWGQGTLVTVSSASTKGPSVFPLAPSSKSTSGGTAALGCLVKDYFPEPVTVSWNSGALTSGVHTFPAVLQSSGLYSLSSVVTVPSSSLGTQTYICNVNHKPSNTKVDKKVEPKSCDKTHTCPPCPAPEAAGPSVFLFPPKPKDTLMISRTPEVTCVVVDVSHEDPEVKFNWYVDGVEVHNAKTKPREEQYNSTYRVVSVLTVLHQDWLNGKEYKCKVSNKALPAPIEKTISKAKGQPREPQVYTLPPSREEMTKNQVSLSCAVKGFYPSDIAVEWESNGQPENNYKTTPPVLDSDGSFFLVSKLTVDKSRWQQGNVFSCSVMHEALHNRFTQKSLSLSPGGGGGSGGGGSGGGGSGGGGSDIQMTQSPSSLSASVGDRVTITCRASQDIRSNLNWYQQKPGGAVKLLIYYTSRLHSGVPSRFSGSGSGTDYTLTISSLQPEDFATYFCQQSEKLPRTFGGGTKVEIR

SEQ ID NO: 269 - protein, 735 aa, synthetic construct
QVQLVESGGGLVKPGESLRLSCAASGFTFSDYYMYWVRQAPGKGLEWVAIISDGGYYTYYSDIIKGRFTISRDNAKNSLYLQMNSLKAEDTAVYYCARGFPLLRHGAMDYWGQGTLVTVSSASTKGPSVFPLAPSSKSTSGGTAALGCLVKDYFPEPVTVSWNSGALTSGVHTFPAVLQSSGLYSLSSVVTVPSSSLGTQTYICNVNHKPSNTKVDKKVEPKSCGGGGSGGGGSGGGGSGGGGSEVQLVESGGGLVQPGGSLRLSCAASGFTFSTYAMNWVRQAPGKGLEWVGRIRSKYNNYATYYADSVKGRFTISRDDSKNSLYLQMNSLKTEDTAVYYCVRHGNFGNSYVSWFAYWGQGTLVTVSSGGGGSDKTHTCPPCPAPEAAGPSVFLFPPKPKDTLMISRTPEVTCVVVDVSHEDPEVKFNWYVDGVEVHNAKTKPREEQYNSTYRVVSVLTVLHQDWLNGKEYKCKVSNKALPAPIEKTISKAKGQPREPQVYTLPPSREEMTKNQVSLWCLVKGFYPSDIAVEWESNGQPENNYKTTPPVLDSDGSFFLYSKLTVDKSRWQQGNVFSCSVMHEALHNHYTQKSLSLSPGGGGGSGGGGSGGGGSGGGGSQVQLVQSGAEVKKPGASVKVSCKASGYTFAGFEMHWVRQAPGQGLEWMGAIDPKTGGTDYNQKFKDRVTMTRDTSISTAYMELSRLRSDDTAVYYCARDLGYFDVWGQGTLVTVSS

SEQ ID NO: 270 - protein, 599 aa, synthetic construct
QVQLVESGGGLVKPGESLRLSCAASGFTFSDYYMYWVRQAPGKGLEWVAIISDGGYYTYYSDIIKGRFTISRDNAKNSLYLQMNSLKAEDTAVYYCARGFPLLRHGAMDYWGQGTLVTVSSASTKGPSVFPLAPSSKSTSGGTAALGCLVKDYFPEPVTVSWNSGALTSGVHTFPAVLQSSGLYSLSSVVTVPSSSLGTQTYICNVNHKPSNTKVDKKVEPKSCGGGGSGGGGSGGGGSGGGGSEVQLVESGGGLVQPGGSLRLSCAASGFTFSTYAMNWVRQAPGKGLEWVGRIRSKYNNYATYYADSVKGRFTISRDDSKNSLYLQMNSLKTEDTAVYYCVRHGNFGNSYVSWFAYWGQGTLVTVSSGGGGSDKTHTCPPCPAPEAAGPSVFLFPPKPKDTLMISRTPEVTCVVVDVSHEDPEVKFNWYVDGVEVHNAKTKPREEQYNSTYRVVSVLTVLHQDWLNGKEYKCKVSNKALPAPIEKTISKAKGQPREPQVYTLPPSREEMTKNQVSLWCLVKGFYPSDIAVEWESNGQPENNYKTTPPVLDSDGSFFLYSKLTVDKSRWQQGNVFSCSVMHEALHNHYTQKSLSLSPG

SEQ ID NO: 271 - protein, 710 aa, synthetic construct
QVQLVESGGGLVKPGESLRLSCAASGFTFSDYYMYWVRQAPGKGLEWVAIISDGGYYTYYSDIIKGRFTISRDNAKNSLYLQMNSLKAEDTAVYYCARGFPLLRHGAMDYWGQGTLVTVSSASTKGPSVFPLAPSSKSTSGGTAALGCLVKDYFPEPVTVSWNSGALTSGVHTFPAVLQSSGLYSLSSVVTVPSSSLGTQTYICNVNHKPSNTKVDKKVEPKSCGGGGSGGGGSGGGGSGGGGSQAVVTQEPSLTVSPGGTVTLTCRSSTGAVTTSNYANWVQQKPGQAPRGLIGGTNKRAPWTPARFSGSLLGGKAALTITGAQAEDEADYYCALWYSNLWVFGGGTKLTVLGGGGSDKTHTCPPCPAPEAAGPSVFLFPPKPKDTLMISRTPEVTCVVVDVSHEDPEVKFNWYVDGVEVHNAKTKPREEQYNSTYRVVSVLTVLHQDWLNGKEYKCKVSNKALPAPIEKTISKAKGQPREPQVYTLPPSREEMTKNQVSLSCAVKGFYPSDIAVEWESNGQPENNYKTTPPVLDSDGSFFLVSKLTVDKSRWQQGNVFSCSVMHEALHNRFTQKSLSLSPGGGGGSGGGGSGGGGSGGGGSDIQMTQSPSSLSASVGDRVTITCRASQDIRSNLNWYQQKPGGAVKLLIYYTSRLHSGVPSRFSGSGSGTDYTLTISSLQPEDFATYFCQQSEKLPRTFGGGTKVEIR

SEQ ID NO: 272 - protein, 583 aa, synthetic construct
QVQLVESGGGLVKPGESLRLSCAASGFTFSDYYMYWVRQAPGKGLEWVAIISDGGYYTYYSDIIKGRFTISRDNAKNSLYLQMNSLKAEDTAVYYCARGFPLLRHGAMDYWGQGTLVTVSSASTKGPSVFPLAPSSKSTSGGTAALGCLVKDYFPEPVTVSWNSGALTSGVHTFPAVLQSSGLYSLSSVVTVPSSSLGTQTYICNVNHKPSNTKVDKKVEPKSCGGGGSGGGGSGGGGSGGGGSQAVVTQEPSLTVSPGGTVTLTCRSSTGAVTTSNYANWVQQKPGQAPRGLIGGTNKRAPWTPARFSGSLLGGKAALTITGAQAEDEADYYCALWYSNLWVFGGGTKLTVLGGGGSDKTHTCPPCPAPEAAGPSVFLFPPKPKDTLMISRTPEVTCVVVDVSHEDPEVKFNWYVDGVEVHNAKTKPREEQYNSTYRVVSVLTVLHQDWLNGKEYKCKVSNKALPAPIEKTISKAKGQPREPQVYTLPPSREEMTKNQVSLSCAVKGFYPSDIAVEWESNGQPENNYKTTPPVLDSDGSFFLVSKLTVDKSRWQQGNVFSCSVMHEALHNRFTQKSLSLSPG

SEQ ID NO: 273 - protein, 596 aa, synthetic construct
QVQLVQSGAEVKKPGASVKVSCKASGYTFTDFWMSWVRQAPGQGLEWMGQIYPNTGTTHSNEKFKGRVTMTRDTSTSTVYMELSSLRSEDTAVYYCARSYHISTTPNWFAYWGQGTLVTVSSASTKGPSVFPLAPSSKSTSGGTAALGCLVKDYFPEPVTVSWNSGALTSGVHTFPAVLQSSGLYSLSSVVTVPSSSLGTQTYICNVNHKPSNTKVDKKVEPKSCDKTHTCPPCPAPEAAGPSVFLFPPKPKDTLMISRTPEVTCVVVDVSHEDPEVKFNWYVDGVEVHNAKTKPREEQYNSTYRVVSVLTVLHQDWLNGKEYKCKVSNKALPAPIEKTISKAKGQPREPQVYTLPPSREEMTKNQVSLWCLVKGFYPSDIAVEWESNGQPENNYKTTPPVLDSDGSFFLYSKLTVDKSRWQQGNVFSCSVMHEALHNHYTQKSLSLSPGGGGGSGGGGSGGGGSGGGGSQVQLVQSGAEVKKPGASVKVSCKASGYTFTGYYMHWVRQAPGQGLEWMGWINPDSGGTNYAQKFQGRVTMTRDTSISTAYMELNRLRSDDTAVYYCARDQPLGYCTNGVCSYFDYWGQGTLVTVSS

SEQ ID NO: 274 - protein, 577 aa, synthetic construct
QVQLVQSGAEVKKPGASVKVSCKASGYTFTDFWMSWVRQAPGQGLEWMGQIYPNTGTTHSNEKFKGRVTMTRDTSTSTVYMELSSLRSEDTAVYYCARSYHISTTPNWFAYWGQGTLVTVSSASTKGPSVFPLAPSSKSTSGGTAALGCLVKDYFPEPVTVSWNSGALTSGVHTFPAVLQSSGLYSLSSVVTVPSSSLGTQTYICNVNHKPSNTKVDKKVEPKSCDKTHTCPPCPAPEAAGPSVFLFPPKPKDTLMISRTPEVTCVVVDVSHEDPEVKFNWYVDGVEVHNAKTKPREEQYNSTYRVVSVLTVLHQDWLNGKEYKCKVSNKALPAPIEKTISKAKGQPREPQVYTLPPSREEMTKNQVSLSCAVKGFYPSDIAVEWESNGQPENNYKTTPPVLDSDGSFFLVSKLTVDKSRWQQGNVFSCSVMHEALHNRFTQKSLSLSPGGGGGSGGGGSGGGGSGGGGSDIQMTQSPSSVSASVGDRVTITCRASQGIYSWLAWYQQKPGKAPNLLIYTASTLQSGVPSRFSGSGSGTDFTLTISSLQPEDFATYYCQQANIFPLTFGGGTKVEIK

SEQ ID NO: 275 - protein, 592 aa, synthetic construct
QVQLVQSGAEVKKPGASVKVSCKASGYTFTDFWMSWVRQAPGQGLEWMGQIYPNTGTTHSNEKFKGRVTMTRDTSTSTVYMELSSLRSEDTAVYYCARSYHISTTPNWFAYWGQGTLVTVSSASTKGPSVFPLAPSSKSTSGGTAALGCLVKDYFPEPVTVSWNSGALTSGVHTFPAVLQSSGLYSLSSVVTVPSSSLGTQTYICNVNHKPSNTKVDKKVEPKSCDKTHTCPPCPAPEAAGPSVFLFPPKPKDTLMISRTPEVTCVVVDVSHEDPEVKFNWYVDGVEVHNAKTKPREEQYNSTYRVVSVLTVLHQDWLNGKEYKCKVSNKALPAPIEKTISKAKGQPREPQVYTLPPSREEMTKNQVSLWCLVKGFYPSDIAVEWESNGQPENNYKTTPPVLDSDGSFFLYSKLTVDKSRWQQGNVFSCSVMHEALHNHYTQKSLSLSPGGGGGSGGGGSGGGGSGGGGSEVQLVESGGGLVQPGGSLRLSCAASGFTFTNYGLHWVRQAPGKGLEWVSSISPSGGVTYYRDSVKGRFTISRDNSKNTLYLQMNSLRAEDTAVYYCAKPFLGWGGANWIAHWGQGTLVTVSS

SEQ ID NO: 276 - protein, 577 aa, synthetic construct
QVQLVQSGAEVKKPGASVKVSCKASGYTFTDFWMSWVRQAPGQGLEWMGQIYPNTGTTHSNEKFKGRVTMTRDTSTSTVYMELSSLRSEDTAVYYCARSYHISTTPNWFAYWGQGTLVTVSSASTKGPSVFPLAPSSKSTSGGTAALGCLVKDYFPEPVTVSWNSGALTSGVHTFPAVLQSSGLYSLSSVVTVPSSSLGTQTYICNVNHKPSNTKVDKKVEPKSCDKTHTCPPCPAPEAAGPSVFLFPPKPKDTLMISRTPEVTCVVVDVSHEDPEVKFNWYVDGVEVHNAKTKPREEQYNSTYRVVSVLTVLHQDWLNGKEYKCKVSNKALPAPIEKTISKAKGQPREPQVYTLPPSREEMTKNQVSLSCAVKGFYPSDIAVEWESNGQPENNYKTTPPVLDSDGSFFLVSKLTVDKSRWQQGNVFSCSVMHEALHNRFTQKSLSLSPGGGGGSGGGGSGGGGSGGGGSDIQMTQSPSSLSASVGDRVTITCLASEDISNDLAWYQQKPGKAPKLLIYFVDRLLDGVPSRFSGSGSGTDFTLTISSLQPEDFATYYCQQSYKYPPTFGQGTKLEIK

SEQ ID NO: 277 - protein, 618 aa, synthetic construct
QVQLVQSGAEVKKPGASVKVSCKASGYTFTDFWMSWVRQAPGQGLEWMGQIYPNTGTTHSNEKFKGRVTMTRDTSTSTVYMELSSLRSEDTAVYYCARSYHISTTPNWFAYWGQGTLVTVSSASTKGPSVFPLAPSSKSTSGGTAALGCLVKDYFPEPVTVSWNSGALTSGVHTFPAVLQSSGLYSLSSVVTVPSSSLGTQTYICNVNHKPSNTKVDKKVEPKSCDKTHTCPPCPAPEAAGPSVFLFPPKPKDTLMISRTPEVTCVVVDVSHEDPEVKFNWYVDGVEVHNAKTKPREEQYNSTYRVVSVLTVLHQDWLNGKEYKCKVSNKALPAPIEKTISKAKGQPREPQVYTLPPSREEMTKNQVSLWCLVKGFYPSDIAVEWESNGQPENNYKTTPPVLDSDGSFFLYSKLTVDKSRWQQGNVFSCSVMHEALHNHYTQKSLSLSPGGGGGSGGGGSGGGGSGGGGSQVQLVQSGAEVKKPGASVKVSCKASGYTFTGYYMHWVRQAPGQGLEWMGWINPDSGGTNYAQKFQGRVTMTRDTSISTAYMELNRLRSDDTAVYYCARDQPLGYCTNGVCSYFDYWGQGTLVTVSSGGGGSDKTHTCPPCPAPEAAGP

SEQ ID NO: 278 - protein, 599 aa, synthetic construct
QVQLVQSGAEVKKPGASVKVSCKASGYTFTDFWMSWVRQAPGQGLEWMGQIYPNTGTTHSNEKFKGRVTMTRDTSTSTVYMELSSLRSEDTAVYYCARSYHISTTPNWFAYWGQGTLVTVSSASTKGPSVFPLAPSSKSTSGGTAALGCLVKDYFPEPVTVSWNSGALTSGVHTFPAVLQSSGLYSLSSVVTVPSSSLGTQTYICNVNHKPSNTKVDKKVEPKSCDKTHTCPPCPAPEAAGPSVFLFPPKPKDTLMISRTPEVTCVVVDVSHEDPEVKFNWYVDGVEVHNAKTKPREEQYNSTYRVVSVLTVLHQDWLNGKEYKCKVSNKALPAPIEKTISKAKGQPREPQVYTLPPSREEMTKNQVSLSCAVKGFYPSDIAVEWESNGQPENNYKTTPPVLDSDGSFFLVSKLTVDKSRWQQGNVFSCSVMHEALHNRFTQKSLSLSPGGGGGSGGGGSGGGGSGGGGSDIQMTQSPSSVSASVGDRVTITCRASQGIYSWLAWYQQKPGKAPNLLIYTASTLQSGVPSRFSGSGSGTDFTLTISSLQPEDFATYYCQQANIFPLTFGGGTKVEIKGGGGSDKTHTCPPCPAPEAAGP

SEQ ID NO: 279 - protein, 614 aa, synthetic construct
QVQLVQSGAEVKKPGASVKVSCKASGYTFTDFWMSWVRQAPGQGLEWMGQIYPNTGTTHSNEKFKGRVTMTRDTSTSTVYMELSSLRSEDTAVYYCARSYHISTTPNWFAYWGQGTLVTVSSASTKGPSVFPLAPSSKSTSGGTAALGCLVKDYFPEPVTVSWNSGALTSGVHTFPAVLQSSGLYSLSSVVTVPSSSLGTQTYICNVNHKPSNTKVDKKVEPKSCDKTHTCPPCPAPEAAGPSVFLFPPKPKDTLMISRTPEVTCVVVDVSHEDPEVKFNWYVDGVEVHNAKTKPREEQYNSTYRVVSVLTVLHQDWLNGKEYKCKVSNKALPAPIEKTISKAKGQPREPQVYTLPPSREEMTKNQVSLWCLVKGFYPSDIAVEWESNGQPENNYKTTPPVLDSDGSFFLYSKLTVDKSRWQQGNVFSCSVMHEALHNHYTQKSLSLSPGGGGGSGGGGSGGGGSGGGGSEVQLVESGGGLVQPGGSLRLSCAASGFTFTNYGLHWVRQAPGKGLEWVSSISPSGGVTYYRDSVKGRFTISRDNSKNTLYLQMNSLRAEDTAVYYCAKPFLGWGGANWIAHWGQGTLVTVSSGGGGSDKTHTCPPCPAPEAAGP

SEQ ID NO: 280 - protein, 599 aa, synthetic construct
QVQLVQSGAEVKKPGASVKVSCKASGYTFTDFWMSWVRQAPGQGLEWMGQIYPNTGTTHSNEKFKGRVTMTRDTSTSTVYMELSSLRSEDTAVYYCARSYHISTTPNWFAYWGQGTLVTVSSASTKGPSVFPLAPSSKSTSGGTAALGCLVKDYFPEPVTVSWNSGALTSGVHTFPAVLQSSGLYSLSSVVTVPSSSLGTQTYICNVNHKPSNTKVDKKVEPKSCDKTHTCPPCPAPEAAGPSVFLFPPKPKDTLMISRTPEVTCVVVDVSHEDPEVKFNWYVDGVEVHNAKTKPREEQYNSTYRVVSVLTVLHQDWLNGKEYKCKVSNKALPAPIEKTISKAKGQPREPQVYTLPPSREEMTKNQVSLSCAVKGFYPSDIAVEWESNGQPENNYKTTPPVLDSDGSFFLVSKLTVDKSRWQQGNVFSCSVMHEALHNRFTQKSLSLSPGGGGGSGGGGSGGGGSGGGGSDIQMTQSPSSLSASVGDRVTITCLASEDISNDLAWYQQKPGKAPKLLIYFVDRLLDGVPSRFSGSGSGTDFTLTISSLQPEDFATYYCQQSYKYPPTFGQGTKLEIKGGGGSDKTHTCPPCPAPEAAGP

SEQ ID NO: 281 - protein, 586 aa, synthetic construct
QVQLVQSGAEVKKPGASVKVSCKASGYTFTDFWMSWVRQAPGQGLEWMGQIYPNTGTTHSNEKFKGRVTMTRDTSTSTVYMELSSLRSEDTAVYYCARSYHISTTPNWFAYWGQGTLVTVSSASTKGPSVFPLAPSSKSTSGGTAALGCLVKDYFPEPVTVSWNSGALTSGVHTFPAVLQSSGLYSLSSVVTVPSSSLGTQTYICNVNHKPSNTKVDKKVEPKSCDKTHTCPPCPAPEAAGPSVFLFPPKPKDTLMISRTPEVTCVVVDVSHEDPEVKFNWYVDGVEVHNAKTKPREEQYNSTYRVVSVLTVLHQDWLNGKEYKCKVSNKALPAPIEKTISKAKGQPREPQVYTLPPSREEMTKNQVSLWCLVKGFYPSDIAVEWESNGQPENNYKTTPPVLDSDGSFFLYSKLTVDKSRWQQGNVFSCSVMHEALHNHYTQKSLSLSPGGGGGSGGGGSGGGGSGGGGSQVQLVQSGAEVKKPGASVKVSCKASGYTFAGFEMHWVRQAPGQGLEWMGAIDPKTGGTDYNQKFKDRVTMTRDTSISTAYMELSRLRSDDTAVYYCARDLGYFDVWGQGTLVTVSS

SEQ ID NO: 282 - protein, 577 aa, synthetic construct
QVQLVQSGAEVKKPGASVKVSCKASGYTFTDFWMSWVRQAPGQGLEWMGQIYPNTGTTHSNEKFKGRVTMTRDTSTSTVYMELSSLRSEDTAVYYCARSYHISTTPNWFAYWGQGTLVTVSSASTKGPSVFPLAPSSKSTSGGTAALGCLVKDYFPEPVTVSWNSGALTSGVHTFPAVLQSSGLYSLSSVVTVPSSSLGTQTYICNVNHKPSNTKVDKKVEPKSCDKTHTCPPCPAPEAAGPSVFLFPPKPKDTLMISRTPEVTCVVVDVSHEDPEVKFNWYVDGVEVHNAKTKPREEQYNSTYRVVSVLTVLHQDWLNGKEYKCKVSNKALPAPIEKTISKAKGQPREPQVYTLPPSREEMTKNQVSLSCAVKGFYPSDIAVEWESNGQPENNYKTTPPVLDSDGSFFLVSKLTVDKSRWQQGNVFSCSVMHEALHNRFTQKSLSLSPGGGGGSGGGGSGGGGSGGGGSDIQMTQSPSSLSASVGDRVTITCRASQDIRSNLNWYQQKPGGAVKLLIYYTSRLHSGVPSRFSGSGSGTDYTLTISSLQPEDFATYFCQQSEKLPRTFGGGTKVEIR

SEQ ID NO: 283 - protein, 582 aa, synthetic construct
QVQLVQSGAEVKKPGASVKVSCKASGYTFTDFWMSWVRQAPGQGLEWMGQIYPNTGTTHSNEKFKGRVTMTRDTSTSTVYMELSSLRSEDTAVYYCARSYHISTTPNWFAYWGQGTLVTVSSASTKGPSVFPLAPSSKSTSGGTAALGCLVKDYFPEPVTVSWNSGALTSGVHTFPAVLQSSGLYSLSSVVTVPSSSLGTQTYICNVNHKPSNTKVDKKVEPKSCGGGGSGGGGSGGGGSGGGGSDIQMTQSPSSVSASVGDRVTITCRASQGIYSWLAWYQQKPGKAPNLLIYTASTLQSGVPSRFSGSGSGTDFTLTISSLQPEDFATYYCQQANIFPLTFGGGTKVEIKGGGGSDKTHTCPPCPAPEAAGPSVFLFPPKPKDTLMISRTPEVTCVVVDVSHEDPEVKFNWYVDGVEVHNAKTKPREEQYNSTYRVVSVLTVLHQDWLNGKEYKCKVSNKALPAPIEKTISKAKGQPREPQVYTLPPSREEMTKNQVSLSCAVKGFYPSDIAVEWESNGQPENNYKTTPPVLDSDGSFFLVSKLTVDKSRWQQGNVFSCSVMHEALHNRFTQKSLSLSPG

SEQ ID NO: 284 - protein, 582 aa, synthetic construct
QVQLVQSGAEVKKPGASVKVSCKASGYTFTDFWMSWVRQAPGQGLEWMGQIYPNTGTTHSNEKFKGRVTMTRDTSTSTVYMELSSLRSEDTAVYYCARSYHISTTPNWFAYWGQGTLVTVSSASTKGPSVFPLAPSSKSTSGGTAALGCLVKDYFPEPVTVSWNSGALTSGVHTFPAVLQSSGLYSLSSVVTVPSSSLGTQTYICNVNHKPSNTKVDKKVEPKSCGGGGSGGGGSGGGGSGGGGSDIQMTQSPSSLSASVGDRVTITCLASEDISNDLAWYQQKPGKAPKLLIYFVDRLLDGVPSRFSGSGSGTDFTLTISSLQPEDFATYYCQQSYKYPPTFGQGTKLEIKGGGGSDKTHTCPPCPAPEAAGPSVFLFPPKPKDTLMISRTPEVTCVVVDVSHEDPEVKFNWYVDGVEVHNAKTKPREEQYNSTYRVVSVLTVLHQDWLNGKEYKCKVSNKALPAPIEKTISKAKGQPREPQVYTLPPSREEMTKNQVSLSCAVKGFYPSDIAVEWESNGQPENNYKTTPPVLDSDGSFFLVSKLTVDKSRWQQGNVFSCSVMHEALHNRFTQKSLSLSPG

SEQ ID NO: 285 - protein, 709 aa, synthetic construct
QVQLVQSGAEVKKPGASVKVSCKASGYTFTDFWMSWVRQAPGQGLEWMGQIYPNTGTTHSNEKFKGRVTMTRDTSTSTVYMELSSLRSEDTAVYYCARSYHISTTPNWFAYWGQGTLVTVSSASTKGPSVFPLAPSSKSTSGGTAALGCLVKDYFPEPVTVSWNSGALTSGVHTFPAVLQSSGLYSLSSVVTVPSSSLGTQTYICNVNHKPSNTKVDKKVEPKSCGGGGSGGGGSGGGGSGGGGSDIQMTQSPSSVSASVGDRVTITCRASQGIYSWLAWYQQKPGKAPNLLIYTASTLQSGVPSRFSGSGSGTDFTLTISSLQPEDFATYYCQQANIFPLTFGGGTKVEIKGGGGSDKTHTCPPCPAPEAAGPSVFLFPPKPKDTLMISRTPEVTCVVVDVSHEDPEVKFNWYVDGVEVHNAKTKPREEQYNSTYRVVSVLTVLHQDWLNGKEYKCKVSNKALPAPIEKTISKAKGQPREPQVYTLPPSREEMTKNQVSLSCAVKGFYPSDIAVEWESNGQPENNYKTTPPVLDSDGSFFLVSKLTVDKSRWQQGNVFSCSVMHEALHNRFTQKSLSLSPGGGGGSGGGGSGGGGSGGGGSDIQMTQSPSSLSASVGDRVTITCRASQDIRSNLNWYQQKPGGAVKLLIYYTSRLHSGVPSRFSGSGSGTDYTLTISSLQPEDFATYFCQQSEKLPRTFGGGTKVEIR

SEQ ID NO: 286 - protein, 709 aa, synthetic construct
QVQLVQSGAEVKKPGASVKVSCKASGYTFTDFWMSWVRQAPGQGLEWMGQIYPNTGTTHSNEKFKGRVTMTRDTSTSTVYMELSSLRSEDTAVYYCARSYHISTTPNWFAYWGQGTLVTVSSASTKGPSVFPLAPSSKSTSGGTAALGCLVKDYFPEPVTVSWNSGALTSGVHTFPAVLQSSGLYSLSSVVTVPSSSLGTQTYICNVNHKPSNTKVDKKVEPKSCGGGGSGGGGSGGGGSGGGGSDIQMTQSPSSLSASVGDRVTITCLASEDISNDLAWYQQKPGKAPKLLIYFVDRLLDGVPSRFSGSGSGTDFTLTISSLQPEDFATYYCQQSYKYPPTFGQGTKLEIKGGGGSDKTHTCPPCPAPEAAGPSVFLFPPKPKDTLMISRTPEVTCVVVDVSHEDPEVKFNWYVDGVEVHNAKTKPREEQYNSTYRVVSVLTVLHQDWLNGKEYKCKVSNKALPAPIEKTISKAKGQPREPQVYTLPPSREEMTKNQVSLSCAVKGFYPSDIAVEWESNGQPENNYKTTPPVLDSDGSFFLVSKLTVDKSRWQQGNVFSCSVMHEALHNRFTQKSLSLSPGGGGGSGGGGSGGGGSGGGGSDIQMTQSPSSLSASVGDRVTITCRASQDIRSNLNWYQQKPGGAVKLLIYYTSRLHSGVPSRFSGSGSGTDYTLTISSLQPEDFATYFCQQSEKLPRTFGGGTKVEIR

SEQ ID NO: 287 - protein, 709 aa, synthetic construct
QVQLVQSGAEVKKPGASVKVSCKASGYTFTDFWMSWVRQAPGQGLEWMGQIYPNTGTTHSNEKFKGRVTMTRDTSTSTVYMELSSLRSEDTAVYYCARSYHISTTPNWFAYWGQGTLVTVSSASTKGPSVFPLAPSSKSTSGGTAALGCLVKDYFPEPVTVSWNSGALTSGVHTFPAVLQSSGLYSLSSVVTVPSSSLGTQTYICNVNHKPSNTKVDKKVEPKSCGGGGSGGGGSGGGGSGGGGSDIQMTQSPSSLSASVGDRVTITCRASQDIRSNLNWYQQKPGGAVKLLIYYTSRLHSGVPSRFSGSGSGTDYTLTISSLQPEDFATYFCQQSEKLPRTFGGGTKVEIRGGGGSDKTHTCPPCPAPEAAGPSVFLFPPKPKDTLMISRTPEVTCVVVDVSHEDPEVKFNWYVDGVEVHNAKTKPREEQYNSTYRVVSVLTVLHQDWLNGKEYKCKVSNKALPAPIEKTISKAKGQPREPQVYTLPPSREEMTKNQVSLSCAVKGFYPSDIAVEWESNGQPENNYKTTPPVLDSDGSFFLVSKLTVDKSRWQQGNVFSCSVMHEALHNRFTQKSLSLSPGGGGGSGGGGSGGGGSGGGGSDIQMTQSPSSVSASVGDRVTITCRASQGIYSWLAWYQQKPGKAPNLLIYTASTLQSGVPSRFSGSGSGTDFTLTISSLQPEDFATYYCQQANIFPLTFGGGTKVEIK

SEQ ID NO: 288 - protein, 709 aa, synthetic construct
QVQLVQSGAEVKKPGASVKVSCKASGYTFTDFWMSWVRQAPGQGLEWMGQIYPNTGTTHSNEKFKGRVTMTRDTSTSTVYMELSSLRSEDTAVYYCARSYHISTTPNWFAYWGQGTLVTVSSASTKGPSVFPLAPSSKSTSGGTAALGCLVKDYFPEPVTVSWNSGALTSGVHTFPAVLQSSGLYSLSSVVTVPSSSLGTQTYICNVNHKPSNTKVDKKVEPKSCGGGGSGGGGSGGGGSGGGGSDIQMTQSPSSLSASVGDRVTITCRASQDIRSNLNWYQQKPGGAVKLLIYYTSRLHSGVPSRFSGSGSGTDYTLTISSLQPEDFATYFCQQSEKLPRTFGGGTKVEIRGGGGSDKTHTCPPCPAPEAAGPSVFLFPPKPKDTLMISRTPEVTCVVVDVSHEDPEVKFNWYVDGVEVHNAKTKPREEQYNSTYRVVSVLTVLHQDWLNGKEYKCKVSNKALPAPIEKTISKAKGQPREPQVYTLPPSREEMTKNQVSLSCAVKGFYPSDIAVEWESNGQPENNYKTTPPVLDSDGSFFLVSKLTVDKSRWQQGNVFSCSVMHEALHNRFTQKSLSLSPGGGGGSGGGGSGGGGSGGGGSDIQMTQSPSSLSASVGDRVTITCLASEDISNDLAWYQQKPGKAPKLLIYFVDRLLDGVPSRFSGSGSGTDFTLTISSLQPEDFATYYCQQSYKYPPTFGQGTKLEIK

SEQ ID NO: 289 - protein, 582 aa, synthetic construct
QVQLVQSGAEVKKPGASVKVSCKASGYTFTDFWMSWVRQAPGQGLEWMGQIYPNTGTTHSNEKFKGRVTMTRDTSTSTVYMELSSLRSEDTAVYYCARSYHISTTPNWFAYWGQGTLVTVSSASTKGPSVFPLAPSSKSTSGGTAALGCLVKDYFPEPVTVSWNSGALTSGVHTFPAVLQSSGLYSLSSVVTVPSSSLGTQTYICNVNHKPSNTKVDKKVEPKSCGGGGSGGGGSGGGGSGGGGSDIQMTQSPSSLSASVGDRVTITCRASQDIRSNLNWYQQKPGGAVKLLIYYTSRLHSGVPSRFSGSGSGTDYTLTISSLQPEDFATYFCQQSEKLPRTFGGGTKVEIRGGGGSDKTHTCPPCPAPEAAGPSVFLFPPKPKDTLMISRTPEVTCVVVDVSHEDPEVKFNWYVDGVEVHNAKTKPREEQYNSTYRVVSVLTVLHQDWLNGKEYKCKVSNKALPAPIEKTISKAKGQPREPQVYTLPPSREEMTKNQVSLSCAVKGFYPSDIAVEWESNGQPENNYKTTPPVLDSDGSFFLVSKLTVDKSRWQQGNVFSCSVMHEALHNRFTQKSLSLSPG

SEQ ID NO: 290 - protein, 597 aa, synthetic construct
QVQLVQSGAEVKKPGASVKVSCKASGYTFTDFWMSWVRQAPGQGLEWMGQIYPNTGTTHSNEKFKGRVTMTRDTSTSTVYMELSSLRSEDTAVYYCARSYHISTTPNWFAYWGQGTLVTVSSASTKGPSVFPLAPSSKSTSGGTAALGCLVKDYFPEPVTVSWNSGALTSGVHTFPAVLQSSGLYSLSSVVTVPSSSLGTQTYICNVNHKPSNTKVDKKVEPKSCGGGGSGGGGSGGGGSGGGGSEVQLVESGGGLVQPGGSLRLSCAASGFTFTNYGLHWVRQAPGKGLEWVSSISPSGGVTYYRDSVKGRFTISRDNSKNTLYLQMNSLRAEDTAVYYCAKPFLGWGGANWIAHWGQGTLVTVSSGGGGSDKTHTCPPCPAPEAAGPSVFLFPPKPKDTLMISRTPEVTCVVVDVSHEDPEVKFNWYVDGVEVHNAKTKPREEQYNSTYRVVSVLTVLHQDWLNGKEYKCKVSNKALPAPIEKTISKAKGQPREPQVYTLPPSREEMTKNQVSLWCLVKGFYPSDIAVEWESNGQPENNYKTTPPVLDSDGSFFLYSKLTVDKSRWQQGNVFSCSVMHEALHNHYTQKSLSLSPG

SEQ ID NO: 291 - protein, 600 aa, synthetic construct
QVQLVQSGAEVKKPGASVKVSCKASGYTFTDFWMSWVRQAPGQGLEWMGQIYPNTGTTHSNEKFKGRVTMTRDTSTSTVYMELSSLRSEDTAVYYCARSYHISTTPNWFAYWGQGTLVTVSSASTKGPSVFPLAPSSKSTSGGTAALGCLVKDYFPEPVTVSWNSGALTSGVHTFPAVLQSSGLYSLSSVVTVPSSSLGTQTYICNVNHKPSNTKVDKKVEPKSCGGGGSGGGGSGGGGSGGGGSEVQLVESGGGLVQPGGSLRLSCAASGFTFSTYAMNWVRQAPGKGLEWVGRIRSKYNNYATYYADSVKGRFTISRDDSKNSLYLQMNSLKTEDTAVYYCVRHGNFGNSYVSWFAYWGQGTLVTVSSGGGGSDKTHTCPPCPAPEAAGPSVFLFPPKPKDTLMISRTPEVTCVVVDVSHEDPEVKFNWYVDGVEVHNAKTKPREEQYNSTYRVVSVLTVLHQDWLNGKEYKCKVSNKALPAPIEKTISKAKGQPREPQVYTLPPSREEMTKNQVSLWCLVKGFYPSDIAVEWESNGQPENNYKTTPPVLDSDGSFFLYSKLTVDKSRWQQGNVFSCSVMHEALHNHYTQKSLSLSPG

SEQ ID NO: 292 - protein, 736 aa, synthetic construct
QVQLVQSGAEVKKPGASVKVSCKASGYTFTDFWMSWVRQAPGQGLEWMGQIYPNTGTTHSNEKFKGRVTMTRDTSTSTVYMELSSLRSEDTAVYYCARSYHISTTPNWFAYWGQGTLVTVSSASTKGPSVFPLAPSSKSTSGGTAALGCLVKDYFPEPVTVSWNSGALTSGVHTFPAVLQSSGLYSLSSVVTVPSSSLGTQTYICNVNHKPSNTKVDKKVEPKSCGGGGSGGGGSGGGGSGGGGSEVQLVESGGGLVQPGGSLRLSCAASGFTFSTYAMNWVRQAPGKGLEWVGRIRSKYNNYATYYADSVKGRFTISRDDSKNSLYLQMNSLKTEDTAVYYCVRHGNFGNSYVSWFAYWGQGTLVTVSSGGGGSDKTHTCPPCPAPEAAGPSVFLFPPKPKDTLMISRTPEVTCVVVDVSHEDPEVKFNWYVDGVEVHNAKTKPREEQYNSTYRVVSVLTVLHQDWLNGKEYKCKVSNKALPAPIEKTISKAKGQPREPQVYTLPPSREEMTKNQVSLWCLVKGFYPSDIAVEWESNGQPENNYKTTPPVLDSDGSFFLYSKLTVDKSRWQQGNVFSCSVMHEALHNHYTQKSLSLSPGGGGGSGGGGSGGGGSGGGGSQVQLVQSGAEVKKPGASVKVSCKASGYTFAGFEMHWVRQAPGQGLEWMGAIDPKTGGTDYNQKFKDRVTMTRDTSISTAYMELSRLRSDDTAVYYCARDLGYFDVWGQGTLVTVSS

SEQ ID NO: 293 - protein, 740 aa, synthetic construct
QVQLVQSGAEVKKPGASVKVSCKASGYTFTDFWMSWVRQAPGQGLEWMGQIYPNTGTTHSNEKFKGRVTMTRDTSTSTVYMELSSLRSEDTAVYYCARSYHISTTPNWFAYWGQGTLVTVSSASTKGPSVFPLAPSSKSTSGGTAALGCLVKDYFPEPVTVSWNSGALTSGVHTFPAVLQSSGLYSLSSVVTVPSSSLGTQTYICNVNHKPSNTKVDKKVEPKSCGGGGSGGGGSGGGGSGGGGSEVQLVESGGGLVQPGGSLRLSCAASGFTFSTYAMNWVRQAPGKGLEWVGRIRSKYNNYATYYADSVKGRFTISRDDSKNSLYLQMNSLKTEDTAVYYCVRHGNFGNSYVSWFAYWGQGTLVTVSSGGGGSDKTHTCPPCPAPEAAGPSVFLFPPKPKDTLMISRTPEVTCVVVDVSHEDPEVKFNWYVDGVEVHNAKTKPREEQYNSTYRVVSVLTVLHQDWLNGKEYKCKVSNKALPAPIEKTISKAKGQPREPQVYTLPPSREEMTKNQVSLWCLVKGFYPSDIAVEWESNGQPENNYKTTPPVLDSDGSFFLYSKLTVDKSRWQQGNVFSCSVMHEALHNHYTQKSLSLSPGGGGGSGGGGSGGGGSGGGGSQVQLVQSGAEVKKPGASVKVSCKASGYTFTSYYIHWVRQAPGQGLEWIGCIYPGNVNTNYNEKFKDRATLTVDTSISTAYMELSRLRSDDTAVYFCTRSHYGLDWNFDVWGQGTTVTVSS

SEQ ID NO: 294 - protein, 733 aa, synthetic construct
QVQLVQSGAEVKKPGASVKVSCKASGYTFTDFWMSWVRQAPGQGLEWMGQIYPNTGTTHSNEKFKGRVTMTRDTSTSTVYMELSSLRSEDTAVYYCARSYHISTTPNWFAYWGQGTLVTVSSASTKGPSVFPLAPSSKSTSGGTAALGCLVKDYFPEPVTVSWNSGALTSGVHTFPAVLQSSGLYSLSSVVTVPSSSLGTQTYICNVNHKPSNTKVDKKVEPKSCGGGGSGGGGSGGGGSGGGGSEVQLVESGGGLVQPGGSLRLSCAASGFTFTNYGLHWVRQAPGKGLEWVSSISPSGGVTYYRDSVKGRFTISRDNSKNTLYLQMNSLRAEDTAVYYCAKPFLGWGGANWIAHWGQGTLVTVSSGGGGSDKTHTCPPCPAPEAAGPSVFLFPPKPKDTLMISRTPEVTCVVVDVSHEDPEVKFNWYVDGVEVHNAKTKPREEQYNSTYRVVSVLTVLHQDWLNGKEYKCKVSNKALPAPIEKTISKAKGQPREPQVYTLPPSREEMTKNQVSLWCLVKGFYPSDIAVEWESNGQPENNYKTTPPVLDSDGSFFLYSKLTVDKSRWQQGNVFSCSVMHEALHNHYTQKSLSLSPGGGGGSGGGGSGGGGSGGGGSQVQLVQSGAEVKKPGASVKVSCKASGYTFAGFEMHWVRQAPGQGLEWMGAIDPKTGGTDYNQKFKDRVTMTRDTSISTAYMELSRLRSDDTAVYYCARDLGYFDVWGQGTLVTVSS

SEQ ID NO: 295 - protein, 584 aa, synthetic construct
QVQLVQSGAEVKKPGASVKVSCKASGYTFTDFWMSWVRQAPGQGLEWMGQIYPNTGTTHSNEKFKGRVTMTRDTSTSTVYMELSSLRSEDTAVYYCARSYHISTTPNWFAYWGQGTLVTVSSASTKGPSVFPLAPSSKSTSGGTAALGCLVKDYFPEPVTVSWNSGALTSGVHTFPAVLQSSGLYSLSSVVTVPSSSLGTQTYICNVNHKPSNTKVDKKVEPKSCGGGGSGGGGSGGGGSGGGGSQAVVTQEPSLTVSPGGTVTLTCRSSTGAVTTSNYANWVQQKPGQAPRGLIGGTNKRAPWTPARFSGSLLGGKAALTITGAQAEDEADYYCALWYSNLWVFGGGTKLTVLGGGGSDKTHTCPPCPAPEAAGPSVFLFPPKPKDTLMISRTPEVTCVVVDVSHEDPEVKFNWYVDGVEVHNAKTKPREEQYNSTYRVVSVLTVLHQDWLNGKEYKCKVSNKALPAPIEKTISKAKGQPREPQVYTLPPSREEMTKNQVSLSCAVKGFYPSDIAVEWESNGQPENNYKTTPPVLDSDGSFFLVSKLTVDKSRWQQGNVFSCSVMHEALHNRFTQKSLSLSPG

SEQ ID NO: 296 - protein, 711 aa, synthetic construct
QVQLVQSGAEVKKPGASVKVSCKASGYTFTDFWMSWVRQAPGQGLEWMGQIYPNTGTTHSNEKFKGRVTMTRDTSTSTVYMELSSLRSEDTAVYYCARSYHISTTPNWFAYWGQGTLVTVSSASTKGPSVFPLAPSSKSTSGGTAALGCLVKDYFPEPVTVSWNSGALTSGVHTFPAVLQSSGLYSLSSVVTVPSSSLGTQTYICNVNHKPSNTKVDKKVEPKSCGGGGSGGGGSGGGGSGGGGSQAVVTQEPSLTVSPGGTVTLTCRSSTGAVTTSNYANWVQQKPGQAPRGLIGGTNKRAPWTPARFSGSLLGGKAALTITGAQAEDEADYYCALWYSNLWVFGGGTKLTVLGGGGSDKTHTCPPCPAPEAAGPSVFLFPPKPKDTLMISRTPEVTCVVVDVSHEDPEVKFNWYVDGVEVHNAKTKPREEQYNSTYRVVSVLTVLHQDWLNGKEYKCKVSNKALPAPIEKTISKAKGQPREPQVYTLPPSREEMTKNQVSLSCAVKGFYPSDIAVEWESNGQPENNYKTTPPVLDSDGSFFLVSKLTVDKSRWQQGNVFSCSVMHEALHNRFTQKSLSLSPGGGGGSGGGGSGGGGSGGGGSDIQMTQSPSSLSASVGDRVTITCRASQDIRSNLNWYQQKPGGAVKLLIYYTSRLHSGVPSRFSGSGSGTDYTLTISSLQPEDFATYFCQQSEKLPRTFGGGTKVEIR

SEQ ID NO: 297 - protein, 711 aa, synthetic construct
QVQLVQSGAEVKKPGASVKVSCKASGYTFTDFWMSWVRQAPGQGLEWMGQIYPNTGTTHSNEKFKGRVTMTRDTSTSTVYMELSSLRSEDTAVYYCARSYHISTTPNWFAYWGQGTLVTVSSASTKGPSVFPLAPSSKSTSGGTAALGCLVKDYFPEPVTVSWNSGALTSGVHTFPAVLQSSGLYSLSSVVTVPSSSLGTQTYICNVNHKPSNTKVDKKVEPKSCGGGGSGGGGSGGGGSGGGGSQAVVTQEPSLTVSPGGTVTLTCRSSTGAVTTSNYANWVQQKPGQAPRGLIGGTNKRAPWTPARFSGSLLGGKAALTITGAQAEDEADYYCALWYSNLWVFGGGTKLTVLGGGGSDKTHTCPPCPAPEAAGPSVFLFPPKPKDTLMISRTPEVTCVVVDVSHEDPEVKFNWYVDGVEVHNAKTKPREEQYNSTYRVVSVLTVLHQDWLNGKEYKCKVSNKALPAPIEKTISKAKGQPREPQVYTLPPSREEMTKNQVSLSCAVKGFYPSDIAVEWESNGQPENNYKTTPPVLDSDGSFFLVSKLTVDKSRWQQGNVFSCSVMHEALHNRFTQKSLSLSPGGGGGSGGGGSGGGGSGGGGSDIQMTQSPSSLSASVGDRVTITCHASQNIYVWLNWYQQKPGKAPKLLIYKASNLHTGVPSRFSGSGSGTDFTLTISSLQPEDFATYYCQQGQTYPYTFGGGTKVEIK

SEQ ID NO: 298 - protein, 601 aa, synthetic construct
QVQLVQSGAEVKKPGASVKVSCKASGYTFTDFWMSWVRQAPGQGLEWMGQIYPNTGTTHSNEKFKGRVTMTRDTSTSTVYMELSSLRSEDTAVYYCARSYHISTTPNWFAYWGQGTLVTVSSASTKGPSVFPLAPSSKSTSGGTAALGCLVKDYFPEPVTVSWNSGALTSGVHTFPAVLQSSGLYSLSSVVTVPSSSLGTQTYICNVNHKPSNTKVDKKVEPKSCGGGGSGGGGSGGGGSGGGGSQVQLVQSGAEVKKPGASVKVSCKASGYTFTGYYMHWVRQAPGQGLEWMGWINPDSGGTNYAQKFQGRVTMTRDTSISTAYMELNRLRSDDTAVYYCARDQPLGYCTNGVCSYFDYWGQGTLVTVSSGGGGSDKTHTCPPCPAPEAAGPSVFLFPPKPKDTLMISRTPEVTCVVVDVSHEDPEVKFNWYVDGVEVHNAKTKPREEQYNSTYRVVSVLTVLHQDWLNGKEYKCKVSNKALPAPIEKTISKAKGQPREPQVYTLPPSREEMTKNQVSLWCLVKGFYPSDIAVEWESNGQPENNYKTTPPVLDSDGSFFLYSKLTVDKSRWQQGNVFSCSVMHEALHNHYTQKSLSLSPG

SEQ ID NO: 299 - protein, 737 aa, synthetic construct
QVQLVQSGAEVKKPGASVKVSCKASGYTFTDFWMSWVRQAPGQGLEWMGQIYPNTGTTHSNEKFKGRVTMTRDTSTSTVYMELSSLRSEDTAVYYCARSYHISTTPNWFAYWGQGTLVTVSSASTKGPSVFPLAPSSKSTSGGTAALGCLVKDYFPEPVTVSWNSGALTSGVHTFPAVLQSSGLYSLSSVVTVPSSSLGTQTYICNVNHKPSNTKVDKKVEPKSCGGGGSGGGGSGGGGSGGGGSQVQLVQSGAEVKKPGASVKVSCKASGYTFTGYYMHWVRQAPGQGLEWMGWINPDSGGTNYAQKFQGRVTMTRDTSISTAYMELNRLRSDDTAVYYCARDQPLGYCTNGVCSYFDYWGQGTLVTVSSGGGGSDKTHTCPPCPAPEAAGPSVFLFPPKPKDTLMISRTPEVTCVVVDVSHEDPEVKFNWYVDGVEVHNAKTKPREEQYNSTYRVVSVLTVLHQDWLNGKEYKCKVSNKALPAPIEKTISKAKGQPREPQVYTLPPSREEMTKNQVSLWCLVKGFYPSDIAVEWESNGQPENNYKTTPPVLDSDGSFFLYSKLTVDKSRWQQGNVFSCSVMHEALHNHYTQKSLSLSPGGGGGSGGGGSGGGGSGGGGSQVQLVQSGAEVKKPGASVKVSCKASGYTFAGFEMHWVRQAPGQGLEWMGAIDPKTGGTDYNQKFKDRVTMTRDTSISTAYMELSRLRSDDTAVYYCARDLGYFDVWGQGTLVTVSS

SEQ ID NO: 300 - protein, 737 aa, synthetic construct
QVQLVQSGAEVKKPGASVKVSCKASGYTFTDFWMSWVRQAPGQGLEWMGQIYPNTGTTHSNEKFKGRVTMTRDTSTSTVYMELSSLRSEDTAVYYCARSYHISTTPNWFAYWGQGTLVTVSSASTKGPSVFPLAPSSKSTSGGTAALGCLVKDYFPEPVTVSWNSGALTSGVHTFPAVLQSSGLYSLSSVVTVPSSSLGTQTYICNVNHKPSNTKVDKKVEPKSCGGGGSGGGGSGGGGSGGGGSQVQLVQSGAEVKKPGASVKVSCKASGYTFAGFEMHWVRQAPGQGLEWMGAIDPKTGGTDYNQKFKDRVTMTRDTSISTAYMELSRLRSDDTAVYYCARDLGYFDVWGQGTLVTVSSGGGGSDKTHTCPPCPAPEAAGPSVFLFPPKPKDTLMISRTPEVTCVVVDVSHEDPEVKFNWYVDGVEVHNAKTKPREEQYNSTYRVVSVLTVLHQDWLNGKEYKCKVSNKALPAPIEKTISKAKGQPREPQVYTLPPSREEMTKNQVSLWCLVKGFYPSDIAVEWESNGQPENNYKTTPPVLDSDGSFFLYSKLTVDKSRWQQGNVFSCSVMHEALHNHYTQKSLSLSPGGGGGSGGGGSGGGGSGGGGSQVQLVQSGAEVKKPGASVKVSCKASGYTFTGYYMHWVRQAPGQGLEWMGWINPDSGGTNYAQKFQGRVTMTRDTSISTAYMELNRLRSDDTAVYYCARDQPLGYCTNGVCSYFDYWGQGTLVTVSS

SEQ ID NO: 301 - protein, 733 aa, synthetic construct
QVQLVQSGAEVKKPGASVKVSCKASGYTFTDFWMSWVRQAPGQGLEWMGQIYPNTGTTHSNEKFKGRVTMTRDTSTSTVYMELSSLRSEDTAVYYCARSYHISTTPNWFAYWGQGTLVTVSSASTKGPSVFPLAPSSKSTSGGTAALGCLVKDYFPEPVTVSWNSGALTSGVHTFPAVLQSSGLYSLSSVVTVPSSSLGTQTYICNVNHKPSNTKVDKKVEPKSCGGGGSGGGGSGGGGSGGGGSQVQLVQSGAEVKKPGASVKVSCKASGYTFAGFEMHWVRQAPGQGLEWMGAIDPKTGGTDYNQKFKDRVTMTRDTSISTAYMELSRLRSDDTAVYYCARDLGYFDVWGQGTLVTVSSGGGGSDKTHTCPPCPAPEAAGPSVFLFPPKPKDTLMISRTPEVTCVVVDVSHEDPEVKFNWYVDGVEVHNAKTKPREEQYNSTYRVVSVLTVLHQDWLNGKEYKCKVSNKALPAPIEKTISKAKGQPREPQVYTLPPSREEMTKNQVSLWCLVKGFYPSDIAVEWESNGQPENNYKTTPPVLDSDGSFFLYSKLTVDKSRWQQGNVFSCSVMHEALHNHYTQKSLSLSPGGGGGSGGGGSGGGGSGGGGSEVQLVESGGGLVQPGGSLRLSCAASGFTFTNYGLHWVRQAPGKGLEWVSSISPSGGVTYYRDSVKGRFTISRDNSKNTLYLQMNSLRAEDTAVYYCAKPFLGWGGANWIAHWGQGTLVTVSS

SEQ ID NO: 302 - protein, 591 aa, synthetic construct
QVQLVQSGAEVKKPGASVKVSCKASGYTFTDFWMSWVRQAPGQGLEWMGQIYPNTGTTHSNEKFKGRVTMTRDTSTSTVYMELSSLRSEDTAVYYCARSYHISTTPNWFAYWGQGTLVTVSSASTKGPSVFPLAPSSKSTSGGTAALGCLVKDYFPEPVTVSWNSGALTSGVHTFPAVLQSSGLYSLSSVVTVPSSSLGTQTYICNVNHKPSNTKVDKKVEPKSCGGGGSGGGGSGGGGSGGGGSQVQLVQSGAEVKKPGASVKVSCKASGYTFAGFEMHWVRQAPGQGLEWMGAIDPKTGGTDYNQKFKDRVTMTRDTSISTAYMELSRLRSDDTAVYYCARDLGYFDVWGQGTLVTVSSGGGGSDKTHTCPPCPAPEAAGPSVFLFPPKPKDTLMISRTPEVTCVVVDVSHEDPEVKFNWYVDGVEVHNAKTKPREEQYNSTYRVVSVLTVLHQDWLNGKEYKCKVSNKALPAPIEKTISKAKGQPREPQVYTLPPSREEMTKNQVSLWCLVKGFYPSDIAVEWESNGQPENNYKTTPPVLDSDGSFFLYSKLTVDKSRWQQGNVFSCSVMHEALHNHYTQKSLSLSPG

SEQ ID NO: 303 - protein, 585 aa, synthetic construct
QVQLVQSGAEVKKPGASVKVSCKASGYTFTEFGMNWVRQAPGQGLEWMGWINTKTGEATYVEEFKGRVTFTTDTSTSTAYMELRSLRSDDTAVYYCARWDFAYYVEAMDYWGQGTTVTVSSASTKGPSVFPLAPSSKSTSGGTAALGCLVKDYFPEPVTVSWNSGALTSGVHTFPAVLQSSGLYSLSSVVTVPSSSLGTQTYICNVNHKPSNTKVDKKVEPKSCDKTHTCPPCPAPEAAGPSVFLFPPKPKDTLMISRTPEVTCVVVDVSHEDPEVKFNWYVDGVEVHNAKTKPREEQYNSTYRVVSVLTVLHQDWLNGKEYKCKVSNKALPAPIEKTISKAKGQPREPQVYTLPPSREEMTKNQVSLWCLVKGFYPSDIAVEWESNGQPENNYKTTPPVLDSDGSFFLYSKLTVDKSRWQQGNVFSCSVMHEALHNHYTQKSLSLSPGGGGGSGGGGSGGGGSGGGGSQVQLVQSGAEVKKPGASVKVSCKASGYTFAGFEMHWVRQAPGQGLEWMGAIDPKTGGTDYNQKFKDRVTMTRDTSISTAYMELSRLRSDDTAVYYCARDLGYFDVWGQGTLVTVSS

SEQ ID NO: 304 - protein, 576 aa, synthetic construct
QVQLVQSGAEVKKPGASVKVSCKASGYTFTEFGMNWVRQAPGQGLEWMGWINTKTGEATYVEEFKGRVTFTTDTSTSTAYMELRSLRSDDTAVYYCARWDFAYYVEAMDYWGQGTTVTVSSASTKGPSVFPLAPSSKSTSGGTAALGCLVKDYFPEPVTVSWNSGALTSGVHTFPAVLQSSGLYSLSSVVTVPSSSLGTQTYICNVNHKPSNTKVDKKVEPKSCDKTHTCPPCPAPEAAGPSVFLFPPKPKDTLMISRTPEVTCVVVDVSHEDPEVKFNWYVDGVEVHNAKTKPREEQYNSTYRVVSVLTVLHQDWLNGKEYKCKVSNKALPAPIEKTISKAKGQPREPQVYTLPPSREEMTKNQVSLSCAVKGFYPSDIAVEWESNGQPENNYKTTPPVLDSDGSFFLVSKLTVDKSRWQQGNVFSCSVMHEALHNRFTQKSLSLSPGGGGGSGGGGSGGGGSGGGGSDIQMTQSPSSLSASVGDRVTITCRASQDIRSNLNWYQQKPGGAVKLLIYYTSRLHSGVPSRFSGSGSGTDYTLTISSLQPEDFATYFCQQSEKLPRTFGGGTKVEIR

SEQ ID NO: 305 - protein, 735 aa, synthetic construct
QVQLVQSGAEVKKPGASVKVSCKASGYTFTEFGMNWVRQAPGQGLEWMGWINTKTGEATYVEEFKGRVTFTTDTSTSTAYMELRSLRSDDTAVYYCARWDFAYYVEAMDYWGQGTTVTVSSASTKGPSVFPLAPSSKSTSGGTAALGCLVKDYFPEPVTVSWNSGALTSGVHTFPAVLQSSGLYSLSSVVTVPSSSLGTQTYICNVNHKPSNTKVDKKVEPKSCGGGGSGGGGSGGGGSGGGGSEVQLVESGGGLVQPGGSLRLSCAASGFTFSTYAMNWVRQAPGKGLEWVGRIRSKYNNYATYYADSVKGRFTISRDDSKNSLYLQMNSLKTEDTAVYYCVRHGNFGNSYVSWFAYWGQGTLVTVSSGGGGSDKTHTCPPCPAPEAAGPSVFLFPPKPKDTLMISRTPEVTCVVVDVSHEDPEVKFNWYVDGVEVHNAKTKPREEQYNSTYRVVSVLTVLHQDWLNGKEYKCKVSNKALPAPIEKTISKAKGQPREPQVYTLPPSREEMTKNQVSLWCLVKGFYPSDIAVEWESNGQPENNYKTTPPVLDSDGSFFLYSKLTVDKSRWQQGNVFSCSVMHEALHNHYTQKSLSLSPGGGGGSGGGGSGGGGSGGGGSQVQLVQSGAEVKKPGASVKVSCKASGYTFAGFEMHWVRQAPGQGLEWMGAIDPKTGGTDYNQKFKDRVTMTRDTSISTAYMELSRLRSDDTAVYYCARDLGYFDVWGQGTLVTVSS

SEQ ID NO: 306 - protein, 599 aa, synthetic construct
QVQLVQSGAEVKKPGASVKVSCKASGYTFTEFGMNWVRQAPGQGLEWMGWINTKTGEATYVEEFKGRVTFTTDTSTSTAYMELRSLRSDDTAVYYCARWDFAYYVEAMDYWGQGTTVTVSSASTKGPSVFPLAPSSKSTSGGTAALGCLVKDYFPEPVTVSWNSGALTSGVHTFPAVLQSSGLYSLSSVVTVPSSSLGTQTYICNVNHKPSNTKVDKKVEPKSCGGGGSGGGGSGGGGSGGGGSEVQLVESGGGLVQPGGSLRLSCAASGFTFSTYAMNWVRQAPGKGLEWVGRIRSKYNNYATYYADSVKGRFTISRDDSKNSLYLQMNSLKTEDTAVYYCVRHGNFGNSYVSWFAYWGQGTLVTVSSGGGGSDKTHTCPPCPAPEAAGPSVFLFPPKPKDTLMISRTPEVTCVVVDVSHEDPEVKFNWYVDGVEVHNAKTKPREEQYNSTYRVVSVLTVLHQDWLNGKEYKCKVSNKALPAPIEKTISKAKGQPREPQVYTLPPSREEMTKNQVSLWCLVKGFYPSDIAVEWESNGQPENNYKTTPPVLDSDGSFFLYSKLTVDKSRWQQGNVFSCSVMHEALHNHYTQKSLSLSPG

SEQ ID NO: 307 - protein, 710 aa, synthetic construct
QVQLVQSGAEVKKPGASVKVSCKASGYTFTEFGMNWVRQAPGQGLEWMGWINTKTGEATYVEEFKGRVTFTTDTSTSTAYMELRSLRSDDTAVYYCARWDFAYYVEAMDYWGQGTTVTVSSASTKGPSVFPLAPSSKSTSGGTAALGCLVKDYFPEPVTVSWNSGALTSGVHTFPAVLQSSGLYSLSSVVTVPSSSLGTQTYICNVNHKPSNTKVDKKVEPKSCGGGGSGGGGSGGGGSGGGGSQAVVTQEPSLTVSPGGTVTLTCRSSTGAVTTSNYANWVQQKPGQAPRGLIGGTNKRAPWTPARFSGSLLGGKAALTITGAQAEDEADYYCALWYSNLWVFGGGTKLTVLGGGGSDKTHTCPPCPAPEAAGPSVFLFPPKPKDTLMISRTPEVTCVVVDVSHEDPEVKFNWYVDGVEVHNAKTKPREEQYNSTYRVVSVLTVLHQDWLNGKEYKCKVSNKALPAPIEKTISKAKGQPREPQVYTLPPSREEMTKNQVSLSCAVKGFYPSDIAVEWESNGQPENNYKTTPPVLDSDGSFFLVSKLTVDKSRWQQGNVFSCSVMHEALHNRFTQKSLSLSPGGGGGSGGGGSGGGGSGGGGSDIQMTQSPSSLSASVGDRVTITCRASQDIRSNLNWYQQKPGGAVKLLIYYTSRLHSGVPSRFSGSGSGTDYTLTISSLQPEDFATYFCQQSEKLPRTFGGGTKVEIR

SEQ ID NO: 308 - protein, 583 aa, synthetic construct
QVQLVQSGAEVKKPGASVKVSCKASGYTFTEFGMNWVRQAPGQGLEWMGWINTKTGEATYVEEFKGRVTFTTDTSTSTAYMELRSLRSDDTAVYYCARWDFAYYVEAMDYWGQGTTVTVSSASTKGPSVFPLAPSSKSTSGGTAALGCLVKDYFPEPVTVSWNSGALTSGVHTFPAVLQSSGLYSLSSVVTVPSSSLGTQTYICNVNHKPSNTKVDKKVEPKSCGGGGSGGGGSGGGGSGGGGSQAVVTQEPSLTVSPGGTVTLTCRSSTGAVTTSNYANWVQQKPGQAPRGLIGGTNKRAPWTPARFSGSLLGGKAALTITGAQAEDEADYYCALWYSNLWVFGGGTKLTVLGGGGSDKTHTCPPCPAPEAAGPSVFLFPPKPKDTLMISRTPEVTCVVVDVSHEDPEVKFNWYVDGVEVHNAKTKPREEQYNSTYRVVSVLTVLHQDWLNGKEYKCKVSNKALPAPIEKTISKAKGQPREPQVYTLPPSREEMTKNQVSLSCAVKGFYPSDIAVEWESNGQPENNYKTTPPVLDSDGSFFLVSKLTVDKSRWQQGNVFSCSVMHEALHNRFTQKSLSLSPG

SEQ ID NO: 309 - protein, 585 aa, synthetic construct
QVQLVQSGAEVKKPGASVKVSCKASGYTFTNHIIHWVRQAPGQGLEWMGYINPYPGYHAYNEKFQGRATMTSDTSTSTVYMELSSLRSEDTAVYYCARDGYYRDTDVLDYWGQGTLVTVSSASTKGPSVFPLAPSSKSTSGGTAALGCLVKDYFPEPVTVSWNSGALTSGVHTFPAVLQSSGLYSLSSVVTVPSSSLGTQTYICNVNHKPSNTKVDKKVEPKSCDKTHTCPPCPAPEAAGPSVFLFPPKPKDTLMISRTPEVTCVVVDVSHEDPEVKFNWYVDGVEVHNAKTKPREEQYNSTYRVVSVLTVLHQDWLNGKEYKCKVSNKALPAPIEKTISKAKGQPREPQVYTLPPSREEMTKNQVSLWCLVKGFYPSDIAVEWESNGQPENNYKTTPPVLDSDGSFFLYSKLTVDKSRWQQGNVFSCSVMHEALHNHYTQKSLSLSPGGGGGSGGGGSGGGGSGGGGSQVQLVQSGAEVKKPGASVKVSCKASGYTFAGFEMHWVRQAPGQGLEWMGAIDPKTGGTDYNQKFKDRVTMTRDTSISTAYMELSRLRSDDTAVYYCARDLGYFDVWGQGTLVTVSS

SEQ ID NO: 310 - protein, 576 aa, synthetic construct
QVQLVQSGAEVKKPGASVKVSCKASGYTFTNHIIHWVRQAPGQGLEWMGYINPYPGYHAYNEKFQGRATMTSDTSTSTVYMELSSLRSEDTAVYYCARDGYYRDTDVLDYWGQGTLVTVSSASTKGPSVFPLAPSSKSTSGGTAALGCLVKDYFPEPVTVSWNSGALTSGVHTFPAVLQSSGLYSLSSVVTVPSSSLGTQTYICNVNHKPSNTKVDKKVEPKSCDKTHTCPPCPAPEAAGPSVFLFPPKPKDTLMISRTPEVTCVVVDVSHEDPEVKFNWYVDGVEVHNAKTKPREEQYNSTYRVVSVLTVLHQDWLNGKEYKCKVSNKALPAPIEKTISKAKGQPREPQVYTLPPSREEMTKNQVSLSCAVKGFYPSDIAVEWESNGQPENNYKTTPPVLDSDGSFFLVSKLTVDKSRWQQGNVFSCSVMHEALHNRFTQKSLSLSPGGGGGSGGGGSGGGGSGGGGSDIQMTQSPSSLSASVGDRVTITCRASQDIRSNLNWYQQKPGGAVKLLIYYTSRLHSGVPSRFSGSGSGTDYTLTISSLQPEDFATYFCQQSEKLPRTFGGGTKVEIR

SEQ ID NO: 311 - protein, 735 aa, synthetic construct
QVQLVQSGAEVKKPGASVKVSCKASGYTFTNHIIHWVRQAPGQGLEWMGYINPYPGYHAYNEKFQGRATMTSDTSTSTVYMELSSLRSEDTAVYYCARDGYYRDTDVLDYWGQGTLVTVSSASTKGPSVFPLAPSSKSTSGGTAALGCLVKDYFPEPVTVSWNSGALTSGVHTFPAVLQSSGLYSLSSVVTVPSSSLGTQTYICNVNHKPSNTKVDKKVEPKSCGGGGSGGGGSGGGGSGGGGSEVQLVESGGGLVQPGGSLRLSCAASGFTFSTYAMNWVRQAPGKGLEWVGRIRSKYNNYATYYADSVKGRFTISRDDSKNSLYLQMNSLKTEDTAVYYCVRHGNFGNSYVSWFAYWGQGTLVTVSSGGGGSDKTHTCPPCPAPEAAGPSVFLFPPKPKDTLMISRTPEVTCVVVDVSHEDPEVKFNWYVDGVEVHNAKTKPREEQYNSTYRVVSVLTVLHQDWLNGKEYKCKVSNKALPAPIEKTISKAKGQPREPQVYTLPPSREEMTKNQVSLWCLVKGFYPSDIAVEWESNGQPENNYKTTPPVLDSDGSFFLYSKLTVDKSRWQQGNVFSCSVMHEALHNHYTQKSLSLSPGGGGGSGGGGSGGGGSGGGGSQVQLVQSGAEVKKPGASVKVSCKASGYTFAGFEMHWVRQAPGQGLEWMGAIDPKTGGTDYNQKFKDRVTMTRDTSISTAYMELSRLRSDDTAVYYCARDLGYFDVWGQGTLVTVSS

SEQ ID NO: 312 - protein, 599 aa, synthetic construct
QVQLVQSGAEVKKPGASVKVSCKASGYTFTNHIIHWVRQAPGQGLEWMGYINPYPGYHAYNEKFQGRATMTSDTSTSTVYMELSSLRSEDTAVYYCARDGYYRDTDVLDYWGQGTLVTVSSASTKGPSVFPLAPSSKSTSGGTAALGCLVKDYFPEPVTVSWNSGALTSGVHTFPAVLQSSGLYSLSSVVTVPSSSLGTQTYICNVNHKPSNTKVDKKVEPKSCGGGGSGGGGSGGGGSGGGGSEVQLVESGGGLVQPGGSLRLSCAASGFTFSTYAMNWVRQAPGKGLEWVGRIRSKYNNYATYYADSVKGRFTISRDDSKNSLYLQMNSLKTEDTAVYYCVRHGNFGNSYVSWFAYWGQGTLVTVSSGGGGSDKTHTCPPCPAPEAAGPSVFLFPPKPKDTLMISRTPEVTCVVVDVSHEDPEVKFNWYVDGVEVHNAKTKPREEQYNSTYRVVSVLTVLHQDWLNGKEYKCKVSNKALPAPIEKTISKAKGQPREPQVYTLPPSREEMTKNQVSLWCLVKGFYPSDIAVEWESNGQPENNYKTTPPVLDSDGSFFLYSKLTVDKSRWQQGNVFSCSVMHEALHNHYTQKSLSLSPG

SEQ ID NO: 313 - protein, 740 aa, synthetic construct
QVQLVQSGAEVKKPGASVKVSCKASGYTFTNHIIHWVRQAPGQGLEWMGYINPYPGYHAYNEKFQGRATMTSDTSTSTVYMELSSLRSEDTAVYYCARDGYYRDTDVLDYWGQGTLVTVSSASTKGPSVFPLAPSSKSTSGGTAALGCLVKDYFPEPVTVSWNSGALTSGVHTFPAVLQSSGLYSLSSVVTVPSSSLGTQTYICNVNHKPSNTKVDKKVEPKSCGGGGSGGGGSGGGGSGGGGSEVQLVESGGGLVQPGGSLRLSCAASGFTFSTYAMNWVRQAPGKGLEWVGRIRSKYNNYATYYADSVKGRFTISRDDSKNSLYLQMNSLKTEDTAVYYCVRHGNFGNSYVSWFAYWGQGTLVTVSSGGGGSDKTHTCPPCPAPELLGPSVFLFPPKPKDTLMISRTPEVTCVVVDVSHEDPEVKFNWYVDGVEVHNAKTKPREEQYNSTYRVVSVLTVLHQDWLNGKEYKCKVSNKALGAPIEKTISKAKGQPREPQVYTLPPSREEMTKNQVSLWCLVKGFYPSDIAVEWESNGQPENNYKTTPPVLDSDGSFFLYSKLTVDKSRWQQGNVFSCSVMHEALHNHYTQKSLSLSPGKGGGGSGGGGSGGGGSGGGGSQVQLVQSGAEVKKPGASVKVSCKASGYTFTSYYIHWVRQAPGQGLEWIGCIYPGNVNTNYNEKFKDRATLTVDTSISTAYMELSRLRSDDTAVYFCTRSHYGLDWNFDVWGQGTTVTVSS

SEQ ID NO: 314 - protein, 600 aa, synthetic construct
QVQLVQSGAEVKKPGASVKVSCKASGYTFTNHIIHWVRQAPGQGLEWMGYINPYPGYHAYNEKFQGRATMTSDTSTSTVYMELSSLRSEDTAVYYCARDGYYRDTDVLDYWGQGTLVTVSSASTKGPSVFPLAPSSKSTSGGTAALGCLVKDYFPEPVTVSWNSGALTSGVHTFPAVLQSSGLYSLSSVVTVPSSSLGTQTYICNVNHKPSNTKVDKKVEPKSCGGGGSGGGGSGGGGSGGGGSEVQLVESGGGLVQPGGSLRLSCAASGFTFSTYAMNWVRQAPGKGLEWVGRIRSKYNNYATYYADSVKGRFTISRDDSKNSLYLQMNSLKTEDTAVYYCVRHGNFGNSYVSWFAYWGQGTLVTVSSGGGGSDKTHTCPPCPAPELLGPSVFLFPPKPKDTLMISRTPEVTCVVVDVSHEDPEVKFNWYVDGVEVHNAKTKPREEQYNSTYRVVSVLTVLHQDWLNGKEYKCKVSNKALGAPIEKTISKAKGQPREPQVYTLPPSREEMTKNQVSLWCLVKGFYPSDIAVEWESNGQPENNYKTTPPVLDSDGSFFLYSKLTVDKSRWQQGNVFSCSVMHEALHNHYTQKSLSLSPGK

SEQ ID NO: 315 - protein, 710 aa, synthetic construct
QVQLVQSGAEVKKPGASVKVSCKASGYTFTNHIIHWVRQAPGQGLEWMGYINPYPGYHAYNEKFQGRATMTSDTSTSTVYMELSSLRSEDTAVYYCARDGYYRDTDVLDYWGQGTLVTVSSASTKGPSVFPLAPSSKSTSGGTAALGCLVKDYFPEPVTVSWNSGALTSGVHTFPAVLQSSGLYSLSSVVTVPSSSLGTQTYICNVNHKPSNTKVDKKVEPKSCGGGGSGGGGSGGGGSGGGGSQAVVTQEPSLTVSPGGTVTLTCRSSTGAVTTSNYANWVQQKPGQAPRGLIGGTNKRAPWTPARFSGSLLGGKAALTITGAQAEDEADYYCALWYSNLWVFGGGTKLTVLGGGGSDKTHTCPPCPAPEAAGPSVFLFPPKPKDTLMISRTPEVTCVVVDVSHEDPEVKFNWYVDGVEVHNAKTKPREEQYNSTYRVVSVLTVLHQDWLNGKEYKCKVSNKALPAPIEKTISKAKGQPREPQVYTLPPSREEMTKNQVSLSCAVKGFYPSDIAVEWESNGQPENNYKTTPPVLDSDGSFFLVSKLTVDKSRWQQGNVFSCSVMHEALHNRFTQKSLSLSPGGGGGSGGGGSGGGGSGGGGSDIQMTQSPSSLSASVGDRVTITCRASQDIRSNLNWYQQKPGGAVKLLIYYTSRLHSGVPSRFSGSGSGTDYTLTISSLQPEDFATYFCQQSEKLPRTFGGGTKVEIR

SEQ ID NO: 316 - protein, 583 aa, synthetic construct
QVQLVQSGAEVKKPGASVKVSCKASGYTFTNHIIHWVRQAPGQGLEWMGYINPYPGYHAYNEKFQGRATMTSDTSTSTVYMELSSLRSEDTAVYYCARDGYYRDTDVLDYWGQGTLVTVSSASTKGPSVFPLAPSSKSTSGGTAALGCLVKDYFPEPVTVSWNSGALTSGVHTFPAVLQSSGLYSLSSVVTVPSSSLGTQTYICNVNHKPSNTKVDKKVEPKSCGGGGSGGGGSGGGGSGGGGSQAVVTQEPSLTVSPGGTVTLTCRSSTGAVTTSNYANWVQQKPGQAPRGLIGGTNKRAPWTPARFSGSLLGGKAALTITGAQAEDEADYYCALWYSNLWVFGGGTKLTVLGGGGSDKTHTCPPCPAPEAAGPSVFLFPPKPKDTLMISRTPEVTCVVVDVSHEDPEVKFNWYVDGVEVHNAKTKPREEQYNSTYRVVSVLTVLHQDWLNGKEYKCKVSNKALPAPIEKTISKAKGQPREPQVYTLPPSREEMTKNQVSLSCAVKGFYPSDIAVEWESNGQPENNYKTTPPVLDSDGSFFLVSKLTVDKSRWQQGNVFSCSVMHEALHNRFTQKSLSLSPG

SEQ ID NO: 317 - protein, 711 aa, synthetic construct
QVQLVQSGAEVKKPGASVKVSCKASGYTFTNHIIHWVRQAPGQGLEWMGYINPYPGYHAYNEKFQGRATMTSDTSTSTVYMELSSLRSEDTAVYYCARDGYYRDTDVLDYWGQGTLVTVSSASTKGPSVFPLAPSSKSTSGGTAALGCLVKDYFPEPVTVSWNSGALTSGVHTFPAVLQSSGLYSLSSVVTVPSSSLGTQTYICNVNHKPSNTKVDKKVEPKSCGGGGSGGGGSGGGGSGGGGSQAVVTQEPSLTVSPGGTVTLTCRSSTGAVTTSNYANWVQQKPGQAPRGLIGGTNKRAPWTPARFSGSLLGGKAALTITGAQAEDEADYYCALWYSNLWVFGGGTKLTVLGGGGSDKTHTCPPCPAPELLGPSVFLFPPKPKDTLMISRTPEVTCVVVDVSHEDPEVKFNWYVDGVEVHNAKTKPREEQYNSTYRVVSVLTVLHQDWLNGKEYKCKVSNKALGAPIEKTISKAKGQPREPQVYTLPPSREEMTKNQVSLSCAVKGFYPSDIAVEWESNGQPENNYKTTPPVLDSDGSFFLVSKLTVDKSRWQQGNVFSCSVMHEALHNRFTQKSLSLSPGKGGGGSGGGGSGGGGSGGGGSDIQMTQSPSSLSASVGDRVTITCHASQNIYVWLNWYQQKPGKAPKLLIYKASNLHTGVPSRFSGSGSGTDFTLTISSLQPEDFATYYCQQGQTYPYTFGGGTKVEIK

SEQ ID NO: 318 - protein, 584 aa, synthetic construct
QVQLVQSGAEVKKPGASVKVSCKASGYTFTNHIIHWVRQAPGQGLEWMGYINPYPGYHAYNEKFQGRATMTSDTSTSTVYMELSSLRSEDTAVYYCARDGYYRDTDVLDYWGQGTLVTVSSASTKGPSVFPLAPSSKSTSGGTAALGCLVKDYFPEPVTVSWNSGALTSGVHTFPAVLQSSGLYSLSSVVTVPSSSLGTQTYICNVNHKPSNTKVDKKVEPKSCGGGGSGGGGSGGGGSGGGGSQAVVTQEPSLTVSPGGTVTLTCRSSTGAVTTSNYANWVQQKPGQAPRGLIGGTNKRAPWTPARFSGSLLGGKAALTITGAQAEDEADYYCALWYSNLWVFGGGTKLTVLGGGGSDKTHTCPPCPAPELLGPSVFLFPPKPKDTLMISRTPEVTCVVVDVSHEDPEVKFNWYVDGVEVHNAKTKPREEQYNSTYRVVSVLTVLHQDWLNGKEYKCKVSNKALGAPIEKTISKAKGQPREPQVYTLPPSREEMTKNQVSLSCAVKGFYPSDIAVEWESNGQPENNYKTTPPVLDSDGSFFLVSKLTVDKSRWQQGNVFSCSVMHEALHNRFTQKSLSLSPGK

SEQ ID NO: 319 - protein, 585 aa, synthetic construct
QVQLVQSGAEVKKPGASVKVSCKASGYTFTSYVMHWVRQKPGQGLEWIGYINPYNEGTESTDKFKGRATMTSDKSTSTVYMELSSLRSEDTAVYYCASIYYGYEGTYFGVWGQGTLVTVSSASTKGPSVFPLAPSSKSTSGGTAALGCLVKDYFPEPVTVSWNSGALTSGVHTFPAVLQSSGLYSLSSVVTVPSSSLGTQTYICNVNHKPSNTKVDKKVEPKSCDKTHTCPPCPAPEAAGPSVFLFPPKPKDTLMISRTPEVTCVVVDVSHEDPEVKFNWYVDGVEVHNAKTKPREEQYNSTYRVVSVLTVLHQDWLNGKEYKCKVSNKALPAPIEKTISKAKGQPREPQVYTLPPSREEMTKNQVSLWCLVKGFYPSDIAVEWESNGQPENNYKTTPPVLDSDGSFFLYSKLTVDKSRWQQGNVFSCSVMHEALHNHYTQKSLSLSPGGGGGSGGGGSGGGGSGGGGSQVQLVQSGAEVKKPGASVKVSCKASGYTFAGFEMHWVRQAPGQGLEWMGAIDPKTGGTDYNQKFKDRVTMTRDTSISTAYMELSRLRSDDTAVYYCARDLGYFDVWGQGTLVTVSS

SEQ ID NO: 320 - protein, 576 aa, synthetic construct
QVQLVQSGAEVKKPGASVKVSCKASGYTFTSYVMHWVRQKPGQGLEWIGYINPYNEGTESTDKFKGRATMTSDKSTSTVYMELSSLRSEDTAVYYCASIYYGYEGTYFGVWGQGTLVTVSSASTKGPSVFPLAPSSKSTSGGTAALGCLVKDYFPEPVTVSWNSGALTSGVHTFPAVLQSSGLYSLSSVVTVPSSSLGTQTYICNVNHKPSNTKVDKKVEPKSCDKTHTCPPCPAPEAAGPSVFLFPPKPKDTLMISRTPEVTCVVVDVSHEDPEVKFNWYVDGVEVHNAKTKPREEQYNSTYRVVSVLTVLHQDWLNGKEYKCKVSNKALPAPIEKTISKAKGQPREPQVYTLPPSREEMTKNQVSLSCAVKGFYPSDIAVEWESNGQPENNYKTTPPVLDSDGSFFLVSKLTVDKSRWQQGNVFSCSVMHEALHNRFTQKSLSLSPGGGGGSGGGGSGGGGSGGGGSDIQMTQSPSSLSASVGDRVTITCRASQDIRSNLNWYQQKPGGAVKLLIYYTSRLHSGVPSRFSGSGSGTDYTLTISSLQPEDFATYFCQQSEKLPRTFGGGTKVEIR

SEQ ID NO: 321 - protein, 595 aa, synthetic construct
QVQLVQSGAEVKKPGASVKVSCKASGYTFTSYVMHWVRQKPGQGLEWIGYINPYNEGTESTDKFKGRATMTSDKSTSTVYMELSSLRSEDTAVYYCASIYYGYEGTYFGVWGQGTLVTVSSASTKGPSVFPLAPSSKSTSGGTAALGCLVKDYFPEPVTVSWNSGALTSGVHTFPAVLQSSGLYSLSSVVTVPSSSLGTQTYICNVNHKPSNTKVDKKVEPKSCDKTHTCPPCPAPEAAGPSVFLFPPKPKDTLMISRTPEVTCVVVDVSHEDPEVKFNWYVDGVEVHNAKTKPREEQYNSTYRVVSVLTVLHQDWLNGKEYKCKVSNKALPAPIEKTISKAKGQPREPQVYTLPPSREEMTKNQVSLWCLVKGFYPSDIAVEWESNGQPENNYKTTPPVLDSDGSFFLYSKLTVDKSRWQQGNVFSCSVMHEALHNHYTQKSLSLSPGGGGGSGGGGSGGGGSGGGGSQVQLVQSGAEVKKPGASVKVSCKASGYTFTGYYMHWVRQAPGQGLEWMGWINPDSGGTNYAQKFQGRVTMTRDTSISTAYMELNRLRSDDTAVYYCARDQPLGYCTNGVCSYFDYWGQGTLVTVSS

SEQ ID NO: 322 - protein, 576 aa, synthetic construct
QVQLVQSGAEVKKPGASVKVSCKASGYTFTSYVMHWVRQKPGQGLEWIGYINPYNEGTESTDKFKGRATMTSDKSTSTVYMELSSLRSEDTAVYYCASIYYGYEGTYFGVWGQGTLVTVSSASTKGPSVFPLAPSSKSTSGGTAALGCLVKDYFPEPVTVSWNSGALTSGVHTFPAVLQSSGLYSLSSVVTVPSSSLGTQTYICNVNHKPSNTKVDKKVEPKSCDKTHTCPPCPAPEAAGPSVFLFPPKPKDTLMISRTPEVTCVVVDVSHEDPEVKFNWYVDGVEVHNAKTKPREEQYNSTYRVVSVLTVLHQDWLNGKEYKCKVSNKALPAPIEKTISKAKGQPREPQVYTLPPSREEMTKNQVSLSCAVKGFYPSDIAVEWESNGQPENNYKTTPPVLDSDGSFFLVSKLTVDKSRWQQGNVFSCSVMHEALHNRFTQKSLSLSPGGGGGSGGGGSGGGGSGGGGSDIQMTQSPSSVSASVGDRVTITCRASQGIYSWLAWYQQKPGKAPNLLIYTASTLQSGVPSRFSGSGSGTDFTLTISSLQPEDFATYYCQQANIFPLTFGGGTKVEIK

SEQ ID NO: 323 - protein, 591 aa, synthetic construct
QVQLVQSGAEVKKPGASVKVSCKASGYTFTSYVMHWVRQKPGQGLEWIGYINPYNEGTESTDKFKGRATMTSDKSTSTVYMELSSLRSEDTAVYYCASIYYGYEGTYFGVWGQGTLVTVSSASTKGPSVFPLAPSSKSTSGGTAALGCLVKDYFPEPVTVSWNSGALTSGVHTFPAVLQSSGLYSLSSVVTVPSSSLGTQTYICNVNHKPSNTKVDKKVEPKSCDKTHTCPPCPAPEAAGPSVFLFPPKPKDTLMISRTPEVTCVVVDVSHEDPEVKFNWYVDGVEVHNAKTKPREEQYNSTYRVVSVLTVLHQDWLNGKEYKCKVSNKALPAPIEKTISKAKGQPREPQVYTLPPSREEMTKNQVSLWCLVKGFYPSDIAVEWESNGQPENNYKTTPPVLDSDGSFFLYSKLTVDKSRWQQGNVFSCSVMHEALHNHYTQKSLSLSPGGGGGSGGGGSGGGGSGGGGSEVQLVESGGGLVQPGGSLRLSCAASGFTFTNYGLHWVRQAPGKGLEWVSSISPSGGVTYYRDSVKGRFTISRDNSKNTLYLQMNSLRAEDTAVYYCAKPFLGWGGANWIAHWGQGTLVTVSS

SEQ ID NO: 324 - protein, 576 aa, synthetic construct
QVQLVQSGAEVKKPGASVKVSCKASGYTFTSYVMHWVRQKPGQGLEWIGYINPYNEGTESTDKFKGRATMTSDKSTSTVYMELSSLRSEDTAVYYCASIYYGYEGTYFGVWGQGTLVTVSSASTKGPSVFPLAPSSKSTSGGTAALGCLVKDYFPEPVTVSWNSGALTSGVHTFPAVLQSSGLYSLSSVVTVPSSSLGTQTYICNVNHKPSNTKVDKKVEPKSCDKTHTCPPCPAPEAAGPSVFLFPPKPKDTLMISRTPEVTCVVVDVSHEDPEVKFNWYVDGVEVHNAKTKPREEQYNSTYRVVSVLTVLHQDWLNGKEYKCKVSNKALPAPIEKTISKAKGQPREPQVYTLPPSREEMTKNQVSLSCAVKGFYPSDIAVEWESNGQPENNYKTTPPVLDSDGSFFLVSKLTVDKSRWQQGNVFSCSVMHEALHNRFTQKSLSLSPGGGGGSGGGGSGGGGSGGGGSDIQMTQSPSSLSASVGDRVTITCLASEDISNDLAWYQQKPGKAPKLLIYFVDRLLDGVPSRFSGSGSGTDFTLTISSLQPEDFATYYCQQSYKYPPTFGQGTKLEIK

SEQ ID NO: 325 - protein, 617 aa, synthetic construct
QVQLVQSGAEVKKPGASVKVSCKASGYTFTSYVMHWVRQKPGQGLEWIGYINPYNEGTESTDKFKGRATMTSDKSTSTVYMELSSLRSEDTAVYYCASIYYGYEGTYFGVWGQGTLVTVSSASTKGPSVFPLAPSSKSTSGGTAALGCLVKDYFPEPVTVSWNSGALTSGVHTFPAVLQSSGLYSLSSVVTVPSSSLGTQTYICNVNHKPSNTKVDKKVEPKSCDKTHTCPPCPAPEAAGPSVFLFPPKPKDTLMISRTPEVTCVVVDVSHEDPEVKFNWYVDGVEVHNAKTKPREEQYNSTYRVVSVLTVLHQDWLNGKEYKCKVSNKALPAPIEKTISKAKGQPREPQVYTLPPSREEMTKNQVSLWCLVKGFYPSDIAVEWESNGQPENNYKTTPPVLDSDGSFFLYSKLTVDKSRWQQGNVFSCSVMHEALHNHYTQKSLSLSPGGGGGSGGGGSGGGGSGGGGSQVQLVQSGAEVKKPGASVKVSCKASGYTFTGYYMHWVRQAPGQGLEWMGWINPDSGGTNYAQKFQGRVTMTRDTSISTAYMELNRLRSDDTAVYYCARDQPLGYCTNGVCSYFDYWGQGTLVTVSSGGGGSDKTHTCPPCPAPEAAGP

SEQ ID NO: 326 - protein, 598 aa, synthetic construct
QVQLVQSGAEVKKPGASVKVSCKASGYTFTSYVMHWVRQKPGQGLEWIGYINPYNEGTESTDKFKGRATMTSDKSTSTVYMELSSLRSEDTAVYYCASIYYGYEGTYFGVWGQGTLVTVSSASTKGPSVFPLAPSSKSTSGGTAALGCLVKDYFPEPVTVSWNSGALTSGVHTFPAVLQSSGLYSLSSVVTVPSSSLGTQTYICNVNHKPSNTKVDKKVEPKSCDKTHTCPPCPAPEAAGPSVFLFPPKPKDTLMISRTPEVTCVVVDVSHEDPEVKFNWYVDGVEVHNAKTKPREEQYNSTYRVVSVLTVLHQDWLNGKEYKCKVSNKALPAPIEKTISKAKGQPREPQVYTLPPSREEMTKNQVSLSCAVKGFYPSDIAVEWESNGQPENNYKTTPPVLDSDGSFFLVSKLTVDKSRWQQGNVFSCSVMHEALHNRFTQKSLSLSPGGGGGSGGGGSGGGGSGGGGSDIQMTQSPSSVSASVGDRVTITCRASQGIYSWLAWYQQKPGKAPNLLIYTASTLQSGVPSRFSGSGSGTDFTLTISSLQPEDFATYYCQQANIFPLTFGGGTKVEIKGGGGSDKTHTCPPCPAPEAAGP

SEQ ID NO: 327 - protein, 613 aa, synthetic construct
QVQLVQSGAEVKKPGASVKVSCKASGYTFTSYVMHWVRQKPGQGLEWIGYINPYNEGTESTDKFKGRATMTSDKSTSTVYMELSSLRSEDTAVYYCASIYYGYEGTYFGVWGQGTLVTVSSASTKGPSVFPLAPSSKSTSGGTAALGCLVKDYFPEPVTVSWNSGALTSGVHTFPAVLQSSGLYSLSSVVTVPSSSLGTQTYICNVNHKPSNTKVDKKVEPKSCDKTHTCPPCPAPEAAGPSVFLFPPKPKDTLMISRTPEVTCVVVDVSHEDPEVKFNWYVDGVEVHNAKTKPREEQYNSTYRVVSVLTVLHQDWLNGKEYKCKVSNKALPAPIEKTISKAKGQPREPQVYTLPPSREEMTKNQVSLWCLVKGFYPSDIAVEWESNGQPENNYKTTPPVLDSDGSFFLYSKLTVDKSRWQQGNVFSCSVMHEALHNHYTQKSLSLSPGGGGGSGGGGSGGGGSGGGGSEVQLVESGGGLVQPGGSLRLSCAASGFTFTNYGLHWVRQAPGKGLEWVSSISPSGGVTYYRDSVKGRFTISRDNSKNTLYLQMNSLRAEDTAVYYCAKPFLGWGGANWIAHWGQGTLVTVSSGGGGSDKTHTCPPCPAPEAAGP

SEQ ID NO: 328 - protein, 598 aa, synthetic construct
QVQLVQSGAEVKKPGASVKVSCKASGYTFTSYVMHWVRQKPGQGLEWIGYINPYNEGTESTDKFKGRATMTSDKSTSTVYMELSSLRSEDTAVYYCASIYYGYEGTYFGVWGQGTLVTVSSASTKGPSVFPLAPSSKSTSGGTAALGCLVKDYFPEPVTVSWNSGALTSGVHTFPAVLQSSGLYSLSSVVTVPSSSLGTQTYICNVNHKPSNTKVDKKVEPKSCDKTHTCPPCPAPEAAGPSVFLFPPKPKDTLMISRTPEVTCVVVDVSHEDPEVKFNWYVDGVEVHNAKTKPREEQYNSTYRVVSVLTVLHQDWLNGKEYKCKVSNKALPAPIEKTISKAKGQPREPQVYTLPPSREEMTKNQVSLSCAVKGFYPSDIAVEWESNGQPENNYKTTPPVLDSDGSFFLVSKLTVDKSRWQQGNVFSCSVMHEALHNRFTQKSLSLSPGGGGGSGGGGSGGGGSGGGGSDIQMTQSPSSLSASVGDRVTITCLASEDISNDLAWYQQKPGKAPKLLIYFVDRLLDGVPSRFSGSGSGTDFTLTISSLQPEDFATYYCQQSYKYPPTFGQGTKLEIKGGGGSDKTHTCPPCPAPEAAGP

SEQ ID NO: 329 - protein, 586 aa, synthetic construct
QVQLVQSGAEVKKPGASVKVSCKASGYTFTSYVMHWVRQKPGQGLEWIGYINPYNEGTESTDKFKGRATMTSDKSTSTVYMELSSLRSEDTAVYYCASIYYGYEGTYFGVWGQGTLVTVSSASTKGPSVFPLAPSSKSTSGGTAALGCLVKDYFPEPVTVSWNSGALTSGVHTFPAVLQSSGLYSLSSVVTVPSSSLGTQTYICNVNHKPSNTKVDKKVEPKSCDKTHTCPPCPAPELLGPSVFLFPPKPKDTLMISRTPEVTCVVVDVSHEDPEVKFNWYVDGVEVHNAKTKPREEQYNSTYRVVSVLTVLHQDWLNGKEYKCKVSNKALGAPIEKTISKAKGQPREPQVYTLPPSREEMTKNQVSLWCLVKGFYPSDIAVEWESNGQPENNYKTTPPVLDSDGSFFLYSKLTVDKSRWQQGNVFSCSVMHEALHNHYTQKSLSLSPGKGGGGSGGGGSGGGGSGGGGSQVQLVQSGAEVKKPGASVKVSCKASGYTFAGFEMHWVRQAPGQGLEWMGAIDPKTGGTDYNQKFKDRVTMTRDTSISTAYMELSRLRSDDTAVYYCARDLGYFDVWGQGTLVTVSS

SEQ ID NO: 330 - protein, 577 aa, synthetic construct
QVQLVQSGAEVKKPGASVKVSCKASGYTFTSYVMHWVRQKPGQGLEWIGYINPYNEGTESTDKFKGRATMTSDKSTSTVYMELSSLRSEDTAVYYCASIYYGYEGTYFGVWGQGTLVTVSSASTKGPSVFPLAPSSKSTSGGTAALGCLVKDYFPEPVTVSWNSGALTSGVHTFPAVLQSSGLYSLSSVVTVPSSSLGTQTYICNVNHKPSNTKVDKKVEPKSCDKTHTCPPCPAPELLGPSVFLFPPKPKDTLMISRTPEVTCVVVDVSHEDPEVKFNWYVDGVEVHNAKTKPREEQYNSTYRVVSVLTVLHQDWLNGKEYKCKVSNKALGAPIEKTISKAKGQPREPQVYTLPPSREEMTKNQVSLSCAVKGFYPSDIAVEWESNGQPENNYKTTPPVLDSDGSFFLVSKLTVDKSRWQQGNVFSCSVMHEALHNRFTQKSLSLSPGKGGGGSGGGGSGGGGSGGGGSDIQMTQSPSSLSASVGDRVTITCRASQDIRSNLNWYQQKPGGAVKLLIYYTSRLHSGVPSRFSGSGSGTDYTLTISSLQPEDFATYFCQQSEKLPRTFGGGTKVEIR

SEQ ID NO: 331 - protein, 715 aa, synthetic construct
QVQLVQSGAEVKKPGASVKVSCKASGYTFTSYVMHWVRQKPGQGLEWIGYINPYNEGTESTDKFKGRATMTSDKSTSTVYMELSSLRSEDTAVYYCASIYYGYEGTYFGVWGQGTLVTVSSASTKGPSVFPLAPSSKSTSGGTAALGCLVKDYFPEPVTVSWNSGALTSGVHTFPAVLQSSGLYSLSSVVTVPSSSLGTQTYICNVNHKPSNTKVDKKVEPKSCEVQLVESGGGLVQPGGSLRLSCAASGFTFSTYAMNWVRQAPGKGLEWVGRIRSKYNNYATYYADSVKGRFTISRDDSKNSLYLQMNSLKTEDTAVYYCVRHGNFGNSYVSWFAYWGQGTLVTVSSGGGGSDKTHTCPPCPAPEAAGPSVFLFPPKPKDTLMISRTPEVTCVVVDVSHEDPEVKFNWYVDGVEVHNAKTKPREEQYNSTYRVVSVLTVLHQDWLNGKEYKCKVSNKALPAPIEKTISKAKGQPREPQVYTLPPSREEMTKNQVSLWCLVKGFYPSDIAVEWESNGQPENNYKTTPPVLDSDGSFFLYSKLTVDKSRWQQGNVFSCSVMHEALHNHYTQKSLSLSPGGGGGSGGGGSGGGGSGGGGSQVQLVQSGAEVKKPGASVKVSCKASGYTFAGFEMHWVRQAPGQGLEWMGAIDPKTGGTDYNQKFKDRVTMTRDTSISTAYMELSRLRSDDTAVYYCARDLGYFDVWGQGTLVTVSS

SEQ ID NO: 332 - protein, 724 aa, synthetic construct
QVQLVQSGAEVKKPGASVKVSCKASGYTFTSYVMHWVRQKPGQGLEWIGYINPYNEGTESTDKFKGRATMTSDKSTSTVYMELSSLRSEDTAVYYCASIYYGYEGTYFGVWGQGTLVTVSSASTKGPSVFPLAPSSKSTSGGTAALGCLVKDYFPEPVTVSWNSGALTSGVHTFPAVLQSSGLYSLSSVVTVPSSSLGTQTYICNVNHKPSNTKVDKKVEPKSCGGGGSEVQLVESGGGLVQPGGSLRLSCAASGFTFSTYAMNWVRQAPGKGLEWVGRIRSKYNNYATYYADSVKGRFTISRDDSKNSLYLQMNSLKTEDTAVYYCVRHGNFGNSYVSWFAYWGQGTLVTVSSGGGGSDKTHTCPPCPAPEAAGPSVFLFPPKPKDTLMISRTPEVTCVVVDVSHEDPEVKFNWYVDGVEVHNAKTKPREEQYNSTYRVVSVLTVLHQDWLNGKEYKCKVSNKALPAPIEKTISKAKGQPREPQVYTLPPSREEMTKNQVSLWCLVKGFYPSDIAVEWESNGQPENNYKTTPPVLDSDGSFFLYSKLTVDKSRWQQGNVFSCSVMHEALHNHYTQKSLSLSPGGGGGSGGGGSGGGGSGGGGSQVQLVQSGAEVKKPGASVKVSCKASGYTFTSYYIHWVRQAPGQGLEWIGCIYPGNVNTNYNEKFKDRATLTVDTSISTAYMELSRLRSDDTAVYFCTRSHYGLDWNFDVWGQGTTVTVSS

SEQ ID NO: 333 - protein, 720 aa, synthetic construct
QVQLVQSGAEVKKPGASVKVSCKASGYTFTSYVMHWVRQKPGQGLEWIGYINPYNEGTESTDKFKGRATMTSDKSTSTVYMELSSLRSEDTAVYYCASIYYGYEGTYFGVWGQGTLVTVSSASTKGPSVFPLAPSSKSTSGGTAALGCLVKDYFPEPVTVSWNSGALTSGVHTFPAVLQSSGLYSLSSVVTVPSSSLGTQTYICNVNHKPSNTKVDKKVEPKSCGGGGSEVQLVESGGGLVQPGGSLRLSCAASGFTFSTYAMNWVRQAPGKGLEWVGRIRSKYNNYATYYADSVKGRFTISRDDSKNSLYLQMNSLKTEDTAVYYCVRHGNFGNSYVSWFAYWGQGTLVTVSSGGGGSDKTHTCPPCPAPEAAGPSVFLFPPKPKDTLMISRTPEVTCVVVDVSHEDPEVKFNWYVDGVEVHNAKTKPREEQYNSTYRVVSVLTVLHQDWLNGKEYKCKVSNKALPAPIEKTISKAKGQPREPQVYTLPPSREEMTKNQVSLWCLVKGFYPSDIAVEWESNGQPENNYKTTPPVLDSDGSFFLYSKLTVDKSRWQQGNVFSCSVMHEALHNHYTQKSLSLSPGGGGGSGGGGSGGGGSGGGGSQVQLVQSGAEVKKPGASVKVSCKASGYTFAGFEMHWVRQAPGQGLEWMGAIDPKTGGTDYNQKFKDRVTMTRDTSISTAYMELSRLRSDDTAVYYCARDLGYFDVWGQGTLVTVSS

SEQ ID NO: 334 - protein, 729 aa, synthetic construct
QVQLVQSGAEVKKPGASVKVSCKASGYTFTSYVMHWVRQKPGQGLEWIGYINPYNEGTESTDKFKGRATMTSDKSTSTVYMELSSLRSEDTAVYYCASIYYGYEGTYFGVWGQGTLVTVSSASTKGPSVFPLAPSSKSTSGGTAALGCLVKDYFPEPVTVSWNSGALTSGVHTFPAVLQSSGLYSLSSVVTVPSSSLGTQTYICNVNHKPSNTKVDKKVEPKSCGGGGSGGGGSEVQLVESGGGLVQPGGSLRLSCAASGFTFSTYAMNWVRQAPGKGLEWVGRIRSKYNNYATYYADSVKGRFTISRDDSKNSLYLQMNSLKTEDTAVYYCVRHGNFGNSYVSWFAYWGQGTLVTVSSGGGGSDKTHTCPPCPAPEAAGPSVFLFPPKPKDTLMISRTPEVTCVVVDVSHEDPEVKFNWYVDGVEVHNAKTKPREEQYNSTYRVVSVLTVLHQDWLNGKEYKCKVSNKALPAPIEKTISKAKGQPREPQVYTLPPSREEMTKNQVSLWCLVKGFYPSDIAVEWESNGQPENNYKTTPPVLDSDGSFFLYSKLTVDKSRWQQGNVFSCSVMHEALHNHYTQKSLSLSPGGGGGSGGGGSGGGGSGGGGSQVQLVQSGAEVKKPGASVKVSCKASGYTFTSYYIHWVRQAPGQGLEWIGCIYPGNVNTNYNEKFKDRATLTVDTSISTAYMELSRLRSDDTAVYFCTRSHYGLDWNFDVWGQGTTVTVSS

SEQ ID NO: 335 - protein, 725 aa, synthetic construct
QVQLVQSGAEVKKPGASVKVSCKASGYTFTSYVMHWVRQKPGQGLEWIGYINPYNEGTESTDKFKGRATMTSDKSTSTVYMELSSLRSEDTAVYYCASIYYGYEGTYFGVWGQGTLVTVSSASTKGPSVFPLAPSSKSTSGGTAALGCLVKDYFPEPVTVSWNSGALTSGVHTFPAVLQSSGLYSLSSVVTVPSSSLGTQTYICNVNHKPSNTKVDKKVEPKSCGGGGSGGGGSEVQLVESGGGLVQPGGSLRLSCAASGFTFSTYAMNWVRQAPGKGLEWVGRIRSKYNNYATYYADSVKGRFTISRDDSKNSLYLQMNSLKTEDTAVYYCVRHGNFGNSYVSWFAYWGQGTLVTVSSGGGGSDKTHTCPPCPAPEAAGPSVFLFPPKPKDTLMISRTPEVTCVVVDVSHEDPEVKFNWYVDGVEVHNAKTKPREEQYNSTYRVVSVLTVLHQDWLNGKEYKCKVSNKALPAPIEKTISKAKGQPREPQVYTLPPSREEMTKNQVSLWCLVKGFYPSDIAVEWESNGQPENNYKTTPPVLDSDGSFFLYSKLTVDKSRWQQGNVFSCSVMHEALHNHYTQKSLSLSPGGGGGSGGGGSGGGGSGGGGSQVQLVQSGAEVKKPGASVKVSCKASGYTFAGFEMHWVRQAPGQGLEWMGAIDPKTGGTDYNQKFKDRVTMTRDTSISTAYMELSRLRSDDTAVYYCARDLGYFDVWGQGTLVTVSS

SEQ ID NO: 336 - protein, 734 aa, synthetic construct
QVQLVQSGAEVKKPGASVKVSCKASGYTFTSYVMHWVRQKPGQGLEWIGYINPYNEGTESTDKFKGRATMTSDKSTSTVYMELSSLRSEDTAVYYCASIYYGYEGTYFGVWGQGTLVTVSSASTKGPSVFPLAPSSKSTSGGTAALGCLVKDYFPEPVTVSWNSGALTSGVHTFPAVLQSSGLYSLSSVVTVPSSSLGTQTYICNVNHKPSNTKVDKKVEPKSCGGGGSGGGGSGGGGSEVQLVESGGGLVQPGGSLRLSCAASGFTFSTYAMNWVRQAPGKGLEWVGRIRSKYNNYATYYADSVKGRFTISRDDSKNSLYLQMNSLKTEDTAVYYCVRHGNFGNSYVSWFAYWGQGTLVTVSSGGGGSDKTHTCPPCPAPEAAGPSVFLFPPKPKDTLMISRTPEVTCVVVDVSHEDPEVKFNWYVDGVEVHNAKTKPREEQYNSTYRVVSVLTVLHQDWLNGKEYKCKVSNKALPAPIEKTISKAKGQPREPQVYTLPPSREEMTKNQVSLWCLVKGFYPSDIAVEWESNGQPENNYKTTPPVLDSDGSFFLYSKLTVDKSRWQQGNVFSCSVMHEALHNHYTQKSLSLSPGGGGGSGGGGSGGGGSGGGGSQVQLVQSGAEVKKPGASVKVSCKASGYTFTSYYIHWVRQAPGQGLEWIGCIYPGNVNTNYNEKFKDRATLTVDTSISTAYMELSRLRSDDTAVYFCTRSHYGLDWNFDVWGQGTTVTVSS

SEQ ID NO: 337 - protein, 730 aa, synthetic construct
QVQLVQSGAEVKKPGASVKVSCKASGYTFTSYVMHWVRQKPGQGLEWIGYINPYNEGTESTDKFKGRATMTSDKSTSTVYMELSSLRSEDTAVYYCASIYYGYEGTYFGVWGQGTLVTVSSASTKGPSVFPLAPSSKSTSGGTAALGCLVKDYFPEPVTVSWNSGALTSGVHTFPAVLQSSGLYSLSSVVTVPSSSLGTQTYICNVNHKPSNTKVDKKVEPKSCGGGGSGGGGSGGGGSEVQLVESGGGLVQPGGSLRLSCAASGFTFSTYAMNWVRQAPGKGLEWVGRIRSKYNNYATYYADSVKGRFTISRDDSKNSLYLQMNSLKTEDTAVYYCVRHGNFGNSYVSWFAYWGQGTLVTVSSGGGGSDKTHTCPPCPAPEAAGPSVFLFPPKPKDTLMISRTPEVTCVVVDVSHEDPEVKFNWYVDGVEVHNAKTKPREEQYNSTYRVVSVLTVLHQDWLNGKEYKCKVSNKALPAPIEKTISKAKGQPREPQVYTLPPSREEMTKNQVSLWCLVKGFYPSDIAVEWESNGQPENNYKTTPPVLDSDGSFFLYSKLTVDKSRWQQGNVFSCSVMHEALHNHYTQKSLSLSPGGGGGSGGGGSGGGGSGGGGSQVQLVQSGAEVKKPGASVKVSCKASGYTFAGFEMHWVRQAPGQGLEWMGAIDPKTGGTDYNQKFKDRVTMTRDTSISTAYMELSRLRSDDTAVYYCARDLGYFDVWGQGTLVTVSS

SEQ ID NO: 338 - protein, 581 aa, synthetic construct
QVQLVQSGAEVKKPGASVKVSCKASGYTFTSYVMHWVRQKPGQGLEWIGYINPYNEGTESTDKFKGRATMTSDKSTSTVYMELSSLRSEDTAVYYCASIYYGYEGTYFGVWGQGTLVTVSSASTKGPSVFPLAPSSKSTSGGTAALGCLVKDYFPEPVTVSWNSGALTSGVHTFPAVLQSSGLYSLSSVVTVPSSSLGTQTYICNVNHKPSNTKVDKKVEPKSCGGGGSGGGGSGGGGSGGGGSDIQMTQSPSSLSASVGDRVTITCLASEDISNDLAWYQQKPGKAPKLLIYFVDRLLDGVPSRFSGSGSGTDFTLTISSLQPEDFATYYCQQSYKYPPTFGQGTKLEIKGGGGSDKTHTCPPCPAPEAAGPSVFLFPPKPKDTLMISRTPEVTCVVVDVSHEDPEVKFNWYVDGVEVHNAKTKPREEQYNSTYRVVSVLTVLHQDWLNGKEYKCKVSNKALPAPIEKTISKAKGQPREPQVYTLPPSREEMTKNQVSLSCAVKGFYPSDIAVEWESNGQPENNYKTTPPVLDSDGSFFLVSKLTVDKSRWQQGNVFSCSVMHEALHNRFTQKSLSLSPG

SEQ ID NO: 339 - protein, 707 aa, synthetic construct
QVQLVQSGAEVKKPGASVKVSCKASGYTFTSYVMHWVRQKPGQGLEWIGYINPYNEGTESTDKFKGRATMTSDKSTSTVYMELSSLRSEDTAVYYCASIYYGYEGTYFGVWGQGTLVTVSSASTKGPSVFPLAPSSKSTSGGTAALGCLVKDYFPEPVTVSWNSGALTSGVHTFPAVLQSSGLYSLSSVVTVPSSSLGTQTYICNVNHKPSNTKVDKKVEPKSCGGGGSGGGGSGGGGSGGGGSDIQMTQSPSSLSASVGDRVTITCRASQDIRSNLNWYQQKPGGAVKLLIYYTSRLHSGVPSRFSGSGSGTDYTLTISSLQPEDFATYFCQQSEKLPRTFGGGTKVEIRGGGGSDKTHTCPPCPAPEAAGPSVFLFPPKPKDTLMISRTPEVTCVVVDVSHEDPEVKFNWYVDGVEVHNAKTKPREEQYNSTYRVVSVLTVLHQDWLNGKEYKCKVSNKALPAPIEKTISKAKGQPREPQVYTLPPSREEMTKNQVSLSCAVKGFYPSDIAVEWESNGQPENNYKTTPPVLDSDGSFFLVSKLTVDKSRWQQGNVFSCSVMHEALHNRFTQKSLSLSPGGGGGSGGGGSGGGGSGGGGSNIQMTQSPSSLSASVGDRVTITCKAGQNVNNYLAWYQQKPGKAPKVLIFNANSLQTGVPSRFSGSGSGTDFTLTISSLQPEDFATYYCQQYNSWPTFGGGTKVEIK

SEQ ID NO: 340 - protein, 708 aa, synthetic construct
QVQLVQSGAEVKKPGASVKVSCKASGYTFTSYVMHWVRQKPGQGLEWIGYINPYNEGTESTDKFKGRATMTSDKSTSTVYMELSSLRSEDTAVYYCASIYYGYEGTYFGVWGQGTLVTVSSASTKGPSVFPLAPSSKSTSGGTAALGCLVKDYFPEPVTVSWNSGALTSGVHTFPAVLQSSGLYSLSSVVTVPSSSLGTQTYICNVNHKPSNTKVDKKVEPKSCGGGGSGGGGSGGGGSGGGGSDIQMTQSPSSLSASVGDRVTITCLASEDISNDLAWYQQKPGKAPKLLIYFVDRLLDGVPSRFSGSGSGTDFTLTISSLQPEDFATYYCQQSYKYPPTFGQGTKLEIKGGGGSDKTHTCPPCPAPEAAGPSVFLFPPKPKDTLMISRTPEVTCVVVDVSHEDPEVKFNWYVDGVEVHNAKTKPREEQYNSTYRVVSVLTVLHQDWLNGKEYKCKVSNKALPAPIEKTISKAKGQPREPQVYTLPPSREEMTKNQVSLSCAVKGFYPSDIAVEWESNGQPENNYKTTPPVLDSDGSFFLVSKLTVDKSRWQQGNVFSCSVMHEALHNRFTQKSLSLSPGGGGGSGGGGSGGGGSGGGGSDIQMTQSPSSLSASVGDRVTITCRASQDIRSNLNWYQQKPGGAVKLLIYYTSRLHSGVPSRFSGSGSGTDYTLTISSLQPEDFATYFCQQSEKLPRTFGGGTKVEIR

SEQ ID NO: 341 - protein, 708 aa, synthetic construct
QVQLVQSGAEVKKPGASVKVSCKASGYTFTSYVMHWVRQKPGQGLEWIGYINPYNEGTESTDKFKGRATMTSDKSTSTVYMELSSLRSEDTAVYYCASIYYGYEGTYFGVWGQGTLVTVSSASTKGPSVFPLAPSSKSTSGGTAALGCLVKDYFPEPVTVSWNSGALTSGVHTFPAVLQSSGLYSLSSVVTVPSSSLGTQTYICNVNHKPSNTKVDKKVEPKSCGGGGSGGGGSGGGGSGGGGSDIQMTQSPSSLSASVGDRVTITCRASQDIRSNLNWYQQKPGGAVKLLIYYTSRLHSGVPSRFSGSGSGTDYTLTISSLQPEDFATYFCQQSEKLPRTFGGGTKVEIRGGGGSDKTHTCPPCPAPEAAGPSVFLFPPKPKDTLMISRTPEVTCVVVDVSHEDPEVKFNWYVDGVEVHNAKTKPREEQYNSTYRVVSVLTVLHQDWLNGKEYKCKVSNKALPAPIEKTISKAKGQPREPQVYTLPPSREEMTKNQVSLSCAVKGFYPSDIAVEWESNGQPENNYKTTPPVLDSDGSFFLVSKLTVDKSRWQQGNVFSCSVMHEALHNRFTQKSLSLSPGGGGGSGGGGSGGGGSGGGGSDIQMTQSPSSVSASVGDRVTITCRASQGIYSWLAWYQQKPGKAPNLLIYTASTLQSGVPSRFSGSGSGTDFTLTISSLQPEDFATYYCQQANIFPLTFGGGTKVEIK

SEQ ID NO: 342 - protein, 708 aa, synthetic construct
QVQLVQSGAEVKKPGASVKVSCKASGYTFTSYVMHWVRQKPGQGLEWIGYINPYNEGTESTDKFKGRATMTSDKSTSTVYMELSSLRSEDTAVYYCASIYYGYEGTYFGVWGQGTLVTVSSASTKGPSVFPLAPSSKSTSGGTAALGCLVKDYFPEPVTVSWNSGALTSGVHTFPAVLQSSGLYSLSSVVTVPSSSLGTQTYICNVNHKPSNTKVDKKVEPKSCGGGGSGGGGSGGGGSGGGGSDIQMTQSPSSLSASVGDRVTITCRASQDIRSNLNWYQQKPGGAVKLLIYYTSRLHSGVPSRFSGSGSGTDYTLTISSLQPEDFATYFCQQSEKLPRTFGGGTKVEIRGGGGSDKTHTCPPCPAPEAAGPSVFLFPPKPKDTLMISRTPEVTCVVVDVSHEDPEVKFNWYVDGVEVHNAKTKPREEQYNSTYRVVSVLTVLHQDWLNGKEYKCKVSNKALPAPIEKTISKAKGQPREPQVYTLPPSREEMTKNQVSLSCAVKGFYPSDIAVEWESNGQPENNYKTTPPVLDSDGSFFLVSKLTVDKSRWQQGNVFSCSVMHEALHNRFTQKSLSLSPGGGGGSGGGGSGGGGSGGGGSDIQMTQSPSSLSASVGDRVTITCLASEDISNDLAWYQQKPGKAPKLLIYFVDRLLDGVPSRFSGSGSGTDFTLTISSLQPEDFATYYCQQSYKYPPTFGQGTKLEIK

SEQ ID NO: 343 - protein, 581 aa, synthetic construct
QVQLVQSGAEVKKPGASVKVSCKASGYTFTSYVMHWVRQKPGQGLEWIGYINPYNEGTESTDKFKGRATMTSDKSTSTVYMELSSLRSEDTAVYYCASIYYGYEGTYFGVWGQGTLVTVSSASTKGPSVFPLAPSSKSTSGGTAALGCLVKDYFPEPVTVSWNSGALTSGVHTFPAVLQSSGLYSLSSVVTVPSSSLGTQTYICNVNHKPSNTKVDKKVEPKSCGGGGSGGGGSGGGGSGGGGSDIQMTQSPSSVSASVGDRVTITCRASQGIYSWLAWYQQKPGKAPNLLIYTASTLQSGVPSRFSGSGSGTDFTLTISSLQPEDFATYYCQQANIFPLTFGGGTKVEIKGGGGSDKTHTCPPCPAPEAAGPSVFLFPPKPKDTLMISRTPEVTCVVVDVSHEDPEVKFNWYVDGVEVHNAKTKPREEQYNSTYRVVSVLTVLHQDWLNGKEYKCKVSNKALPAPIEKTISKAKGQPREPQVYTLPPSREEMTKNQVSLSCAVKGFYPSDIAVEWESNGQPENNYKTTPPVLDSDGSFFLVSKLTVDKSRWQQGNVFSCSVMHEALHNRFTQKSLSLSPG

SEQ ID NO: 344 - protein, 707 aa, synthetic construct
QVQLVQSGAEVKKPGASVKVSCKASGYTFTSYVMHWVRQKPGQGLEWIGYINPYNEGTESTDKFKGRATMTSDKSTSTVYMELSSLRSEDTAVYYCASIYYGYEGTYFGVWGQGTLVTVSSASTKGPSVFPLAPSSKSTSGGTAALGCLVKDYFPEPVTVSWNSGALTSGVHTFPAVLQSSGLYSLSSVVTVPSSSLGTQTYICNVNHKPSNTKVDKKVEPKSCGGGGSGGGGSGGGGSGGGGSDIQMTQSPSSVSASVGDRVTITCRASQGIYSWLAWYQQKPGKAPNLLIYTASTLQSGVPSRFSGSGSGTDFTLTISSLQPEDFATYYCQQANIFPLTFGGGTKVEIKGGGGSDKTHTCPPCPAPEAAGPSVFLFPPKPKDTLMISRTPEVTCVVVDVSHEDPEVKFNWYVDGVEVHNAKTKPREEQYNSTYRVVSVLTVLHQDWLNGKEYKCKVSNKALPAPIEKTISKAKGQPREPQVYTLPPSREEMTKNQVSLSCAVKGFYPSDIAVEWESNGQPENNYKTTPPVLDSDGSFFLVSKLTVDKSRWQQGNVFSCSVMHEALHNRFTQKSLSLSPGGGGGSGGGGSGGGGSGGGGSNIQMTQSPSSLSASVGDRVTITCKAGQNVNNYLAWYQQKPGKAPKVLIFNANSLQTGVPSRFSGSGSGTDFTLTISSLQPEDFATYYCQQYNSWPTFGGGTKVEIK

SEQ ID NO: 345 - protein, 708 aa, synthetic construct
QVQLVQSGAEVKKPGASVKVSCKASGYTFTSYVMHWVRQKPGQGLEWIGYINPYNEGTESTDKFKGRATMTSDKSTSTVYMELSSLRSEDTAVYYCASIYYGYEGTYFGVWGQGTLVTVSSASTKGPSVFPLAPSSKSTSGGTAALGCLVKDYFPEPVTVSWNSGALTSGVHTFPAVLQSSGLYSLSSVVTVPSSSLGTQTYICNVNHKPSNTKVDKKVEPKSCGGGGSGGGGSGGGGSGGGGSDIQMTQSPSSVSASVGDRVTITCRASQGIYSWLAWYQQKPGKAPNLLIYTASTLQSGVPSRFSGSGSGTDFTLTISSLQPEDFATYYCQQANIFPLTFGGGTKVEIKGGGGSDKTHTCPPCPAPEAAGPSVFLFPPKPKDTLMISRTPEVTCVVVDVSHEDPEVKFNWYVDGVEVHNAKTKPREEQYNSTYRVVSVLTVLHQDWLNGKEYKCKVSNKALPAPIEKTISKAKGQPREPQVYTLPPSREEMTKNQVSLSCAVKGFYPSDIAVEWESNGQPENNYKTTPPVLDSDGSFFLVSKLTVDKSRWQQGNVFSCSVMHEALHNRFTQKSLSLSPGGGGGSGGGGSGGGGSGGGGSDIQMTQSPSSLSASVGDRVTITCRASQDIRSNLNWYQQKPGGAVKLLIYYTSRLHSGVPSRFSGSGSGTDYTLTISSLQPEDFATYFCQQSEKLPRTFGGGTKVEIR

SEQ ID NO: 346 - protein, 739 aa, synthetic construct
QVQLVQSGAEVKKPGASVKVSCKASGYTFTSYVMHWVRQKPGQGLEWIGYINPYNEGTESTDKFKGRATMTSDKSTSTVYMELSSLRSEDTAVYYCASIYYGYEGTYFGVWGQGTLVTVSSASTKGPSVFPLAPSSKSTSGGTAALGCLVKDYFPEPVTVSWNSGALTSGVHTFPAVLQSSGLYSLSSVVTVPSSSLGTQTYICNVNHKPSNTKVDKKVEPKSCGGGGSGGGGSGGGGSGGGGSEVQLVESGGGLVQPGGSLRLSCAASGFTFSTYAMNWVRQAPGKGLEWVGRIRSKYNNYATYYADSVKGRFTISRDDSKNSLYLQMNSLKTEDTAVYYCVRHGNFGNSYVSWFAYWGQGTLVTVSSGGGGSDKTHTCPPCPAPEAAGPSVFLFPPKPKDTLMISRTPEVTCVVVDVSHEDPEVKFNWYVDGVEVHNAKTKPREEQYNSTYRVVSVLTVLHQDWLNGKEYKCKVSNKALPAPIEKTISKAKGQPREPQVYTLPPSREEMTKNQVSLWCLVKGFYPSDIAVEWESNGQPENNYKTTPPVLDSDGSFFLYSKLTVDKSRWQQGNVFSCSVMHEALHNHYTQKSLSLSPGGGGGSGGGGSGGGGSGGGGSQVQLVQSGAEVKKPGASVKVSCKASGYTFTSYYIHWVRQAPGQGLEWIGCIYPGNVNTNYNEKFKDRATLTVDTSISTAYMELSRLRSDDTAVYFCTRSHYGLDWNFDVWGQGTTVTVSS

SEQ ID NO: 347 - protein, 739 aa, synthetic construct
QVQLVQSGAEVKKPGASVKVSCKASGYTFTSYVMHWVRQKPGQGLEWIGYINPYNEGTESTDKFKGRATMTSDKSTSTVYMELSSLRSEDTAVYYCASIYYGYEGTYFGVWGQGTLVTVSSASTKGPSVFPLAPSSKSTSGGTAALGCLVKDYFPEPVTVSWNSGALTSGVHTFPAVLQSSGLYSLSSVVTVPSSSLGTQTYICNVNHKPSNTKVDKKVEPKSCGGGGSGGGGSGGGGSGGGGSEVQLVESGGGLVQPGGSLRLSCAASGFTFSTYAMNWVRQAPGKGLEWVGRIRSKYNNYATYYADSVKGRFTISRDDSKNSLYLQMNSLKTEDTAVYYCVRHGNFGNSYVSWFAYWGQGTLVTVSSGGGGSDKTHTCPPCPAPEAAGPSVFLFPPKPKDTLMISRTPEVTCVVVDVSHEDPEVKFNWYVDGVEVHNAKTKPREEQYNSTYRVVSVLTVLHQDWLNGKEYKCKVSNKALPAPIEKTISKAKGQPREPQVYTLPPSREEMTKNQVSLWCLVKGFYPSDIAVEWESNGQPENNYKTTPPVLDSDGSFFLYSKLTVDKSRWQQGNVFSCSVMHEALHNHYTQKSLSLSPGGGGGSGGGGSGGGGSGGGGSQVQLVQSGAEVVKPGASVKVSCKASGYTFTSYYIHWVRQAPGQGLEWIGSIYPGNVNTNYAQKFQGRATLTVDTSISTAYMELSRLRSDDTAVYYCTRSHYGLDWNFDVWGKGTTVTVSS

SEQ ID NO: 348 - protein, 741 aa, synthetic construct
QVQLVQSGAEVKKPGASVKVSCKASGYTFTSYVMHWVRQKPGQGLEWIGYINPYNEGTESTDKFKGRATMTSDKSTSTVYMELSSLRSEDTAVYYCASIYYGYEGTYFGVWGQGTLVTVSSASTKGPSVFPLAPSSKSTSGGTAALGCLVKDYFPEPVTVSWNSGALTSGVHTFPAVLQSSGLYSLSSVVTVPSSSLGTQTYICNVNHKPSNTKVDKKVEPKSCGGGGSGGGGSGGGGSGGGGSEVQLVESGGGLVQPGGSLRLSCAASGFTFSTYAMNWVRQAPGKGLEWVGRIRSKYNNYATYYADSVKGRFTISRDDSKNSLYLQMNSLKTEDTAVYYCVRHGNFGNSYVSWFAYWGQGTLVTVSSGGGGSDKTHTCPPCPAPEAAGPSVFLFPPKPKDTLMISRTPEVTCVVVDVSHEDPEVKFNWYVDGVEVHNAKTKPREEQYNSTYRVVSVLTVLHQDWLNGKEYKCKVSNKALPAPIEKTISKAKGQPREPQVYTLPPSREEMTKNQVSLWCLVKGFYPSDIAVEWESNGQPENNYKTTPPVLDSDGSFFLYSKLTVDKSRWQQGNVFSCSVMHEALHNHYTQKSLSLSPGGGGGSGGGGSGGGGSGGGGSQVQLQESGPGLVKPSETLSLTCTVSGGSISSYYWSWIRQPPGKGLEWIGYIYYSGITHYNPSLKSRVTISVDTSKIQFSLKLSSVTAADTAVYYCARWGVRRDYYYYGMDVWGQGTTVTVSS

SEQ ID NO: 349 - protein, 734 aa, synthetic construct
QVQLVQSGAEVKKPGASVKVSCKASGYTFTSYVMHWVRQKPGQGLEWIGYINPYNEGTESTDKFKGRATMTSDKSTSTVYMELSSLRSEDTAVYYCASIYYGYEGTYFGVWGQGTLVTVSSASTKGPSVFPLAPSSKSTSGGTAALGCLVKDYFPEPVTVSWNSGALTSGVHTFPAVLQSSGLYSLSSVVTVPSSSLGTQTYICNVNHKPSNTKVDKKVEPKSCGGGGSGGGGSGGGGSGGGGSEVQLVESGGGLVQPGGSLRLSCAASGFTFSTYAMNWVRQAPGKGLEWVGRIRSKYNNYATYYADSVKGRFTISRDDSKNSLYLQMNSLKTEDTAVYYCVRHGNFGNSYVSWFAYWGQGTLVTVSSDKTHTCPPCPAPEAAGPSVFLFPPKPKDTLMISRTPEVTCVVVDVSHEDPEVKFNWYVDGVEVHNAKTKPREEQYNSTYRVVSVLTVLHQDWLNGKEYKCKVSNKALPAPIEKTISKAKGQPREPQVYTLPPSREEMTKNQVSLWCLVKGFYPSDIAVEWESNGQPENNYKTTPPVLDSDGSFFLYSKLTVDKSRWQQGNVFSCSVMHEALHNHYTQKSLSLSPGGGGGSGGGGSGGGGSGGGGSQVQLVQSGAEVKKPGASVKVSCKASGYTFTSYYIHWVRQAPGQGLEWIGCIYPGNVNTNYNEKFKDRATLTVDTSISTAYMELSRLRSDDTAVYFCTRSHYGLDWNFDVWGQGTTVTVSS

SEQ ID NO: 350 - protein, 737 aa, synthetic construct
QVQLVQSGAEVKKPGASVKVSCKASGYTFTSYVMHWVRQKPGQGLEWIGYINPYNEGTESTDKFKGRATMTSDKSTSTVYMELSSLRSEDTAVYYCASIYYGYEGTYFGVWGQGTLVTVSSASTKGPSVFPLAPSSKSTSGGTAALGCLVKDYFPEPVTVSWNSGALTSGVHTFPAVLQSSGLYSLSSVVTVPSSSLGTQTYICNVNHKPSNTKVDKKVEPKSCGGGGSGGGGSGGGGSGGGGSEVQLVESGGGLVQPGGSLRLSCAASGFTFSTYAMNWVRQAPGKGLEWVGRIRSKYNNYATYYADSVKGRFTISRDDSKNSLYLQMNSLKTEDTAVYYCVRHGNFGNSYVSWFAYWGQGTLVTVSSGGSDKTHTCPPCPAPEAAGPSVFLFPPKPKDTLMISRTPEVTCVVVDVSHEDPEVKFNWYVDGVEVHNAKTKPREEQYNSTYRVVSVLTVLHQDWLNGKEYKCKVSNKALPAPIEKTISKAKGQPREPQVYTLPPSREEMTKNQVSLWCLVKGFYPSDIAVEWESNGQPENNYKTTPPVLDSDGSFFLYSKLTVDKSRWQQGNVFSCSVMHEALHNHYTQKSLSLSPGGGGGSGGGGSGGGGSGGGGSQVQLVQSGAEVKKPGASVKVSCKASGYTFTSYYIHWVRQAPGQGLEWIGCIYPGNVNTNYNEKFKDRATLTVDTSISTAYMELSRLRSDDTAVYFCTRSHYGLDWNFDVWGQGTTVTVSS

SEQ ID NO: 351 - protein, 738 aa, synthetic construct
QVQLVQSGAEVKKPGASVKVSCKASGYTFTSYVMHWVRQKPGQGLEWIGYINPYNEGTESTDKFKGRATMTSDKSTSTVYMELSSLRSEDTAVYYCASIYYGYEGTYFGVWGQGTLVTVSSASTKGPSVFPLAPSSKSTSGGTAALGCLVKDYFPEPVTVSWNSGALTSGVHTFPAVLQSSGLYSLSSVVTVPSSSLGTQTYICNVNHKPSNTKVDKKVEPKSCGGGGSGGGGSGGGGSGGGGSEVQLVESGGGLVQPGGSLRLSCAASGFTFSTYAMNWVRQAPGKGLEWVGRIRSKYNNYATYYADSVKGRFTISRDDSKNSLYLQMNSLKTEDTAVYYCVRHGNFGNSYVSWFAYWGQGTLVTVSSGGGSDKTHTCPPCPAPEAAGPSVFLFPPKPKDTLMISRTPEVTCVVVDVSHEDPEVKFNWYVDGVEVHNAKTKPREEQYNSTYRVVSVLTVLHQDWLNGKEYKCKVSNKALPAPIEKTISKAKGQPREPQVYTLPPSREEMTKNQVSLWCLVKGFYPSDIAVEWESNGQPENNYKTTPPVLDSDGSFFLYSKLTVDKSRWQQGNVFSCSVMHEALHNHYTQKSLSLSPGGGGGSGGGGSGGGGSGGGGSQVQLVQSGAEVKKPGASVKVSCKASGYTFTSYYIHWVRQAPGQGLEWIGCIYPGNVNTNYNEKFKDRATLTVDTSISTAYMELSRLRSDDTAVYFCTRSHYGLDWNFDVWGQGTTVTVSS

SEQ ID NO: 352 - protein, 742 aa, synthetic construct
QVQLVQSGAEVKKPGASVKVSCKASGYTFTSYVMHWVRQKPGQGLEWIGYINPYNEGTESTDKFKGRATMTSDKSTSTVYMELSSLRSEDTAVYYCASIYYGYEGTYFGVWGQGTLVTVSSASTKGPSVFPLAPSSKSTSGGTAALGCLVKDYFPEPVTVSWNSGALTSGVHTFPAVLQSSGLYSLSSVVTVPSSSLGTQTYICNVNHKPSNTKVDKKVEPKSCGGGGSGGGGSGGGGSGGGGSEVQLVESGGGLVQPGGSLRLSCAASGFTFSTYAMNWVRQAPGKGLEWVGRIRSKYNNYATYYADSVKGRFTISRDDSKNSLYLQMNSLKTEDTAVYYCVRHGNFGNSYVSWFAYWGQGTLVTVSSGGGSGGGSDKTHTCPPCPAPEAAGPSVFLFPPKPKDTLMISRTPEVTCVVVDVSHEDPEVKFNWYVDGVEVHNAKTKPREEQYNSTYRVVSVLTVLHQDWLNGKEYKCKVSNKALPAPIEKTISKAKGQPREPQVYTLPPSREEMTKNQVSLWCLVKGFYPSDIAVEWESNGQPENNYKTTPPVLDSDGSFFLYSKLTVDKSRWQQGNVFSCSVMHEALHNHYTQKSLSLSPGGGGGSGGGGSGGGGSGGGGSQVQLVQSGAEVKKPGASVKVSCKASGYTFTSYYIHWVRQAPGQGLEWIGCIYPGNVNTNYNEKFKDRATLTVDTSISTAYMELSRLRSDDTAVYFCTRSHYGLDWNFDVWGQGTTVTVSS

SEQ ID NO: 353 - protein, 744 aa, synthetic construct
QVQLVQSGAEVKKPGASVKVSCKASGYTFTSYVMHWVRQKPGQGLEWIGYINPYNEGTESTDKFKGRATMTSDKSTSTVYMELSSLRSEDTAVYYCASIYYGYEGTYFGVWGQGTLVTVSSASTKGPSVFPLAPSSKSTSGGTAALGCLVKDYFPEPVTVSWNSGALTSGVHTFPAVLQSSGLYSLSSVVTVPSSSLGTQTYICNVNHKPSNTKVDKKVEPKSCGGGGSGGGGSGGGGSGGGGSEVQLVESGGGLVQPGGSLRLSCAASGFTFSTYAMNWVRQAPGKGLEWVGRIRSKYNNYATYYADSVKGRFTISRDDSKNSLYLQMNSLKTEDTAVYYCVRHGNFGNSYVSWFAYWGQGTLVTVSSGGGGSGGGGSDKTHTCPPCPAPEAAGPSVFLFPPKPKDTLMISRTPEVTCVVVDVSHEDPEVKFNWYVDGVEVHNAKTKPREEQYNSTYRVVSVLTVLHQDWLNGKEYKCKVSNKALPAPIEKTISKAKGQPREPQVYTLPPSREEMTKNQVSLWCLVKGFYPSDIAVEWESNGQPENNYKTTPPVLDSDGSFFLYSKLTVDKSRWQQGNVFSCSVMHEALHNHYTQKSLSLSPGGGGGSGGGGSGGGGSGGGGSQVQLVQSGAEVKKPGASVKVSCKASGYTFTSYYIHWVRQAPGQGLEWIGCIYPGNVNTNYNEKFKDRATLTVDTSISTAYMELSRLRSDDTAVYFCTRSHYGLDWNFDVWGQGTTVTVSS

SEQ ID NO: 354 - protein, 749 aa, synthetic construct
QVQLVQSGAEVKKPGASVKVSCKASGYTFTSYVMHWVRQKPGQGLEWIGYINPYNEGTESTDKFKGRATMTSDKSTSTVYMELSSLRSEDTAVYYCASIYYGYEGTYFGVWGQGTLVTVSSASTKGPSVFPLAPSSKSTSGGTAALGCLVKDYFPEPVTVSWNSGALTSGVHTFPAVLQSSGLYSLSSVVTVPSSSLGTQTYICNVNHKPSNTKVDKKVEPKSCGGGGSGGGGSGGGGSGGGGSEVQLVESGGGLVQPGGSLRLSCAASGFTFSTYAMNWVRQAPGKGLEWVGRIRSKYNNYATYYADSVKGRFTISRDDSKNSLYLQMNSLKTEDTAVYYCVRHGNFGNSYVSWFAYWGQGTLVTVSSGGGGSGGGGSGGGGSDKTHTCPPCPAPEAAGPSVFLFPPKPKDTLMISRTPEVTCVVVDVSHEDPEVKFNWYVDGVEVHNAKTKPREEQYNSTYRVVSVLTVLHQDWLNGKEYKCKVSNKALPAPIEKTISKAKGQPREPQVYTLPPSREEMTKNQVSLWCLVKGFYPSDIAVEWESNGQPENNYKTTPPVLDSDGSFFLYSKLTVDKSRWQQGNVFSCSVMHEALHNHYTQKSLSLSPGGGGGSGGGGSGGGGSGGGGSQVQLVQSGAEVKKPGASVKVSCKASGYTFTSYYIHWVRQAPGQGLEWIGCIYPGNVNTNYNEKFKDRATLTVDTSISTAYMELSRLRSDDTAVYFCTRSHYGLDWNFDVWGQGTTVTVSS

SEQ ID NO: 355 - protein, 734 aa, synthetic construct
QVQLVQSGAEVKKPGASVKVSCKASGYTFTSYVMHWVRQKPGQGLEWIGYINPYNEGTESTDKFKGRATMTSDKSTSTVYMELSSLRSEDTAVYYCASIYYGYEGTYFGVWGQGTLVTVSSASTKGPSVFPLAPSSKSTSGGTAALGCLVKDYFPEPVTVSWNSGALTSGVHTFPAVLQSSGLYSLSSVVTVPSSSLGTQTYICNVNHKPSNTKVDKKVEPKSCGGGGSGGGGSGGGGSGGGGSEVQLVESGGGLVQPGGSLRLSCAASGFTFSTYAMNWVRQAPGKGLEWVGRIRSKYNNYATYYADSVKGRFTISRDDSKNSLYLQMNSLKTEDTAVYYCVRHGNFGNSYVSWFAYWGQGTLVTVSSGGGGSDKTHTCPPCPAPEAAGPSVFLFPPKPKDTLMISRTPEVTCVVVDVSHEDPEVKFNWYVDGVEVHNAKTKPREEQYNSTYRVVSVLTVLHQDWLNGKEYKCKVSNKALPAPIEKTISKAKGQPREPQVYTLPPSREEMTKNQVSLWCLVKGFYPSDIAVEWESNGQPENNYKTTPPVLDSDGSFFLYSKLTVDKSRWQQGNVFSCSVMHEALHNHYTQKSLSLSPGGGGGSGGGGSGGGGSQVQLVQSGAEVKKPGASVKVSCKASGYTFTSYYIHWVRQAPGQGLEWIGCIYPGNVNTNYNEKFKDRATLTVDTSISTAYMELSRLRSDDTAVYFCTRSHYGLDWNFDVWGQGTTVTVSS

SEQ ID NO: 356 - protein, 729 aa, synthetic construct
QVQLVQSGAEVKKPGASVKVSCKASGYTFTSYVMHWVRQKPGQGLEWIGYINPYNEGTESTDKFKGRATMTSDKSTSTVYMELSSLRSEDTAVYYCASIYYGYEGTYFGVWGQGTLVTVSSASTKGPSVFPLAPSSKSTSGGTAALGCLVKDYFPEPVTVSWNSGALTSGVHTFPAVLQSSGLYSLSSVVTVPSSSLGTQTYICNVNHKPSNTKVDKKVEPKSCGGGGSGGGGSGGGGSGGGGSEVQLVESGGGLVQPGGSLRLSCAASGFTFSTYAMNWVRQAPGKGLEWVGRIRSKYNNYATYYADSVKGRFTISRDDSKNSLYLQMNSLKTEDTAVYYCVRHGNFGNSYVSWFAYWGQGTLVTVSSGGGGSDKTHTCPPCPAPEAAGPSVFLFPPKPKDTLMISRTPEVTCVVVDVSHEDPEVKFNWYVDGVEVHNAKTKPREEQYNSTYRVVSVLTVLHQDWLNGKEYKCKVSNKALPAPIEKTISKAKGQPREPQVYTLPPSREEMTKNQVSLWCLVKGFYPSDIAVEWESNGQPENNYKTTPPVLDSDGSFFLYSKLTVDKSRWQQGNVFSCSVMHEALHNHYTQKSLSLSPGGGGGSGGGGSQVQLVQSGAEVKKPGASVKVSCKASGYTFTSYYIHWVRQAPGQGLEWIGCIYPGNVNTNYNEKFKDRATLTVDTSISTAYMELSRLRSDDTAVYFCTRSHYGLDWNFDVWGQGTTVTVSS

SEQ ID NO: 357 - protein, 724 aa, synthetic construct
QVQLVQSGAEVKKPGASVKVSCKASGYTFTSYVMHWVRQKPGQGLEWIGYINPYNEGTESTDKFKGRATMTSDKSTSTVYMELSSLRSEDTAVYYCASIYYGYEGTYFGVWGQGTLVTVSSASTKGPSVFPLAPSSKSTSGGTAALGCLVKDYFPEPVTVSWNSGALTSGVHTFPAVLQSSGLYSLSSVVTVPSSSLGTQTYICNVNHKPSNTKVDKKVEPKSCGGGGSGGGGSGGGGSGGGGSEVQLVESGGGLVQPGGSLRLSCAASGFTFSTYAMNWVRQAPGKGLEWVGRIRSKYNNYATYYADSVKGRFTISRDDSKNSLYLQMNSLKTEDTAVYYCVRHGNFGNSYVSWFAYWGQGTLVTVSSGGGGSDKTHTCPPCPAPEAAGPSVFLFPPKPKDTLMISRTPEVTCVVVDVSHEDPEVKFNWYVDGVEVHNAKTKPREEQYNSTYRVVSVLTVLHQDWLNGKEYKCKVSNKALPAPIEKTISKAKGQPREPQVYTLPPSREEMTKNQVSLWCLVKGFYPSDIAVEWESNGQPENNYKTTPPVLDSDGSFFLYSKLTVDKSRWQQGNVFSCSVMHEALHNHYTQKSLSLSPGGGGGSQVQLVQSGAEVKKPGASVKVSCKASGYTFTSYYIHWVRQAPGQGLEWIGCIYPGNVNTNYNEKFKDRATLTVDTSISTAYMELSRLRSDDTAVYFCTRSHYGLDWNFDVWGQGTTVTVSS

SEQ ID NO: 358 - protein, 744 aa, synthetic construct
QVQLVQSGAEVKKPGASVKVSCKASGYTFTSYVMHWVRQKPGQGLEWIGYINPYNEGTESTDKFKGRATMTSDKSTSTVYMELSSLRSEDTAVYYCASIYYGYEGTYFGVWGQGTLVTVSSASTKGPSVFPLAPSSKSTSGGTAALGCLVKDYFPEPVTVSWNSGALTSGVHTFPAVLQSSGLYSLSSVVTVPSSSLGTQTYICNVNHKPSNTKVDKKVEPKSCGGGGSGGGGSGGGGSGGGGSEVQLVESGGGLVQPGGSLRLSCAASGFTFSTYAMNWVRQAPGKGLEWVGRIRSKYNNYATYYADSVKGRFTISRDDSKNSLYLQMNSLKTEDTAVYYCVRHGNFGNSYVSWFAYWGQGTLVTVSSGGGGSDKTHTCPPCPAPEAAGPSVFLFPPKPKDTLMISRTPEVTCVVVDVSHEDPEVKFNWYVDGVEVHNAKTKPREEQYNSTYRVVSVLTVLHQDWLNGKEYKCKVSNKALPAPIEKTISKAKGQPREPQVYTLPPSREEMTKNQVSLWCLVKGFYPSDIAVEWESNGQPENNYKTTPPVLDSDGSFFLYSKLTVDKSRWQQGNVFSCSVMHEALHNHYTQKSLSLSPGDKTHTCPPCPGGGGSGGGGSGGGGSQVQLVQSGAEVKKPGASVKVSCKASGYTFTSYYIHWVRQAPGQGLEWIGCIYPGNVNTNYNEKFKDRATLTVDTSISTAYMELSRLRSDDTAVYFCTRSHYGLDWNFDVWGQGTTVTVSS

SEQ ID NO: 359 - protein, 848 aa, synthetic construct
QVQLVQSGAEVKKPGASVKVSCKASGYTFTSYVMHWVRQKPGQGLEWIGYINPYNEGTESTDKFKGRATMTSDKSTSTVYMELSSLRSEDTAVYYCASIYYGYEGTYFGVWGQGTLVTVSSASTKGPSVFPLAPSSKSTSGGTAALGCLVKDYFPEPVTVSWNSGALTSGVHTFPAVLQSSGLYSLSSVVTVPSSSLGTQTYICNVNHKPSNTKVDKKVEPKSCGGGGSGGGGSGGGGSGGGGSEVQLVESGGGLVQPGGSLRLSCAASGFTFSTYAMNWVRQAPGKGLEWVGRIRSKYNNYATYYADSVKGRFTISRDDSKNSLYLQMNSLKTEDTAVYYCVRHGNFGNSYVSWFAYWGQGTLVTVSSPAPEAAGPSVFLFPPKPKDTLMISRTPEVTCVVVDVSHEDPEVKFNWYVDGVEVHNAKTKPREEQYNSTYRVVSVLTVLHQDWLNGKEYKCKVSNKALPAPIEKTISKAKGQPREPQVYTLPPSREEMTKNQVSLWCLVKGFYPSDIAVEWESNGQPENNYKTTPPVLDSDGSFFLYSKLTVDKSRWQQGNVFSCSVMHEALHNHYTQKSLSLSPGGGGGSGGGGSGGGGSGGGGSQVQLVQSGAEVKKPGASVKVSCKASGYTFAGFEMHWVRQAPGQGLEWMGAIDPKTGGTDYNQKFKDRVTMTRDTSISTAYMELSRLRSDDTAVYYCARDLGYFDVWGQGTLVTVSSGGGGSGGGGSGGGGSGGGGSDIQMTQSPSSLSASVGDRVTITCRASQDIRSNLNWYQQKPGGAVKLLIYYTSRLHSGVPSRFSGSGSGTDYTLTISSLQPEDFATYFCQQSEKLPRTFGGGTKVEIR

SEQ ID NO: 360 - protein, 862 aa, synthetic construct
QVQLVQSGAEVKKPGASVKVSCKASGYTFTSYVMHWVRQKPGQGLEWIGYINPYNEGTESTDKFKGRATMTSDKSTSTVYMELSSLRSEDTAVYYCASIYYGYEGTYFGVWGQGTLVTVSSASTKGPSVFPLAPSSKSTSGGTAALGCLVKDYFPEPVTVSWNSGALTSGVHTFPAVLQSSGLYSLSSVVTVPSSSLGTQTYICNVNHKPSNTKVDKKVEPKSCGGGGSGGGGSGGGGSGGGGSEVQLVESGGGLVQPGGSLRLSCAASGFTFSTYAMNWVRQAPGKGLEWVGRIRSKYNNYATYYADSVKGRFTISRDDSKNSLYLQMNSLKTEDTAVYYCVRHGNFGNSYVSWFAYWGQGTLVTVSSGGGGSDKTHTCPPCPAPEAAGPSVFLFPPKPKDTLMISRTPEVTCVVVDVSHEDPEVKFNWYVDGVEVHNAKTKPREEQYNSTYRVVSVLTVLHQDWLNGKEYKCKVSNKALPAPIEKTISKAKGQPREPQVYTLPPSREEMTKNQVSLWCLVKGFYPSDIAVEWESNGQPENNYKTTPPVLDSDGSFFLYSKLTVDKSRWQQGNVFSCSVMHEALHNHYTQKSLSLSPGGGGGSGGGGSGGGGSGGGGSQVQLVQSGAEVKKPGASVKVSCKASGYTFAGFEMHWVRQAPGQGLEWMGAIDPKTGGTDYNQKFKDRVTMTRDTSISTAYMELSRLRSDDTAVYYCARDLGYFDVWGQGTLVTVSSGGGGSGGGGSGGGGSGGGGSDIQMTQSPSSLSASVGDRVTITCRASQDIRSNLNWYQQKPGGAVKLLIYYTSRLHSGVPSRFSGSGSGTDYTLTISSLQPEDFATYFCQQSEKLPRTFGGGTKVEIR

SEQ ID NO: 361 - protein, 721 aa, synthetic construct
QVQLVQSGAEVKKPGASVKVSCKASGYTFTSYVMHWVRQKPGQGLEWIGYINPYNEGTESTDKFKGRATMTSDKSTSTVYMELSSLRSEDTAVYYCASIYYGYEGTYFGVWGQGTLVTVSSASTKGPSVFPLAPSSKSTSGGTAALGCLVKDYFPEPVTVSWNSGALTSGVHTFPAVLQSSGLYSLSSVVTVPSSSLGTQTYICNVNHKPSNTKVDKKVEPKSCGGGGSGGGGSGGGGSGGGGSEVQLVESGGGLVQPGGSLRLSCAASGFTFSTYAMNWVRQAPGKGLEWVGRIRSKYNNYATYYADSVKGRFTISRDDSKNSLYLQMNSLKTEDTAVYYCVRHGNFGNSYVSWFAYWGQGTLVTVSSPAPEAAGPSVFLFPPKPKDTLMISRTPEVTCVVVDVSHEDPEVKFNWYVDGVEVHNAKTKPREEQYNSTYRVVSVLTVLHQDWLNGKEYKCKVSNKALPAPIEKTISKAKGQPREPQVYTLPPSREEMTKNQVSLWCLVKGFYPSDIAVEWESNGQPENNYKTTPPVLDSDGSFFLYSKLTVDKSRWQQGNVFSCSVMHEALHNHYTQKSLSLSPGGGGGSGGGGSGGGGSGGGGSQVQLVQSGAEVKKPGASVKVSCKASGYTFAGFEMHWVRQAPGQGLEWMGAIDPKTGGTDYNQKFKDRVTMTRDTSISTAYMELSRLRSDDTAVYYCARDLGYFDVWGQGTLVTVSS

SEQ ID NO: 362 - protein, 735 aa, synthetic construct
QVQLVQSGAEVKKPGASVKVSCKASGYTFTSYVMHWVRQKPGQGLEWIGYINPYNEGTESTDKFKGRATMTSDKSTSTVYMELSSLRSEDTAVYYCASIYYGYEGTYFGVWGQGTLVTVSSASTKGPSVFPLAPSSKSTSGGTAALGCLVKDYFPEPVTVSWNSGALTSGVHTFPAVLQSSGLYSLSSVVTVPSSSLGTQTYICNVNHKPSNTKVDKKVEPKSCGGGGSGGGGSGGGGSGGGGSEVQLVESGGGLVQPGGSLRLSCAASGFTFSTYAMNWVRQAPGKGLEWVGRIRSKYNNYATYYADSVKGRFTISRDDSKNSLYLQMNSLKTEDTAVYYCVRHGNFGNSYVSWFAYWGQGTLVTVSSGGGGSDKTHTCPPCPAPEAAGPSVFLFPPKPKDTLMISRTPEVTCVVVDVSHEDPEVKFNWYVDGVEVHNAKTKPREEQYNSTYRVVSVLTVLHQDWLNGKEYKCKVSNKALPAPIEKTISKAKGQPREPQVYTLPPSREEMTKNQVSLWCLVKGFYPSDIAVEWESNGQPENNYKTTPPVLDSDGSFFLYSKLTVDKSRWQQGNVFSCSVMHEALHNHYTQKSLSLSPGGGGGSGGGGSGGGGSGGGGSQVQLVQSGAEVKKPGASVKVSCKASGYTFAGFEMHWVRQAPGQGLEWMGAIDPKTGGTDYNQKFKDRVTMTRDTSISTAYMELSRLRSDDTAVYYCARDLGYFDVWGQGTLVTVSS

SEQ ID NO: 363 - protein, 721 aa, synthetic construct; identical to SEQ ID NO: 361

SEQ ID NO: 364 - protein, 735 aa, synthetic construct; identical to SEQ ID NO: 362

SEQ ID NO: 365 - protein, 735 aa, synthetic construct
QVQLVQSGAEVKKPGASVKVSCKASGYTFTSYVMHWVRQKPGQGLEWIGYINPYNEGTESTDKFKGRATMTSDKSTSTVYMELSSLRSEDTAVYYCASIYYGYEGTYFGVWGQGTLVTVSSASTKGPSVFPLAPSSKSTSGGTAALGCLVKDYFPEPVTVSWNSGALTSGVHTFPAVLQSSGLYSLSSVVTVPSSSLGTQTYICNVNHKPSNTKVDKKVEPKSCGGGGSGGGGSGGGGSGGGGSEVQLVESGGGLVQPGGSLRLSCAASGFTFSTYAMNWVRQAPGKGLEWVGRIRSKYNNYATYYADSVKGRFTISRDDSKNSLYLQMNSLKTEDTAVYYCVRHGNFGNSYVSWFAYWGQGTLVTVSSGGGGSDKTHTCPPCPAPELLGPSVFLFPPKPKDTLMISRTPEVTCVVVAVSHEDPEVKFNWYVDGVEVHNAKTKPREEQYASTYRVVSVLTVLHQDWLNGKEYKCKVSNKALPAPIEKTISKAKGQPREPQVYTLPPSREEMTKNQVSLWCLVKGFYPSDIAVEWESNGQPENNYKTTPPVLDSDGSFFLYSKLTVDKSRWQQGNVFSCSVMHEALHNHYTQKSLSLSPGGGGGSGGGGSGGGGSGGGGSQVQLVQSGAEVKKPGASVKVSCKASGYTFAGFEMHWVRQAPGQGLEWMGAIDPKTGGTDYNQKFKDRVTMTRDTSISTAYMELSRLRSDDTAVYYCARDLGYFDVWGQGTLVTVSS

SEQ ID NO: 366 - protein, 737 aa, synthetic construct
QVQLVQSGAEVKKPGASVKVSCKASGYTFTSYVMHWVRQKPGQGLEWIGYINPYNEGTESTDKFKGRATMTSDKSTSTVYMELSSLRSEDTAVYYCASIYYGYEGTYFGVWGQGTLVTVSSASTKGPSVFPLAPSSKSTSGGTAALGCLVKDYFPEPVTVSWNSGALTSGVHTFPAVLQSSGLYSLSSVVTVPSSSLGTQTYICNVNHKPSNTKVDKKVEPKSCGGGGSGGGGSGGGGSGGGGSEVQLVESGGGLVQPGGSLRLSCAASGFTFSTYAMNWVRQAPGKGLEWVGRIRSKYNNYATYYADSVKGRFTISRDDSKNSLYLQMNSLKTEDTAVYYCVRHGNFGNSYVSWFAYWGQGTLVTVSSGGGGSDKTHTCPPCPAPEAAGGPSVFLFPPKPKDTLMISRTPEVTCVVVDVSHEDPEVKFNWYVDGVEVHNAKTKPREEQYNSTYRVVSVLTVLHQDWLNGKEYKCKVSNKALGAPIEKTISKAKGQPREPQVYTLPPSREEMTKNQVSLWCLVKGFYPSDIAVEWESNGQPENNYKTTPPVLDSDGSFFLYSKLTVDKSRWQQGNVFSCSVMHEALHNHYTQKSLSLSPGKGGGGSGGGGSGGGGSGGGGSQVQLVQSGAEVKKPGASVKVSCKASGYTFAGFEMHWVRQAPGQGLEWMGAIDPKTGGTDYNQKFKDRVTMTRDTSISTAYMELSRLRSDDTAVYYCARDLGYFDVWGQGTLVTVSS

SEQ ID NO: 367 - protein, 736 aa, synthetic construct
QVQLVQSGAEVKKPGASVKVSCKASGYTFTSYVMHWVRQKPGQGLEWIGYINPYNEGTESTDKFKGRATMTSDKSTSTVYMELSSLRSEDTAVYYCASIYYGYEGTYFGVWGQGTLVTVSSASTKGPSVFPLAPSSKSTSGGTAALGCLVKDYFPEPVTVSWNSGALTSGVHTFPAVLQSSGLYSLSSVVTVPSSSLGTQTYICNVNHKPSNTKVDKKVEPKSCGGGGSGGGGSGGGGSGGGGSEVQLVESGGGLVQPGGSLRLSCAASGFTFSTYAMNWVRQAPGKGLEWVGRIRSKYNNYATYYADSVKGRFTISRDDSKNSLYLQMNSLKTEDTAVYYCVRHGNFGNSYVSWFAYWGQGTLVTVSSGGGGSDKTHTCPPCPAPEAAGPSVFLFPPKPKDTLMISRTPEVTCVVVDVSHEDPEVKFNWYVDGVEVHNAKTKPREEQYNSTYRVVSVLTVLHQDWLNGKEYKCKVSNKALGAPIEKTISKAKGQPREPQVYTLPPSREEMTKNQVSLWCLVKGFYPSDIAVEWESNGQPENNYKTTPPVLDSDGSFFLYSKLTVDKSRWQQGNVFSCSVMHEALHNHYTQKSLSLSPGKGGGGSGGGGSGGGGSGGGGSQVQLVQSGAEVKKPGASVKVSCKASGYTFAGFEMHWVRQAPGQGLEWMGAIDPKTGGTDYNQKFKDRVTMTRDTSISTAYMELSRLRSDDTAVYYCARDLGYFDVWGQGTLVTVSS

SEQ ID NO: 368 - protein, 735 aa, synthetic construct
QVQLVQSGAEVKKPGASVKVSCKASGYTFTSYVMHWVRQKPGQGLEWIGYINPYNEGTESTDKFKGRATMTSDKSTSTVYMELSSLRSEDTAVYYCASIYYGYEGTYFGVWGQGTLVTVSSASTKGPSVFPLAPSSKSTSGGTAALGCLVKDYFPEPVTVSWNSGALTSGVHTFPAVLQSSGLYSLSSVVTVPSSSLGTQTYICNVNHKPSNTKVDKKVEPKSCGGGGSGGGGSGGGGSGGGGSEVQLVESGGGLVQPGGSLRLSCAASGFTFSTYAMNWVRQAPGKGLEWVGRIRSKYNNYATYYADSVKGRFTISRDDSKNSLYLQMNSLKTEDTAVYYCVRHGNFGNSYVSWFAYWGQGTLVTVSSGGGGSDKTHTCPPCPAPELLGPSVFLFPPKPKDTLMISRTPEVTCVVVDVSHEDPEVKFNWYVDGVEVHNAKTKPREEQYNSTYRVVSVLTVLHQDWLNGKEYKCKVSNKALGAPIEKTISKAKGQPREPQVYTLPPSREEMTKNQVSLWCLVKGFYPSDIAVEWESNGQPENNYKTTPPVLDSDGSFFLYSKLTVDKSRWQQGNVFSCSVMHEALHNHYTQKSLSLSPGGGGGSGGGGSGGGGSGGGGSQVQLVQSGAEVKKPGASVKVSCKASGYTFAGFEMHWVRQAPGQGLEWMGAIDPKTGGTDYNQKFKDRVTMTRDTSISTAYMELSRLRSDDTAVYYCARDLGYFDVWGQGTLVTVSS

SEQ ID NO: 369 - protein, 599 aa, synthetic construct
QVQLVQSGAEVKKPGASVKVSCKASGYTFTSYVMHWVRQKPGQGLEWIGYINPYNEGTESTDKFKGRATMTSDKSTSTVYMELSSLRSEDTAVYYCASIYYGYEGTYFGVWGQGTLVTVSSASTKGPSVFPLAPSSKSTSGGTAALGCLVKDYFPEPVTVSWNSGALTSGVHTFPAVLQSSGLYSLSSVVTVPSSSLGTQTYICNVNHKPSNTKVDKKVEPKSCGGGGSGGGGSGGGGSGGGGSEVQLVESGGGLVQPGGSLRLSCAASGFTFSTYAMNWVRQAPGKGLEWVGRIRSKYNNYATYYADSVKGRFTISRDDSKNSLYLQMNSLKTEDTAVYYCVRHGNFGNSYVSWFAYWGQGTLVTVSSGGGGSDKTHTCPPCPAPEAAGPSVFLFPPKPKDTLMISRTPEVTCVVVDVSHEDPEVKFNWYVDGVEVHNAKTKPREEQYNSTYRVVSVLTVLHQDWLNGKEYKCKVSNKALPAPIEKTISKAKGQPREPQVYTLPPSREEMTKNQVSLWCLVKGFYPSDIAVEWESNGQPENNYKTTPPVLDSDGSFFLYSKLTVDKSRWQQGNVFSCSVMHEALHNHYTQKSLSLSPG

SEQ ID NO: 370 - protein, 730 aa, synthetic construct
QVQLVQSGAEVKKPGASVKVSCKASGYTFTSYVMHWVRQKPGQGLEWIGYINPYNEGTESTDKFKGRATMTSDKSTSTVYMELSSLRSEDTAVYYCASIYYGYEGTYFGVWGQGTLVTVSSASTKGPSVFPLAPSSKSTSGGTAALGCLVKDYFPEPVTVSWNSGALTSGVHTFPAVLQSSGLYSLSSVVTVPSSSLGTQTYICNVNHKPSNTKVDKKVEPKSCGGGGSGGGGSGGGGSGGGGSEVQLVESGGGLVQPGGSLRLSCAASGFTFSTYAMNWVRQAPGKGLEWVGRIRSKYNNYATYYADSVKGRFTISRDDSKNSLYLQMNSLKTEDTAVYYCVRHGNFGNSYVSWFAYWGQGTLVTVSSDKTHTCPPCPAPEAAGPSVFLFPPKPKDTLMISRTPEVTCVVVDVSHEDPEVKFNWYVDGVEVHNAKTKPREEQYNSTYRVVSVLTVLHQDWLNGKEYKCKVSNKALPAPIEKTISKAKGQPREPQVYTLPPSREEMTKNQVSLWCLVKGFYPSDIAVEWESNGQPENNYKTTPPVLDSDGSFFLYSKLTVDKSRWQQGNVFSCSVMHEALHNHYTQKSLSLSPGGGGGSGGGGSGGGGSGGGGSQVQLVQSGAEVKKPGASVKVSCKASGYTFAGFEMHWVRQAPGQGLEWMGAIDPKTGGTDYNQKFKDRVTMTRDTSISTAYMELSRLRSDDTAVYYCARDLGYFDVWGQGTLVTVSS

SEQ ID NO: 371 - protein, 733 aa, synthetic construct
QVQLVQSGAEVKKPGASVKVSCKASGYTFTSYVMHWVRQKPGQGLEWIGYINPYNEGTESTDKFKGRATMTSDKSTSTVYMELSSLRSEDTAVYYCASIYYGYEGTYFGVWGQGTLVTVSSASTKGPSVFPLAPSSKSTSGGTAALGCLVKDYFPEPVTVSWNSGALTSGVHTFPAVLQSSGLYSLSSVVTVPSSSLGTQTYICNVNHKPSNTKVDKKVEPKSCGGGGSGGGGSGGGGSGGGGSEVQLVESGGGLVQPGGSLRLSCAASGFTFSTYAMNWVRQAPGKGLEWVGRIRSKYNNYATYYADSVKGRFTISRDDSKNSLYLQMNSLKTEDTAVYYCVRHGNFGNSYVSWFAYWGQGTLVTVSSGGSDKTHTCPPCPAPEAAGPSVFLFPPKPKDTLMISRTPEVTCVVVDVSHEDPEVKFNWYVDGVEVHNAKTKPREEQYNSTYRVVSVLTVLHQDWLNGKEYKCKVSNKALPAPIEKTISKAKGQPREPQVYTLPPSREEMTKNQVSLWCLVKGFYPSDIAVEWESNGQPENNYKTTPPVLDSDGSFFLYSKLTVDKSRWQQGNVFSCSVMHEALHNHYTQKSLSLSPGGGGGSGGGGSGGGGSGGGGSQVQLVQSGAEVKKPGASVKVSCKASGYTFAGFEMHWVRQAPGQGLEWMGAIDPKTGGTDYNQKFKDRVTMTRDTSISTAYMELSRLRSDDTAVYYCARDLGYFDVWGQGTLVTVSS

SEQ ID NO: 372 - protein, 734 aa, synthetic construct
QVQLVQSGAEVKKPGASVKVSCKASGYTFTSYVMHWVRQKPGQGLEWIGYINPYNEGTESTDKFKGRATMTSDKSTSTVYMELSSLRSEDTAVYYCASIYYGYEGTYFGVWGQGTLVTVSSASTKGPSVFPLAPSSKSTSGGTAALGCLVKDYFPEPVTVSWNSGALTSGVHTFPAVLQSSGLYSLSSVVTVPSSSLGTQTYICNVNHKPSNTKVDKKVEPKSCGGGGSGGGGSGGGGSGGGGSEVQLVESGGGLVQPGGSLRLSCAASGFTFSTYAMNWVRQAPGKGLEWVGRIRSKYNNYATYYADSVKGRFTISRDDSKNSLYLQMNSLKTEDTAVYYCVRHGNFGNSYVSWFAYWGQGTLVTVSSGGGSDKTHTCPPCPAPEAAGPSVFLFPPKPKDTLMISRTPEVTCVVVDVSHEDPEVKFNWYVDGVEVHNAKTKPREEQYNSTYRVVSVLTVLHQDWLNGKEYKCKVSNKALPAPIEKTISKAKGQPREPQVYTLPPSREEMTKNQVSLWCLVKGFYPSDIAVEWESNGQPENNYKTTPPVLDSDGSFFLYSKLTVDKSRWQQGNVFSCSVMHEALHNHYTQKSLSLSPGGGGGSGGGGSGGGGSGGGGSQVQLVQSGAEVKKPGASVKVSCKASGYTFAGFEMHWVRQAPGQGLEWMGAIDPKTGGTDYNQKFKDRVTMTRDTSISTAYMELSRLRSDDTAVYYCARDLGYFDVWGQGTLVTVSS

SEQ ID NO: 373 - protein, 738 aa, synthetic construct
QVQLVQSGAEVKKPGASVKVSCKASGYTFTSYVMHWVRQKPGQGLEWIGYINPYNEGTESTDKFKGRATMTSDKSTSTVYMELSSLRSEDTAVYYCASIYYGYEGTYFGVWGQGTLVTVSSASTKGPSVFPLAPSSKSTSGGTAALGCLVKDYFPEPVTVSWNSGALTSGVHTFPAVLQSSGLYSLSSVVTVPSSSLGTQTYICNVNHKPSNTKVDKKVEPKSCGGGGSGGGGSGGGGSGGGGSEVQLVESGGGLVQPGGSLRLSCAASGFTFSTYAMNWVRQAPGKGLEWVGRIRSKYNNYATYYADSVKGRFTISRDDSKNSLYLQMNSLKTEDTAVYYCVRHGNFGNSYVSWFAYWGQGTLVTVSSGGGSGGGSDKTHTCPPCPAPEAAGPSVFLFPPKPKDTLMISRTPEVTCVVVDVSHEDPEVKFNWYVDGVEVHNAKTKPREEQYNSTYRVVSVLTVLHQDWLNGKEYKCKVSNKALPAPIEKTISKAKGQPREPQVYTLPPSREEMTKNQVSLWCLVKGFYPSDIAVEWESNGQPENNYKTTPPVLDSDGSFFLYSKLTVDKSRWQQGNVFSCSVMHEALHNHYTQKSLSLSPGGGGGSGGGGSGGGGSGGGGSQVQLVQSGAEVKKPGASVKVSCKASGYTFAGFEMHWVRQAPGQGLEWMGAIDPKTGGTDYNQKFKDRVTMTRDTSISTAYMELSRLRSDDTAVYYCARDLGYFDVWGQGTLVTVSS

SEQ ID NO: 374 - protein, 740 aa, synthetic construct
QVQLVQSGAEVKKPGASVKVSCKASGYTFTSYVMHWVRQKPGQGLEWIGYINPYNEGTESTDKFKGRATMTSDKSTSTVYMELSSLRSEDTAVYYCASIYYGYEGTYFGVWGQGTLVTVSSASTKGPSVFPLAPSSKSTSGGTAALGCLVKDYFPEPVTVSWNSGALTSGVHTFPAVLQSSGLYSLSSVVTVPSSSLGTQTYICNVNHKPSNTKVDKKVEPKSCGGGGSGGGGSGGGGSGGGGSEVQLVESGGGLVQPGGSLRLSCAASGFTFSTYAMNWVRQAPGKGLEWVGRIRSKYNNYATYYADSVKGRFTISRDDSKNSLYLQMNSLKTEDTAVYYCVRHGNFGNSYVSWFAYWGQGTLVTVSSGGGGSGGGGSDKTHTCPPCPAPEAAGPSVFLFPPKPKDTLMISRTPEVTCVVVDVSHEDPEVKFNWYVDGVEVHNAKTKPREEQYNSTYRVVSVLTVLHQDWLNGKEYKCKVSNKALPAPIEKTISKAKGQPREPQVYTLPPSREEMTKNQVSLWCLVKGFYPSDIAVEWESNGQPENNYKTTPPVLDSDGSFFLYSKLTVDKSRWQQGNVFSCSVMHEALHNHYTQKSLSLSPGGGGGSGGGGSGGGGSGGGGSQVQLVQSGAEVKKPGASVKVSCKASGYTFAGFEMHWVRQAPGQGLEWMGAIDPKTGGTDYNQKFKDRVTMTRDTSISTAYMELSRLRSDDTAVYYCARDLGYFDVWGQGTLVTVSS

SEQ ID NO: 375 - protein, 745 aa, synthetic construct
QVQLVQSGAEVKKPGASVKVSCKASGYTFTSYVMHWVRQKPGQGLEWIGYINPYNEGTESTDKFKGRATMTSDKSTSTVYMELSSLRSEDTAVYYCASIYYGYEGTYFGVWGQGTLVTVSSASTKGPSVFPLAPSSKSTSGGTAALGCLVKDYFPEPVTVSWNSGALTSGVHTFPAVLQSSGLYSLSSVVTVPSSSLGTQTYICNVNHKPSNTKVDKKVEPKSCGGGGSGGGGSGGGGSGGGGSEVQLVESGGGLVQPGGSLRLSCAASGFTFSTYAMNWVRQAPGKGLEWVGRIRSKYNNYATYYADSVKGRFTISRDDSKNSLYLQMNSLKTEDTAVYYCVRHGNFGNSYVSWFAYWGQGTLVTVSSGGGGSGGGGSGGGGSDKTHTCPPCPAPEAAGPSVFLFPPKPKDTLMISRTPEVTCVVVDVSHEDPEVKFNWYVDGVEVHNAKTKPREEQYNSTYRVVSVLTVLHQDWLNGKEYKCKVSNKALPAPIEKTISKAKGQPREPQVYTLPPSREEMTKNQVSLWCLVKGFYPSDIAVEWESNGQPENNYKTTPPVLDSDGSFFLYSKLTVDKSRWQQGNVFSCSVMHEALHNHYTQKSLSLSPGGGGGSGGGGSGGGGSGGGGSQVQLVQSGAEVKKPGASVKVSCKASGYTFAGFEMHWVRQAPGQGLEWMGAIDPKTGGTDYNQKFKDRVTMTRDTSISTAYMELSRLRSDDTAVYYCARDLGYFDVWGQGTLVTVSS

SEQ ID NO: 376 - protein, 730 aa, synthetic construct
QVQLVQSGAEVKKPGASVKVSCKASGYTFTSYVMHWVRQKPGQGLEWIGYINPYNEGTESTDKFKGRATMTSDKSTSTVYMELSSLRSEDTAVYYCASIYYGYEGTYFGVWGQGTLVTVSSASTKGPSVFPLAPSSKSTSGGTAALGCLVKDYFPEPVTVSWNSGALTSGVHTFPAVLQSSGLYSLSSVVTVPSSSLGTQTYICNVNHKPSNTKVDKKVEPKSCGGGGSGGGGSGGGGSGGGGSEVQLVESGGGLVQPGGSLRLSCAASGFTFSTYAMNWVRQAPGKGLEWVGRIRSKYNNYATYYADSVKGRFTISRDDSKNSLYLQMNSLKTEDTAVYYCVRHGNFGNSYVSWFAYWGQGTLVTVSSGGGGSDKTHTCPPCPAPEAAGPSVFLFPPKPKDTLMISRTPEVTCVVVDVSHEDPEVKFNWYVDGVEVHNAKTKPREEQYNSTYRVVSVLTVLHQDWLNGKEYKCKVSNKALPAPIEKTISKAKGQPREPQVYTLPPSREEMTKNQVSLWCLVKGFYPSDIAVEWESNGQPENNYKTTPPVLDSDGSFFLYSKLTVDKSRWQQGNVFSCSVMHEALHNHYTQKSLSLSPGGGGGSGGGGSGGGGSQVQLVQSGAEVKKPGASVKVSCKASGYTFAGFEMHWVRQAPGQGLEWMGAIDPKTGGTDYNQKFKDRVTMTRDTSISTAYMELSRLRSDDTAVYYCARDLGYFDVWGQGTLVTVSS

SEQ ID NO: 377 - protein, 725 aa, synthetic construct
QVQLVQSGAEVKKPGASVKVSCKASGYTFTSYVMHWVRQKPGQGLEWIGYINPYNEGTESTDKFKGRATMTSDKSTSTVYMELSSLRSEDTAVYYCASIYYGYEGTYFGVWGQGTLVTVSSASTKGPSVFPLAPSSKSTSGGTAALGCLVKDYFPEPVTVSWNSGALTSGVHTFPAVLQSSGLYSLSSVVTVPSSSLGTQTYICNVNHKPSNTKVDKKVEPKSCGGGGSGGGGSGGGGSGGGGSEVQLVESGGGLVQPGGSLRLSCAASGFTFSTYAMNWVRQAPGKGLEWVGRIRSKYNNYATYYADSVKGRFTISRDDSKNSLYLQMNSLKTEDTAVYYCVRHGNFGNSYVSWFAYWGQGTLVTVSSGGGGSDKTHTCPPCPAPEAAGPSVFLFPPKPKDTLMISRTPEVTCVVVDVSHEDPEVKFNWYVDGVEVHNAKTKPREEQYNSTYRVVSVLTVLHQDWLNGKEYKCKVSNKALPAPIEKTISKAKGQPREPQVYTLPPSREEMTKNQVSLWCLVKGFYPSDIAVEWESNGQPENNYKTTPPVLDSDGSFFLYSKLTVDKSRWQQGNVFSCSVMHEALHNHYTQKSLSLSPGGGGGSGGGGSQVQLVQSGAEVKKPGASVKVSCKASGYTFAGFEMHWVRQAPGQGLEWMGAIDPKTGGTDYNQKFKDRVTMTRDTSISTAYMELSRLRSDDTAVYYCARDLGYFDVWGQGTLVTVSS

SEQ ID NO: 378 - protein, 720 aa, synthetic construct
QVQLVQSGAEVKKPGASVKVSCKASGYTFTSYVMHWVRQKPGQGLEWIGYINPYNEGTESTDKFKGRATMTSDKSTSTVYMELSSLRSEDTAVYYCASIYYGYEGTYFGVWGQGTLVTVSSASTKGPSVFPLAPSSKSTSGGTAALGCLVKDYFPEPVTVSWNSGALTSGVHTFPAVLQSSGLYSLSSVVTVPSSSLGTQTYICNVNHKPSNTKVDKKVEPKSCGGGGSGGGGSGGGGSGGGGSEVQLVESGGGLVQPGGSLRLSCAASGFTFSTYAMNWVRQAPGKGLEWVGRIRSKYNNYATYYADSVKGRFTISRDDSKNSLYLQMNSLKTEDTAVYYCVRHGNFGNSYVSWFAYWGQGTLVTVSSGGGGSDKTHTCPPCPAPEAAGPSVFLFPPKPKDTLMISRTPEVTCVVVDVSHEDPEVKFNWYVDGVEVHNAKTKPREEQYNSTYRVVSVLTVLHQDWLNGKEYKCKVSNKALPAPIEKTISKAKGQPREPQVYTLPPSREEMTKNQVSLWCLVKGFYPSDIAVEWESNGQPENNYKTTPPVLDSDGSFFLYSKLTVDKSRWQQGNVFSCSVMHEALHNHYTQKSLSLSPGGGGGSQVQLVQSGAEVKKPGASVKVSCKASGYTFAGFEMHWVRQAPGQGLEWMGAIDPKTGGTDYNQKFKDRVTMTRDTSISTAYMELSRLRSDDTAVYYCARDLGYFDVWGQGTLVTVSS

SEQ ID NO: 379 - protein, 739 aa, synthetic construct
QVQLVQSGAEVKKPGASVKVSCKASGYTFTSYVMHWVRQKPGQGLEWIGYINPYNEGTESTDKFKGRATMTSDKSTSTVYMELSSLRSEDTAVYYCASIYYGYEGTYFGVWGQGTLVTVSSASTKGPSVFPLAPSSKSTSGGTAALGCLVKDYFPEPVTVSWNSGALTSGVHTFPAVLQSSGLYSLSSVVTVPSSSLGTQTYICNVNHKPSNTKVDKKVEPKSCGGGGSGGGGSGGGGSGGGGSEVQLVESGGGLVQPGGSLRLSCAASGFTFSTYAMNWVRQAPGKGLEWVGRIRSKYNNYATYYADSVKGRFTISRDDSKNSLYLQMNSLKTEDTAVYYCVRHGNFGNSYVSWFAYWGQGTLVTVSSGGGGSDKTHTCPPCPAPEAAGPSVFLFPPKPKDTLMISRTPEVTCVVVDVSHEDPEVKFNWYVDGVEVHNAKTKPREEQYNSTYRVVSVLTVLHQDWLNGKEYKCKVSNKALPAPIEKTISKAKGQPREPQVYTLPPSREEMTKNQVSLWCLVKGFYPSDIAVEWESNGQPENNYKTTPPVLDSDGSFFLYSKLTVDKSRWQQGNVFSCSVMHEALHNHYTQKSLSLSPGDKTHTCPPCGGGGSGGGGSGGGGSQVQLVQSGAEVKKPGASVKVSCKASGYTFAGFEMHWVRQAPGQGLEWMGAIDPKTGGTDYNQKFKDRVTMTRDTSISTAYMELSRLRSDDTAVYYCARDLGYFDVWGQGTLVTVSS

SEQ ID NO: 380 - protein, 744 aa, synthetic construct
QVQLVQSGAEVKKPGASVKVSCKASGYTFTSYVMHWVRQKPGQGLEWIGYINPYNEGTESTDKFKGRATMTSDKSTSTVYMELSSLRSEDTAVYYCASIYYGYEGTYFGVWGQGTLVTVSSASTKGPSVFPLAPSSKSTSGGTAALGCLVKDYFPEPVTVSWNSGALTSGVHTFPAVLQSSGLYSLSSVVTVPSSSLGTQTYICNVNHKPSNTKVDKKVEPKSCGGGGSGGGGSGGGGSGGGGSEVQLVESGGGLVQPGGSLRLSCAASGFTFSTYAMNWVRQAPGKGLEWVGRIRSKYNNYATYYADSVKGRFTISRDDSKNSLYLQMNSLKTEDTAVYYCVRHGNFGNSYVSWFAYWGQGTLVTVSSGGGGSDKTHTCPPCPAPEAAGPSVFLFPPKPKDTLMISRTPEVTCVVVDVSHEDPEVKFNWYVDGVEVHNAKTKPREEQYNSTYRVVSVLTVLHQDWLNGKEYKCKVSNKALPAPIEKTISKAKGQPREPQVYTLPPSREEMTKNQVSLWCLVKGFYPSDIAVEWESNGQPENNYKTTPPVLDSDGSFFLYSKLTVDKSRWQQGNVFSCSVMHEALHNHYTQKSLSLSPGDKTHTCPPCGGGGSGGGGSGGGGSGGGGSQVQLVQSGAEVKKPGASVKVSCKASGYTFAGFEMHWVRQAPGQGLEWMGAIDPKTGGTDYNQKFKDRVTMTRDTSISTAYMELSRLRSDDTAVYYCARDLGYFDVWGQGTLVTVSS

SEQ ID NO: 381 - protein, 734 aa, synthetic construct
QVQLVQSGAEVKKPGASVKVSCKASGYTFTSYVMHWVRQKPGQGLEWIGYINPYNEGTESTDKFKGRATMTSDKSTSTVYMELSSLRSEDTAVYYCASIYYGYEGTYFGVWGQGTLVTVSSASTKGPSVFPLAPSSKSTSGGTAALGCLVKDYFPEPVTVSWNSGALTSGVHTFPAVLQSSGLYSLSSVVTVPSSSLGTQTYICNVNHKPSNTKVDKKVEPKSCGGGGSGGGGSGGGGSGGGGSEVQLVESGGGLVQPGGSLRLSCAASGFTFSTYAMNWVRQAPGKGLEWVGRIRSKYNNYATYYADSVKGRFTISRDDSKNSLYLQMNSLKTEDTAVYYCVRHGNFGNSYVSWFAYWGQGTLVTVSSGGGGSDKTHTCPPCPAPEAAGPSVFLFPPKPKDTLMISRTPEVTCVVVDVSHEDPEVKFNWYVDGVEVHNAKTKPREEQYNSTYRVVSVLTVLHQDWLNGKEYKCKVSNKALPAPIEKTISKAKGQPREPQVYTLPPSREEMTKNQVSLWCLVKGFYPSDIAVEWESNGQPENNYKTTPPVLDSDGSFFLYSKLTVDKSRWQQGNVFSCSVMHEALHNHYTQKSLSLSPGDKTHTCPPCGGGGSGGGGSQVQLVQSGAEVKKPGASVKVSCKASGYTFAGFEMHWVRQAPGQGLEWMGAIDPKTGGTDYNQKFKDRVTMTRDTSISTAYMELSRLRSDDTAVYYCARDLGYFDVWGQGTLVTVSS

SEQ ID NO: 382 - protein, 729 aa, synthetic construct
QVQLVQSGAEVKKPGASVKVSCKASGYTFTSYVMHWVRQKPGQGLEWIGYINPYNEGTESTDKFKGRATMTSDKSTSTVYMELSSLRSEDTAVYYCASIYYGYEGTYFGVWGQGTLVTVSSASTKGPSVFPLAPSSKSTSGGTAALGCLVKDYFPEPVTVSWNSGALTSGVHTFPAVLQSSGLYSLSSVVTVPSSSLGTQTYICNVNHKPSNTKVDKKVEPKSCGGGGSGGGGSGGGGSGGGGSEVQLVESGGGLVQPGGSLRLSCAASGFTFSTYAMNWVRQAPGKGLEWVGRIRSKYNNYATYYADSVKGRFTISRDDSKNSLYLQMNSLKTEDTAVYYCVRHGNFGNSYVSWFAYWGQGTLVTVSSGGGGSDKTHTCPPCPAPEAAGPSVFLFPPKPKDTLMISRTPEVTCVVVDVSHEDPEVKFNWYVDGVEVHNAKTKPREEQYNSTYRVVSVLTVLHQDWLNGKEYKCKVSNKALPAPIEKTISKAKGQPREPQVYTLPPSREEMTKNQVSLWCLVKGFYPSDIAVEWESNGQPENNYKTTPPVLDSDGSFFLYSKLTVDKSRWQQGNVFSCSVMHEALHNHYTQKSLSLSPGDKTHTCPPCGGGGSQVQLVQSGAEVKKPGASVKVSCKASGYTFAGFEMHWVRQAPGQGLEWMGAIDPKTGGTDYNQKFKDRVTMTRDTSISTAYMELSRLRSDDTAVYYCARDLGYFDVWGQGTLVTVSS

SEQ ID NO: 383 - protein, 724 aa, synthetic construct
QVQLVQSGAEVKKPGASVKVSCKASGYTFTSYVMHWVRQKPGQGLEWIGYINPYNEGTESTDKFKGRATMTSDKSTSTVYMELSSLRSEDTAVYYCASIYYGYEGTYFGVWGQGTLVTVSSASTKGPSVFPLAPSSKSTSGGTAALGCLVKDYFPEPVTVSWNSGALTSGVHTFPAVLQSSGLYSLSSVVTVPSSSLGTQTYICNVNHKPSNTKVDKKVEPKSCGGGGSGGGGSGGGGSGGGGSEVQLVESGGGLVQPGGSLRLSCAASGFTFSTYAMNWVRQAPGKGLEWVGRIRSKYNNYATYYADSVKGRFTISRDDSKNSLYLQMNSLKTEDTAVYYCVRHGNFGNSYVSWFAYWGQGTLVTVSSGGGGSDKTHTCPPCPAPEAAGPSVFLFPPKPKDTLMISRTPEVTCVVVDVSHEDPEVKFNWYVDGVEVHNAKTKPREEQYNSTYRVVSVLTVLHQDWLNGKEYKCKVSNKALPAPIEKTISKAKGQPREPQVYTLPPSREEMTKNQVSLWCLVKGFYPSDIAVEWESNGQPENNYKTTPPVLDSDGSFFLYSKLTVDKSRWQQGNVFSCSVMHEALHNHYTQKSLSLSPGDKTHTCPPCQVQLVQSGAEVKKPGASVKVSCKASGYTFAGFEMHWVRQAPGQGLEWMGAIDPKTGGTDYNQKFKDRVTMTRDTSISTAYMELSRLRSDDTAVYYCARDLGYFDVWGQGTLVTVSS

SEQ ID NO: 384 - protein, 715 aa, synthetic construct
QVQLVQSGAEVKKPGASVKVSCKASGYTFTSYVMHWVRQKPGQGLEWIGYINPYNEGTESTDKFKGRATMTSDKSTSTVYMELSSLRSEDTAVYYCASIYYGYEGTYFGVWGQGTLVTVSSASTKGPSVFPLAPSSKSTSGGTAALGCLVKDYFPEPVTVSWNSGALTSGVHTFPAVLQSSGLYSLSSVVTVPSSSLGTQTYICNVNHKPSNTKVDKKVEPKSCGGGGSGGGGSGGGGSGGGGSEVQLVESGGGLVQPGGSLRLSCAASGFTFSTYAMNWVRQAPGKGLEWVGRIRSKYNNYATYYADSVKGRFTISRDDSKNSLYLQMNSLKTEDTAVYYCVRHGNFGNSYVSWFAYWGQGTLVTVSSGGGGSDKTHTCPPCPAPEAAGPSVFLFPPKPKDTLMISRTPEVTCVVVDVSHEDPEVKFNWYVDGVEVHNAKTKPREEQYNSTYRVVSVLTVLHQDWLNGKEYKCKVSNKALPAPIEKTISKAKGQPREPQVYTLPPSREEMTKNQVSLWCLVKGFYPSDIAVEWESNGQPENNYKTTPPVLDSDGSFFLYSKLTVDKSRWQQGNVFSCSVMHEALHNHYTQKSLSLSPGQVQLVQSGAEVKKPGASVKVSCKASGYTFAGFEMHWVRQAPGQGLEWMGAIDPKTGGTDYNQKFKDRVTMTRDTSISTAYMELSRLRSDDTAVYYCARDLGYFDVWGQGTLVTVSS

SEQ ID NO: 385 - protein, 596 aa, synthetic construct
QVQLVQSGAEVKKPGASVKVSCKASGYTFTSYVMHWVRQKPGQGLEWIGYINPYNEGTESTDKFKGRATMTSDKSTSTVYMELSSLRSEDTAVYYCASIYYGYEGTYFGVWGQGTLVTVSSASTKGPSVFPLAPSSKSTSGGTAALGCLVKDYFPEPVTVSWNSGALTSGVHTFPAVLQSSGLYSLSSVVTVPSSSLGTQTYICNVNHKPSNTKVDKKVEPKSCGGGGSGGGGSGGGGSGGGGSEVQLVESGGGLVQPGGSLRLSCAASGFTFTNYGLHWVRQAPGKGLEWVSSISPSGGVTYYRDSVKGRFTISRDNSKNTLYLQMNSLRAEDTAVYYCAKPFLGWGGANWIAHWGQGTLVTVSSGGGGSDKTHTCPPCPAPEAAGPSVFLFPPKPKDTLMISRTPEVTCVVVDVSHEDPEVKFNWYVDGVEVHNAKTKPREEQYNSTYRVVSVLTVLHQDWLNGKEYKCKVSNKALPAPIEKTISKAKGQPREPQVYTLPPSREEMTKNQVSLWCLVKGFYPSDIAVEWESNGQPENNYKTTPPVLDSDGSFFLYSKLTVDKSRWQQGNVFSCSVMHEALHNHYTQKSLSLSPG

SEQ ID NO: 386 - protein, 732 aa, synthetic construct
QVQLVQSGAEVKKPGASVKVSCKASGYTFTSYVMHWVRQKPGQGLEWIGYINPYNEGTESTDKFKGRATMTSDKSTSTVYMELSSLRSEDTAVYYCASIYYGYEGTYFGVWGQGTLVTVSSASTKGPSVFPLAPSSKSTSGGTAALGCLVKDYFPEPVTVSWNSGALTSGVHTFPAVLQSSGLYSLSSVVTVPSSSLGTQTYICNVNHKPSNTKVDKKVEPKSCGGGGSGGGGSGGGGSGGGGSEVQLVESGGGLVQPGGSLRLSCAASGFTFTNYGLHWVRQAPGKGLEWVSSISPSGGVTYYRDSVKGRFTISRDNSKNTLYLQMNSLRAEDTAVYYCAKPFLGWGGANWIAHWGQGTLVTVSSGGGGSDKTHTCPPCPAPEAAGPSVFLFPPKPKDTLMISRTPEVTCVVVDVSHEDPEVKFNWYVDGVEVHNAKTKPREEQYNSTYRVVSVLTVLHQDWLNGKEYKCKVSNKALPAPIEKTISKAKGQPREPQVYTLPPSREEMTKNQVSLWCLVKGFYPSDIAVEWESNGQPENNYKTTPPVLDSDGSFFLYSKLTVDKSRWQQGNVFSCSVMHEALHNHYTQKSLSLSPGGGGGSGGGGSGGGGSGGGGSQVQLVQSGAEVKKPGASVKVSCKASGYTFAGFEMHWVRQAPGQGLEWMGAIDPKTGGTDYNQKFKDRVTMTRDTSISTAYMELSRLRSDDTAVYYCARDLGYFDVWGQGTLVTVSS

SEQ ID NO: 387 - protein, 736 aa, synthetic construct
QVQLVQSGAEVKKPGASVKVSCKASGYTFTSYVMHWVRQKPGQGLEWIGYINPYNEGTESTDKFKGRATMTSDKSTSTVYMELSSLRSEDTAVYYCASIYYGYEGTYFGVWGQGTLVTVSSASTKGPSVFPLAPSSKSTSGGTAALGCLVKDYFPEPVTVSWNSGALTSGVHTFPAVLQSSGLYSLSSVVTVPSSSLGTQTYICNVNHKPSNTKVDKKVEPKSCGGGGSGGGGSGGGGSGGGGSEVQLVESGGGLVQPGGSLRLSCAASGFTFSTYAMNWVRQAPGKGLEWVGRIRSKYNNYATYYADSVKGRFTISRDDSKNSLYLQMNSLKTEDTAVYYCVRHGNFGNSYVSWFAYWGQGTLVTVSSGGGGSDKTHTCPPCPAPELLGPSVFLFPPKPKDTLMISRTPEVTCVVVDVSHEDPEVKFNWYVDGVEVHNAKTKPREEQYNSTYRVVSVLTVLHQDWLNGKEYKCKVSNKALGAPIEKTISKAKGQPREPQVYTLPPSREEMTKNQVSLWCLVKGFYPSDIAVEWESNGQPENNYKTTPPVLDSDGSFFLYSKLTVDKSRWQQGNVFSCSVMHEALHNHYTQKSLSLSPGKGGGGSGGGGSGGGGSGGGGSQVQLVQSGAEVKKPGASVKVSCKASGYTFAGFEMHWVRQAPGQGLEWMGAIDPKTGGTDYNQKFKDRVTMTRDTSISTAYMELSRLRSDDTAVYYCARDLGYFDVWGQGTLVTVSS

SEQ ID NO: 388 - protein, 740 aa, synthetic construct
QVQLVQSGAEVKKPGASVKVSCKASGYTFTSYVMHWVRQKPGQGLEWIGYINPYNEGTESTDKFKGRATMTSDKSTSTVYMELSSLRSEDTAVYYCASIYYGYEGTYFGVWGQGTLVTVSSASTKGPSVFPLAPSSKSTSGGTAALGCLVKDYFPEPVTVSWNSGALTSGVHTFPAVLQSSGLYSLSSVVTVPSSSLGTQTYICNVNHKPSNTKVDKKVEPKSCGGGGSGGGGSGGGGSGGGGSEVQLVESGGGLVQPGGSLRLSCAASGFTFSTYAMNWVRQAPGKGLEWVGRIRSKYNNYATYYADSVKGRFTISRDDSKNSLYLQMNSLKTEDTAVYYCVRHGNFGNSYVSWFAYWGQGTLVTVSSGGGGSDKTHTCPPCPAPELLGPSVFLFPPKPKDTLMISRTPEVTCVVVDVSHEDPEVKFNWYVDGVEVHNAKTKPREEQYNSTYRVVSVLTVLHQDWLNGKEYKCKVSNKALGAPIEKTISKAKGQPREPQVYTLPPSREEMTKNQVSLWCLVKGFYPSDIAVEWESNGQPENNYKTTPPVLDSDGSFFLYSKLTVDKSRWQQGNVFSCSVMHEALHNHYTQKSLSLSPGKGGGGSGGGGSGGGGSGGGGSQVQLVQSGAEVKKPGASVKVSCKASGYTFTSYYIHWVRQAPGQGLEWIGCIYPGNVNTNYNEKFKDRATLTVDTSISTAYMELSRLRSDDTAVYFCTRSHYGLDWNFDVWGQGTTVTVSS

SEQ ID NO: 389 - protein, 600 aa, synthetic construct
QVQLVQSGAEVKKPGASVKVSCKASGYTFTSYVMHWVRQKPGQGLEWIGYINPYNEGTESTDKFKGRATMTSDKSTSTVYMELSSLRSEDTAVYYCASIYYGYEGTYFGVWGQGTLVTVSSASTKGPSVFPLAPSSKSTSGGTAALGCLVKDYFPEPVTVSWNSGALTSGVHTFPAVLQSSGLYSLSSVVTVPSSSLGTQTYICNVNHKPSNTKVDKKVEPKSCGGGGSGGGGSGGGGSGGGGSEVQLVESGGGLVQPGGSLRLSCAASGFTFSTYAMNWVRQAPGKGLEWVGRIRSKYNNYATYYADSVKGRFTISRDDSKNSLYLQMNSLKTEDTAVYYCVRHGNFGNSYVSWFAYWGQGTLVTVSSGGGGSDKTHTCPPCPAPELLGPSVFLFPPKPKDTLMISRTPEVTCVVVDVSHEDPEVKFNWYVDGVEVHNAKTKPREEQYNSTYRVVSVLTVLHQDWLNGKEYKCKVSNKALGAPIEKTISKAKGQPREPQVYTLPPSREEMTKNQVSLWCLVKGFYPSDIAVEWESNGQPENNYKTTPPVLDSDGSFFLYSKLTVDKSRWQQGNVFSCSVMHEALHNHYTQKSLSLSPGK

SEQ ID NO: 390 - protein, 738 aa, synthetic construct
QVQLVQSGAEVKKPGASVKVSCKASGYTFTSYVMHWVRQKPGQGLEWIGYINPYNEGTESTDKFKGRATMTSDKSTSTVYMELSSLRSEDTAVYYCASIYYGYEGTYFGVWGQGTLVTVSSASTKGPSVFPLAPSSKSTSGGTAALGCLVKDYFPEPVTVSWNSGALTSGVHTFPAVLQSSGLYSLSSVVTVPSSSLGTQTYICNVNHKPSNTKVDKKVEPKSCGGGGSGGGGSGGGGSGGGGSEVQLVESGGGLVQPGGSLRLSCAASGFTFSTYAMNWVRQAPGKGLEWVGRIRSKYNNYATYYADSVKGRFTISRDDSKNSLYLQMNSLKTEDTAVYYCVRHGNFGNSYVSWFAYWGQGTLVTVSSGGGGSDKTHTCPPCPAPELLGPSVFLFPPKPKDTLMISRTPEVTCVVVDVSHEDPEVKFNWYVDGVEVHNAKTKPREEQYNSTYRVVSVLTVLHQDWLNGKEYKCKVSNKALGAPIEKTISKAKGQPREPQVYTLPPSREEMTKNQVSLWCLVKGFYPSDIAVEWESNGQPENNYKTTPPVLDSDGSFFLYSKLTVDKSRWQQGNVFSCSVMHEALHNHYTQKSLSLSPGKGGGGSGGGGSGGGGSGGGGSQVQLVESGGGVVQPGRSLRLSCAASGFTFSSYTMHWVRQAPGKGLEWVTFISYDGNNKYYADSVKGRFTISRDNSKNTLYLQMNSLRAEDTAIYYCARTGWLGPFDYWGQGTLVTVSS

SEQ ID NO: 391 - protein, 745 aa, synthetic construct
QVQLVQSGAEVKKPGASVKVSCKASGYTFTSYVMHWVRQKPGQGLEWIGYINPYNEGTESTDKFKGRATMTSDKSTSTVYMELSSLRSEDTAVYYCASIYYGYEGTYFGVWGQGTLVTVSSASTKGPSVFPLAPSSKSTSGGTAALGCLVKDYFPEPVTVSWNSGALTSGVHTFPAVLQSSGLYSLSSVVTVPSSSLGTQTYICNVNHKPSNTKVDKKVEPKSCGGGGSGGGGSGGGGSGGGGSEVQLVESGGGLVQPGGSLRLSCAASGFTFSTYAMNWVRQAPGKGLEWVGRIRSKYNNYATYYADSVKGRFTISRDDSKNSLYLQMNSLKTEDTAVYYCVRHGNFGNSYVSWFAYWGQGTLVTVSSGGGGSDKTHTCPPCPAPELLGPSVFLFPPKPKDTLMISRTPEVTCVVVDVSHEDPEVKFNWYVDGVEVHNAKTKPREEQYNSTYRVVSVLTVLHQDWLNGKEYKCKVSNKALGAPIEKTISKAKGQPREPQVYTLPPSREEMTKNQVSLWCLVKGFYPSDIAVEWESNGQPENNYKTTPPVLDSDGSFFLYSKLTVDKSRWQQGNVFSCSVMHEALHNHYTQKSLSLSPGKGGGGSGGGGSGGGGSGGGGSQVQLVESGGGVVQPGRSLRLSCAASGFTFSSYGMHWVRQAPGKGLEWVAVIWYDGSNKYYADSVKGRFTISRDNSKNTLYLQMNSLRAEDTAVYYCARDPRGATLYYYYYGMDVWGQGTTVTVSS

SEQ ID NO: 392 - protein, 735 aa, synthetic construct
QVQLVQSGAEVKKPGASVKVSCKASGYTFTSYVMHWVRQKPGQGLEWIGYINPYNEGTESTDKFKGRATMTSDKSTSTVYMELSSLRSEDTAVYYCASIYYGYEGTYFGVWGQGTLVTVSSASTKGPSVFPLAPSSKSTSGGTAALGCLVKDYFPEPVTVSWNSGALTSGVHTFPAVLQSSGLYSLSSVVTVPSSSLGTQTYICNVNHKPSNTKVDKKVEPKSCGGGGSGGGGSGGGGSGGGGSEVQLVESGGGLVQPGGSLRLSCAASGFTFSTYAMNWVRQAPGKGLEWVGRIRSKYNNYATYYADSVKGRFTISRDDSKNSLYLQMNSLKTEDTAVYYCVRHGNFGNSYVSWFAYWGQGTLVTVSSGGGGSDKTHTCPPCPAPELLGPSVFLFPPKPKDTLMISRTPEVTCVVVDVSHEDPEVKFNWYVDGVEVHNAKTKPREEQYNSTYRVVSVLTVLHQDWLNGKEYKCKVSNKALGAPIEKTISKAKGQPREPQVYTLPPSREEMTKNQVSLWCLVKGFYPSDIAVEWESNGQPENNYKTTPPVLDSDGSFFLYSKLTVDKSRWQQGNVFSCSVMHEALHNHYTQKSLSLSPGKGGGGSGGGGSGGGGSGGGGSQVQLVESGAEVKKPGASVKVSCKASGYSFTGYTMNWVRQAPGQCLEWIGLINPYNNITNYAQKFQGRVTFTVDTSISTAYMELSRLRSDDTGVYFCARLDYRSYWGQGTLVTVSA

SEQ ID NO: 393 - protein, 741 aa, synthetic construct
QVQLVQSGAEVKKPGASVKVSCKASGYTFTSYVMHWVRQKPGQGLEWIGYINPYNEGTESTDKFKGRATMTSDKSTSTVYMELSSLRSEDTAVYYCASIYYGYEGTYFGVWGQGTLVTVSSASTKGPSVFPLAPSSKSTSGGTAALGCLVKDYFPEPVTVSWNSGALTSGVHTFPAVLQSSGLYSLSSVVTVPSSSLGTQTYICNVNHKPSNTKVDKKVEPKSCGGGGSGGGGSGGGGSGGGGSEVQLVESGGGLVQPGGSLRLSCAASGFTFSTYAMNWVRQAPGKGLEWVGRIRSKYNNYATYYADSVKGRFTISRDDSKNSLYLQMNSLKTEDTAVYYCVRHGNFGNSYVSWFAYWGQGTLVTVSSGGGGSDKTHTCPPCPAPELLGPSVFLFPPKPKDTLMISRTPEVTCVVVDVSHEDPEVKFNWYVDGVEVHNAKTKPREEQYNSTYRVVSVLTVLHQDWLNGKEYKCKVSNKALGAPIEKTISKAKGQPREPQVYTLPPSREEMTKNQVSLWCLVKGFYPSDIAVEWESNGQPENNYKTTPPVLDSDGSFFLYSKLTVDKSRWQQGNVFSCSVMHEALHNHYTQKSLSLSPGKGGGGSGGGGSGGGGSGGGGSQVTLKESGPALVKPTQTLTLTCTFSGFSLSTSGTCVSWIRQPPGKALEWLATICWEDSKGYNPSLKSRLTISKDTSKNQAVLTMTNMDPVDTATYYCARREDSGYFWFPYWGQGTLVTVSS

SEQ ID NO: 394 - protein, 742 aa, synthetic construct
QVQLVQSGAEVKKPGASVKVSCKASGYTFTSYVMHWVRQKPGQGLEWIGYINPYNEGTESTDKFKGRATMTSDKSTSTVYMELSSLRSEDTAVYYCASIYYGYEGTYFGVWGQGTLVTVSSASTKGPSVFPLAPSSKSTSGGTAALGCLVKDYFPEPVTVSWNSGALTSGVHTFPAVLQSSGLYSLSSVVTVPSSSLGTQTYICNVNHKPSNTKVDKKVEPKSCGGGGSGGGGSGGGGSGGGGSEVQLVESGGGLVQPGGSLRLSCAASGFTFSTYAMNWVRQAPGKGLEWVGRIRSKYNNYATYYADSVKGRFTISRDDSKNSLYLQMNSLKTEDTAVYYCVRHGNFGNSYVSWFAYWGQGTLVTVSSGGGGSDKTHTCPPCPAPELLGPSVFLFPPKPKDTLMISRTPEVTCVVVDVSHEDPEVKFNWYVDGVEVHNAKTKPREEQYNSTYRVVSVLTVLHQDWLNGKEYKCKVSNKALGAPIEKTISKAKGQPREPQVYTLPPSREEMTKNQVSLWCLVKGFYPSDIAVEWESNGQPENNYKTTPPVLDSDGSFFLYSKLTVDKSRWQQGNVFSCSVMHEALHNHYTQKSLSLSPGKGGGGSGGGGSGGGGSGGGGSQVQLVQSGAEVKKPGASVKVSCKASGYTFTDFWMSWVRQAPGQGLEWMGQIYPNTGTTHSNEKFKGRVTMTRDTSTSTVYMELSSLRSEDTAVYYCARSYHISTTPNWFAYWGQGTLVTVSS

SEQ ID NO: 395 - protein, 738 aa, synthetic construct
QVQLVQSGAEVKKPGASVKVSCKASGYTFTSYVMHWVRQKPGQGLEWIGYINPYNEGTESTDKFKGRATMTSDKSTSTVYMELSSLRSEDTAVYYCASIYYGYEGTYFGVWGQGTLVTVSSASTKGPSVFPLAPSSKSTSGGTAALGCLVKDYFPEPVTVSWNSGALTSGVHTFPAVLQSSGLYSLSSVVTVPSSSLGTQTYICNVNHKPSNTKVDKKVEPKSCGGGGSGGGGSGGGGSGGGGSEVQLVESGGGLVQPGGSLRLSCAASGFTFSTYAMNWVRQAPGKGLEWVGRIRSKYNNYATYYADSVKGRFTISRDDSKNSLYLQMNSLKTEDTAVYYCVRHGNFGNSYVSWFAYWGQGTLVTVSSGGGGSDKTHTCPPCPAPELLGPSVFLFPPKPKDTLMISRTPEVTCVVVDVSHEDPEVKFNWYVDGVEVHNAKTKPREEQYNSTYRVVSVLTVLHQDWLNGKEYKCKVSNKALGAPIEKTISKAKGQPREPQVYTLPPSREEMTKNQVSLWCLVKGFYPSDIAVEWESNGQPENNYKTTPPVLDSDGSFFLYSKLTVDKSRWQQGNVFSCSVMHEALHNHYTQKSLSLSPGKGGGGSGGGGSGGGGSGGGGSEVQLVESGGGLVQPGGSLRLSCAASGFTFSDSWIHWVRQAPGKGLEWVAWISPYGGSTYYADSVKGRFTISADTSKNTAYLQMNSLRAEDTAVYYCARRHWPGGFDYWGQGTLVTVSS

SEQ ID NO: 396 - protein, 744 aa, synthetic construct
QVQLVQSGAEVKKPGASVKVSCKASGYTFTSYVMHWVRQKPGQGLEWIGYINPYNEGTESTDKFKGRATMTSDKSTSTVYMELSSLRSEDTAVYYCASIYYGYEGTYFGVWGQGTLVTVSSASTKGPSVFPLAPSSKSTSGGTAALGCLVKDYFPEPVTVSWNSGALTSGVHTFPAVLQSSGLYSLSSVVTVPSSSLGTQTYICNVNHKPSNTKVDKKVEPKSCGGGGSGGGGSGGGGSGGGGSGGGGSEVQLVESGGGLVQPGGSLRLSCAASGFTFSTYAMNWVRQAPGKGLEWVGRIRSKYNNYATYYADSVKGRFTISRDDSKNSLYLQMNSLKTEDTAVYYCVRHGNFGNSYVSWFAYWGQGTLVTVSSGGGGSDKTHTCPPCPAPEAAGPSVFLFPPKPKDTLMISRTPEVTCVVVDVSHEDPEVKFNWYVDGVEVHNAKTKPREEQYNSTYRVVSVLTVLHQDWLNGKEYKCKVSNKALPAPIEKTISKAKGQPREPQVYTLPPSREEMTKNQVSLWCLVKGFYPSDIAVEWESNGQPENNYKTTPPVLDSDGSFFLYSKLTVDKSRWQQGNVFSCSVMHEALHNHYTQKSLSLSPGGGGGSGGGGSGGGGSGGGGSQVQLVQSGAEVKKPGASVKVSCKASGYTFTSYYIHWVRQAPGQGLEWIGCIYPGNVNTNYNEKFKDRATLTVDTSISTAYMELSRLRSDDTAVYFCTRSHYGLDWNFDVWGQGTTVTVSS

SEQ ID NO: 397 - protein, 740 aa, synthetic construct
QVQLVQSGAEVKKPGASVKVSCKASGYTFTSYVMHWVRQKPGQGLEWIGYINPYNEGTESTDKFKGRATMTSDKSTSTVYMELSSLRSEDTAVYYCASIYYGYEGTYFGVWGQGTLVTVSSASTKGPSVFPLAPSSKSTSGGTAALGCLVKDYFPEPVTVSWNSGALTSGVHTFPAVLQSSGLYSLSSVVTVPSSSLGTQTYICNVNHKPSNTKVDKKVEPKSCGGGGSGGGGSGGGGSGGGGSGGGGSEVQLVESGGGLVQPGGSLRLSCAASGFTFSTYAMNWVRQAPGKGLEWVGRIRSKYNNYATYYADSVKGRFTISRDDSKNSLYLQMNSLKTEDTAVYYCVRHGNFGNSYVSWFAYWGQGTLVTVSSGGGGSDKTHTCPPCPAPEAAGPSVFLFPPKPKDTLMISRTPEVTCVVVDVSHEDPEVKFNWYVDGVEVHNAKTKPREEQYNSTYRVVSVLTVLHQDWLNGKEYKCKVSNKALPAPIEKTISKAKGQPREPQVYTLPPSREEMTKNQVSLWCLVKGFYPSDIAVEWESNGQPENNYKTTPPVLDSDGSFFLYSKLTVDKSRWQQGNVFSCSVMHEALHNHYTQKSLSLSPGGGGGSGGGGSGGGGSGGGGSQVQLVQSGAEVKKPGASVKVSCKASGYTFAGFEMHWVRQAPGQGLEWMGAIDPKTGGTDYNQKFKDRVTMTRDTSISTAYMELSRLRSDDTAVYYCARDLGYFDVWGQGTLVTVSS

SEQ ID NO: 398 - protein, 715 aa, synthetic construct
QVQLVQSGAEVKKPGASVKVSCKASGYTFTSYVMHWVRQKPGQGLEWIGYINPYNEGTESTDKFKGRATMTSDKSTSTVYMELSSLRSEDTAVYYCASIYYGYEGTYFGVWGQGTLVTVSSASTKGPSVFPLAPSSKSTSGGTAALGCLVKDYFPEPVTVSWNSGALTSGVHTFPAVLQSSGLYSLSSVVTVPSSSLGTQTYICNVNHKPSNTKVDKKVEPKSCGGGGSGGGGSGGGGSGGGGSGGGGSQAVVTQEPSLTVSPGGTVTLTCRSSTGAVTTSNYANWVQQKPGQAPRGLIGGTNKRAPWTPARFSGSLLGGKAALTITGAQAEDEADYYCALWYSNLWVFGGGTKLTVLGGGGSDKTHTCPPCPAPEAAGPSVFLFPPKPKDTLMISRTPEVTCVVVDVSHEDPEVKFNWYVDGVEVHNAKTKPREEQYNSTYRVVSVLTVLHQDWLNGKEYKCKVSNKALPAPIEKTISKAKGQPREPQVYTLPPSREEMTKNQVSLSCAVKGFYPSDIAVEWESNGQPENNYKTTPPVLDSDGSFFLVSKLTVDKSRWQQGNVFSCSVMHEALHNRFTQKSLSLSPGGGGGSGGGGSGGGGSGGGGSDIQMTQSPSSLSASVGDRVTITCHASQNIYVWLNWYQQKPGKAPKLLIYKASNLHTGVPSRFSGSGSGTDFTLTISSLQPEDFATYYCQQGQTYPYTFGGGTKVEIK

SEQ ID NO: 399 - protein, 715 aa, synthetic construct
QVQLVQSGAEVKKPGASVKVSCKASGYTFTSYVMHWVRQKPGQGLEWIGYINPYNEGTESTDKFKGRATMTSDKSTSTVYMELSSLRSEDTAVYYCASIYYGYEGTYFGVWGQGTLVTVSSASTKGPSVFPLAPSSKSTSGGTAALGCLVKDYFPEPVTVSWNSGALTSGVHTFPAVLQSSGLYSLSSVVTVPSSSLGTQTYICNVNHKPSNTKVDKKVEPKSCGGGGSGGGGSGGGGSGGGGSGGGGSQAVVTQEPSLTVSPGGTVTLTCRSSTGAVTTSNYANWVQQKPGQAPRGLIGGTNKRAPWTPARFSGSLLGGKAALTITGAQAEDEADYYCALWYSNLWVFGGGTKLTVLGGGGSDKTHTCPPCPAPEAAGPSVFLFPPKPKDTLMISRTPEVTCVVVDVSHEDPEVKFNWYVDGVEVHNAKTKPREEQYNSTYRVVSVLTVLHQDWLNGKEYKCKVSNKALPAPIEKTISKAKGQPREPQVYTLPPSREEMTKNQVSLSCAVKGFYPSDIAVEWESNGQPENNYKTTPPVLDSDGSFFLVSKLTVDKSRWQQGNVFSCSVMHEALHNRFTQKSLSLSPGGGGGSGGGGSGGGGSGGGGSDIQMTQSPSSLSASVGDRVTITCRASQDIRSNLNWYQQKPGGAVKLLIYYTSRLHSGVPSRFSGSGSGTDYTLTISSLQPEDFATYFCQQSEKLPRTFGGGTKVEIR

SEQ ID NO: 400 - protein, 710 aa, synthetic construct
QVQLVQSGAEVKKPGASVKVSCKASGYTFTSYVMHWVRQKPGQGLEWIGYINPYNEGTESTDKFKGRATMTSDKSTSTVYMELSSLRSEDTAVYYCASIYYGYEGTYFGVWGQGTLVTVSSASTKGPSVFPLAPSSKSTSGGTAALGCLVKDYFPEPVTVSWNSGALTSGVHTFPAVLQSSGLYSLSSVVTVPSSSLGTQTYICNVNHKPSNTKVDKKVEPKSCGGGGSGGGGSGGGGSGGGGSQAVVTQEPSLTVSPGGTVTLTCRSSTGAVTTSNYANWVQQKPGQAPRGLIGGTNKRAPWTPARFSGSLLGGKAALTITGAQAEDEADYYCALWYSNLWVFGGGTKLTVLGGGGSDKTHTCPPCPAPEAAGPSVFLFPPKPKDTLMISRTPEVTCVVVDVSHEDPEVKFNWYVDGVEVHNAKTKPREEQYNSTYRVVSVLTVLHQDWLNGKEYKCKVSNKALPAPIEKTISKAKGQPREPQVYTLPPSREEMTKNQVSLSCAVKGFYPSDIAVEWESNGQPENNYKTTPPVLDSDGSFFLVSKLTVDKSRWQQGNVFSCSVMHEALHNRFTQKSLSLSPGGGGGSGGGGSGGGGSGGGGSDIQMTQSPSSLSASVGDRVTITCHASQNIYVWLNWYQQKPGKAPKLLIYKASNLHTGVPSRFSGSGSGTDFTLTISSLQPEDFATYYCQQGQTYPYTFGGGTKVEIK

SEQ ID NO: 401 - protein, 710 aa, synthetic construct
QVQLVQSGAEVKKPGASVKVSCKASGYTFTSYVMHWVRQKPGQGLEWIGYINPYNEGTESTDKFKGRATMTSDKSTSTVYMELSSLRSEDTAVYYCASIYYGYEGTYFGVWGQGTLVTVSSASTKGPSVFPLAPSSKSTSGGTAALGCLVKDYFPEPVTVSWNSGALTSGVHTFPAVLQSSGLYSLSSVVTVPSSSLGTQTYICNVNHKPSNTKVDKKVEPKSCGGGGSGGGGSGGGGSGGGGSQAVVTQEPSLTVSPGGTVTLTCRSSTGAVTTSNYANWVQQKPGQAPRGLIGGTNKRAPWTPARFSGSLLGGKAALTITGAQAEDEADYYCALWYSNLWVFGGGTKLTVLGGGGSDKTHTCPPCPAPEAAGPSVFLFPPKPKDTLMISRTPEVTCVVVDVSHEDPEVKFNWYVDGVEVHNAKTKPREEQYNSTYRVVSVLTVLHQDWLNGKEYKCKVSNKALPAPIEKTISKAKGQPREPQVYTLPPSREEMTKNQVSLSCAVKGFYPSDIAVEWESNGQPENNYKTTPPVLDSDGSFFLVSKLTVDKSRWQQGNVFSCSVMHEALHNRFTQKSLSLSPGGGGGSGGGGSGGGGSGGGGSDIQMTQSPSSLSASVGDRVTITCQASQNIYVWLNWYQQKPGKAPKLLIYKASNLHTGVPSRFSGSGSGTDFTLTISSLQPEDIATYYCQQGQTYPYTFGQGTKLEIK

SEQ ID NO: 402 - protein, 711 aa, synthetic construct
QVQLVQSGAEVKKPGASVKVSCKASGYTFTSYVMHWVRQKPGQGLEWIGYINPYNEGTESTDKFKGRATMTSDKSTSTVYMELSSLRSEDTAVYYCASIYYGYEGTYFGVWGQGTLVTVSSASTKGPSVFPLAPSSKSTSGGTAALGCLVKDYFPEPVTVSWNSGALTSGVHTFPAVLQSSGLYSLSSVVTVPSSSLGTQTYICNVNHKPSNTKVDKKVEPKSCGGGGSGGGGSGGGGSGGGGSQAVVTQEPSLTVSPGGTVTLTCRSSTGAVTTSNYANWVQQKPGQAPRGLIGGTNKRAPWTPARFSGSLLGGKAALTITGAQAEDEADYYCALWYSNLWVFGGGTKLTVLGGGGSDKTHTCPPCPAPEAAGPSVFLFPPKPKDTLMISRTPEVTCVVVDVSHEDPEVKFNWYVDGVEVHNAKTKPREEQYNSTYRVVSVLTVLHQDWLNGKEYKCKVSNKALPAPIEKTISKAKGQPREPQVYTLPPSREEMTKNQVSLSCAVKGFYPSDIAVEWESNGQPENNYKTTPPVLDSDGSFFLVSKLTVDKSRWQQGNVFSCSVMHEALHNRFTQKSLSLSPGGGGGSGGGGSGGGGSGGGGSEIVLTQSPGTLSLSPGERATLSCRASQSVSSSYLAWYQQKPGQAPRLLIYGASSRATGIPDRFSGSGSGTDFTLTISRLEPEDFAVYYCQQYGSSPWTFGQGTKVEIK

SEQ ID NO: 403 - protein, 705 aa, synthetic construct
QVQLVQSGAEVKKPGASVKVSCKASGYTFTSYVMHWVRQKPGQGLEWIGYINPYNEGTESTDKFKGRATMTSDKSTSTVYMELSSLRSEDTAVYYCASIYYGYEGTYFGVWGQGTLVTVSSASTKGPSVFPLAPSSKSTSGGTAALGCLVKDYFPEPVTVSWNSGALTSGVHTFPAVLQSSGLYSLSSVVTVPSSSLGTQTYICNVNHKPSNTKVDKKVEPKSCGGGGSGGGGSGGGGSGGGGSQAVVTQEPSLTVSPGGTVTLTCRSSTGAVTTSNYANWVQQKPGQAPRGLIGGTNKRAPWTPARFSGSLLGGKAALTITGAQAEDEADYYCALWYSNLWVFGGGTKLTVLDKTHTCPPCPAPEAAGPSVFLFPPKPKDTLMISRTPEVTCVVVDVSHEDPEVKFNWYVDGVEVHNAKTKPREEQYNSTYRVVSVLTVLHQDWLNGKEYKCKVSNKALPAPIEKTISKAKGQPREPQVYTLPPSREEMTKNQVSLSCAVKGFYPSDIAVEWESNGQPENNYKTTPPVLDSDGSFFLVSKLTVDKSRWQQGNVFSCSVMHEALHNRFTQKSLSLSPGGGGGSGGGGSGGGGSGGGGSDIQMTQSPSSLSASVGDRVTITCHASQNIYVWLNWYQQKPGKAPKLLIYKASNLHTGVPSRFSGSGSGTDFTLTISSLQPEDFATYYCQQGQTYPYTFGGGTKVEIK

SEQ ID NO: 404 - protein, 708 aa, synthetic construct
QVQLVQSGAEVKKPGASVKVSCKASGYTFTSYVMHWVRQKPGQGLEWIGYINPYNEGTESTDKFKGRATMTSDKSTSTVYMELSSLRSEDTAVYYCASIYYGYEGTYFGVWGQGTLVTVSSASTKGPSVFPLAPSSKSTSGGTAALGCLVKDYFPEPVTVSWNSGALTSGVHTFPAVLQSSGLYSLSSVVTVPSSSLGTQTYICNVNHKPSNTKVDKKVEPKSCGGGGSGGGGSGGGGSGGGGSQAVVTQEPSLTVSPGGTVTLTCRSSTGAVTTSNYANWVQQKPGQAPRGLIGGTNKRAPWTPARFSGSLLGGKAALTITGAQAEDEADYYCALWYSNLWVFGGGTKLTVLGGSDKTHTCPPCPAPEAAGPSVFLFPPKPKDTLMISRTPEVTCVVVDVSHEDPEVKFNWYVDGVEVHNAKTKPREEQYNSTYRVVSVLTVLHQDWLNGKEYKCKVSNKALPAPIEKTISKAKGQPREPQVYTLPPSREEMTKNQVSLSCAVKGFYPSDIAVEWESNGQPENNYKTTPPVLDSDGSFFLVSKLTVDKSRWQQGNVFSCSVMHEALHNRFTQKSLSLSPGGGGGSGGGGSGGGGSGGGGSDIQMTQSPSSLSASVGDRVTITCHASQNIYVWLNWYQQKPGKAPKLLIYKASNLHTGVPSRFSGSGSGTDFTLTISSLQPEDFATYYCQQGQTYPYTFGGGTKVEIK

SEQ ID NO: 405 - protein, 709 aa, synthetic construct
QVQLVQSGAEVKKPGASVKVSCKASGYTFTSYVMHWVRQKPGQGLEWIGYINPYNEGTESTDKFKGRATMTSDKSTSTVYMELSSLRSEDTAVYYCASIYYGYEGTYFGVWGQGTLVTVSSASTKGPSVFPLAPSSKSTSGGTAALGCLVKDYFPEPVTVSWNSGALTSGVHTFPAVLQSSGLYSLSSVVTVPSSSLGTQTYICNVNHKPSNTKVDKKVEPKSCGGGGSGGGGSGGGGSGGGGSQAVVTQEPSLTVSPGGTVTLTCRSSTGAVTTSNYANWVQQKPGQAPRGLIGGTNKRAPWTPARFSGSLLGGKAALTITGAQAEDEADYYCALWYSNLWVFGGGTKLTVLGGGSDKTHTCPPCPAPEAAGPSVFLFPPKPKDTLMISRTPEVTCVVVDVSHEDPEVKFNWYVDGVEVHNAKTKPREEQYNSTYRVVSVLTVLHQDWLNGKEYKCKVSNKALPAPIEKTISKAKGQPREPQVYTLPPSREEMTKNQVSLSCAVKGFYPSDIAVEWESNGQPENNYKTTPPVLDSDGSFFLVSKLTVDKSRWQQGNVFSCSVMHEALHNRFTQKSLSLSPGGGGGSGGGGSGGGGSGGGGSDIQMTQSPSSLSASVGDRVTITCHASQNIYVWLNWYQQKPGKAPKLLIYKASNLHTGVPSRFSGSGSGTDFTLTISSLQPEDFATYYCQQGQTYPYTFGGGTKVEIK

SEQ ID NO: 406 - protein, 713 aa, synthetic construct
QVQLVQSGAEVKKPGASVKVSCKASGYTFTSYVMHWVRQKPGQGLEWIGYINPYNEGTESTDKFKGRATMTSDKSTSTVYMELSSLRSEDTAVYYCASIYYGYEGTYFGVWGQGTLVTVSSASTKGPSVFPLAPSSKSTSGGTAALGCLVKDYFPEPVTVSWNSGALTSGVHTFPAVLQSSGLYSLSSVVTVPSSSLGTQTYICNVNHKPSNTKVDKKVEPKSCGGGGSGGGGSGGGGSGGGGSQAVVTQEPSLTVSPGGTVTLTCRSSTGAVTTSNYANWVQQKPGQAPRGLIGGTNKRAPWTPARFSGSLLGGKAALTITGAQAEDEADYYCALWYSNLWVFGGGTKLTVLGGGSGGGSDKTHTCPPCPAPEAAGPSVFLFPPKPKDTLMISRTPEVTCVVVDVSHEDPEVKFNWYVDGVEVHNAKTKPREEQYNSTYRVVSVLTVLHQDWLNGKEYKCKVSNKALPAPIEKTISKAKGQPREPQVYTLPPSREEMTKNQVSLSCAVKGFYPSDIAVEWESNGQPENNYKTTPPVLDSDGSFFLVSKLTVDKSRWQQGNVFSCSVMHEALHNRFTQKSLSLSPGGGGGSGGGGSGGGGSGGGGSDIQMTQSPSSLSASVGDRVTITCHASQNIYVWLNWYQQKPGKAPKLLIYKASNLHTGVPSRFSGSGSGTDFTLTISSLQPEDFATYYCQQGQTYPYTFGGGTKVEIK

SEQ ID NO: 407 - protein, 715 aa, synthetic construct
QVQLVQSGAEVKKPGASVKVSCKASGYTFTSYVMHWVRQKPGQGLEWIGYINPYNEGTESTDKFKGRATMTSDKSTSTVYMELSSLRSEDTAVYYCASIYYGYEGTYFGVWGQGTLVTVSSASTKGPSVFPLAPSSKSTSGGTAALGCLVKDYFPEPVTVSWNSGALTSGVHTFPAVLQSSGLYSLSSVVTVPSSSLGTQTYICNVNHKPSNTKVDKKVEPKSCGGGGSGGGGSGGGGSGGGGSQAVVTQEPSLTVSPGGTVTLTCRSSTGAVTTSNYANWVQQKPGQAPRGLIGGTNKRAPWTPARFSGSLLGGKAALTITGAQAEDEADYYCALWYSNLWVFGGGTKLTVLGGGGSGGGGSDKTHTCPPCPAPEAAGPSVFLFPPKPKDTLMISRTPEVTCVVVDVSHEDPEVKFNWYVDGVEVHNAKTKPREEQYNSTYRVVSVLTVLHQDWLNGKEYKCKVSNKALPAPIEKTISKAKGQPREPQVYTLPPSREEMTKNQVSLSCAVKGFYPSDIAVEWESNGQPENNYKTTPPVLDSDGSFFLVSKLTVDKSRWQQGNVFSCSVMHEALHNRFTQKSLSLSPGGGGGSGGGGSGGGGSGGGGSDIQMTQSPSSLSASVGDRVTITCHASQNIYVWLNWYQQKPGKAPKLLIYKASNLHTGVPSRFSGSGSGTDFTLTISSLQPEDFATYYCQQGQTYPYTFGGGTKVEIK

SEQ ID NO: 408 - protein, 720 aa, synthetic construct
QVQLVQSGAEVKKPGASVKVSCKASGYTFTSYVMHWVRQKPGQGLEWIGYINPYNEGTESTDKFKGRATMTSDKSTSTVYMELSSLRSEDTAVYYCASIYYGYEGTYFGVWGQGTLVTVSSASTKGPSVFPLAPSSKSTSGGTAALGCLVKDYFPEPVTVSWNSGALTSGVHTFPAVLQSSGLYSLSSVVTVPSSSLGTQTYICNVNHKPSNTKVDKKVEPKSCGGGGSGGGGSGGGGSGGGGSQAVVTQEPSLTVSPGGTVTLTCRSSTGAVTTSNYANWVQQKPGQAPRGLIGGTNKRAPWTPARFSGSLLGGKAALTITGAQAEDEADYYCALWYSNLWVFGGGTKLTVLGGGGSGGGGSGGGGSDKTHTCPPCPAPEAAGPSVFLFPPKPKDTLMISRTPEVTCVVVDVSHEDPEVKFNWYVDGVEVHNAKTKPREEQYNSTYRVVSVLTVLHQDWLNGKEYKCKVSNKALPAPIEKTISKAKGQPREPQVYTLPPSREEMTKNQVSLSCAVKGFYPSDIAVEWESNGQPENNYKTTPPVLDSDGSFFLVSKLTVDKSRWQQGNVFSCSVMHEALHNRFTQKSLSLSPGGGGGSGGGGSGGGGSGGGGSDIQMTQSPSSLSASVGDRVTITCHASQNIYVWLNWYQQKPGKAPKLLIYKASNLHTGVPSRFSGSGSGTDFTLTISSLQPEDFATYYCQQGQTYPYTFGGGTKVEIK

SEQ ID NO: 409 - protein, 705 aa, synthetic construct
QVQLVQSGAEVKKPGASVKVSCKASGYTFTSYVMHWVRQKPGQGLEWIGYINPYNEGTESTDKFKGRATMTSDKSTSTVYMELSSLRSEDTAVYYCASIYYGYEGTYFGVWGQGTLVTVSSASTKGPSVFPLAPSSKSTSGGTAALGCLVKDYFPEPVTVSWNSGALTSGVHTFPAVLQSSGLYSLSSVVTVPSSSLGTQTYICNVNHKPSNTKVDKKVEPKSCGGGGSGGGGSGGGGSGGGGSQAVVTQEPSLTVSPGGTVTLTCRSSTGAVTTSNYANWVQQKPGQAPRGLIGGTNKRAPWTPARFSGSLLGGKAALTITGAQAEDEADYYCALWYSNLWVFGGGTKLTVLGGGGSDKTHTCPPCPAPEAAGPSVFLFPPKPKDTLMISRTPEVTCVVVDVSHEDPEVKFNWYVDGVEVHNAKTKPREEQYNSTYRVVSVLTVLHQDWLNGKEYKCKVSNKALPAPIEKTISKAKGQPREPQVYTLPPSREEMTKNQVSLSCAVKGFYPSDIAVEWESNGQPENNYKTTPPVLDSDGSFFLVSKLTVDKSRWQQGNVFSCSVMHEALHNRFTQKSLSLSPGGGGGSGGGGSGGGGSDIQMTQSPSSLSASVGDRVTITCHASQNIYVWLNWYQQKPGKAPKLLIYKASNLHTGVPSRFSGSGSGTDFTLTISSLQPEDFATYYCQQGQTYPYTFGGGTKVEIK

SEQ ID NO: 410 - protein, 700 aa, synthetic construct
QVQLVQSGAEVKKPGASVKVSCKASGYTFTSYVMHWVRQKPGQGLEWIGYINPYNEGTESTDKFKGRATMTSDKSTSTVYMELSSLRSEDTAVYYCASIYYGYEGTYFGVWGQGTLVTVSSASTKGPSVFPLAPSSKSTSGGTAALGCLVKDYFPEPVTVSWNSGALTSGVHTFPAVLQSSGLYSLSSVVTVPSSSLGTQTYICNVNHKPSNTKVDKKVEPKSCGGGGSGGGGSGGGGSGGGGSQAVVTQEPSLTVSPGGTVTLTCRSSTGAVTTSNYANWVQQKPGQAPRGLIGGTNKRAPWTPARFSGSLLGGKAALTITGAQAEDEADYYCALWYSNLWVFGGGTKLTVLGGGGSDKTHTCPPCPAPEAAGPSVFLFPPKPKDTLMISRTPEVTCVVVDVSHEDPEVKFNWYVDGVEVHNAKTKPREEQYNSTYRVVSVLTVLHQDWLNGKEYKCKVSNKALPAPIEKTISKAKGQPREPQVYTLPPSREEMTKNQVSLSCAVKGFYPSDIAVEWESNGQPENNYKTTPPVLDSDGSFFLVSKLTVDKSRWQQGNVFSCSVMHEALHNRFTQKSLSLSPGGGGGSGGGGSDIQMTQSPSSLSASVGDRVTITCHASQNIYVWLNWYQQKPGKAPKLLIYKASNLHTGVPSRFSGSGSGTDFTLTISSLQPEDFATYYCQQGQTYPYTFGGGTKVEIK

SEQ ID NO: 411 - protein, 695 aa, synthetic construct
QVQLVQSGAEVKKPGASVKVSCKASGYTFTSYVMHWVRQKPGQGLEWIGYINPYNEGTESTDKFKGRATMTSDKSTSTVYMELSSLRSEDTAVYYCASIYYGYEGTYFGVWGQGTLVTVSSASTKGPSVFPLAPSSKSTSGGTAALGCLVKDYFPEPVTVSWNSGALTSGVHTFPAVLQSSGLYSLSSVVTVPSSSLGTQTYICNVNHKPSNTKVDKKVEPKSCGGGGSGGGGSGGGGSGGGGSQAVVTQEPSLTVSPGGTVTLTCRSSTGAVTTSNYANWVQQKPGQAPRGLIGGTNKRAPWTPARFSGSLLGGKAALTITGAQAEDEADYYCALWYSNLWVFGGGTKLTVLGGGGSDKTHTCPPCPAPEAAGPSVFLFPPKPKDTLMISRTPEVTCVVVDVSHEDPEVKFNWYVDGVEVHNAKTKPREEQYNSTYRVVSVLTVLHQDWLNGKEYKCKVSNKALPAPIEKTISKAKGQPREPQVYTLPPSREEMTKNQVSLSCAVKGFYPSDIAVEWESNGQPENNYKTTPPVLDSDGSFFLVSKLTVDKSRWQQGNVFSCSVMHEALHNRFTQKSLSLSPGGGGGSDIQMTQSPSSLSASVGDRVTITCHASQNIYVWLNWYQQKPGKAPKLLIYKASNLHTGVPSRFSGSGSGTDFTLTISSLQPEDFATYYCQQGQTYPYTFGGGTKVEIK

SEQ ID NO: 412 - protein, 715 aa, synthetic construct
QVQLVQSGAEVKKPGASVKVSCKASGYTFTSYVMHWVRQKPGQGLEWIGYINPYNEGTESTDKFKGRATMTSDKSTSTVYMELSSLRSEDTAVYYCASIYYGYEGTYFGVWGQGTLVTVSSASTKGPSVFPLAPSSKSTSGGTAALGCLVKDYFPEPVTVSWNSGALTSGVHTFPAVLQSSGLYSLSSVVTVPSSSLGTQTYICNVNHKPSNTKVDKKVEPKSCGGGGSGGGGSGGGGSGGGGSQAVVTQEPSLTVSPGGTVTLTCRSSTGAVTTSNYANWVQQKPGQAPRGLIGGTNKRAPWTPARFSGSLLGGKAALTITGAQAEDEADYYCALWYSNLWVFGGGTKLTVLGGGGSDKTHTCPPCPAPEAAGPSVFLFPPKPKDTLMISRTPEVTCVVVDVSHEDPEVKFNWYVDGVEVHNAKTKPREEQYNSTYRVVSVLTVLHQDWLNGKEYKCKVSNKALPAPIEKTISKAKGQPREPQVYTLPPSREEMTKNQVSLSCAVKGFYPSDIAVEWESNGQPENNYKTTPPVLDSDGSFFLVSKLTVDKSRWQQGNVFSCSVMHEALHNRFTQKSLSLSPGDKTHTCPPCPGGGGSGGGGSGGGGSDIQMTQSPSSLSASVGDRVTITCHASQNIYVWLNWYQQKPGKAPKLLIYKASNLHTGVPSRFSGSGSGTDFTLTISSLQPEDFATYYCQQGQTYPYTFGGGTKVEIK

SEQ ID NO: 413 - protein, 832 aa, synthetic construct
QVQLVQSGAEVKKPGASVKVSCKASGYTFTSYVMHWVRQKPGQGLEWIGYINPYNEGTESTDKFKGRATMTSDKSTSTVYMELSSLRSEDTAVYYCASIYYGYEGTYFGVWGQGTLVTVSSASTKGPSVFPLAPSSKSTSGGTAALGCLVKDYFPEPVTVSWNSGALTSGVHTFPAVLQSSGLYSLSSVVTVPSSSLGTQTYICNVNHKPSNTKVDKKVEPKSCGGGGSGGGGSGGGGSGGGGSQAVVTQEPSLTVSPGGTVTLTCRSSTGAVTTSNYANWVQQKPGQAPRGLIGGTNKRAPWTPARFSGSLLGGKAALTITGAQAEDEADYYCALWYSNLWVFGGGTKLTVLPAPEAAGPSVFLFPPKPKDTLMISRTPEVTCVVVDVSHEDPEVKFNWYVDGVEVHNAKTKPREEQYNSTYRVVSVLTVLHQDWLNGKEYKCKVSNKALPAPIEKTISKAKGQPREPQVYTLPPSREEMTKNQVSLSCAVKGFYPSDIAVEWESNGQPENNYKTTPPVLDSDGSFFLVSKLTVDKSRWQQGNVFSCSVMHEALHNRFTQKSLSLSPGGGGGSGGGGSGGGGSGGGGSQVQLVQSGAEVKKPGASVKVSCKASGYTFAGFEMHWVRQAPGQGLEWMGAIDPKTGGTDYNQKFKDRVTMTRDTSISTAYMELSRLRSDDTAVYYCARDLGYFDVWGQGTLVTVSSGGGGSGGGGSGGGGSGGGGSDIQMTQSPSSLSASVGDRVTITCRASQDIRSNLNWYQQKPGGAVKLLIYYTSRLHSGVPSRFSGSGSGTDYTLTISSLQPEDFATYFCQQSEKLPRTFGGGTKVEIR

SEQ ID NO: 414 - protein, 846 aa, synthetic construct
QVQLVQSGAEVKKPGASVKVSCKASGYTFTSYVMHWVRQKPGQGLEWIGYINPYNEGTESTDKFKGRATMTSDKSTSTVYMELSSLRSEDTAVYYCASIYYGYEGTYFGVWGQGTLVTVSSASTKGPSVFPLAPSSKSTSGGTAALGCLVKDYFPEPVTVSWNSGALTSGVHTFPAVLQSSGLYSLSSVVTVPSSSLGTQTYICNVNHKPSNTKVDKKVEPKSCGGGGSGGGGSGGGGSGGGGSQAVVTQEPSLTVSPGGTVTLTCRSSTGAVTTSNYANWVQQKPGQAPRGLIGGTNKRAPWTPARFSGSLLGGKAALTITGAQAEDEADYYCALWYSNLWVFGGGTKLTVLGGGGSDKTHTCPPCPAPEAAGPSVFLFPPKPKDTLMISRTPEVTCVVVDVSHEDPEVKFNWYVDGVEVHNAKTKPREEQYNSTYRVVSVLTVLHQDWLNGKEYKCKVSNKALPAPIEKTISKAKGQPREPQVYTLPPSREEMTKNQVSLSCAVKGFYPSDIAVEWESNGQPENNYKTTPPVLDSDGSFFLVSKLTVDKSRWQQGNVFSCSVMHEALHNRFTQKSLSLSPGGGGGSGGGGSGGGGSGGGGSQVQLVQSGAEVKKPGASVKVSCKASGYTFAGFEMHWVRQAPGQGLEWMGAIDPKTGGTDYNQKFKDRVTMTRDTSISTAYMELSRLRSDDTAVYYCARDLGYFDVWGQGTLVTVSSGGGGSGGGGSGGGGSGGGGSDIQMTQSPSSLSASVGDRVTITCRASQDIRSNLNWYQQKPGGAVKLLIYYTSRLHSGVPSRFSGSGSGTDYTLTISSLQPEDFATYFCQQSEKLPRTFGGGTKVEIR

SEQ ID NO: 415 - protein, 696 aa, synthetic construct
QVQLVQSGAEVKKPGASVKVSCKASGYTFTSYVMHWVRQKPGQGLEWIGYINPYNEGTESTDKFKGRATMTSDKSTSTVYMELSSLRSEDTAVYYCASIYYGYEGTYFGVWGQGTLVTVSSASTKGPSVFPLAPSSKSTSGGTAALGCLVKDYFPEPVTVSWNSGALTSGVHTFPAVLQSSGLYSLSSVVTVPSSSLGTQTYICNVNHKPSNTKVDKKVEPKSCGGGGSGGGGSGGGGSGGGGSQAVVTQEPSLTVSPGGTVTLTCRSSTGAVTTSNYANWVQQKPGQAPRGLIGGTNKRAPWTPARFSGSLLGGKAALTITGAQAEDEADYYCALWYSNLWVFGGGTKLTVLPAPEAAGPSVFLFPPKPKDTLMISRTPEVTCVVVDVSHEDPEVKFNWYVDGVEVHNAKTKPREEQYNSTYRVVSVLTVLHQDWLNGKEYKCKVSNKALPAPIEKTISKAKGQPREPQVYTLPPSREEMTKNQVSLSCAVKGFYPSDIAVEWESNGQPENNYKTTPPVLDSDGSFFLVSKLTVDKSRWQQGNVFSCSVMHEALHNRFTQKSLSLSPGGGGGSGGGGSGGGGSGGGGSDIQMTQSPSSLSASVGDRVTITCRASQDIRSNLNWYQQKPGGAVKLLIYYTSRLHSGVPSRFSGSGSGTDYTLTISSLQPEDFATYFCQQSEKLPRTFGGGTKVEIR

SEQ ID NO: 416 - protein, 710 aa, synthetic construct
QVQLVQSGAEVKKPGASVKVSCKASGYTFTSYVMHWVRQKPGQGLEWIGYINPYNEGTESTDKFKGRATMTSDKSTSTVYMELSSLRSEDTAVYYCASIYYGYEGTYFGVWGQGTLVTVSSASTKGPSVFPLAPSSKSTSGGTAALGCLVKDYFPEPVTVSWNSGALTSGVHTFPAVLQSSGLYSLSSVVTVPSSSLGTQTYICNVNHKPSNTKVDKKVEPKSCGGGGSGGGGSGGGGSGGGGSQAVVTQEPSLTVSPGGTVTLTCRSSTGAVTTSNYANWVQQKPGQAPRGLIGGTNKRAPWTPARFSGSLLGGKAALTITGAQAEDEADYYCALWYSNLWVFGGGTKLTVLGGGGSDKTHTCPPCPAPEAAGPSVFLFPPKPKDTLMISRTPEVTCVVVDVSHEDPEVKFNWYVDGVEVHNAKTKPREEQYNSTYRVVSVLTVLHQDWLNGKEYKCKVSNKALPAPIEKTISKAKGQPREPQVYTLPPSREEMTKNQVSLSCAVKGFYPSDIAVEWESNGQPENNYKTTPPVLDSDGSFFLVSKLTVDKSRWQQGNVFSCSVMHEALHNRFTQKSLSLSPGGGGGSGGGGSGGGGSGGGGSDIQMTQSPSSLSASVGDRVTITCRASQDIRSNLNWYQQKPGGAVKLLIYYTSRLHSGVPSRFSGSGSGTDYTLTISSLQPEDFATYFCQQSEKLPRTFGGGTKVEIR

SEQ ID NO: 417 - protein, 696 aa, synthetic construct
QVQLVQSGAEVKKPGASVKVSCKASGYTFTSYVMHWVRQKPGQGLEWIGYINPYNEGTESTDKFKGRATMTSDKSTSTVYMELSSLRSEDTAVYYCASIYYGYEGTYFGVWGQGTLVTVSSASTKGPSVFPLAPSSKSTSGGTAALGCLVKDYFPEPVTVSWNSGALTSGVHTFPAVLQSSGLYSLSSVVTVPSSSLGTQTYICNVNHKPSNTKVDKKVEPKSCGGGGSGGGGSGGGGSGGGGSQAVVTQEPSLTVSPGGTVTLTCRSSTGAVTTSNYANWVQQKPGQAPRGLIGGTNKRAPWTPARFSGSLLGGKAALTITGAQAEDEADYYCALWYSNLWVFGGGTKLTVLPAPEAAGPSVFLFPPKPKDTLMISRTPEVTCVVVDVSHEDPEVKFNWYVDGVEVHNAKTKPREEQYNSTYRVVSVLTVLHQDWLNGKEYKCKVSNKALPAPIEKTISKAKGQPREPQVYTLPPSREEMTKNQVSLSCAVKGFYPSDIAVEWESNGQPENNYKTTPPVLDSDGSFFLVSKLTVDKSRWQQGNVFSCSVMHEALHNHYTQKSLSLSPGGGGGSGGGGSGGGGSGGGGSDIQMTQSPSSLSASVGDRVTITCRASQDIRSNLNWYQQKPGGAVKLLIYYTSRLHSGVPSRFSGSGSGTDYTLTISSLQPEDFATYFCQQSEKLPRTFGGGTKVEIR

SEQ ID NO: 418 - protein, 710 aa, synthetic construct
QVQLVQSGAEVKKPGASVKVSCKASGYTFTSYVMHWVRQKPGQGLEWIGYINPYNEGTESTDKFKGRATMTSDKSTSTVYMELSSLRSEDTAVYYCASIYYGYEGTYFGVWGQGTLVTVSSASTKGPSVFPLAPSSKSTSGGTAALGCLVKDYFPEPVTVSWNSGALTSGVHTFPAVLQSSGLYSLSSVVTVPSSSLGTQTYICNVNHKPSNTKVDKKVEPKSCGGGGSGGGGSGGGGSGGGGSQAVVTQEPSLTVSPGGTVTLTCRSSTGAVTTSNYANWVQQKPGQAPRGLIGGTNKRAPWTPARFSGSLLGGKAALTITGAQAEDEADYYCALWYSNLWVFGGGTKLTVLGGGGSDKTHTCPPCPAPEAAGPSVFLFPPKPKDTLMISRTPEVTCVVVDVSHEDPEVKFNWYVDGVEVHNAKTKPREEQYNSTYRVVSVLTVLHQDWLNGKEYKCKVSNKALPAPIEKTISKAKGQPREPQVYTLPPSREEMTKNQVSLSCAVKGFYPSDIAVEWESNGQPENNYKTTPPVLDSDGSFFLVSKLTVDKSRWQQGNVFSCSVMHEALHNHYTQKSLSLSPGGGGGSGGGGSGGGGSGGGGSDIQMTQSPSSLSASVGDRVTITCRASQDIRSNLNWYQQKPGGAVKLLIYYTSRLHSGVPSRFSGSGSGTDYTLTISSLQPEDFATYFCQQSEKLPRTFGGGTKVEIR

SEQ ID NO: 419 - protein, 710 aa, synthetic construct
QVQLVQSGAEVKKPGASVKVSCKASGYTFTSYVMHWVRQKPGQGLEWIGYINPYNEGTESTDKFKGRATMTSDKSTSTVYMELSSLRSEDTAVYYCASIYYGYEGTYFGVWGQGTLVTVSSASTKGPSVFPLAPSSKSTSGGTAALGCLVKDYFPEPVTVSWNSGALTSGVHTFPAVLQSSGLYSLSSVVTVPSSSLGTQTYICNVNHKPSNTKVDKKVEPKSCGGGGSGGGGSGGGGSGGGGSQAVVTQEPSLTVSPGGTVTLTCRSSTGAVTTSNYANWVQQKPGQAPRGLIGGTNKRAPWTPARFSGSLLGGKAALTITGAQAEDEADYYCALWYSNLWVFGGGTKLTVLGGGGSDKTHTCPPCPAPELLGPSVFLFPPKPKDTLMISRTPEVTCVVVAVSHEDPEVKFNWYVDGVEVHNAKTKPREEQYASTYRVVSVLTVLHQDWLNGKEYKCKVSNKALPAPIEKTISKAKGQPREPQVYTLPPSREEMTKNQVSLSCAVKGFYPSDIAVEWESNGQPENNYKTTPPVLDSDGSFFLVSKLTVDKSRWQQGNVFSCSVMHEALHNHYTQKSLSLSPGGGGGSGGGGSGGGGSGGGGSDIQMTQSPSSLSASVGDRVTITCRASQDIRSNLNWYQQKPGGAVKLLIYYTSRLHSGVPSRFSGSGSGTDYTLTISSLQPEDFATYFCQQSEKLPRTFGGGTKVEIR

SEQ ID NO: 420 - protein, 712 aa, synthetic construct
QVQLVQSGAEVKKPGASVKVSCKASGYTFTSYVMHWVRQKPGQGLEWIGYINPYNEGTESTDKFKGRATMTSDKSTSTVYMELSSLRSEDTAVYYCASIYYGYEGTYFGVWGQGTLVTVSSASTKGPSVFPLAPSSKSTSGGTAALGCLVKDYFPEPVTVSWNSGALTSGVHTFPAVLQSSGLYSLSSVVTVPSSSLGTQTYICNVNHKPSNTKVDKKVEPKSCGGGGSGGGGSGGGGSGGGGSQAVVTQEPSLTVSPGGTVTLTCRSSTGAVTTSNYANWVQQKPGQAPRGLIGGTNKRAPWTPARFSGSLLGGKAALTITGAQAEDEADYYCALWYSNLWVFGGGTKLTVLGGGGSDKTHTCPPCPAPEAAGGPSVFLFPPKPKDTLMISRTPEVTCVVVDVSHEDPEVKFNWYVDGVEVHNAKTKPREEQYNSTYRVVSVLTVLHQDWLNGKEYKCKVSNKALGAPIEKTISKAKGQPREPQVYTLPPSREEMTKNQVSLSCAVKGFYPSDIAVEWESNGQPENNYKTTPPVLDSDGSFFLVSKLTVDKSRWQQGNVFSCSVMHEALHNHYTQKSLSLSPGKGGGGSGGGGSGGGGSGGGGSDIQMTQSPSSLSASVGDRVTITCRASQDIRSNLNWYQQKPGGAVKLLIYYTSRLHSGVPSRFSGSGSGTDYTLTISSLQPEDFATYFCQQSEKLPRTFGGGTKVEIR

SEQ ID NO: 421 - protein, 711 aa, synthetic construct
QVQLVQSGAEVKKPGASVKVSCKASGYTFTSYVMHWVRQKPGQGLEWIGYINPYNEGTESTDKFKGRATMTSDKSTSTVYMELSSLRSEDTAVYYCASIYYGYEGTYFGVWGQGTLVTVSSASTKGPSVFPLAPSSKSTSGGTAALGCLVKDYFPEPVTVSWNSGALTSGVHTFPAVLQSSGLYSLSSVVTVPSSSLGTQTYICNVNHKPSNTKVDKKVEPKSCGGGGSGGGGSGGGGSGGGGSQAVVTQEPSLTVSPGGTVTLTCRSSTGAVTTSNYANWVQQKPGQAPRGLIGGTNKRAPWTPARFSGSLLGGKAALTITGAQAEDEADYYCALWYSNLWVFGGGTKLTVLGGGGSDKTHTCPPCPAPEAAGPSVFLFPPKPKDTLMISRTPEVTCVVVDVSHEDPEVKFNWYVDGVEVHNAKTKPREEQYNSTYRVVSVLTVLHQDWLNGKEYKCKVSNKALGAPIEKTISKAKGQPREPQVYTLPPSREEMTKNQVSLSCAVKGFYPSDIAVEWESNGQPENNYKTTPPVLDSDGSFFLVSKLTVDKSRWQQGNVFSCSVMHEALHNHYTQKSLSLSPGKGGGGSGGGGSGGGGSGGGGSDIQMTQSPSSLSASVGDRVTITCRASQDIRSNLNWYQQKPGGAVKLLIYYTSRLHSGVPSRFSGSGSGTDYTLTISSLQPEDFATYFCQQSEKLPRTFGGGTKVEIR

SEQ ID NO: 422 - protein, 710 aa, synthetic construct
QVQLVQSGAEVKKPGASVKVSCKASGYTFTSYVMHWVRQKPGQGLEWIGYINPYNEGTESTDKFKGRATMTSDKSTSTVYMELSSLRSEDTAVYYCASIYYGYEGTYFGVWGQGTLVTVSSASTKGPSVFPLAPSSKSTSGGTAALGCLVKDYFPEPVTVSWNSGALTSGVHTFPAVLQSSGLYSLSSVVTVPSSSLGTQTYICNVNHKPSNTKVDKKVEPKSCGGGGSGGGGSGGGGSGGGGSQAVVTQEPSLTVSPGGTVTLTCRSSTGAVTTSNYANWVQQKPGQAPRGLIGGTNKRAPWTPARFSGSLLGGKAALTITGAQAEDEADYYCALWYSNLWVFGGGTKLTVLGGGGSDKTHTCPPCPAPELLGPSVFLFPPKPKDTLMISRTPEVTCVVVDVSHEDPEVKFNWYVDGVEVHNAKTKPREEQYNSTYRVVSVLTVLHQDWLNGKEYKCKVSNKALGAPIEKTISKAKGQPREPQVYTLPPSREEMTKNQVSLSCAVKGFYPSDIAVEWESNGQPENNYKTTPPVLDSDGSFFLVSKLTVDKSRWQQGNVFSCSVMHEALHNHYTQKSLSLSPGGGGGSGGGGSGGGGSGGGGSDIQMTQSPSSLSASVGDRVTITCRASQDIRSNLNWYQQKPGGAVKLLIYYTSRLHSGVPSRFSGSGSGTDYTLTISSLQPEDFATYFCQQSEKLPRTFGGGTKVEIR

SEQ ID NO: 423 - protein, 583 aa, synthetic construct
QVQLVQSGAEVKKPGASVKVSCKASGYTFTSYVMHWVRQKPGQGLEWIGYINPYNEGTESTDKFKGRATMTSDKSTSTVYMELSSLRSEDTAVYYCASIYYGYEGTYFGVWGQGTLVTVSSASTKGPSVFPLAPSSKSTSGGTAALGCLVKDYFPEPVTVSWNSGALTSGVHTFPAVLQSSGLYSLSSVVTVPSSSLGTQTYICNVNHKPSNTKVDKKVEPKSCGGGGSGGGGSGGGGSGGGGSQAVVTQEPSLTVSPGGTVTLTCRSSTGAVTTSNYANWVQQKPGQAPRGLIGGTNKRAPWTPARFSGSLLGGKAALTITGAQAEDEADYYCALWYSNLWVFGGGTKLTVLGGGGSDKTHTCPPCPAPEAAGPSVFLFPPKPKDTLMISRTPEVTCVVVDVSHEDPEVKFNWYVDGVEVHNAKTKPREEQYNSTYRVVSVLTVLHQDWLNGKEYKCKVSNKALPAPIEKTISKAKGQPREPQVYTLPPSREEMTKNQVSLSCAVKGFYPSDIAVEWESNGQPENNYKTTPPVLDSDGSFFLVSKLTVDKSRWQQGNVFSCSVMHEALHNRFTQKSLSLSPG

SEQ ID NO: 424 - protein, 705 aa, synthetic construct
QVQLVQSGAEVKKPGASVKVSCKASGYTFTSYVMHWVRQKPGQGLEWIGYINPYNEGTESTDKFKGRATMTSDKSTSTVYMELSSLRSEDTAVYYCASIYYGYEGTYFGVWGQGTLVTVSSASTKGPSVFPLAPSSKSTSGGTAALGCLVKDYFPEPVTVSWNSGALTSGVHTFPAVLQSSGLYSLSSVVTVPSSSLGTQTYICNVNHKPSNTKVDKKVEPKSCGGGGSGGGGSGGGGSGGGGSQAVVTQEPSLTVSPGGTVTLTCRSSTGAVTTSNYANWVQQKPGQAPRGLIGGTNKRAPWTPARFSGSLLGGKAALTITGAQAEDEADYYCALWYSNLWVFGGGTKLTVLDKTHTCPPCPAPEAAGPSVFLFPPKPKDTLMISRTPEVTCVVVDVSHEDPEVKFNWYVDGVEVHNAKTKPREEQYNSTYRVVSVLTVLHQDWLNGKEYKCKVSNKALPAPIEKTISKAKGQPREPQVYTLPPSREEMTKNQVSLSCAVKGFYPSDIAVEWESNGQPENNYKTTPPVLDSDGSFFLVSKLTVDKSRWQQGNVFSCSVMHEALHNRFTQKSLSLSPGGGGGSGGGGSGGGGSGGGGSDIQMTQSPSSLSASVGDRVTITCRASQDIRSNLNWYQQKPGGAVKLLIYYTSRLHSGVPSRFSGSGSGTDYTLTISSLQPEDFATYFCQQSEKLPRTFGGGTKVEIR

SEQ ID NO: 425 - protein, 708 aa, synthetic construct
QVQLVQSGAEVKKPGASVKVSCKASGYTFTSYVMHWVRQKPGQGLEWIGYINPYNEGTESTDKFKGRATMTSDKSTSTVYMELSSLRSEDTAVYYCASIYYGYEGTYFGVWGQGTLVTVSSASTKGPSVFPLAPSSKSTSGGTAALGCLVKDYFPEPVTVSWNSGALTSGVHTFPAVLQSSGLYSLSSVVTVPSSSLGTQTYICNVNHKPSNTKVDKKVEPKSCGGGGSGGGGSGGGGSGGGGSQAVVTQEPSLTVSPGGTVTLTCRSSTGAVTTSNYANWVQQKPGQAPRGLIGGTNKRAPWTPARFSGSLLGGKAALTITGAQAEDEADYYCALWYSNLWVFGGGTKLTVLGGSDKTHTCPPCPAPEAAGPSVFLFPPKPKDTLMISRTPEVTCVVVDVSHEDPEVKFNWYVDGVEVHNAKTKPREEQYNSTYRVVSVLTVLHQDWLNGKEYKCKVSNKALPAPIEKTISKAKGQPREPQVYTLPPSREEMTKNQVSLSCAVKGFYPSDIAVEWESNGQPENNYKTTPPVLDSDGSFFLVSKLTVDKSRWQQGNVFSCSVMHEALHNRFTQKSLSLSPGGGGGSGGGGSGGGGSGGGGSDIQMTQSPSSLSASVGDRVTITCRASQDIRSNLNWYQQKPGGAVKLLIYYTSRLHSGVPSRFSGSGSGTDYTLTISSLQPEDFATYFCQQSEKLPRTFGGGTKVEIR

SEQ ID NO: 426 - protein, 709 aa, synthetic construct
QVQLVQSGAEVKKPGASVKVSCKASGYTFTSYVMHWVRQKPGQGLEWIGYINPYNEGTESTDKFKGRATMTSDKSTSTVYMELSSLRSEDTAVYYCASIYYGYEGTYFGVWGQGTLVTVSSASTKGPSVFPLAPSSKSTSGGTAALGCLVKDYFPEPVTVSWNSGALTSGVHTFPAVLQSSGLYSLSSVVTVPSSSLGTQTYICNVNHKPSNTKVDKKVEPKSCGGGGSGGGGSGGGGSGGGGSQAVVTQEPSLTVSPGGTVTLTCRSSTGAVTTSNYANWVQQKPGQAPRGLIGGTNKRAPWTPARFSGSLLGGKAALTITGAQAEDEADYYCALWYSNLWVFGGGTKLTVLGGGSDKTHTCPPCPAPEAAGPSVFLFPPKPKDTLMISRTPEVTCVVVDVSHEDPEVKFNWYVDGVEVHNAKTKPREEQYNSTYRVVSVLTVLHQDWLNGKEYKCKVSNKALPAPIEKTISKAKGQPREPQVYTLPPSREEMTKNQVSLSCAVKGFYPSDIAVEWESNGQPENNYKTTPPVLDSDGSFFLVSKLTVDKSRWQQGNVFSCSVMHEALHNRFTQKSLSLSPGGGGGSGGGGSGGGGSGGGGSDIQMTQSPSSLSASVGDRVTITCRASQDIRSNLNWYQQKPGGAVKLLIYYTSRLHSGVPSRFSGSGSGTDYTLTISSLQPEDFATYFCQQSEKLPRTFGGGTKVEIR

SEQ ID NO: 427 - protein, 713 aa, synthetic construct
QVQLVQSGAEVKKPGASVKVSCKASGYTFTSYVMHWVRQKPGQGLEWIGYINPYNEGTESTDKFKGRATMTSDKSTSTVYMELSSLRSEDTAVYYCASIYYGYEGTYFGVWGQGTLVTVSSASTKGPSVFPLAPSSKSTSGGTAALGCLVKDYFPEPVTVSWNSGALTSGVHTFPAVLQSSGLYSLSSVVTVPSSSLGTQTYICNVNHKPSNTKVDKKVEPKSCGGGGSGGGGSGGGGSGGGGSQAVVTQEPSLTVSPGGTVTLTCRSSTGAVTTSNYANWVQQKPGQAPRGLIGGTNKRAPWTPARFSGSLLGGKAALTITGAQAEDEADYYCALWYSNLWVFGGGTKLTVLGGGSGGGSDKTHTCPPCPAPEAAGPSVFLFPPKPKDTLMISRTPEVTCVVVDVSHEDPEVKFNWYVDGVEVHNAKTKPREEQYNSTYRVVSVLTVLHQDWLNGKEYKCKVSNKALPAPIEKTISKAKGQPREPQVYTLPPSREEMTKNQVSLSCAVKGFYPSDIAVEWESNGQPENNYKTTPPVLDSDGSFFLVSKLTVDKSRWQQGNVFSCSVMHEALHNRFTQKSLSLSPGGGGGSGGGGSGGGGSGGGGSDIQMTQSPSSLSASVGDRVTITCRASQDIRSNLNWYQQKPGGAVKLLIYYTSRLHSGVPSRFSGSGSGTDYTLTISSLQPEDFATYFCQQSEKLPRTFGGGTKVEIR

SEQ ID NO: 428 - protein, 715 aa, synthetic construct
QVQLVQSGAEVKKPGASVKVSCKASGYTFTSYVMHWVRQKPGQGLEWIGYINPYNEGTESTDKFKGRATMTSDKSTSTVYMELSSLRSEDTAVYYCASIYYGYEGTYFGVWGQGTLVTVSSASTKGPSVFPLAPSSKSTSGGTAALGCLVKDYFPEPVTVSWNSGALTSGVHTFPAVLQSSGLYSLSSVVTVPSSSLGTQTYICNVNHKPSNTKVDKKVEPKSCGGGGSGGGGSGGGGSGGGGSQAVVTQEPSLTVSPGGTVTLTCRSSTGAVTTSNYANWVQQKPGQAPRGLIGGTNKRAPWTPARFSGSLLGGKAALTITGAQAEDEADYYCALWYSNLWVFGGGTKLTVLGGGGSGGGGSDKTHTCPPCPAPEAAGPSVFLFPPKPKDTLMISRTPEVTCVVVDVSHEDPEVKFNWYVDGVEVHNAKTKPREEQYNSTYRVVSVLTVLHQDWLNGKEYKCKVSNKALPAPIEKTISKAKGQPREPQVYTLPPSREEMTKNQVSLSCAVKGFYPSDIAVEWESNGQPENNYKTTPPVLDSDGSFFLVSKLTVDKSRWQQGNVFSCSVMHEALHNRFTQKSLSLSPGGGGGSGGGGSGGGGSGGGGSDIQMTQSPSSLSASVGDRVTITCRASQDIRSNLNWYQQKPGGAVKLLIYYTSRLHSGVPSRFSGSGSGTDYTLTISSLQPEDFATYFCQQSEKLPRTFGGGTKVEIR

SEQ ID NO: 429 - protein, 720 aa, synthetic construct
QVQLVQSGAEVKKPGASVKVSCKASGYTFTSYVMHWVRQKPGQGLEWIGYINPYNEGTESTDKFKGRATMTSDKSTSTVYMELSSLRSEDTAVYYCASIYYGYEGTYFGVWGQGTLVTVSSASTKGPSVFPLAPSSKSTSGGTAALGCLVKDYFPEPVTVSWNSGALTSGVHTFPAVLQSSGLYSLSSVVTVPSSSLGTQTYICNVNHKPSNTKVDKKVEPKSCGGGGSGGGGSGGGGSGGGGSQAVVTQEPSLTVSPGGTVTLTCRSSTGAVTTSNYANWVQQKPGQAPRGLIGGTNKRAPWTPARFSGSLLGGKAALTITGAQAEDEADYYCALWYSNLWVFGGGTKLTVLGGGGSGGGGSGGGGSDKTHTCPPCPAPEAAGPSVFLFPPKPKDTLMISRTPEVTCVVVDVSHEDPEVKFNWYVDGVEVHNAKTKPREEQYNSTYRVVSVLTVLHQDWLNGKEYKCKVSNKALPAPIEKTISKAKGQPREPQVYTLPPSREEMTKNQVSLSCAVKGFYPSDIAVEWESNGQPENNYKTTPPVLDSDGSFFLVSKLTVDKSRWQQGNVFSCSVMHEALHNRFTQKSLSLSPGGGGGSGGGGSGGGGSGGGGSDIQMTQSPSSLSASVGDRVTITCRASQDIRSNLNWYQQKPGGAVKLLIYYTSRLHSGVPSRFSGSGSGTDYTLTISSLQPEDFATYFCQQSEKLPRTFGGGTKVEIR

SEQ ID NO: 430 - protein, 705 aa, synthetic construct
QVQLVQSGAEVKKPGASVKVSCKASGYTFTSYVMHWVRQKPGQGLEWIGYINPYNEGTESTDKFKGRATMTSDKSTSTVYMELSSLRSEDTAVYYCASIYYGYEGTYFGVWGQGTLVTVSSASTKGPSVFPLAPSSKSTSGGTAALGCLVKDYFPEPVTVSWNSGALTSGVHTFPAVLQSSGLYSLSSVVTVPSSSLGTQTYICNVNHKPSNTKVDKKVEPKSCGGGGSGGGGSGGGGSGGGGSQAVVTQEPSLTVSPGGTVTLTCRSSTGAVTTSNYANWVQQKPGQAPRGLIGGTNKRAPWTPARFSGSLLGGKAALTITGAQAEDEADYYCALWYSNLWVFGGGTKLTVLGGGGSDKTHTCPPCPAPEAAGPSVFLFPPKPKDTLMISRTPEVTCVVVDVSHEDPEVKFNWYVDGVEVHNAKTKPREEQYNSTYRVVSVLTVLHQDWLNGKEYKCKVSNKALPAPIEKTISKAKGQPREPQVYTLPPSREEMTKNQVSLSCAVKGFYPSDIAVEWESNGQPENNYKTTPPVLDSDGSFFLVSKLTVDKSRWQQGNVFSCSVMHEALHNRFTQKSLSLSPGGGGGSGGGGSGGGGSDIQMTQSPSSLSASVGDRVTITCRASQDIRSNLNWYQQKPGGAVKLLIYYTSRLHSGVPSRFSGSGSGTDYTLTISSLQPEDFATYFCQQSEKLPRTFGGGTKVEIR

SEQ ID NO: 431 - protein, 700 aa, synthetic construct
QVQLVQSGAEVKKPGASVKVSCKASGYTFTSYVMHWVRQKPGQGLEWIGYINPYNEGTESTDKFKGRATMTSDKSTSTVYMELSSLRSEDTAVYYCASIYYGYEGTYFGVWGQGTLVTVSSASTKGPSVFPLAPSSKSTSGGTAALGCLVKDYFPEPVTVSWNSGALTSGVHTFPAVLQSSGLYSLSSVVTVPSSSLGTQTYICNVNHKPSNTKVDKKVEPKSCGGGGSGGGGSGGGGSGGGGSQAVVTQEPSLTVSPGGTVTLTCRSSTGAVTTSNYANWVQQKPGQAPRGLIGGTNKRAPWTPARFSGSLLGGKAALTITGAQAEDEADYYCALWYSNLWVFGGGTKLTVLGGGGSDKTHTCPPCPAPEAAGPSVFLFPPKPKDTLMISRTPEVTCVVVDVSHEDPEVKFNWYVDGVEVHNAKTKPREEQYNSTYRVVSVLTVLHQDWLNGKEYKCKVSNKALPAPIEKTISKAKGQPREPQVYTLPPSREEMTKNQVSLSCAVKGFYPSDIAVEWESNGQPENNYKTTPPVLDSDGSFFLVSKLTVDKSRWQQGNVFSCSVMHEALHNRFTQKSLSLSPGGGGGSGGGGSDIQMTQSPSSLSASVGDRVTITCRASQDIRSNLNWYQQKPGGAVKLLIYYTSRLHSGVPSRFSGSGSGTDYTLTISSLQPEDFATYFCQQSEKLPRTFGGGTKVEIR

SEQ ID NO: 432 - protein, 695 aa, synthetic construct
QVQLVQSGAEVKKPGASVKVSCKASGYTFTSYVMHWVRQKPGQGLEWIGYINPYNEGTESTDKFKGRATMTSDKSTSTVYMELSSLRSEDTAVYYCASIYYGYEGTYFGVWGQGTLVTVSSASTKGPSVFPLAPSSKSTSGGTAALGCLVKDYFPEPVTVSWNSGALTSGVHTFPAVLQSSGLYSLSSVVTVPSSSLGTQTYICNVNHKPSNTKVDKKVEPKSCGGGGSGGGGSGGGGSGGGGSQAVVTQEPSLTVSPGGTVTLTCRSSTGAVTTSNYANWVQQKPGQAPRGLIGGTNKRAPWTPARFSGSLLGGKAALTITGAQAEDEADYYCALWYSNLWVFGGGTKLTVLGGGGSDKTHTCPPCPAPEAAGPSVFLFPPKPKDTLMISRTPEVTCVVVDVSHEDPEVKFNWYVDGVEVHNAKTKPREEQYNSTYRVVSVLTVLHQDWLNGKEYKCKVSNKALPAPIEKTISKAKGQPREPQVYTLPPSREEMTKNQVSLSCAVKGFYPSDIAVEWESNGQPENNYKTTPPVLDSDGSFFLVSKLTVDKSRWQQGNVFSCSVMHEALHNRFTQKSLSLSPGGGGGSDIQMTQSPSSLSASVGDRVTITCRASQDIRSNLNWYQQKPGGAVKLLIYYTSRLHSGVPSRFSGSGSGTDYTLTISSLQPEDFATYFCQQSEKLPRTFGGGTKVEIR

SEQ ID NO: 433 - protein, 714 aa, synthetic construct
QVQLVQSGAEVKKPGASVKVSCKASGYTFTSYVMHWVRQKPGQGLEWIGYINPYNEGTESTDKFKGRATMTSDKSTSTVYMELSSLRSEDTAVYYCASIYYGYEGTYFGVWGQGTLVTVSSASTKGPSVFPLAPSSKSTSGGTAALGCLVKDYFPEPVTVSWNSGALTSGVHTFPAVLQSSGLYSLSSVVTVPSSSLGTQTYICNVNHKPSNTKVDKKVEPKSCGGGGSGGGGSGGGGSGGGGSQAVVTQEPSLTVSPGGTVTLTCRSSTGAVTTSNYANWVQQKPGQAPRGLIGGTNKRAPWTPARFSGSLLGGKAALTITGAQAEDEADYYCALWYSNLWVFGGGTKLTVLGGGGSDKTHTCPPCPAPEAAGPSVFLFPPKPKDTLMISRTPEVTCVVVDVSHEDPEVKFNWYVDGVEVHNAKTKPREEQYNSTYRVVSVLTVLHQDWLNGKEYKCKVSNKALPAPIEKTISKAKGQPREPQVYTLPPSREEMTKNQVSLSCAVKGFYPSDIAVEWESNGQPENNYKTTPPVLDSDGSFFLVSKLTVDKSRWQQGNVFSCSVMHEALHNRFTQKSLSLSPGDKTHTCPPCGGGGSGGGGSGGGGSDIQMTQSPSSLSASVGDRVTITCRASQDIRSNLNWYQQKPGGAVKLLIYYTSRLHSGVPSRFSGSGSGTDYTLTISSLQPEDFATYFCQQSEKLPRTFGGGTKVEIR

SEQ ID NO: 434 - protein, 719 aa, synthetic construct
QVQLVQSGAEVKKPGASVKVSCKASGYTFTSYVMHWVRQKPGQGLEWIGYINPYNEGTESTDKFKGRATMTSDKSTSTVYMELSSLRSEDTAVYYCASIYYGYEGTYFGVWGQGTLVTVSSASTKGPSVFPLAPSSKSTSGGTAALGCLVKDYFPEPVTVSWNSGALTSGVHTFPAVLQSSGLYSLSSVVTVPSSSLGTQTYICNVNHKPSNTKVDKKVEPKSCGGGGSGGGGSGGGGSGGGGSQAVVTQEPSLTVSPGGTVTLTCRSSTGAVTTSNYANWVQQKPGQAPRGLIGGTNKRAPWTPARFSGSLLGGKAALTITGAQAEDEADYYCALWYSNLWVFGGGTKLTVLGGGGSDKTHTCPPCPAPEAAGPSVFLFPPKPKDTLMISRTPEVTCVVVDVSHEDPEVKFNWYVDGVEVHNAKTKPREEQYNSTYRVVSVLTVLHQDWLNGKEYKCKVSNKALPAPIEKTISKAKGQPREPQVYTLPPSREEMTKNQVSLSCAVKGFYPSDIAVEWESNGQPENNYKTTPPVLDSDGSFFLVSKLTVDKSRWQQGNVFSCSVMHEALHNRFTQKSLSLSPGDKTHTCPPCGGGGSGGGGSGGGGSGGGGSDIQMTQSPSSLSASVGDRVTITCRASQDIRSNLNWYQQKPGGAVKLLIYYTSRLHSGVPSRFSGSGSGTDYTLTISSLQPEDFATYFCQQSEKLPRTFGGGTKVEIR

SEQ ID NO: 435 - protein, 709 aa, synthetic construct
QVQLVQSGAEVKKPGASVKVSCKASGYTFTSYVMHWVRQKPGQGLEWIGYINPYNEGTESTDKFKGRATMTSDKSTSTVYMELSSLRSEDTAVYYCASIYYGYEGTYFGVWGQGTLVTVSSASTKGPSVFPLAPSSKSTSGGTAALGCLVKDYFPEPVTVSWNSGALTSGVHTFPAVLQSSGLYSLSSVVTVPSSSLGTQTYICNVNHKPSNTKVDKKVEPKSCGGGGSGGGGSGGGGSGGGGSQAVVTQEPSLTVSPGGTVTLTCRSSTGAVTTSNYANWVQQKPGQAPRGLIGGTNKRAPWTPARFSGSLLGGKAALTITGAQAEDEADYYCALWYSNLWVFGGGTKLTVLGGGGSDKTHTCPPCPAPEAAGPSVFLFPPKPKDTLMISRTPEVTCVVVDVSHEDPEVKFNWYVDGVEVHNAKTKPREEQYNSTYRVVSVLTVLHQDWLNGKEYKCKVSNKALPAPIEKTISKAKGQPREPQVYTLPPSREEMTKNQVSLSCAVKGFYPSDIAVEWESNGQPENNYKTTPPVLDSDGSFFLVSKLTVDKSRWQQGNVFSCSVMHEALHNRFTQKSLSLSPGDKTHTCPPCGGGGSGGGGSDIQMTQSPSSLSASVGDRVTITCRASQDIRSNLNWYQQKPGGAVKLLIYYTSRLHSGVPSRFSGSGSGTDYTLTISSLQPEDFATYFCQQSEKLPRTFGGGTKVEIR

SEQ ID NO: 436 - protein, 704 aa, synthetic construct
QVQLVQSGAEVKKPGASVKVSCKASGYTFTSYVMHWVRQKPGQGLEWIGYINPYNEGTESTDKFKGRATMTSDKSTSTVYMELSSLRSEDTAVYYCASIYYGYEGTYFGVWGQGTLVTVSSASTKGPSVFPLAPSSKSTSGGTAALGCLVKDYFPEPVTVSWNSGALTSGVHTFPAVLQSSGLYSLSSVVTVPSSSLGTQTYICNVNHKPSNTKVDKKVEPKSCGGGGSGGGGSGGGGSGGGGSQAVVTQEPSLTVSPGGTVTLTCRSSTGAVTTSNYANWVQQKPGQAPRGLIGGTNKRAPWTPARFSGSLLGGKAALTITGAQAEDEADYYCALWYSNLWVFGGGTKLTVLGGGGSDKTHTCPPCPAPEAAGPSVFLFPPKPKDTLMISRTPEVTCVVVDVSHEDPEVKFNWYVDGVEVHNAKTKPREEQYNSTYRVVSVLTVLHQDWLNGKEYKCKVSNKALPAPIEKTISKAKGQPREPQVYTLPPSREEMTKNQVSLSCAVKGFYPSDIAVEWESNGQPENNYKTTPPVLDSDGSFFLVSKLTVDKSRWQQGNVFSCSVMHEALHNRFTQKSLSLSPGDKTHTCPPCGGGGSDIQMTQSPSSLSASVGDRVTITCRASQDIRSNLNWYQQKPGGAVKLLIYYTSRLHSGVPSRFSGSGSGTDYTLTISSLQPEDFATYFCQQSEKLPRTFGGGTKVEIR

SEQ ID NO: 437 - protein, 699 aa, synthetic construct
QVQLVQSGAEVKKPGASVKVSCKASGYTFTSYVMHWVRQKPGQGLEWIGYINPYNEGTESTDKFKGRATMTSDKSTSTVYMELSSLRSEDTAVYYCASIYYGYEGTYFGVWGQGTLVTVSSASTKGPSVFPLAPSSKSTSGGTAALGCLVKDYFPEPVTVSWNSGALTSGVHTFPAVLQSSGLYSLSSVVTVPSSSLGTQTYICNVNHKPSNTKVDKKVEPKSCGGGGSGGGGSGGGGSGGGGSQAVVTQEPSLTVSPGGTVTLTCRSSTGAVTTSNYANWVQQKPGQAPRGLIGGTNKRAPWTPARFSGSLLGGKAALTITGAQAEDEADYYCALWYSNLWVFGGGTKLTVLGGGGSDKTHTCPPCPAPEAAGPSVFLFPPKPKDTLMISRTPEVTCVVVDVSHEDPEVKFNWYVDGVEVHNAKTKPREEQYNSTYRVVSVLTVLHQDWLNGKEYKCKVSNKALPAPIEKTISKAKGQPREPQVYTLPPSREEMTKNQVSLSCAVKGFYPSDIAVEWESNGQPENNYKTTPPVLDSDGSFFLVSKLTVDKSRWQQGNVFSCSVMHEALHNRFTQKSLSLSPGDKTHTCPPCDIQMTQSPSSLSASVGDRVTITCRASQDIRSNLNWYQQKPGGAVKLLIYYTSRLHSGVPSRFSGSGSGTDYTLTISSLQPEDFATYFCQQSEKLPRTFGGGTKVEIR

SEQ ID NO: 438 - protein, 690 aa, synthetic construct
QVQLVQSGAEVKKPGASVKVSCKASGYTFTSYVMHWVRQKPGQGLEWIGYINPYNEGTESTDKFKGRATMTSDKSTSTVYMELSSLRSEDTAVYYCASIYYGYEGTYFGVWGQGTLVTVSSASTKGPSVFPLAPSSKSTSGGTAALGCLVKDYFPEPVTVSWNSGALTSGVHTFPAVLQSSGLYSLSSVVTVPSSSLGTQTYICNVNHKPSNTKVDKKVEPKSCGGGGSGGGGSGGGGSGGGGSQAVVTQEPSLTVSPGGTVTLTCRSSTGAVTTSNYANWVQQKPGQAPRGLIGGTNKRAPWTPARFSGSLLGGKAALTITGAQAEDEADYYCALWYSNLWVFGGGTKLTVLGGGGSDKTHTCPPCPAPEAAGPSVFLFPPKPKDTLMISRTPEVTCVVVDVSHEDPEVKFNWYVDGVEVHNAKTKPREEQYNSTYRVVSVLTVLHQDWLNGKEYKCKVSNKALPAPIEKTISKAKGQPREPQVYTLPPSREEMTKNQVSLSCAVKGFYPSDIAVEWESNGQPENNYKTTPPVLDSDGSFFLVSKLTVDKSRWQQGNVFSCSVMHEALHNRFTQKSLSLSPGDIQMTQSPSSLSASVGDRVTITCRASQDIRSNLNWYQQKPGGAVKLLIYYTSRLHSGVPSRFSGSGSGTDYTLTISSLQPEDFATYFCQQSEKLPRTFGGGTKVEIR

SEQ ID NO: 439 - protein, 711 aa, synthetic construct
QVQLVQSGAEVKKPGASVKVSCKASGYTFTSYVMHWVRQKPGQGLEWIGYINPYNEGTESTDKFKGRATMTSDKSTSTVYMELSSLRSEDTAVYYCASIYYGYEGTYFGVWGQGTLVTVSSASTKGPSVFPLAPSSKSTSGGTAALGCLVKDYFPEPVTVSWNSGALTSGVHTFPAVLQSSGLYSLSSVVTVPSSSLGTQTYICNVNHKPSNTKVDKKVEPKSCGGGGSGGGGSGGGGSGGGGSQAVVTQEPSLTVSPGGTVTLTCRSSTGAVTTSNYANWVQQKPGQAPRGLIGGTNKRAPWTPARFSGSLLGGKAALTITGAQAEDEADYYCALWYSNLWVFGGGTKLTVLGGGGSDKTHTCPPCPAPELLGPSVFLFPPKPKDTLMISRTPEVTCVVVDVSHEDPEVKFNWYVDGVEVHNAKTKPREEQYNSTYRVVSVLTVLHQDWLNGKEYKCKVSNKALGAPIEKTISKAKGQPREPQVYTLPPSREEMTKNQVSLSCAVKGFYPSDIAVEWESNGQPENNYKTTPPVLDSDGSFFLVSKLTVDKSRWQQGNVFSCSVMHEALHNRFTQKSLSLSPGKGGGGSGGGGSGGGGSGGGGSDIQMTQSPSSLSASVGDRVTITCRASQDIRSNLNWYQQKPGGAVKLLIYYTSRLHSGVPSRFSGSGSGTDYTLTISSLQPEDFATYFCQQSEKLPRTFGGGTKVEIR

SEQ ID NO: 440 - protein, 711 aa, synthetic construct
QVQLVQSGAEVKKPGASVKVSCKASGYTFTSYVMHWVRQKPGQGLEWIGYINPYNEGTESTDKFKGRATMTSDKSTSTVYMELSSLRSEDTAVYYCASIYYGYEGTYFGVWGQGTLVTVSSASTKGPSVFPLAPSSKSTSGGTAALGCLVKDYFPEPVTVSWNSGALTSGVHTFPAVLQSSGLYSLSSVVTVPSSSLGTQTYICNVNHKPSNTKVDKKVEPKSCGGGGSGGGGSGGGGSGGGGSQAVVTQEPSLTVSPGGTVTLTCRSSTGAVTTSNYANWVQQKPGQAPRGLIGGTNKRAPWTPARFSGSLLGGKAALTITGAQAEDEADYYCALWYSNLWVFGGGTKLTVLGGGGSDKTHTCPPCPAPELLGPSVFLFPPKPKDTLMISRTPEVTCVVVDVSHEDPEVKFNWYVDGVEVHNAKTKPREEQYNSTYRVVSVLTVLHQDWLNGKEYKCKVSNKALGAPIEKTISKAKGQPREPQVYTLPPSREEMTKNQVSLSCAVKGFYPSDIAVEWESNGQPENNYKTTPPVLDSDGSFFLVSKLTVDKSRWQQGNVFSCSVMHEALHNRFTQKSLSLSPGKGGGGSGGGGSGGGGSGGGGSDIQMTQSPSSLSASVGDRVTITCHASQNIYVWLNWYQQKPGKAPKLLIYKASNLHTGVPSRFSGSGSGTDFTLTISSLQPEDFATYYCQQGQTYPYTFGGGTKVEIK

SEQ ID NO: 441 - protein, 584 aa, synthetic construct
QVQLVQSGAEVKKPGASVKVSCKASGYTFTSYVMHWVRQKPGQGLEWIGYINPYNEGTESTDKFKGRATMTSDKSTSTVYMELSSLRSEDTAVYYCASIYYGYEGTYFGVWGQGTLVTVSSASTKGPSVFPLAPSSKSTSGGTAALGCLVKDYFPEPVTVSWNSGALTSGVHTFPAVLQSSGLYSLSSVVTVPSSSLGTQTYICNVNHKPSNTKVDKKVEPKSCGGGGSGGGGSGGGGSGGGGSQAVVTQEPSLTVSPGGTVTLTCRSSTGAVTTSNYANWVQQKPGQAPRGLIGGTNKRAPWTPARFSGSLLGGKAALTITGAQAEDEADYYCALWYSNLWVFGGGTKLTVLGGGGSDKTHTCPPCPAPELLGPSVFLFPPKPKDTLMISRTPEVTCVVVDVSHEDPEVKFNWYVDGVEVHNAKTKPREEQYNSTYRVVSVLTVLHQDWLNGKEYKCKVSNKALGAPIEKTISKAKGQPREPQVYTLPPSREEMTKNQVSLSCAVKGFYPSDIAVEWESNGQPENNYKTTPPVLDSDGSFFLVSKLTVDKSRWQQGNVFSCSVMHEALHNRFTQKSLSLSPGK

SEQ ID NO: 442 - protein, 712 aa, synthetic construct
QVQLVQSGAEVKKPGASVKVSCKASGYTFTSYVMHWVRQKPGQGLEWIGYINPYNEGTESTDKFKGRATMTSDKSTSTVYMELSSLRSEDTAVYYCASIYYGYEGTYFGVWGQGTLVTVSSASTKGPSVFPLAPSSKSTSGGTAALGCLVKDYFPEPVTVSWNSGALTSGVHTFPAVLQSSGLYSLSSVVTVPSSSLGTQTYICNVNHKPSNTKVDKKVEPKSCGGGGSGGGGSGGGGSGGGGSQAVVTQEPSLTVSPGGTVTLTCRSSTGAVTTSNYANWVQQKPGQAPRGLIGGTNKRAPWTPARFSGSLLGGKAALTITGAQAEDEADYYCALWYSNLWVFGGGTKLTVLGGGGSDKTHTCPPCPAPELLGPSVFLFPPKPKDTLMISRTPEVTCVVVDVSHEDPEVKFNWYVDGVEVHNAKTKPREEQYNSTYRVVSVLTVLHQDWLNGKEYKCKVSNKALGAPIEKTISKAKGQPREPQVYTLPPSREEMTKNQVSLSCAVKGFYPSDIAVEWESNGQPENNYKTTPPVLDSDGSFFLVSKLTVDKSRWQQGNVFSCSVMHEALHNRFTQKSLSLSPGKGGGGSGGGGSGGGGSGGGGSEIVLTQSPGTLSLSPGERATLSCRASQSVGSSYLAWYQQKPGQAPRLLIYGAFSRATGIPDRFSGSGSGTDFTLTISRLEPEDFAVYYCQQYGSSPWTFGQGTKVEIK

SEQ ID NO: 443 - protein, 711 aa, synthetic construct
QVQLVQSGAEVKKPGASVKVSCKASGYTFTSYVMHWVRQKPGQGLEWIGYINPYNEGTESTDKFKGRATMTSDKSTSTVYMELSSLRSEDTAVYYCASIYYGYEGTYFGVWGQGTLVTVSSASTKGPSVFPLAPSSKSTSGGTAALGCLVKDYFPEPVTVSWNSGALTSGVHTFPAVLQSSGLYSLSSVVTVPSSSLGTQTYICNVNHKPSNTKVDKKVEPKSCGGGGSGGGGSGGGGSGGGGSQAVVTQEPSLTVSPGGTVTLTCRSSTGAVTTSNYANWVQQKPGQAPRGLIGGTNKRAPWTPARFSGSLLGGKAALTITGAQAEDEADYYCALWYSNLWVFGGGTKLTVLGGGGSDKTHTCPPCPAPELLGPSVFLFPPKPKDTLMISRTPEVTCVVVDVSHEDPEVKFNWYVDGVEVHNAKTKPREEQYNSTYRVVSVLTVLHQDWLNGKEYKCKVSNKALGAPIEKTISKAKGQPREPQVYTLPPSREEMTKNQVSLSCAVKGFYPSDIAVEWESNGQPENNYKTTPPVLDSDGSFFLVSKLTVDKSRWQQGNVFSCSVMHEALHNRFTQKSLSLSPGKGGGGSGGGGSGGGGSGGGGSDIQMTQSPSSLSASVGDRVTITCRASQSINSYLDWYQQKPGKAPKLLIYAASSLQSGVPSRFSGSGSGTDFTLTISSLQPEDFATYYCQQYYSTPFTFGPGTKVEIK

SEQ ID NO: 444 - protein, 713 aa, synthetic construct
QVQLVQSGAEVKKPGASVKVSCKASGYTFTSYVMHWVRQKPGQGLEWIGYINPYNEGTESTDKFKGRATMTSDKSTSTVYMELSSLRSEDTAVYYCASIYYGYEGTYFGVWGQGTLVTVSSASTKGPSVFPLAPSSKSTSGGTAALGCLVKDYFPEPVTVSWNSGALTSGVHTFPAVLQSSGLYSLSSVVTVPSSSLGTQTYICNVNHKPSNTKVDKKVEPKSCGGGGSGGGGSGGGGSGGGGSQAVVTQEPSLTVSPGGTVTLTCRSSTGAVTTSNYANWVQQKPGQAPRGLIGGTNKRAPWTPARFSGSLLGGKAALTITGAQAEDEADYYCALWYSNLWVFGGGTKLTVLGGGGSDKTHTCPPCPAPELLGPSVFLFPPKPKDTLMISRTPEVTCVVVDVSHEDPEVKFNWYVDGVEVHNAKTKPREEQYNSTYRVVSVLTVLHQDWLNGKEYKCKVSNKALGAPIEKTISKAKGQPREPQVYTLPPSREEMTKNQVSLSCAVKGFYPSDIAVEWESNGQPENNYKTTPPVLDSDGSFFLVSKLTVDKSRWQQGNVFSCSVMHEALHNRFTQKSLSLSPGKGGGGSGGGGSGGGGSGGGGSQAVVTQEPSLTVSPGGTVTLTCGSSTGAVTTSNFPNWVQQKPGQAPRSLIGGTNNKASWTPARFSGSLLGGKAALTISGAQPEDEAEYYCALWYSNHWVFGCGTKLTVL

SEQ ID NO: 445 - protein, 710 aa, synthetic construct
QVQLVQSGAEVKKPGASVKVSCKASGYTFTSYVMHWVRQKPGQGLEWIGYINPYNEGTESTDKFKGRATMTSDKSTSTVYMELSSLRSEDTAVYYCASIYYGYEGTYFGVWGQGTLVTVSSASTKGPSVFPLAPSSKSTSGGTAALGCLVKDYFPEPVTVSWNSGALTSGVHTFPAVLQSSGLYSLSSVVTVPSSSLGTQTYICNVNHKPSNTKVDKKVEPKSCGGGGSGGGGSGGGGSGGGGSQAVVTQEPSLTVSPGGTVTLTCRSSTGAVTTSNYANWVQQKPGQAPRGLIGGTNKRAPWTPARFSGSLLGGKAALTITGAQAEDEADYYCALWYSNLWVFGGGTKLTVLGGGGSDKTHTCPPCPAPELLGPSVFLFPPKPKDTLMISRTPEVTCVVVDVSHEDPEVKFNWYVDGVEVHNAKTKPREEQYNSTYRVVSVLTVLHQDWLNGKEYKCKVSNKALGAPIEKTISKAKGQPREPQVYTLPPSREEMTKNQVSLSCAVKGFYPSDIAVEWESNGQPENNYKTTPPVLDSDGSFFLVSKLTVDKSRWQQGNVFSCSVMHEALHNRFTQKSLSLSPGKGGGGSGGGGSGGGGSGGGGSNIQMTQSPSSLSASVGDRVTITCKAGQNVNNYLAWYQQKPGKAPKVLIFNANSLQTGVPSRFSGSGSGTDFTLTISSLQPEDFATYYCQQYNSWPTFGGGTKVEIK

SEQ ID NO: 446 - protein, 710 aa, synthetic construct
QVQLVQSGAEVKKPGASVKVSCKASGYTFTSYVMHWVRQKPGQGLEWIGYINPYNEGTESTDKFKGRATMTSDKSTSTVYMELSSLRSEDTAVYYCASIYYGYEGTYFGVWGQGTLVTVSSASTKGPSVFPLAPSSKSTSGGTAALGCLVKDYFPEPVTVSWNSGALTSGVHTFPAVLQSSGLYSLSSVVTVPSSSLGTQTYICNVNHKPSNTKVDKKVEPKSCGGGGSGGGGSGGGGSGGGGSQAVVTQEPSLTVSPGGTVTLTCRSSTGAVTTSNYANWVQQKPGQAPRGLIGGTNKRAPWTPARFSGSLLGGKAALTITGAQAEDEADYYCALWYSNLWVFGGGTKLTVLGGGGSDKTHTCPPCPAPELLGPSVFLFPPKPKDTLMISRTPEVTCVVVDVSHEDPEVKFNWYVDGVEVHNAKTKPREEQYNSTYRVVSVLTVLHQDWLNGKEYKCKVSNKALGAPIEKTISKAKGQPREPQVYTLPPSREEMTKNQVSLSCAVKGFYPSDIAVEWESNGQPENNYKTTPPVLDSDGSFFLVSKLTVDKSRWQQGNVFSCSVMHEALHNRFTQKSLSLSPGKGGGGSGGGGSGGGGSGGGGSDIQMTQSPSSLSASVGDRVTITCKASQNVYKKLEWYQQKPGKVPKVLIYHTNILQTGVPSRFSGSGSGTDYTLTISSLQPEDVATYYCYQWNSGPTFGGGTKVEIK

SEQ ID NO: 447 - protein, 711 aa, synthetic construct
QVQLVQSGAEVKKPGASVKVSCKASGYTFTSYVMHWVRQKPGQGLEWIGYINPYNEGTESTDKFKGRATMTSDKSTSTVYMELSSLRSEDTAVYYCASIYYGYEGTYFGVWGQGTLVTVSSASTKGPSVFPLAPSSKSTSGGTAALGCLVKDYFPEPVTVSWNSGALTSGVHTFPAVLQSSGLYSLSSVVTVPSSSLGTQTYICNVNHKPSNTKVDKKVEPKSCGGGGSGGGGSGGGGSGGGGSQAVVTQEPSLTVSPGGTVTLTCRSSTGAVTTSNYANWVQQKPGQAPRGLIGGTNKRAPWTPARFSGSLLGGKAALTITGAQAEDEADYYCALWYSNLWVFGGGTKLTVLGGGGSDKTHTCPPCPAPELLGPSVFLFPPKPKDTLMISRTPEVTCVVVDVSHEDPEVKFNWYVDGVEVHNAKTKPREEQYNSTYRVVSVLTVLHQDWLNGKEYKCKVSNKALGAPIEKTISKAKGQPREPQVYTLPPSREEMTKNQVSLSCAVKGFYPSDIAVEWESNGQPENNYKTTPPVLDSDGSFFLVSKLTVDKSRWQQGNVFSCSVMHEALHNRFTQKSLSLSPGKGGGGSGGGGSGGGGSGGGGSDIQMTQSPSSLSASVGDRVTITCRASQDVSTAVAWYQQKPGKAPKLLIYSASFLYSGVPSRFSGSGSGTDFTLTISSLQPEDFATYYCQQYLYHPATFGQGTKVEIK

SEQ ID NO: 448 - protein, 708 aa, synthetic construct
QVQLVQSGAEVKKPGASVKVSCKASGYTFTSYVMHWVRQKPGQGLEWIGYINPYNEGTESTDKFKGRATMTSDKSTSTVYMELSSLRSEDTAVYYCASIYYGYEGTYFGVWGQGTLVTVSSASTKGPSVFPLAPSSKSTSGGTAALGCLVKDYFPEPVTVSWNSGALTSGVHTFPAVLQSSGLYSLSSVVTVPSSSLGTQTYICNVNHKPSNTKVDKKVEPKSCGGGGSGGGGSGGGGSGGGGSQIVLTQSPAIMSASPGEKVTMTCSASSSVSYMNWYQQKSGTSPKRWIYDTSKLASGVPAHFRGSGSGTSYSLTISGMEAEDAATYYCQQWSSNPFTFGSGTKLEINGGGGSDKTHTCPPCPAPELLGPSVFLFPPKPKDTLMISRTPEVTCVVVDVSHEDPEVKFNWYVDGVEVHNAKTKPREEQYNSTYRVVSVLTVLHQDWLNGKEYKCKVSNKALGAPIEKTISKAKGQPREPQVYTLPPSREEMTKNQVSLSCAVKGFYPSDIAVEWESNGQPENNYKTTPPVLDSDGSFFLVSKLTVDKSRWQQGNVFSCSVMHEALHNRFTQKSLSLSPGKGGGGSGGGGSGGGGSGGGGSDIQMTQSPSSLSASVGDRVTITCRASQDIRSNLNWYQQKPGGAVKLLIYYTSRLHSGVPSRFSGSGSGTDYTLTISSLQPEDFATYFCQQSEKLPRTFGGGTKVEIR

SEQ ID NO: 449 - protein, 730 aa, synthetic construct
QVQLVQSGAEVKKPGASVKVSCKASGYTFTSYVMHWVRQKPGQGLEWIGYINPYNEGTESTDKFKGRATMTSDKSTSTVYMELSSLRSEDTAVYYCASIYYGYEGTYFGVWGQGTLVTVSSASTKGPSVFPLAPSSKSTSGGTAALGCLVKDYFPEPVTVSWNSGALTSGVHTFPAVLQSSGLYSLSSVVTVPSSSLGTQTYICNVNHKPSNTKVDKKVEPKSCGGGGSGGGGSGGGGSGGGGSQVQLQQSGAELARPGASVKMSCKASGYTFTRYTMHWVKQRPGQGLEWIGYINPSRGYTNYNQKFKDKATLTTDKSSSTAYMQLSSLTSEDSAVYYCARYYDDHYCLDYWGQGTTLTVSSGGGGSDKTHTCPPCPAPELLGPSVFLFPPKPKDTLMISRTPEVTCVVVDVSHEDPEVKFNWYVDGVEVHNAKTKPREEQYNSTYRVVSVLTVLHQDWLNGKEYKCKVSNKALGAPIEKTISKAKGQPREPQVYTLPPSREEMTKNQVSLWCLVKGFYPSDIAVEWESNGQPENNYKTTPPVLDSDGSFFLYSKLTVDKSRWQQGNVFSCSVMHEALHNHYTQKSLSLSPGKGGGGSGGGGSGGGGSGGGGSQVQLVQSGAEVKKPGASVKVSCKASGYTFAGFEMHWVRQAPGQGLEWMGAIDPKTGGTDYNQKFKDRVTMTRDTSISTAYMELSRLRSDDTAVYYCARDLGYFDVWGQGTLVTVSS

SEQ ID NO: 450 - protein, 600 aa, synthetic construct
QVQLVQSGAEVKKPGASVKVSCKASGYTFTSYVMHWVRQKPGQGLEWIGYINPYNEGTESTDKFKGRATMTSDKSTSTVYMELSSLRSEDTAVYYCASIYYGYEGTYFGVWGQGTLVTVSSASTKGPSVFPLAPSSKSTSGGTAALGCLVKDYFPEPVTVSWNSGALTSGVHTFPAVLQSSGLYSLSSVVTVPSSSLGTQTYICNVNHKPSNTKVDKKVEPKSCGGGGSGGGGSGGGGSGGGGSQVQLVQSGAEVKKPGASVKVSCKASGYTFTGYYMHWVRQAPGQGLEWMGWINPDSGGTNYAQKFQGRVTMTRDTSISTAYMELNRLRSDDTAVYYCARDQPLGYCTNGVCSYFDYWGQGTLVTVSSGGGGSDKTHTCPPCPAPEAAGPSVFLFPPKPKDTLMISRTPEVTCVVVDVSHEDPEVKFNWYVDGVEVHNAKTKPREEQYNSTYRVVSVLTVLHQDWLNGKEYKCKVSNKALPAPIEKTISKAKGQPREPQVYTLPPSREEMTKNQVSLWCLVKGFYPSDIAVEWESNGQPENNYKTTPPVLDSDGSFFLYSKLTVDKSRWQQGNVFSCSVMHEALHNHYTQKSLSLSPG

SEQ ID NO: 451 - protein, 731 aa, synthetic construct
QVQLVQSGAEVKKPGASVKVSCKASGYTFTSYVMHWVRQKPGQGLEWIGYINPYNEGTESTDKFKGRATMTSDKSTSTVYMELSSLRSEDTAVYYCASIYYGYEGTYFGVWGQGTLVTVSSASTKGPSVFPLAPSSKSTSGGTAALGCLVKDYFPEPVTVSWNSGALTSGVHTFPAVLQSSGLYSLSSVVTVPSSSLGTQTYICNVNHKPSNTKVDKKVEPKSCGGGGSGGGGSGGGGSGGGGSQVQLVQSGAEVKKPGASVKVSCKASGYTFAGFEMHWVRQAPGQGLEWMGAIDPKTGGTDYNQKFKDRVTMTRDTSISTAYMELSRLRSDDTAVYYCARDLGYFDVWGQGTLVTVSSGGGGSDKTHTCPPCPAPEAAGPSVFLFPPKPKDTLMISRTPEVTCVVVDVSHEDPEVKFNWYVDGVEVHNAKTKPREEQYNSTYRVVSVLTVLHQDWLNGKEYKCKVSNKALPAPIEKTISKAKGQPREPQVYTLPPSREEMTKNQVSLWCLVKGFYPSDIAVEWESNGQPENNYKTTPPVLDSDGSFFLYSKLTVDKSRWQQGNVFSCSVMHEALHNHYTQKSLSLSPGGGGGSGGGGSGGGGSGGGGSQVTLKESGPALVKPTQTLTLTCTFSGFSLSTSGTCVSWIRQPPGKALEWLATICWEDSKGYNPSLKSRLTISKDTSKNQAVLTMTNMDPVDTATYYCARREDSGYFWFPYWGQGTLVTVSS

SEQ ID NO: 452 - protein, 741 aa, synthetic construct
QVQLVQSGAEVKKPGASVKVSCKASGYTFTSYVMHWVRQKPGQGLEWIGYINPYNEGTESTDKFKGRATMTSDKSTSTVYMELSSLRSEDTAVYYCASIYYGYEGTYFGVWGQGTLVTVSSASTKGPSVFPLAPSSKSTSGGTAALGCLVKDYFPEPVTVSWNSGALTSGVHTFPAVLQSSGLYSLSSVVTVPSSSLGTQTYICNVNHKPSNTKVDKKVEPKSCGGGGSGGGGSGGGGSGGGGSQVQLVQSGAEVKKPGASVKVSCKASGYTFTGYYMHWVRQAPGQGLEWMGWINPDSGGTNYAQKFQGRVTMTRDTSISTAYMELNRLRSDDTAVYYCARDQPLGYCTNGVCSYFDYWGQGTLVTVSSGGGGSDKTHTCPPCPAPEAAGPSVFLFPPKPKDTLMISRTPEVTCVVVDVSHEDPEVKFNWYVDGVEVHNAKTKPREEQYNSTYRVVSVLTVLHQDWLNGKEYKCKVSNKALPAPIEKTISKAKGQPREPQVYTLPPSREEMTKNQVSLWCLVKGFYPSDIAVEWESNGQPENNYKTTPPVLDSDGSFFLYSKLTVDKSRWQQGNVFSCSVMHEALHNHYTQKSLSLSPGGGGGSGGGGSGGGGSGGGGSQVTLKESGPALVKPTQTLTLTCTFSGFSLSTSGTCVSWIRQPPGKALEWLATICWEDSKGYNPSLKSRLTISKDTSKNQAVLTMTNMDPVDTATYYCARREDSGYFWFPYWGQGTLVTVSS

SEQ ID NO: 453 - protein, 736 aa, synthetic construct
QVQLVQSGAEVKKPGASVKVSCKASGYTFTSYVMHWVRQKPGQGLEWIGYINPYNEGTESTDKFKGRATMTSDKSTSTVYMELSSLRSEDTAVYYCASIYYGYEGTYFGVWGQGTLVTVSSASTKGPSVFPLAPSSKSTSGGTAALGCLVKDYFPEPVTVSWNSGALTSGVHTFPAVLQSSGLYSLSSVVTVPSSSLGTQTYICNVNHKPSNTKVDKKVEPKSCGGGGSGGGGSGGGGSGGGGSQVQLVQSGAEVKKPGASVKVSCKASGYTFTGYYMHWVRQAPGQGLEWMGWINPDSGGTNYAQKFQGRVTMTRDTSISTAYMELNRLRSDDTAVYYCARDQPLGYCTNGVCSYFDYWGQGTLVTVSSGGGGSDKTHTCPPCPAPEAAGPSVFLFPPKPKDTLMISRTPEVTCVVVDVSHEDPEVKFNWYVDGVEVHNAKTKPREEQYNSTYRVVSVLTVLHQDWLNGKEYKCKVSNKALPAPIEKTISKAKGQPREPQVYTLPPSREEMTKNQVSLWCLVKGFYPSDIAVEWESNGQPENNYKTTPPVLDSDGSFFLYSKLTVDKSRWQQGNVFSCSVMHEALHNHYTQKSLSLSPGGGGGSGGGGSGGGGSGGGGSQVQLVQSGAEVKKPGASVKVSCKASGYTFAGFEMHWVRQAPGQGLEWMGAIDPKTGGTDYNQKFKDRVTMTRDTSISTAYMELSRLRSDDTAVYYCARDLGYFDVWGQGTLVTVSS

SEQ ID NO: 454 - protein, 736 aa, synthetic construct
QVQLVQSGAEVKKPGASVKVSCKASGYTFTSYVMHWVRQKPGQGLEWIGYINPYNEGTESTDKFKGRATMTSDKSTSTVYMELSSLRSEDTAVYYCASIYYGYEGTYFGVWGQGTLVTVSSASTKGPSVFPLAPSSKSTSGGTAALGCLVKDYFPEPVTVSWNSGALTSGVHTFPAVLQSSGLYSLSSVVTVPSSSLGTQTYICNVNHKPSNTKVDKKVEPKSCGGGGSGGGGSGGGGSGGGGSQVQLVQSGAEVKKPGASVKVSCKASGYTFAGFEMHWVRQAPGQGLEWMGAIDPKTGGTDYNQKFKDRVTMTRDTSISTAYMELSRLRSDDTAVYYCARDLGYFDVWGQGTLVTVSSGGGGSDKTHTCPPCPAPEAAGPSVFLFPPKPKDTLMISRTPEVTCVVVDVSHEDPEVKFNWYVDGVEVHNAKTKPREEQYNSTYRVVSVLTVLHQDWLNGKEYKCKVSNKALPAPIEKTISKAKGQPREPQVYTLPPSREEMTKNQVSLWCLVKGFYPSDIAVEWESNGQPENNYKTTPPVLDSDGSFFLYSKLTVDKSRWQQGNVFSCSVMHEALHNHYTQKSLSLSPGGGGGSGGGGSGGGGSGGGGSQVQLVQSGAEVKKPGASVKVSCKASGYTFTGYYMHWVRQAPGQGLEWMGWINPDSGGTNYAQKFQGRVTMTRDTSISTAYMELNRLRSDDTAVYYCARDQPLGYCTNGVCSYFDYWGQGTLVTVSS

SEQ ID NO: 455 - protein, 732 aa, synthetic construct
QVQLVQSGAEVKKPGASVKVSCKASGYTFTSYVMHWVRQKPGQGLEWIGYINPYNEGTESTDKFKGRATMTSDKSTSTVYMELSSLRSEDTAVYYCASIYYGYEGTYFGVWGQGTLVTVSSASTKGPSVFPLAPSSKSTSGGTAALGCLVKDYFPEPVTVSWNSGALTSGVHTFPAVLQSSGLYSLSSVVTVPSSSLGTQTYICNVNHKPSNTKVDKKVEPKSCGGGGSGGGGSGGGGSGGGGSQVQLVQSGAEVKKPGASVKVSCKASGYTFAGFEMHWVRQAPGQGLEWMGAIDPKTGGTDYNQKFKDRVTMTRDTSISTAYMELSRLRSDDTAVYYCARDLGYFDVWGQGTLVTVSSGGGGSDKTHTCPPCPAPEAAGPSVFLFPPKPKDTLMISRTPEVTCVVVDVSHEDPEVKFNWYVDGVEVHNAKTKPREEQYNSTYRVVSVLTVLHQDWLNGKEYKCKVSNKALPAPIEKTISKAKGQPREPQVYTLPPSREEMTKNQVSLWCLVKGFYPSDIAVEWESNGQPENNYKTTPPVLDSDGSFFLYSKLTVDKSRWQQGNVFSCSVMHEALHNHYTQKSLSLSPGGGGGSGGGGSGGGGSGGGGSEVQLVESGGGLVQPGGSLRLSCAASGFTFTNYGLHWVRQAPGKGLEWVSSISPSGGVTYYRDSVKGRFTISRDNSKNTLYLQMNSLRAEDTAVYYCAKPFLGWGGANWIAHWGQGTLVTVSS

SEQ ID NO: 456 - protein, 705 aa, synthetic construct
QVQLVQSGAEVKKPGASVKVSCKASGYTFTSYVMHWVRQKPGQGLEWIGYINPYNEGTESTDKFKGRATMTSDKSTSTVYMELSSLRSEDTAVYYCASIYYGYEGTYFGVWGQGTLVTVSSASTKGPSVFPLAPSSKSTSGGTAALGCLVKDYFPEPVTVSWNSGALTSGVHTFPAVLQSSGLYSLSSVVTVPSSSLGTQTYICNVNHKPSNTKVDKKVEPKSCGGGGSGGGGSGGGGSQAVVTQEPSLTVSPGGTVTLTCRSSTGAVTTSNYANWVQQKPGQAPRGLIGGTNKRAPWTPARFSGSLLGGKAALTITGAQAEDEADYYCALWYSNLWVFGGGTKLTVLGGGGSDKTHTCPPCPAPEAAGPSVFLFPPKPKDTLMISRTPEVTCVVVDVSHEDPEVKFNWYVDGVEVHNAKTKPREEQYNSTYRVVSVLTVLHQDWLNGKEYKCKVSNKALPAPIEKTISKAKGQPREPQVYTLPPSREEMTKNQVSLSCAVKGFYPSDIAVEWESNGQPENNYKTTPPVLDSDGSFFLVSKLTVDKSRWQQGNVFSCSVMHEALHNRFTQKSLSLSPGGGGGSGGGGSGGGGSGGGGSDIQMTQSPSSLSASVGDRVTITCHASQNIYVWLNWYQQKPGKAPKLLIYKASNLHTGVPSRFSGSGSGTDFTLTISSLQPEDFATYYCQQGQTYPYTFGGGTKVEIK

SEQ ID NO: 457 - protein, 705 aa, synthetic construct
QVQLVQSGAEVKKPGASVKVSCKASGYTFTSYVMHWVRQKPGQGLEWIGYINPYNEGTESTDKFKGRATMTSDKSTSTVYMELSSLRSEDTAVYYCASIYYGYEGTYFGVWGQGTLVTVSSASTKGPSVFPLAPSSKSTSGGTAALGCLVKDYFPEPVTVSWNSGALTSGVHTFPAVLQSSGLYSLSSVVTVPSSSLGTQTYICNVNHKPSNTKVDKKVEPKSCGGGGSGGGGSGGGGSQAVVTQEPSLTVSPGGTVTLTCRSSTGAVTTSNYANWVQQKPGQAPRGLIGGTNKRAPWTPARFSGSLLGGKAALTITGAQAEDEADYYCALWYSNLWVFGGGTKLTVLGGGGSDKTHTCPPCPAPEAAGPSVFLFPPKPKDTLMISRTPEVTCVVVDVSHEDPEVKFNWYVDGVEVHNAKTKPREEQYNSTYRVVSVLTVLHQDWLNGKEYKCKVSNKALPAPIEKTISKAKGQPREPQVYTLPPSREEMTKNQVSLSCAVKGFYPSDIAVEWESNGQPENNYKTTPPVLDSDGSFFLVSKLTVDKSRWQQGNVFSCSVMHEALHNRFTQKSLSLSPGGGGGSGGGGSGGGGSGGGGSDIQMTQSPSSLSASVGDRVTITCRASQDIRSNLNWYQQKPGGAVKLLIYYTSRLHSGVPSRFSGSGSGTDYTLTISSLQPEDFATYFCQQSEKLPRTFGGGTKVEIR

SEQ ID NO: 458 - protein, 700 aa, synthetic construct
QVQLVQSGAEVKKPGASVKVSCKASGYTFTSYVMHWVRQKPGQGLEWIGYINPYNEGTESTDKFKGRATMTSDKSTSTVYMELSSLRSEDTAVYYCASIYYGYEGTYFGVWGQGTLVTVSSASTKGPSVFPLAPSSKSTSGGTAALGCLVKDYFPEPVTVSWNSGALTSGVHTFPAVLQSSGLYSLSSVVTVPSSSLGTQTYICNVNHKPSNTKVDKKVEPKSCGGGGSGGGGSQAVVTQEPSLTVSPGGTVTLTCRSSTGAVTTSNYANWVQQKPGQAPRGLIGGTNKRAPWTPARFSGSLLGGKAALTITGAQAEDEADYYCALWYSNLWVFGGGTKLTVLGGGGSDKTHTCPPCPAPEAAGPSVFLFPPKPKDTLMISRTPEVTCVVVDVSHEDPEVKFNWYVDGVEVHNAKTKPREEQYNSTYRVVSVLTVLHQDWLNGKEYKCKVSNKALPAPIEKTISKAKGQPREPQVYTLPPSREEMTKNQVSLSCAVKGFYPSDIAVEWESNGQPENNYKTTPPVLDSDGSFFLVSKLTVDKSRWQQGNVFSCSVMHEALHNRFTQKSLSLSPGGGGGSGGGGSGGGGSGGGGSDIQMTQSPSSLSASVGDRVTITCHASQNIYVWLNWYQQKPGKAPKLLIYKASNLHTGVPSRFSGSGSGTDFTLTISSLQPEDFATYYCQQGQTYPYTFGGGTKVEIK

SEQ ID NO: 459 - protein, 700 aa, synthetic construct
QVQLVQSGAEVKKPGASVKVSCKASGYTFTSYVMHWVRQKPGQGLEWIGYINPYNEGTESTDKFKGRATMTSDKSTSTVYMELSSLRSEDTAVYYCASIYYGYEGTYFGVWGQGTLVTVSSASTKGPSVFPLAPSSKSTSGGTAALGCLVKDYFPEPVTVSWNSGALTSGVHTFPAVLQSSGLYSLSSVVTVPSSSLGTQTYICNVNHKPSNTKVDKKVEPKSCGGGGSGGGGSQAVVTQEPSLTVSPGGTVTLTCRSSTGAVTTSNYANWVQQKPGQAPRGLIGGTNKRAPWTPARFSGSLLGGKAALTITGAQAEDEADYYCALWYSNLWVFGGGTKLTVLGGGGSDKTHTCPPCPAPEAAGPSVFLFPPKPKDTLMISRTPEVTCVVVDVSHEDPEVKFNWYVDGVEVHNAKTKPREEQYNSTYRVVSVLTVLHQDWLNGKEYKCKVSNKALPAPIEKTISKAKGQPREPQVYTLPPSREEMTKNQVSLSCAVKGFYPSDIAVEWESNGQPENNYKTTPPVLDSDGSFFLVSKLTVDKSRWQQGNVFSCSVMHEALHNRFTQKSLSLSPGGGGGSGGGGSGGGGSGGGGSDIQMTQSPSSLSASVGDRVTITCRASQDIRSNLNWYQQKPGGAVKLLIYYTSRLHSGVPSRFSGSGSGTDYTLTISSLQPEDFATYFCQQSEKLPRTFGGGTKVEIR

SEQ ID NO: 460 - protein, 695 aa, synthetic construct
QVQLVQSGAEVKKPGASVKVSCKASGYTFTSYVMHWVRQKPGQGLEWIGYINPYNEGTESTDKFKGRATMTSDKSTSTVYMELSSLRSEDTAVYYCASIYYGYEGTYFGVWGQGTLVTVSSASTKGPSVFPLAPSSKSTSGGTAALGCLVKDYFPEPVTVSWNSGALTSGVHTFPAVLQSSGLYSLSSVVTVPSSSLGTQTYICNVNHKPSNTKVDKKVEPKSCGGGGSQAVVTQEPSLTVSPGGTVTLTCRSSTGAVTTSNYANWVQQKPGQAPRGLIGGTNKRAPWTPARFSGSLLGGKAALTITGAQAEDEADYYCALWYSNLWVFGGGTKLTVLGGGGSDKTHTCPPCPAPEAAGPSVFLFPPKPKDTLMISRTPEVTCVVVDVSHEDPEVKFNWYVDGVEVHNAKTKPREEQYNSTYRVVSVLTVLHQDWLNGKEYKCKVSNKALPAPIEKTISKAKGQPREPQVYTLPPSREEMTKNQVSLSCAVKGFYPSDIAVEWESNGQPENNYKTTPPVLDSDGSFFLVSKLTVDKSRWQQGNVFSCSVMHEALHNRFTQKSLSLSPGGGGGSGGGGSGGGGSGGGGSDIQMTQSPSSLSASVGDRVTITCHASQNIYVWLNWYQQKPGKAPKLLIYKASNLHTGVPSRFSGSGSGTDFTLTISSLQPEDFATYYCQQGQTYPYTFGGGTKVEIK

SEQ ID NO: 461 - protein, 695 aa, synthetic construct
QVQLVQSGAEVKKPGASVKVSCKASGYTFTSYVMHWVRQKPGQGLEWIGYINPYNEGTESTDKFKGRATMTSDKSTSTVYMELSSLRSEDTAVYYCASIYYGYEGTYFGVWGQGTLVTVSSASTKGPSVFPLAPSSKSTSGGTAALGCLVKDYFPEPVTVSWNSGALTSGVHTFPAVLQSSGLYSLSSVVTVPSSSLGTQTYICNVNHKPSNTKVDKKVEPKSCGGGGSQAVVTQEPSLTVSPGGTVTLTCRSSTGAVTTSNYANWVQQKPGQAPRGLIGGTNKRAPWTPARFSGSLLGGKAALTITGAQAEDEADYYCALWYSNLWVFGGGTKLTVLGGGGSDKTHTCPPCPAPEAAGPSVFLFPPKPKDTLMISRTPEVTCVVVDVSHEDPEVKFNWYVDGVEVHNAKTKPREEQYNSTYRVVSVLTVLHQDWLNGKEYKCKVSNKALPAPIEKTISKAKGQPREPQVYTLPPSREEMTKNQVSLSCAVKGFYPSDIAVEWESNGQPENNYKTTPPVLDSDGSFFLVSKLTVDKSRWQQGNVFSCSVMHEALHNRFTQKSLSLSPGGGGGSGGGGSGGGGSGGGGSDIQMTQSPSSLSASVGDRVTITCRASQDIRSNLNWYQQKPGGAVKLLIYYTSRLHSGVPSRFSGSGSGTDYTLTISSLQPEDFATYFCQQSEKLPRTFGGGTKVEIR

SEQ ID NO: 462 - protein, 719 aa, synthetic construct
QVQLVQSGAEVKKPGASVKVSCKASGYTFTSYVMHWVRQKPGQGLEWIGYINPYNEGTESTDKFKGRATMTSDKSTSTVYMELSSLRSEDTAVYYCASIYYGYEGTYFGVWGQGTLVTVSSASTKGPSVFPLAPSSKSTSGGTAALGCLVKDYFPEPVTVSWNSGALTSGVHTFPAVLQSSGLYSLSSVVTVPSSSLGTQTYICNVNHKPSNTKVDKKVEPKSCGGGSEVQLVESGGGLVQPGGSLRLSCAASGFTFSTYAMNWVRQAPGKGLEWVGRIRSKYNNYATYYADSVKGRFTISRDDSKNSLYLQMNSLKTEDTAVYYCVRHGNFGNSYVSWFAYWGQGTLVTVSSGGGGSDKTHTCPPCPAPEAAGPSVFLFPPKPKDTLMISRTPEVTCVVVDVSHEDPEVKFNWYVDGVEVHNAKTKPREEQYNSTYRVVSVLTVLHQDWLNGKEYKCKVSNKALPAPIEKTISKAKGQPREPQVYTLPPSREEMTKNQVSLWCLVKGFYPSDIAVEWESNGQPENNYKTTPPVLDSDGSFFLYSKLTVDKSRWQQGNVFSCSVMHEALHNHYTQKSLSLSPGGGGGSGGGGSGGGGSGGGGSQVQLVQSGAEVKKPGASVKVSCKASGYTFAGFEMHWVRQAPGQGLEWMGAIDPKTGGTDYNQKFKDRVTMTRDTSISTAYMELSRLRSDDTAVYYCARDLGYFDVWGQGTLVTVSS

SEQ ID NO: 463 - protein, 694 aa, synthetic construct
QVQLVQSGAEVKKPGASVKVSCKASGYTFTSYVMHWVRQKPGQGLEWIGYINPYNEGTESTDKFKGRATMTSDKSTSTVYMELSSLRSEDTAVYYCASIYYGYEGTYFGVWGQGTLVTVSSASTKGPSVFPLAPSSKSTSGGTAALGCLVKDYFPEPVTVSWNSGALTSGVHTFPAVLQSSGLYSLSSVVTVPSSSLGTQTYICNVNHKPSNTKVDKKVEPKSCGGGSQAVVTQEPSLTVSPGGTVTLTCRSSTGAVTTSNYANWVQQKPGQAPRGLIGGTNKRAPWTPARFSGSLLGGKAALTITGAQAEDEADYYCALWYSNLWVFGGGTKLTVLGGGGSDKTHTCPPCPAPEAAGPSVFLFPPKPKDTLMISRTPEVTCVVVDVSHEDPEVKFNWYVDGVEVHNAKTKPREEQYNSTYRVVSVLTVLHQDWLNGKEYKCKVSNKALPAPIEKTISKAKGQPREPQVYTLPPSREEMTKNQVSLSCAVKGFYPSDIAVEWESNGQPENNYKTTPPVLDSDGSFFLVSKLTVDKSRWQQGNVFSCSVMHEALHNRFTQKSLSLSPGGGGGSGGGGSGGGGSGGGGSDIQMTQSPSSLSASVGDRVTITCRASQDIRSNLNWYQQKPGGAVKLLIYYTSRLHSGVPSRFSGSGSGTDYTLTISSLQPEDFATYFCQQSEKLPRTFGGGTKVEIR

SEQ ID NO: 464 - protein, 718 aa, synthetic construct
QVQLVQSGAEVKKPGASVKVSCKASGYTFTSYVMHWVRQKPGQGLEWIGYINPYNEGTESTDKFKGRATMTSDKSTSTVYMELSSLRSEDTAVYYCASIYYGYEGTYFGVWGQGTLVTVSSASTKGPSVFPLAPSSKSTSGGTAALGCLVKDYFPEPVTVSWNSGALTSGVHTFPAVLQSSGLYSLSSVVTVPSSSLGTQTYICNVNHKPSNTKVDKKVEPKSCGGSEVQLVESGGGLVQPGGSLRLSCAASGFTFSTYAMNWVRQAPGKGLEWVGRIRSKYNNYATYYADSVKGRFTISRDDSKNSLYLQMNSLKTEDTAVYYCVRHGNFGNSYVSWFAYWGQGTLVTVSSGGGGSDKTHTCPPCPAPEAAGPSVFLFPPKPKDTLMISRTPEVTCVVVDVSHEDPEVKFNWYVDGVEVHNAKTKPREEQYNSTYRVVSVLTVLHQDWLNGKEYKCKVSNKALPAPIEKTISKAKGQPREPQVYTLPPSREEMTKNQVSLWCLVKGFYPSDIAVEWESNGQPENNYKTTPPVLDSDGSFFLYSKLTVDKSRWQQGNVFSCSVMHEALHNHYTQKSLSLSPGGGGGSGGGGSGGGGSGGGGSQVQLVQSGAEVKKPGASVKVSCKASGYTFAGFEMHWVRQAPGQGLEWMGAIDPKTGGTDYNQKFKDRVTMTRDTSISTAYMELSRLRSDDTAVYYCARDLGYFDVWGQGTLVTVSS

SEQ ID NO: 465 - protein, 693 aa, synthetic construct
QVQLVQSGAEVKKPGASVKVSCKASGYTFTSYVMHWVRQKPGQGLEWIGYINPYNEGTESTDKFKGRATMTSDKSTSTVYMELSSLRSEDTAVYYCASIYYGYEGTYFGVWGQGTLVTVSSASTKGPSVFPLAPSSKSTSGGTAALGCLVKDYFPEPVTVSWNSGALTSGVHTFPAVLQSSGLYSLSSVVTVPSSSLGTQTYICNVNHKPSNTKVDKKVEPKSCGGSQAVVTQEPSLTVSPGGTVTLTCRSSTGAVTTSNYANWVQQKPGQAPRGLIGGTNKRAPWTPARFSGSLLGGKAALTITGAQAEDEADYYCALWYSNLWVFGGGTKLTVLGGGGSDKTHTCPPCPAPEAAGPSVFLFPPKPKDTLMISRTPEVTCVVVDVSHEDPEVKFNWYVDGVEVHNAKTKPREEQYNSTYRVVSVLTVLHQDWLNGKEYKCKVSNKALPAPIEKTISKAKGQPREPQVYTLPPSREEMTKNQVSLSCAVKGFYPSDIAVEWESNGQPENNYKTTPPVLDSDGSFFLVSKLTVDKSRWQQGNVFSCSVMHEALHNRFTQKSLSLSPGGGGGSGGGGSGGGGSGGGGSDIQMTQSPSSLSASVGDRVTITCRASQDIRSNLNWYQQKPGGAVKLLIYYTSRLHSGVPSRFSGSGSGTDYTLTISSLQPEDFATYFCQQSEKLPRTFGGGTKVEIR

SEQ ID NO: 466 - protein, 690 aa, synthetic construct
QVQLVQSGAEVKKPGASVKVSCKASGYTFTSYVMHWVRQKPGQGLEWIGYINPYNEGTESTDKFKGRATMTSDKSTSTVYMELSSLRSEDTAVYYCASIYYGYEGTYFGVWGQGTLVTVSSASTKGPSVFPLAPSSKSTSGGTAALGCLVKDYFPEPVTVSWNSGALTSGVHTFPAVLQSSGLYSLSSVVTVPSSSLGTQTYICNVNHKPSNTKVDKKVEPKSCQAVVTQEPSLTVSPGGTVTLTCRSSTGAVTTSNYANWVQQKPGQAPRGLIGGTNKRAPWTPARFSGSLLGGKAALTITGAQAEDEADYYCALWYSNLWVFGGGTKLTVLGGGGSDKTHTCPPCPAPEAAGPSVFLFPPKPKDTLMISRTPEVTCVVVDVSHEDPEVKFNWYVDGVEVHNAKTKPREEQYNSTYRVVSVLTVLHQDWLNGKEYKCKVSNKALPAPIEKTISKAKGQPREPQVYTLPPSREEMTKNQVSLSCAVKGFYPSDIAVEWESNGQPENNYKTTPPVLDSDGSFFLVSKLTVDKSRWQQGNVFSCSVMHEALHNRFTQKSLSLSPGGGGGSGGGGSGGGGSGGGGSDIQMTQSPSSLSASVGDRVTITCRASQDIRSNLNWYQQKPGGAVKLLIYYTSRLHSGVPSRFSGSGSGTDYTLTISSLQPEDFATYFCQQSEKLPRTFGGGTKVEIR

SEQ ID NO: 467 - protein, 674 aa, synthetic construct
QVQLVQSGAEVKKPGSSVKVSCKASGYAFSYSWINWVRQAPGQGLEWMGRIFPGDGDTDYNGKFKGRVTITADKSTSTAYMELSSLRSEDTAVYYCARNVFDGYWLVYWGQGTLVTVSSASTKGPSVFPLAPSSKSTSGGTAALGCLVEDYFPEPVTVSWNSGALTSGVHTFPAVLQSSGLYSLSSVVTVPSSSLGTQTYICNVNHKPSNTKVDEKVEPKSCDGGGGSGGGGSQAVVTQEPSLTVSPGGTVTLTCGSSTGAVTTSNYANWVQEKPGQAFRGLIGGTNKRAPGTPARFSGSLLGGKAALTLSGAQPEDEAEYYCALWYSNLWVFGGGTKLTVLSSASTKGPSVFPLAPSSKSTSGGTAALGCLVKDYFPEPVTVSWNSGALTSGVHTFPAVLQSSGLYSLSSVVTVPSSSLGTQTYICNVNHKPSNTKVDKKVEPKSCDKTHTCPPCPAPEAAGGPSVFLFPPKPKDTLMISRTPEVTCVVVDVSHEDPEVKFNWYVDGVEVHNAKTKPREEQYNSTYRVVSVLTVLHQDWLNGKEYKCKVSNKALGAPIEKTISKAKGQPREPQVYTLPPCRDELTKNQVSLWCLVKGFYPSDIAVEWESNGQPENNYKTTPPVLDSDGSFFLYSKLTVDKSRWQQGNVFSCSVMHEALHNHYTQKSLSLSPGK

SEQ ID NO: 468 - protein, 449 aa, synthetic construct
QVQLVQSGAEVKKPGSSVKVSCKASGYAFSYSWINWVRQAPGQGLEWMGRIFPGDGDTDYNGKFKGRVTITADKSTSTAYMELSSLRSEDTAVYYCARNVFDGYWLVYWGQGTLVTVSSASTKGPSVFPLAPSSKSTSGGTAALGCLVEDYFPEPVTVSWNSGALTSGVHTFPAVLQSSGLYSLSSVVTVPSSSLGTQTYICNVNHKPSNTKVDEKVEPKSCDKTHTCPPCPAPEAAGGPSVFLFPPKPKDTLMISRTPEVTCVVVDVSHEDPEVKFNWYVDGVEVHNAKTKPREEQYNSTYRVVSVLTVLHQDWLNGKEYKCKVSNKALGAPIEKTISKAKGQPREPQVCTLPPSRDELTKNQVSLSCAVKGFYPSDIAVEWESNGQPENNYKTTPPVLDSDGSFFLVSKLTVDKSRWQQGNVFSCSVMHEALHNHYTQKSLSLSPGK

SEQ ID NO: 469 - protein, 585 aa, synthetic construct
QVTLKESGPALVKPTQTLTLTCTFSGFSLSTSGTCVSWIRQPPGKALEWLATICWEDSKGYNPSLKSRLTISKDTSKNQAVLTMTNMDPVDTATYYCARREDSGYFWFPYWGQGTLVTVSSASTKGPSVFPLAPSSKSTSGGTAALGCLVKDYFPEPVTVSWNSGALTSGVHTFPAVLQSSGLYSLSSVVTVPSSSLGTQTYICNVNHKPSNTKVDKKVEPKSCDKTHTCPPCPAPEAAGPSVFLFPPKPKDTLMISRTPEVTCVVVDVSHEDPEVKFNWYVDGVEVHNAKTKPREEQYNSTYRVVSVLTVLHQDWLNGKEYKCKVSNKALPAPIEKTISKAKGQPREPQVYTLPPSREEMTKNQVSLWCLVKGFYPSDIAVEWESNGQPENNYKTTPPVLDSDGSFFLYSKLTVDKSRWQQGNVFSCSVMHEALHNHYTQKSLSLSPGGGGGSGGGGSGGGGSGGGGSQVQLVQSGAEVKKPGASVKVSCKASGYTFAGFEMHWVRQAPGQGLEWMGAIDPKTGGTDYNQKFKDRVTMTRDTSISTAYMELSRLRSDDTAVYYCARDLGYFDVWGQGTLVTVSS

SEQ ID NO: 470 - protein, 576 aa, synthetic construct
QVTLKESGPALVKPTQTLTLTCTFSGFSLSTSGTCVSWIRQPPGKALEWLATICWEDSKGYNPSLKSRLTISKDTSKNQAVLTMTNMDPVDTATYYCARREDSGYFWFPYWGQGTLVTVSSASTKGPSVFPLAPSSKSTSGGTAALGCLVKDYFPEPVTVSWNSGALTSGVHTFPAVLQSSGLYSLSSVVTVPSSSLGTQTYICNVNHKPSNTKVDKKVEPKSCDKTHTCPPCPAPEAAGPSVFLFPPKPKDTLMISRTPEVTCVVVDVSHEDPEVKFNWYVDGVEVHNAKTKPREEQYNSTYRVVSVLTVLHQDWLNGKEYKCKVSNKALPAPIEKTISKAKGQPREPQVYTLPPSREEMTKNQVSLSCAVKGFYPSDIAVEWESNGQPENNYKTTPPVLDSDGSFFLVSKLTVDKSRWQQGNVFSCSVMHEALHNRFTQKSLSLSPGGGGGSGGGGSGGGGSGGGGSDIQMTQSPSSLSASVGDRVTITCRASQDIRSNLNWYQQKPGGAVKLLIYYTSRLHSGVPSRFSGSGSGTDYTLTISSLQPEDFATYFCQQSEKLPRTFGGGTKVEIR

SEQ ID NO: 471 - protein, 607 aa, synthetic construct
QVTLKESGPALVKPTQTLTLTCTFSGFSLSTSGTCVSWIRQPPGKALEWLATICWEDSKGYNPSLKSRLTISKDTSKNQAVLTMTNMDPVDTATYYCARREDSGYFWFPYWGQGTLVTVSSASTKGPSVFPLAPSSKSTSGGTAALGCLVKDYFPEPVTVSWNSGALTSGVHTFPAVLQSSGLYSLSSVVTVPSSSLGTQTYICNVNHKPSNTKVDKKVEPKSCDKTHTCPPCPAPEAAGPSVFLFPPKPKDTLMISRTPEVTCVVVDVSHEDPEVKFNWYVDGVEVHNAKTKPREEQYNSTYRVVSVLTVLHQDWLNGKEYKCKVSNKALPAPIEKTISKAKGQPREPQVYTLPPSREEMTKNQVSLWCLVKGFYPSDIAVEWESNGQPENNYKTTPPVLDSDGSFFLYSKLTVDKSRWQQGNVFSCSVMHEALHNHYTQKSLSLSPGGGGGSGGGGSGGGGSGGGGSQVQLVQSGAEVKKPGASVKVSCKASGYTFAGFEMHWVRQAPGQGLEWMGAIDPKTGGTDYNQKFKDRVTMTRDTSISTAYMELSRLRSDDTAVYYCARDLGYFDVWGQGTLVTVSSGGGGSDKTHTCPPCPAPEAAGP

SEQ ID NO: 472 - protein, 598 aa, synthetic construct
QVTLKESGPALVKPTQTLTLTCTFSGFSLSTSGTCVSWIRQPPGKALEWLATICWEDSKGYNPSLKSRLTISKDTSKNQAVLTMTNMDPVDTATYYCARREDSGYFWFPYWGQGTLVTVSSASTKGPSVFPLAPSSKSTSGGTAALGCLVKDYFPEPVTVSWNSGALTSGVHTFPAVLQSSGLYSLSSVVTVPSSSLGTQTYICNVNHKPSNTKVDKKVEPKSCDKTHTCPPCPAPEAAGPSVFLFPPKPKDTLMISRTPEVTCVVVDVSHEDPEVKFNWYVDGVEVHNAKTKPREEQYNSTYRVVSVLTVLHQDWLNGKEYKCKVSNKALPAPIEKTISKAKGQPREPQVYTLPPSREEMTKNQVSLSCAVKGFYPSDIAVEWESNGQPENNYKTTPPVLDSDGSFFLVSKLTVDKSRWQQGNVFSCSVMHEALHNRFTQKSLSLSPGGGGGSGGGGSGGGGSGGGGSDIQMTQSPSSLSASVGDRVTITCRASQDIRSNLNWYQQKPGGAVKLLIYYTSRLHSGVPSRFSGSGSGTDYTLTISSLQPEDFATYFCQQSEKLPRTFGGGTKVEIRGGGGSDKTHTCPPCPAPEAAGP

SEQ ID NO: 473 - protein, 595 aa, synthetic construct
QVTLKESGPALVKPTQTLTLTCTFSGFSLSTSGTCVSWIRQPPGKALEWLATICWEDSKGYNPSLKSRLTISKDTSKNQAVLTMTNMDPVDTATYYCARREDSGYFWFPYWGQGTLVTVSSASTKGPSVFPLAPSSKSTSGGTAALGCLVKDYFPEPVTVSWNSGALTSGVHTFPAVLQSSGLYSLSSVVTVPSSSLGTQTYICNVNHKPSNTKVDKKVEPKSCDKTHTCPPCPAPEAAGPSVFLFPPKPKDTLMISRTPEVTCVVVDVSHEDPEVKFNWYVDGVEVHNAKTKPREEQYNSTYRVVSVLTVLHQDWLNGKEYKCKVSNKALPAPIEKTISKAKGQPREPQVYTLPPSREEMTKNQVSLWCLVKGFYPSDIAVEWESNGQPENNYKTTPPVLDSDGSFFLYSKLTVDKSRWQQGNVFSCSVMHEALHNHYTQKSLSLSPGGGGGSGGGGSGGGGSGGGGSQVQLVQSGAEVKKPGASVKVSCKASGYTFTGYYMHWVRQAPGQGLEWMGWINPDSGGTNYAQKFQGRVTMTRDTSISTAYMELNRLRSDDTAVYYCARDQPLGYCTNGVCSYFDYWGQGTLVTVSS

SEQ ID NO: 474 - protein, 576 aa, synthetic construct
QVTLKESGPALVKPTQTLTLTCTFSGFSLSTSGTCVSWIRQPPGKALEWLATICWEDSKGYNPSLKSRLTISKDTSKNQAVLTMTNMDPVDTATYYCARREDSGYFWFPYWGQGTLVTVSSASTKGPSVFPLAPSSKSTSGGTAALGCLVKDYFPEPVTVSWNSGALTSGVHTFPAVLQSSGLYSLSSVVTVPSSSLGTQTYICNVNHKPSNTKVDKKVEPKSCDKTHTCPPCPAPEAAGPSVFLFPPKPKDTLMISRTPEVTCVVVDVSHEDPEVKFNWYVDGVEVHNAKTKPREEQYNSTYRVVSVLTVLHQDWLNGKEYKCKVSNKALPAPIEKTISKAKGQPREPQVYTLPPSREEMTKNQVSLSCAVKGFYPSDIAVEWESNGQPENNYKTTPPVLDSDGSFFLVSKLTVDKSRWQQGNVFSCSVMHEALHNRFTQKSLSLSPGGGGGSGGGGSGGGGSGGGGSDIQMTQSPSSVSASVGDRVTITCRASQGIYSWLAWYQQKPGKAPNLLIYTASTLQSGVPSRFSGSGSGTDFTLTISSLQPEDFATYYCQQANIFPLTFGGGTKVEIK

SEQ ID NO: 475 - protein, 591 aa, synthetic construct
QVTLKESGPALVKPTQTLTLTCTFSGFSLSTSGTCVSWIRQPPGKALEWLATICWEDSKGYNPSLKSRLTISKDTSKNQAVLTMTNMDPVDTATYYCARREDSGYFWFPYWGQGTLVTVSSASTKGPSVFPLAPSSKSTSGGTAALGCLVKDYFPEPVTVSWNSGALTSGVHTFPAVLQSSGLYSLSSVVTVPSSSLGTQTYICNVNHKPSNTKVDKKVEPKSCDKTHTCPPCPAPEAAGPSVFLFPPKPKDTLMISRTPEVTCVVVDVSHEDPEVKFNWYVDGVEVHNAKTKPREEQYNSTYRVVSVLTVLHQDWLNGKEYKCKVSNKALPAPIEKTISKAKGQPREPQVYTLPPSREEMTKNQVSLWCLVKGFYPSDIAVEWESNGQPENNYKTTPPVLDSDGSFFLYSKLTVDKSRWQQGNVFSCSVMHEALHNHYTQKSLSLSPGGGGGSGGGGSGGGGSGGGGSEVQLVESGGGLVQPGGSLRLSCAASGFTFTNYGLHWVRQAPGKGLEWVSSISPSGGVTYYRDSVKGRFTISRDNSKNTLYLQMNSLRAEDTAVYYCAKPFLGWGGANWIAHWGQGTLVTVSS

SEQ ID NO: 476 - protein, 576 aa, synthetic construct
QVTLKESGPALVKPTQTLTLTCTFSGFSLSTSGTCVSWIRQPPGKALEWLATICWEDSKGYNPSLKSRLTISKDTSKNQAVLTMTNMDPVDTATYYCARREDSGYFWFPYWGQGTLVTVSSASTKGPSVFPLAPSSKSTSGGTAALGCLVKDYFPEPVTVSWNSGALTSGVHTFPAVLQSSGLYSLSSVVTVPSSSLGTQTYICNVNHKPSNTKVDKKVEPKSCDKTHTCPPCPAPEAAGPSVFLFPPKPKDTLMISRTPEVTCVVVDVSHEDPEVKFNWYVDGVEVHNAKTKPREEQYNSTYRVVSVLTVLHQDWLNGKEYKCKVSNKALPAPIEKTISKAKGQPREPQVYTLPPSREEMTKNQVSLSCAVKGFYPSDIAVEWESNGQPENNYKTTPPVLDSDGSFFLVSKLTVDKSRWQQGNVFSCSVMHEALHNRFTQKSLSLSPGGGGGSGGGGSGGGGSGGGGSDIQMTQSPSSLSASVGDRVTITCLASEDISNDLAWYQQKPGKAPKLLIYFVDRLLDGVPSRFSGSGSGTDFTLTISSLQPEDFATYYCQQSYKYPPTFGQGTKLEIK

SEQ ID NO: 477 - protein, 617 aa, synthetic construct
QVTLKESGPALVKPTQTLTLTCTFSGFSLSTSGTCVSWIRQPPGKALEWLATICWEDSKGYNPSLKSRLTISKDTSKNQAVLTMTNMDPVDTATYYCARREDSGYFWFPYWGQGTLVTVSSASTKGPSVFPLAPSSKSTSGGTAALGCLVKDYFPEPVTVSWNSGALTSGVHTFPAVLQSSGLYSLSSVVTVPSSSLGTQTYICNVNHKPSNTKVDKKVEPKSCDKTHTCPPCPAPEAAGPSVFLFPPKPKDTLMISRTPEVTCVVVDVSHEDPEVKFNWYVDGVEVHNAKTKPREEQYNSTYRVVSVLTVLHQDWLNGKEYKCKVSNKALPAPIEKTISKAKGQPREPQVYTLPPSREEMTKNQVSLWCLVKGFYPSDIAVEWESNGQPENNYKTTPPVLDSDGSFFLYSKLTVDKSRWQQGNVFSCSVMHEALHNHYTQKSLSLSPGGGGGSGGGGSGGGGSGGGGSQVQLVQSGAEVKKPGASVKVSCKASGYTFTGYYMHWVRQAPGQGLEWMGWINPDSGGTNYAQKFQGRVTMTRDTSISTAYMELNRLRSDDTAVYYCARDQPLGYCTNGVCSYFDYWGQGTLVTVSSGGGGSDKTHTCPPCPAPEAAGP

SEQ ID NO: 478 - protein, 598 aa, synthetic construct
QVTLKESGPALVKPTQTLTLTCTFSGFSLSTSGTCVSWIRQPPGKALEWLATICWEDSKGYNPSLKSRLTISKDTSKNQAVLTMTNMDPVDTATYYCARREDSGYFWFPYWGQGTLVTVSSASTKGPSVFPLAPSSKSTSGGTAALGCLVKDYFPEPVTVSWNSGALTSGVHTFPAVLQSSGLYSLSSVVTVPSSSLGTQTYICNVNHKPSNTKVDKKVEPKSCDKTHTCPPCPAPEAAGPSVFLFPPKPKDTLMISRTPEVTCVVVDVSHEDPEVKFNWYVDGVEVHNAKTKPREEQYNSTYRVVSVLTVLHQDWLNGKEYKCKVSNKALPAPIEKTISKAKGQPREPQVYTLPPSREEMTKNQVSLSCAVKGFYPSDIAVEWESNGQPENNYKTTPPVLDSDGSFFLVSKLTVDKSRWQQGNVFSCSVMHEALHNRFTQKSLSLSPGGGGGSGGGGSGGGGSGGGGSDIQMTQSPSSVSASVGDRVTITCRASQGIYSWLAWYQQKPGKAPNLLIYTASTLQSGVPSRFSGSGSGTDFTLTISSLQPEDFATYYCQQANIFPLTFGGGTKVEIKGGGGSDKTHTCPPCPAPEAAGP

SEQ ID NO: 479 - protein, 613 aa, synthetic construct
QVTLKESGPALVKPTQTLTLTCTFSGFSLSTSGTCVSWIRQPPGKALEWLATICWEDSKGYNPSLKSRLTISKDTSKNQAVLTMTNMDPVDTATYYCARREDSGYFWFPYWGQGTLVTVSSASTKGPSVFPLAPSSKSTSGGTAALGCLVKDYFPEPVTVSWNSGALTSGVHTFPAVLQSSGLYSLSSVVTVPSSSLGTQTYICNVNHKPSNTKVDKKVEPKSCDKTHTCPPCPAPEAAGPSVFLFPPKPKDTLMISRTPEVTCVVVDVSHEDPEVKFNWYVDGVEVHNAKTKPREEQYNSTYRVVSVLTVLHQDWLNGKEYKCKVSNKALPAPIEKTISKAKGQPREPQVYTLPPSREEMTKNQVSLWCLVKGFYPSDIAVEWESNGQPENNYKTTPPVLDSDGSFFLYSKLTVDKSRWQQGNVFSCSVMHEALHNHYTQKSLSLSPGGGGGSGGGGSGGGGSGGGGSEVQLVESGGGLVQPGGSLRLSCAASGFTFTNYGLHWVRQAPGKGLEWVSSISPSGGVTYYRDSVKGRFTISRDNSKNTLYLQMNSLRAEDTAVYYCAKPFLGWGGANWIAHWGQGTLVTVSSGGGGSDKTHTCPPCPAPEAAGP

SEQ ID NO: 480 - protein, 598 aa, synthetic construct
QVTLKESGPALVKPTQTLTLTCTFSGFSLSTSGTCVSWIRQPPGKALEWLATICWEDSKGYNPSLKSRLTISKDTSKNQAVLTMTNMDPVDTATYYCARREDSGYFWFPYWGQGTLVTVSSASTKGPSVFPLAPSSKSTSGGTAALGCLVKDYFPEPVTVSWNSGALTSGVHTFPAVLQSSGLYSLSSVVTVPSSSLGTQTYICNVNHKPSNTKVDKKVEPKSCDKTHTCPPCPAPEAAGPSVFLFPPKPKDTLMISRTPEVTCVVVDVSHEDPEVKFNWYVDGVEVHNAKTKPREEQYNSTYRVVSVLTVLHQDWLNGKEYKCKVSNKALPAPIEKTISKAKGQPREPQVYTLPPSREEMTKNQVSLSCAVKGFYPSDIAVEWESNGQPENNYKTTPPVLDSDGSFFLVSKLTVDKSRWQQGNVFSCSVMHEALHNRFTQKSLSLSPGGGGGSGGGGSGGGGSGGGGSDIQMTQSPSSLSASVGDRVTITCLASEDISNDLAWYQQKPGKAPKLLIYFVDRLLDGVPSRFSGSGSGTDFTLTISSLQPEDFATYYCQQSYKYPPTFGQGTKLEIKGGGGSDKTHTCPPCPAPEAAGP

SEQ ID NO: 481 - protein, 581 aa, synthetic construct
QVTLKESGPALVKPTQTLTLTCTFSGFSLSTSGTCVSWIRQPPGKALEWLATICWEDSKGYNPSLKSRLTISKDTSKNQAVLTMTNMDPVDTATYYCARREDSGYFWFPYWGQGTLVTVSSASTKGPSVFPLAPSSKSTSGGTAALGCLVKDYFPEPVTVSWNSGALTSGVHTFPAVLQSSGLYSLSSVVTVPSSSLGTQTYICNVNHKPSNTKVDKKVEPKSCGGGGSGGGGSGGGGSGGGGSDIQMTQSPSSLSASVGDRVTITCRASQDIRSNLNWYQQKPGGAVKLLIYYTSRLHSGVPSRFSGSGSGTDYTLTISSLQPEDFATYFCQQSEKLPRTFGGGTKVEIRGGGGSDKTHTCPPCPAPEAAGPSVFLFPPKPKDTLMISRTPEVTCVVVDVSHEDPEVKFNWYVDGVEVHNAKTKPREEQYNSTYRVVSVLTVLHQDWLNGKEYKCKVSNKALPAPIEKTISKAKGQPREPQVYTLPPSREEMTKNQVSLSCAVKGFYPSDIAVEWESNGQPENNYKTTPPVLDSDGSFFLVSKLTVDKSRWQQGNVFSCSVMHEALHNRFTQKSLSLSPG

SEQ ID NO: 482 - protein, 581 aa, synthetic construct
QVTLKESGPALVKPTQTLTLTCTFSGFSLSTSGTCVSWIRQPPGKALEWLATICWEDSKGYNPSLKSRLTISKDTSKNQAVLTMTNMDPVDTATYYCARREDSGYFWFPYWGQGTLVTVSSASTKGPSVFPLAPSSKSTSGGTAALGCLVKDYFPEPVTVSWNSGALTSGVHTFPAVLQSSGLYSLSSVVTVPSSSLGTQTYICNVNHKPSNTKVDKKVEPKSCGGGGSGGGGSGGGGSGGGGSDIQMTQSPSSLSASVGDRVTITCLASEDISNDLAWYQQKPGKAPKLLIYFVDRLLDGVPSRFSGSGSGTDFTLTISSLQPEDFATYYCQQSYKYPPTFGQGTKLEIKGGGGSDKTHTCPPCPAPEAAGPSVFLFPPKPKDTLMISRTPEVTCVVVDVSHEDPEVKFNWYVDGVEVHNAKTKPREEQYNSTYRVVSVLTVLHQDWLNGKEYKCKVSNKALPAPIEKTISKAKGQPREPQVYTLPPSREEMTKNQVSLSCAVKGFYPSDIAVEWESNGQPENNYKTTPPVLDSDGSFFLVSKLTVDKSRWQQGNVFSCSVMHEALHNRFTQKSLSLSPG

SEQ ID NO: 483 - protein, 707 aa, synthetic construct
QVTLKESGPALVKPTQTLTLTCTFSGFSLSTSGTCVSWIRQPPGKALEWLATICWEDSKGYNPSLKSRLTISKDTSKNQAVLTMTNMDPVDTATYYCARREDSGYFWFPYWGQGTLVTVSSASTKGPSVFPLAPSSKSTSGGTAALGCLVKDYFPEPVTVSWNSGALTSGVHTFPAVLQSSGLYSLSSVVTVPSSSLGTQTYICNVNHKPSNTKVDKKVEPKSCGGGGSGGGGSGGGGSGGGGSDIQMTQSPSSLSASVGDRVTITCRASQDIRSNLNWYQQKPGGAVKLLIYYTSRLHSGVPSRFSGSGSGTDYTLTISSLQPEDFATYFCQQSEKLPRTFGGGTKVEIRGGGGSDKTHTCPPCPAPEAAGPSVFLFPPKPKDTLMISRTPEVTCVVVDVSHEDPEVKFNWYVDGVEVHNAKTKPREEQYNSTYRVVSVLTVLHQDWLNGKEYKCKVSNKALPAPIEKTISKAKGQPREPQVYTLPPSREEMTKNQVSLSCAVKGFYPSDIAVEWESNGQPENNYKTTPPVLDSDGSFFLVSKLTVDKSRWQQGNVFSCSVMHEALHNRFTQKSLSLSPGGGGGSGGGGSGGGGSGGGGSEIVLTQSPATLSLSPGERATLSCRASSSVSYMHWYQQKPGQAPRPWIYATSNLASGIPARFSGSRSGTDYTLTISSLEPEDFAVYYCQQWSSNTLTFGGGTKVEIK

SEQ ID NO: 484 - protein, 708 aa, synthetic construct
QVTLKESGPALVKPTQTLTLTCTFSGFSLSTSGTCVSWIRQPPGKALEWLATICWEDSKGYNPSLKSRLTISKDTSKNQAVLTMTNMDPVDTATYYCARREDSGYFWFPYWGQGTLVTVSSASTKGPSVFPLAPSSKSTSGGTAALGCLVKDYFPEPVTVSWNSGALTSGVHTFPAVLQSSGLYSLSSVVTVPSSSLGTQTYICNVNHKPSNTKVDKKVEPKSCGGGGSGGGGSGGGGSGGGGSDIQMTQSPSSLSASVGDRVTITCLASEDISNDLAWYQQKPGKAPKLLIYFVDRLLDGVPSRFSGSGSGTDFTLTISSLQPEDFATYYCQQSYKYPPTFGQGTKLEIKGGGGSDKTHTCPPCPAPEAAGPSVFLFPPKPKDTLMISRTPEVTCVVVDVSHEDPEVKFNWYVDGVEVHNAKTKPREEQYNSTYRVVSVLTVLHQDWLNGKEYKCKVSNKALPAPIEKTISKAKGQPREPQVYTLPPSREEMTKNQVSLSCAVKGFYPSDIAVEWESNGQPENNYKTTPPVLDSDGSFFLVSKLTVDKSRWQQGNVFSCSVMHEALHNRFTQKSLSLSPGGGGGSGGGGSGGGGSGGGGSDIQMTQSPSSLSASVGDRVTITCRASQDIRSNLNWYQQKPGGAVKLLIYYTSRLHSGVPSRFSGSGSGTDYTLTISSLQPEDFATYFCQQSEKLPRTFGGGTKVEIR

SEQ ID NO: 485 - protein, 708 aa, synthetic construct
QVTLKESGPALVKPTQTLTLTCTFSGFSLSTSGTCVSWIRQPPGKALEWLATICWEDSKGYNPSLKSRLTISKDTSKNQAVLTMTNMDPVDTATYYCARREDSGYFWFPYWGQGTLVTVSSASTKGPSVFPLAPSSKSTSGGTAALGCLVKDYFPEPVTVSWNSGALTSGVHTFPAVLQSSGLYSLSSVVTVPSSSLGTQTYICNVNHKPSNTKVDKKVEPKSCGGGGSGGGGSGGGGSGGGGSDIQMTQSPSSLSASVGDRVTITCRASQDIRSNLNWYQQKPGGAVKLLIYYTSRLHSGVPSRFSGSGSGTDYTLTISSLQPEDFATYFCQQSEKLPRTFGGGTKVEIRGGGGSDKTHTCPPCPAPEAAGPSVFLFPPKPKDTLMISRTPEVTCVVVDVSHEDPEVKFNWYVDGVEVHNAKTKPREEQYNSTYRVVSVLTVLHQDWLNGKEYKCKVSNKALPAPIEKTISKAKGQPREPQVYTLPPSREEMTKNQVSLSCAVKGFYPSDIAVEWESNGQPENNYKTTPPVLDSDGSFFLVSKLTVDKSRWQQGNVFSCSVMHEALHNRFTQKSLSLSPGGGGGSGGGGSGGGGSGGGGSDIQMTQSPSSVSASVGDRVTITCRASQGIYSWLAWYQQKPGKAPNLLIYTASTLQSGVPSRFSGSGSGTDFTLTISSLQPEDFATYYCQQANIFPLTFGGGTKVEIK

SEQ ID NO: 486 - protein, 708 aa, synthetic construct
QVTLKESGPALVKPTQTLTLTCTFSGFSLSTSGTCVSWIRQPPGKALEWLATICWEDSKGYNPSLKSRLTISKDTSKNQAVLTMTNMDPVDTATYYCARREDSGYFWFPYWGQGTLVTVSSASTKGPSVFPLAPSSKSTSGGTAALGCLVKDYFPEPVTVSWNSGALTSGVHTFPAVLQSSGLYSLSSVVTVPSSSLGTQTYICNVNHKPSNTKVDKKVEPKSCGGGGSGGGGSGGGGSGGGGSDIQMTQSPSSLSASVGDRVTITCRASQDIRSNLNWYQQKPGGAVKLLIYYTSRLHSGVPSRFSGSGSGTDYTLTISSLQPEDFATYFCQQSEKLPRTFGGGTKVEIRGGGGSDKTHTCPPCPAPEAAGPSVFLFPPKPKDTLMISRTPEVTCVVVDVSHEDPEVKFNWYVDGVEVHNAKTKPREEQYNSTYRVVSVLTVLHQDWLNGKEYKCKVSNKALPAPIEKTISKAKGQPREPQVYTLPPSREEMTKNQVSLSCAVKGFYPSDIAVEWESNGQPENNYKTTPPVLDSDGSFFLVSKLTVDKSRWQQGNVFSCSVMHEALHNRFTQKSLSLSPGGGGGSGGGGSGGGGSGGGGSDIQMTQSPSSLSASVGDRVTITCLASEDISNDLAWYQQKPGKAPKLLIYFVDRLLDGVPSRFSGSGSGTDFTLTISSLQPEDFATYYCQQSYKYPPTFGQGTKLEIK

SEQ ID NO: 487 - protein, 707 aa, synthetic construct
QVTLKESGPALVKPTQTLTLTCTFSGFSLSTSGTCVSWIRQPPGKALEWLATICWEDSKGYNPSLKSRLTISKDTSKNQAVLTMTNMDPVDTATYYCARREDSGYFWFPYWGQGTLVTVSSASTKGPSVFPLAPSSKSTSGGTAALGCLVKDYFPEPVTVSWNSGALTSGVHTFPAVLQSSGLYSLSSVVTVPSSSLGTQTYICNVNHKPSNTKVDKKVEPKSCGGGGSGGGGSGGGGSGGGGSDIQMTQSPSSLSASVGDRVTITCRASQDIRSNLNWYQQKPGGAVKLLIYYTSRLHSGVPSRFSGSGSGTDYTLTISSLQPEDFATYFCQQSEKLPRTFGGGTKVEIRGGGGSDKTHTCPPCPAPEAAGPSVFLFPPKPKDTLMISRTPEVTCVVVDVSHEDPEVKFNWYVDGVEVHNAKTKPREEQYNSTYRVVSVLTVLHQDWLNGKEYKCKVSNKALPAPIEKTISKAKGQPREPQVYTLPPSREEMTKNQVSLSCAVKGFYPSDIAVEWESNGQPENNYKTTPPVLDSDGSFFLVSKLTVDKSRWQQGNVFSCSVMHEALHNRFTQKSLSLSPGGGGGSGGGGSGGGGSGGGGSEIVLTQSPATLSLSPGERATLSCRASKSVRTGMHWYQQKPGQAPRLLIYGASNLESGIPARFSGSGSGTDFTLTISSLEPEDFAVYYCQQSWNHFTFGQGTKLEIK

SEQ ID NO: 488 - protein, 707 aa, synthetic construct
QVTLKESGPALVKPTQTLTLTCTFSGFSLSTSGTCVSWIRQPPGKALEWLATICWEDSKGYNPSLKSRLTISKDTSKNQAVLTMTNMDPVDTATYYCARREDSGYFWFPYWGQGTLVTVSSASTKGPSVFPLAPSSKSTSGGTAALGCLVKDYFPEPVTVSWNSGALTSGVHTFPAVLQSSGLYSLSSVVTVPSSSLGTQTYICNVNHKPSNTKVDKKVEPKSCGGGGSGGGGSGGGGSGGGGSDIQMTQSPSSLSASVGDRVTITCLASEDISNDLAWYQQKPGKAPKLLIYFVDRLLDGVPSRFSGSGSGTDFTLTISSLQPEDFATYYCQQSYKYPPTFGQGTKLEIKGGGGSDKTHTCPPCPAPEAAGPSVFLFPPKPKDTLMISRTPEVTCVVVDVSHEDPEVKFNWYVDGVEVHNAKTKPREEQYNSTYRVVSVLTVLHQDWLNGKEYKCKVSNKALPAPIEKTISKAKGQPREPQVYTLPPSREEMTKNQVSLSCAVKGFYPSDIAVEWESNGQPENNYKTTPPVLDSDGSFFLVSKLTVDKSRWQQGNVFSCSVMHEALHNRFTQKSLSLSPGGGGGSGGGGSGGGGSGGGGSEIVLTQSPATLSLSPGERATLSCRASKSVRTGMHWYQQKPGQAPRLLIYGASNLESGIPARFSGSGSGTDFTLTISSLEPEDFAVYYCQQSWNHFTFGQGTKLEIK

SEQ ID NO: 489 - protein, 581 aa, synthetic construct
QVTLKESGPALVKPTQTLTLTCTFSGFSLSTSGTCVSWIRQPPGKALEWLATICWEDSKGYNPSLKSRLTISKDTSKNQAVLTMTNMDPVDTATYYCARREDSGYFWFPYWGQGTLVTVSSASTKGPSVFPLAPSSKSTSGGTAALGCLVKDYFPEPVTVSWNSGALTSGVHTFPAVLQSSGLYSLSSVVTVPSSSLGTQTYICNVNHKPSNTKVDKKVEPKSCGGGGSGGGGSGGGGSGGGGSDIQMTQSPSSVSASVGDRVTITCRASQGIYSWLAWYQQKPGKAPNLLIYTASTLQSGVPSRFSGSGSGTDFTLTISSLQPEDFATYYCQQANIFPLTFGGGTKVEIKGGGGSDKTHTCPPCPAPEAAGPSVFLFPPKPKDTLMISRTPEVTCVVVDVSHEDPEVKFNWYVDGVEVHNAKTKPREEQYNSTYRVVSVLTVLHQDWLNGKEYKCKVSNKALPAPIEKTISKAKGQPREPQVYTLPPSREEMTKNQVSLSCAVKGFYPSDIAVEWESNGQPENNYKTTPPVLDSDGSFFLVSKLTVDKSRWQQGNVFSCSVMHEALHNRFTQKSLSLSPG

SEQ ID NO: 490 - protein, 707 aa, synthetic construct
QVTLKESGPALVKPTQTLTLTCTFSGFSLSTSGTCVSWIRQPPGKALEWLATICWEDSKGYNPSLKSRLTISKDTSKNQAVLTMTNMDPVDTATYYCARREDSGYFWFPYWGQGTLVTVSSASTKGPSVFPLAPSSKSTSGGTAALGCLVKDYFPEPVTVSWNSGALTSGVHTFPAVLQSSGLYSLSSVVTVPSSSLGTQTYICNVNHKPSNTKVDKKVEPKSCGGGGSGGGGSGGGGSGGGGSDIQMTQSPSSVSASVGDRVTITCRASQGIYSWLAWYQQKPGKAPNLLIYTASTLQSGVPSRFSGSGSGTDFTLTISSLQPEDFATYYCQQANIFPLTFGGGTKVEIKGGGGSDKTHTCPPCPAPEAAGPSVFLFPPKPKDTLMISRTPEVTCVVVDVSHEDPEVKFNWYVDGVEVHNAKTKPREEQYNSTYRVVSVLTVLHQDWLNGKEYKCKVSNKALPAPIEKTISKAKGQPREPQVYTLPPSREEMTKNQVSLSCAVKGFYPSDIAVEWESNGQPENNYKTTPPVLDSDGSFFLVSKLTVDKSRWQQGNVFSCSVMHEALHNRFTQKSLSLSPGGGGGSGGGGSGGGGSGGGGSEIVLTQSPATLSLSPGERATLSCRASSSVSYMHWYQQKPGQAPRPWIYATSNLASGIPARFSGSRSGTDYTLTISSLEPEDFAVYYCQQWSSNTLTFGGGTKVEIK

SEQ ID NO: 491 - protein, 708 aa, synthetic construct
QVTLKESGPALVKPTQTLTLTCTFSGFSLSTSGTCVSWIRQPPGKALEWLATICWEDSKGYNPSLKSRLTISKDTSKNQAVLTMTNMDPVDTATYYCARREDSGYFWFPYWGQGTLVTVSSASTKGPSVFPLAPSSKSTSGGTAALGCLVKDYFPEPVTVSWNSGALTSGVHTFPAVLQSSGLYSLSSVVTVPSSSLGTQTYICNVNHKPSNTKVDKKVEPKSCGGGGSGGGGSGGGGSGGGGSDIQMTQSPSSVSASVGDRVTITCRASQGIYSWLAWYQQKPGKAPNLLIYTASTLQSGVPSRFSGSGSGTDFTLTISSLQPEDFATYYCQQANIFPLTFGGGTKVEIKGGGGSDKTHTCPPCPAPEAAGPSVFLFPPKPKDTLMISRTPEVTCVVVDVSHEDPEVKFNWYVDGVEVHNAKTKPREEQYNSTYRVVSVLTVLHQDWLNGKEYKCKVSNKALPAPIEKTISKAKGQPREPQVYTLPPSREEMTKNQVSLSCAVKGFYPSDIAVEWESNGQPENNYKTTPPVLDSDGSFFLVSKLTVDKSRWQQGNVFSCSVMHEALHNRFTQKSLSLSPGGGGGSGGGGSGGGGSGGGGSDIQMTQSPSSLSASVGDRVTITCRASQDIRSNLNWYQQKPGGAVKLLIYYTSRLHSGVPSRFSGSGSGTDYTLTISSLQPEDFATYFCQQSEKLPRTFGGGTKVEIR

SEQ ID NO: 492 - protein, 707 aa, synthetic construct
QVTLKESGPALVKPTQTLTLTCTFSGFSLSTSGTCVSWIRQPPGKALEWLATICWEDSKGYNPSLKSRLTISKDTSKNQAVLTMTNMDPVDTATYYCARREDSGYFWFPYWGQGTLVTVSSASTKGPSVFPLAPSSKSTSGGTAALGCLVKDYFPEPVTVSWNSGALTSGVHTFPAVLQSSGLYSLSSVVTVPSSSLGTQTYICNVNHKPSNTKVDKKVEPKSCGGGGSGGGGSGGGGSGGGGSDIQMTQSPSSVSASVGDRVTITCRASQGIYSWLAWYQQKPGKAPNLLIYTASTLQSGVPSRFSGSGSGTDFTLTISSLQPEDFATYYCQQANIFPLTFGGGTKVEIKGGGGSDKTHTCPPCPAPEAAGPSVFLFPPKPKDTLMISRTPEVTCVVVDVSHEDPEVKFNWYVDGVEVHNAKTKPREEQYNSTYRVVSVLTVLHQDWLNGKEYKCKVSNKALPAPIEKTISKAKGQPREPQVYTLPPSREEMTKNQVSLSCAVKGFYPSDIAVEWESNGQPENNYKTTPPVLDSDGSFFLVSKLTVDKSRWQQGNVFSCSVMHEALHNRFTQKSLSLSPGGGGGSGGGGSGGGGSGGGGSEIVLTQSPATLSLSPGERATLSCRASKSVRTGMHWYQQKPGQAPRLLIYGASNLESGIPARFSGSGSGTDFTLTISSLEPEDFAVYYCQQSWNHFTFGQGTKLEIK

SEQ ID NO: 493 - protein, 707 aa, synthetic construct
QVTLKESGPALVKPTQTLTLTCTFSGFSLSTSGTCVSWIRQPPGKALEWLATICWEDSKGYNPSLKSRLTISKDTSKNQAVLTMTNMDPVDTATYYCARREDSGYFWFPYWGQGTLVTVSSASTKGPSVFPLAPSSKSTSGGTAALGCLVKDYFPEPVTVSWNSGALTSGVHTFPAVLQSSGLYSLSSVVTVPSSSLGTQTYICNVNHKPSNTKVDKKVEPKSCGGGGSGGGGSGGGGSGGGGSEIVLTQSPATLSLSPGERATLSCRASKSVRTGMHWYQQKPGQAPRLLIYGASNLESGIPARFSGSGSGTDFTLTISSLEPEDFAVYYCQQSWNHFTFGQGTKLEIKGGGGSDKTHTCPPCPAPEAAGPSVFLFPPKPKDTLMISRTPEVTCVVVDVSHEDPEVKFNWYVDGVEVHNAKTKPREEQYNSTYRVVSVLTVLHQDWLNGKEYKCKVSNKALPAPIEKTISKAKGQPREPQVYTLPPSREEMTKNQVSLSCAVKGFYPSDIAVEWESNGQPENNYKTTPPVLDSDGSFFLVSKLTVDKSRWQQGNVFSCSVMHEALHNRFTQKSLSLSPGGGGGSGGGGSGGGGSGGGGSDIQMTQSPSSLSASVGDRVTITCRASQDIRSNLNWYQQKPGGAVKLLIYYTSRLHSGVPSRFSGSGSGTDYTLTISSLQPEDFATYFCQQSEKLPRTFGGGTKVEIR

SEQ ID NO: 494 - protein, 707 aa, synthetic construct
QVTLKESGPALVKPTQTLTLTCTFSGFSLSTSGTCVSWIRQPPGKALEWLATICWEDSKGYNPSLKSRLTISKDTSKNQAVLTMTNMDPVDTATYYCARREDSGYFWFPYWGQGTLVTVSSASTKGPSVFPLAPSSKSTSGGTAALGCLVKDYFPEPVTVSWNSGALTSGVHTFPAVLQSSGLYSLSSVVTVPSSSLGTQTYICNVNHKPSNTKVDKKVEPKSCGGGGSGGGGSGGGGSGGGGSEIVLTQSPATLSLSPGERATLSCRASKSVRTGMHWYQQKPGQAPRLLIYGASNLESGIPARFSGSGSGTDFTLTISSLEPEDFAVYYCQQSWNHFTFGQGTKLEIKGGGGSDKTHTCPPCPAPEAAGPSVFLFPPKPKDTLMISRTPEVTCVVVDVSHEDPEVKFNWYVDGVEVHNAKTKPREEQYNSTYRVVSVLTVLHQDWLNGKEYKCKVSNKALPAPIEKTISKAKGQPREPQVYTLPPSREEMTKNQVSLSCAVKGFYPSDIAVEWESNGQPENNYKTTPPVLDSDGSFFLVSKLTVDKSRWQQGNVFSCSVMHEALHNRFTQKSLSLSPGGGGGSGGGGSGGGGSGGGGSDIQMTQSPSSVSASVGDRVTITCRASQGIYSWLAWYQQKPGKAPNLLIYTASTLQSGVPSRFSGSGSGTDFTLTISSLQPEDFATYYCQQANIFPLTFGGGTKVEIK

SEQ ID NO: 495 - protein, 707 aa, synthetic construct
QVTLKESGPALVKPTQTLTLTCTFSGFSLSTSGTCVSWIRQPPGKALEWLATICWEDSKGYNPSLKSRLTISKDTSKNQAVLTMTNMDPVDTATYYCARREDSGYFWFPYWGQGTLVTVSSASTKGPSVFPLAPSSKSTSGGTAALGCLVKDYFPEPVTVSWNSGALTSGVHTFPAVLQSSGLYSLSSVVTVPSSSLGTQTYICNVNHKPSNTKVDKKVEPKSCGGGGSGGGGSGGGGSGGGGSEIVLTQSPATLSLSPGERATLSCRASKSVRTGMHWYQQKPGQAPRLLIYGASNLESGIPARFSGSGSGTDFTLTISSLEPEDFAVYYCQQSWNHFTFGQGTKLEIKGGGGSDKTHTCPPCPAPEAAGPSVFLFPPKPKDTLMISRTPEVTCVVVDVSHEDPEVKFNWYVDGVEVHNAKTKPREEQYNSTYRVVSVLTVLHQDWLNGKEYKCKVSNKALPAPIEKTISKAKGQPREPQVYTLPPSREEMTKNQVSLSCAVKGFYPSDIAVEWESNGQPENNYKTTPPVLDSDGSFFLVSKLTVDKSRWQQGNVFSCSVMHEALHNRFTQKSLSLSPGGGGGSGGGGSGGGGSGGGGSDIQMTQSPSSLSASVGDRVTITCLASEDISNDLAWYQQKPGKAPKLLIYFVDRLLDGVPSRFSGSGSGTDFTLTISSLQPEDFATYYCQQSYKYPPTFGQGTKLEIK

SEQ ID NO: 496 - protein, 596 aa, synthetic construct
QVTLKESGPALVKPTQTLTLTCTFSGFSLSTSGTCVSWIRQPPGKALEWLATICWEDSKGYNPSLKSRLTISKDTSKNQAVLTMTNMDPVDTATYYCARREDSGYFWFPYWGQGTLVTVSSASTKGPSVFPLAPSSKSTSGGTAALGCLVKDYFPEPVTVSWNSGALTSGVHTFPAVLQSSGLYSLSSVVTVPSSSLGTQTYICNVNHKPSNTKVDKKVEPKSCGGGGSGGGGSGGGGSGGGGSEVQLVESGGGLVQPGGSLRLSCAASGFTFTNYGLHWVRQAPGKGLEWVSSISPSGGVTYYRDSVKGRFTISRDNSKNTLYLQMNSLRAEDTAVYYCAKPFLGWGGANWIAHWGQGTLVTVSSGGGGSDKTHTCPPCPAPEAAGPSVFLFPPKPKDTLMISRTPEVTCVVVDVSHEDPEVKFNWYVDGVEVHNAKTKPREEQYNSTYRVVSVLTVLHQDWLNGKEYKCKVSNKALPAPIEKTISKAKGQPREPQVYTLPPSREEMTKNQVSLWCLVKGFYPSDIAVEWESNGQPENNYKTTPPVLDSDGSFFLYSKLTVDKSRWQQGNVFSCSVMHEALHNHYTQKSLSLSPG

SEQ ID NO: 497 - protein, 732 aa, synthetic construct
QVTLKESGPALVKPTQTLTLTCTFSGFSLSTSGTCVSWIRQPPGKALEWLATICWEDSKGYNPSLKSRLTISKDTSKNQAVLTMTNMDPVDTATYYCARREDSGYFWFPYWGQGTLVTVSSASTKGPSVFPLAPSSKSTSGGTAALGCLVKDYFPEPVTVSWNSGALTSGVHTFPAVLQSSGLYSLSSVVTVPSSSLGTQTYICNVNHKPSNTKVDKKVEPKSCGGGGSGGGGSGGGGSGGGGSEVQLVESGGGLVQPGGSLRLSCAASGFTFTNYGLHWVRQAPGKGLEWVSSISPSGGVTYYRDSVKGRFTISRDNSKNTLYLQMNSLRAEDTAVYYCAKPFLGWGGANWIAHWGQGTLVTVSSGGGGSDKTHTCPPCPAPEAAGPSVFLFPPKPKDTLMISRTPEVTCVVVDVSHEDPEVKFNWYVDGVEVHNAKTKPREEQYNSTYRVVSVLTVLHQDWLNGKEYKCKVSNKALPAPIEKTISKAKGQPREPQVYTLPPSREEMTKNQVSLWCLVKGFYPSDIAVEWESNGQPENNYKTTPPVLDSDGSFFLYSKLTVDKSRWQQGNVFSCSVMHEALHNHYTQKSLSLSPGGGGGSGGGGSGGGGSGGGGSQVQLVQSGAEVKKPGASVKVSCKASGYTFAGFEMHWVRQAPGQGLEWMGAIDPKTGGTDYNQKFKDRVTMTRDTSISTAYMELSRLRSDDTAVYYCARDLGYFDVWGQGTLVTVSS

SEQ ID NO: 498 - protein, 737 aa, synthetic construct
QVTLKESGPALVKPTQTLTLTCTFSGFSLSTSGTCVSWIRQPPGKALEWLATICWEDSKGYNPSLKSRLTISKDTSKNQAVLTMTNMDPVDTATYYCARREDSGYFWFPYWGQGTLVTVSSASTKGPSVFPLAPSSKSTSGGTAALGCLVKDYFPEPVTVSWNSGALTSGVHTFPAVLQSSGLYSLSSVVTVPSSSLGTQTYICNVNHKPSNTKVDKKVEPKSCGGGGSGGGGSGGGGSGGGGSEVQLVESGGGLVQPGGSLRLSCAASGFTFTNYGLHWVRQAPGKGLEWVSSISPSGGVTYYRDSVKGRFTISRDNSKNTLYLQMNSLRAEDTAVYYCAKPFLGWGGANWIAHWGQGTLVTVSSGGGGSDKTHTCPPCPAPEAAGPSVFLFPPKPKDTLMISRTPEVTCVVVDVSHEDPEVKFNWYVDGVEVHNAKTKPREEQYNSTYRVVSVLTVLHQDWLNGKEYKCKVSNKALPAPIEKTISKAKGQPREPQVYTLPPSREEMTKNQVSLWCLVKGFYPSDIAVEWESNGQPENNYKTTPPVLDSDGSFFLYSKLTVDKSRWQQGNVFSCSVMHEALHNHYTQKSLSLSPGGGGGSGGGGSGGGGSGGGGSQVQLQESGPGLVKPSETLSLTCTVSGFSLTSYNVHWIRQPPGKGLEWIGVIWSGVRTDYNSVLKPRVTISVDTSKNQFSLKLSSVTAADTAVYYCARGTYDDNYHDVMDAWGQGTLVTVSS

SEQ ID NO: 499 - protein, 731 aa, synthetic construct
QVTLKESGPALVKPTQTLTLTCTFSGFSLSTSGTCVSWIRQPPGKALEWLATICWEDSKGYNPSLKSRLTISKDTSKNQAVLTMTNMDPVDTATYYCARREDSGYFWFPYWGQGTLVTVSSASTKGPSVFPLAPSSKSTSGGTAALGCLVKDYFPEPVTVSWNSGALTSGVHTFPAVLQSSGLYSLSSVVTVPSSSLGTQTYICNVNHKPSNTKVDKKVEPKSCGGGGSGGGGSGGGGSGGGGSQVQLQESGPGLVKPSETLSLTCTVSGFSLTSYNVHWIRQPPGKGLEWIGVIWSGVRTDYNSVLKPRVTISVDTSKNQFSLKLSSVTAADTAVYYCARGTYDDNYHDVMDAWGQGTLVTVSSGGGGSDKTHTCPPCPAPEAAGPSVFLFPPKPKDTLMISRTPEVTCVVVDVSHEDPEVKFNWYVDGVEVHNAKTKPREEQYNSTYRVVSVLTVLHQDWLNGKEYKCKVSNKALPAPIEKTISKAKGQPREPQVYTLPPSREEMTKNQVSLWCLVKGFYPSDIAVEWESNGQPENNYKTTPPVLDSDGSFFLYSKLTVDKSRWQQGNVFSCSVMHEALHNHYTQKSLSLSPGGGGGSGGGGSGGGGSGGGGSQVQLVQSGAEVKKPGASVKVSCKASGYTFAGFEMHWVRQAPGQGLEWMGAIDPKTGGTDYNQKFKDRVTMTRDTSISTAYMELSRLRSDDTAVYYCARDLGYFDVWGQGTLVTVSS

SEQ ID NO: 500 - protein, 741 aa, synthetic construct
QVTLKESGPALVKPTQTLTLTCTFSGFSLSTSGTCVSWIRQPPGKALEWLATICWEDSKGYNPSLKSRLTISKDTSKNQAVLTMTNMDPVDTATYYCARREDSGYFWFPYWGQGTLVTVSSASTKGPSVFPLAPSSKSTSGGTAALGCLVKDYFPEPVTVSWNSGALTSGVHTFPAVLQSSGLYSLSSVVTVPSSSLGTQTYICNVNHKPSNTKVDKKVEPKSCGGGGSGGGGSGGGGSGGGGSQVQLQESGPGLVKPSETLSLTCTVSGFSLTSYNVHWIRQPPGKGLEWIGVIWSGVRTDYNSVLKPRVTISVDTSKNQFSLKLSSVTAADTAVYYCARGTYDDNYHDVMDAWGQGTLVTVSSGGGGSDKTHTCPPCPAPEAAGPSVFLFPPKPKDTLMISRTPEVTCVVVDVSHEDPEVKFNWYVDGVEVHNAKTKPREEQYNSTYRVVSVLTVLHQDWLNGKEYKCKVSNKALPAPIEKTISKAKGQPREPQVYTLPPSREEMTKNQVSLWCLVKGFYPSDIAVEWESNGQPENNYKTTPPVLDSDGSFFLYSKLTVDKSRWQQGNVFSCSVMHEALHNHYTQKSLSLSPGGGGGSGGGGSGGGGSGGGGSQVQLVQSGAEVKKPGASVKVSCKASGYTFTGYYMHWVRQAPGQGLEWMGWINPDSGGTNYAQKFQGRVTMTRDTSISTAYMELNRLRSDDTAVYYCARDQPLGYCTNGVCSYFDYWGQGTLVTVSS

SEQ ID NO: 501 - protein, 737 aa, synthetic construct
QVTLKESGPALVKPTQTLTLTCTFSGFSLSTSGTCVSWIRQPPGKALEWLATICWEDSKGYNPSLKSRLTISKDTSKNQAVLTMTNMDPVDTATYYCARREDSGYFWFPYWGQGTLVTVSSASTKGPSVFPLAPSSKSTSGGTAALGCLVKDYFPEPVTVSWNSGALTSGVHTFPAVLQSSGLYSLSSVVTVPSSSLGTQTYICNVNHKPSNTKVDKKVEPKSCGGGGSGGGGSGGGGSGGGGSQVQLQESGPGLVKPSETLSLTCTVSGFSLTSYNVHWIRQPPGKGLEWIGVIWSGVRTDYNSVLKPRVTISVDTSKNQFSLKLSSVTAADTAVYYCARGTYDDNYHDVMDAWGQGTLVTVSSGGGGSDKTHTCPPCPAPEAAGPSVFLFPPKPKDTLMISRTPEVTCVVVDVSHEDPEVKFNWYVDGVEVHNAKTKPREEQYNSTYRVVSVLTVLHQDWLNGKEYKCKVSNKALPAPIEKTISKAKGQPREPQVYTLPPSREEMTKNQVSLWCLVKGFYPSDIAVEWESNGQPENNYKTTPPVLDSDGSFFLYSKLTVDKSRWQQGNVFSCSVMHEALHNHYTQKSLSLSPGGGGGSGGGGSGGGGSGGGGSEVQLVESGGGLVQPGGSLRLSCAASGFTFTNYGLHWVRQAPGKGLEWVSSISPSGGVTYYRDSVKGRFTISRDNSKNTLYLQMNSLRAEDTAVYYCAKPFLGWGGANWIAHWGQGTLVTVSS

SEQ ID NO: 502 - protein, 590 aa, synthetic construct
QVTLKESGPALVKPTQTLTLTCTFSGFSLSTSGTCVSWIRQPPGKALEWLATICWEDSKGYNPSLKSRLTISKDTSKNQAVLTMTNMDPVDTATYYCARREDSGYFWFPYWGQGTLVTVSSASTKGPSVFPLAPSSKSTSGGTAALGCLVKDYFPEPVTVSWNSGALTSGVHTFPAVLQSSGLYSLSSVVTVPSSSLGTQTYICNVNHKPSNTKVDKKVEPKSCGGGGSGGGGSGGGGSGGGGSQVQLVQSGAEVKKPGASVKVSCKASGYTFAGFEMHWVRQAPGQGLEWMGAIDPKTGGTDYNQKFKDRVTMTRDTSISTAYMELSRLRSDDTAVYYCARDLGYFDVWGQGTLVTVSSGGGGSDKTHTCPPCPAPEAAGPSVFLFPPKPKDTLMISRTPEVTCVVVDVSHEDPEVKFNWYVDGVEVHNAKTKPREEQYNSTYRVVSVLTVLHQDWLNGKEYKCKVSNKALPAPIEKTISKAKGQPREPQVYTLPPSREEMTKNQVSLWCLVKGFYPSDIAVEWESNGQPENNYKTTPPVLDSDGSFFLYSKLTVDKSRWQQGNVFSCSVMHEALHNHYTQKSLSLSPG

SEQ ID NO: 503 - protein, 600 aa, synthetic construct
QVTLKESGPALVKPTQTLTLTCTFSGFSLSTSGTCVSWIRQPPGKALEWLATICWEDSKGYNPSLKSRLTISKDTSKNQAVLTMTNMDPVDTATYYCARREDSGYFWFPYWGQGTLVTVSSASTKGPSVFPLAPSSKSTSGGTAALGCLVKDYFPEPVTVSWNSGALTSGVHTFPAVLQSSGLYSLSSVVTVPSSSLGTQTYICNVNHKPSNTKVDKKVEPKSCGGGGSGGGGSGGGGSGGGGSQVQLVQSGAEVKKPGASVKVSCKASGYTFTGYYMHWVRQAPGQGLEWMGWINPDSGGTNYAQKFQGRVTMTRDTSISTAYMELNRLRSDDTAVYYCARDQPLGYCTNGVCSYFDYWGQGTLVTVSSGGGGSDKTHTCPPCPAPEAAGPSVFLFPPKPKDTLMISRTPEVTCVVVDVSHEDPEVKFNWYVDGVEVHNAKTKPREEQYNSTYRVVSVLTVLHQDWLNGKEYKCKVSNKALPAPIEKTISKAKGQPREPQVYTLPPSREEMTKNQVSLWCLVKGFYPSDIAVEWESNGQPENNYKTTPPVLDSDGSFFLYSKLTVDKSRWQQGNVFSCSVMHEALHNHYTQKSLSLSPG

SEQ ID NO: 504 - protein, 731 aa, synthetic construct
QVTLKESGPALVKPTQTLTLTCTFSGFSLSTSGTCVSWIRQPPGKALEWLATICWEDSKGYNPSLKSRLTISKDTSKNQAVLTMTNMDPVDTATYYCARREDSGYFWFPYWGQGTLVTVSSASTKGPSVFPLAPSSKSTSGGTAALGCLVKDYFPEPVTVSWNSGALTSGVHTFPAVLQSSGLYSLSSVVTVPSSSLGTQTYICNVNHKPSNTKVDKKVEPKSCGGGGSGGGGSGGGGSGGGGSQVQLVQSGAEVKKPGASVKVSCKASGYTFAGFEMHWVRQAPGQGLEWMGAIDPKTGGTDYNQKFKDRVTMTRDTSISTAYMELSRLRSDDTAVYYCARDLGYFDVWGQGTLVTVSSGGGGSDKTHTCPPCPAPEAAGPSVFLFPPKPKDTLMISRTPEVTCVVVDVSHEDPEVKFNWYVDGVEVHNAKTKPREEQYNSTYRVVSVLTVLHQDWLNGKEYKCKVSNKALPAPIEKTISKAKGQPREPQVYTLPPSREEMTKNQVSLWCLVKGFYPSDIAVEWESNGQPENNYKTTPPVLDSDGSFFLYSKLTVDKSRWQQGNVFSCSVMHEALHNHYTQKSLSLSPGGGGGSGGGGSGGGGSGGGGSQVQLVQSGAEVKKPGASVKVSCKASGYTFTSYVMHWVRQKPGQGLEWIGYINPYNEGTESTDKFKGRATMTSDKSTSTVYMELSSLRSEDTAVYYCASIYYGYEGTYFGVWGQGTLVTVSS

SEQ ID NO: 505 - protein, 741 aa, synthetic construct
QVTLKESGPALVKPTQTLTLTCTFSGFSLSTSGTCVSWIRQPPGKALEWLATICWEDSKGYNPSLKSRLTISKDTSKNQAVLTMTNMDPVDTATYYCARREDSGYFWFPYWGQGTLVTVSSASTKGPSVFPLAPSSKSTSGGTAALGCLVKDYFPEPVTVSWNSGALTSGVHTFPAVLQSSGLYSLSSVVTVPSSSLGTQTYICNVNHKPSNTKVDKKVEPKSCGGGGSGGGGSGGGGSGGGGSQVQLVQSGAEVKKPGASVKVSCKASGYTFTGYYMHWVRQAPGQGLEWMGWINPDSGGTNYAQKFQGRVTMTRDTSISTAYMELNRLRSDDTAVYYCARDQPLGYCTNGVCSYFDYWGQGTLVTVSSGGGGSDKTHTCPPCPAPEAAGPSVFLFPPKPKDTLMISRTPEVTCVVVDVSHEDPEVKFNWYVDGVEVHNAKTKPREEQYNSTYRVVSVLTVLHQDWLNGKEYKCKVSNKALPAPIEKTISKAKGQPREPQVYTLPPSREEMTKNQVSLWCLVKGFYPSDIAVEWESNGQPENNYKTTPPVLDSDGSFFLYSKLTVDKSRWQQGNVFSCSVMHEALHNHYTQKSLSLSPGGGGGSGGGGSGGGGSGGGGSQVQLVQSGAEVKKPGASVKVSCKASGYTFTSYVMHWVRQKPGQGLEWIGYINPYNEGTESTDKFKGRATMTSDKSTSTVYMELSSLRSEDTAVYYCASIYYGYEGTYFGVWGQGTLVTVSS

SEQ ID NO: 506 - protein, 736 aa, synthetic construct
QVTLKESGPALVKPTQTLTLTCTFSGFSLSTSGTCVSWIRQPPGKALEWLATICWEDSKGYNPSLKSRLTISKDTSKNQAVLTMTNMDPVDTATYYCARREDSGYFWFPYWGQGTLVTVSSASTKGPSVFPLAPSSKSTSGGTAALGCLVKDYFPEPVTVSWNSGALTSGVHTFPAVLQSSGLYSLSSVVTVPSSSLGTQTYICNVNHKPSNTKVDKKVEPKSCGGGGSGGGGSGGGGSGGGGSQVQLVQSGAEVKKPGASVKVSCKASGYTFTGYYMHWVRQAPGQGLEWMGWINPDSGGTNYAQKFQGRVTMTRDTSISTAYMELNRLRSDDTAVYYCARDQPLGYCTNGVCSYFDYWGQGTLVTVSSGGGGSDKTHTCPPCPAPEAAGPSVFLFPPKPKDTLMISRTPEVTCVVVDVSHEDPEVKFNWYVDGVEVHNAKTKPREEQYNSTYRVVSVLTVLHQDWLNGKEYKCKVSNKALPAPIEKTISKAKGQPREPQVYTLPPSREEMTKNQVSLWCLVKGFYPSDIAVEWESNGQPENNYKTTPPVLDSDGSFFLYSKLTVDKSRWQQGNVFSCSVMHEALHNHYTQKSLSLSPGGGGGSGGGGSGGGGSGGGGSQVQLVQSGAEVKKPGASVKVSCKASGYTFAGFEMHWVRQAPGQGLEWMGAIDPKTGGTDYNQKFKDRVTMTRDTSISTAYMELSRLRSDDTAVYYCARDLGYFDVWGQGTLVTVSS

SEQ ID NO: 507 - protein, 736 aa, synthetic construct
QVTLKESGPALVKPTQTLTLTCTFSGFSLSTSGTCVSWIRQPPGKALEWLATICWEDSKGYNPSLKSRLTISKDTSKNQAVLTMTNMDPVDTATYYCARREDSGYFWFPYWGQGTLVTVSSASTKGPSVFPLAPSSKSTSGGTAALGCLVKDYFPEPVTVSWNSGALTSGVHTFPAVLQSSGLYSLSSVVTVPSSSLGTQTYICNVNHKPSNTKVDKKVEPKSCGGGGSGGGGSGGGGSGGGGSQVQLVQSGAEVKKPGASVKVSCKASGYTFAGFEMHWVRQAPGQGLEWMGAIDPKTGGTDYNQKFKDRVTMTRDTSISTAYMELSRLRSDDTAVYYCARDLGYFDVWGQGTLVTVSSGGGGSDKTHTCPPCPAPEAAGPSVFLFPPKPKDTLMISRTPEVTCVVVDVSHEDPEVKFNWYVDGVEVHNAKTKPREEQYNSTYRVVSVLTVLHQDWLNGKEYKCKVSNKALPAPIEKTISKAKGQPREPQVYTLPPSREEMTKNQVSLWCLVKGFYPSDIAVEWESNGQPENNYKTTPPVLDSDGSFFLYSKLTVDKSRWQQGNVFSCSVMHEALHNHYTQKSLSLSPGGGGGSGGGGSGGGGSGGGGSQVQLVQSGAEVKKPGASVKVSCKASGYTFTGYYMHWVRQAPGQGLEWMGWINPDSGGTNYAQKFQGRVTMTRDTSISTAYMELNRLRSDDTAVYYCARDQPLGYCTNGVCSYFDYWGQGTLVTVSS

SEQ ID NO: 508 - protein, 732 aa, synthetic construct
QVTLKESGPALVKPTQTLTLTCTFSGFSLSTSGTCVSWIRQPPGKALEWLATICWEDSKGYNPSLKSRLTISKDTSKNQAVLTMTNMDPVDTATYYCARREDSGYFWFPYWGQGTLVTVSSASTKGPSVFPLAPSSKSTSGGTAALGCLVKDYFPEPVTVSWNSGALTSGVHTFPAVLQSSGLYSLSSVVTVPSSSLGTQTYICNVNHKPSNTKVDKKVEPKSCGGGGSGGGGSGGGGSGGGGSQVQLVQSGAEVKKPGASVKVSCKASGYTFAGFEMHWVRQAPGQGLEWMGAIDPKTGGTDYNQKFKDRVTMTRDTSISTAYMELSRLRSDDTAVYYCARDLGYFDVWGQGTLVTVSSGGGGSDKTHTCPPCPAPEAAGPSVFLFPPKPKDTLMISRTPEVTCVVVDVSHEDPEVKFNWYVDGVEVHNAKTKPREEQYNSTYRVVSVLTVLHQDWLNGKEYKCKVSNKALPAPIEKTISKAKGQPREPQVYTLPPSREEMTKNQVSLWCLVKGFYPSDIAVEWESNGQPENNYKTTPPVLDSDGSFFLYSKLTVDKSRWQQGNVFSCSVMHEALHNHYTQKSLSLSPGGGGGSGGGGSGGGGSGGGGSEVQLVESGGGLVQPGGSLRLSCAASGFTFTNYGLHWVRQAPGKGLEWVSSISPSGGVTYYRDSVKGRFTISRDNSKNTLYLQMNSLRAEDTAVYYCAKPFLGWGGANWIAHWGQGTLVTVSS

SEQ ID NO: 509 - protein, 731 aa, synthetic construct
QVTLKESGPALVKPTQTLTLTCTFSGFSLSTSGTCVSWIRQPPGKALEWLATICWEDSKGYNPSLKSRLTISKDTSKNQAVLTMTNMDPVDTATYYCARREDSGYFWFPYWGQGTLVTVSSASTKGPSVFPLAPSSKSTSGGTAALGCLVKDYFPEPVTVSWNSGALTSGVHTFPAVLQSSGLYSLSSVVTVPSSSLGTQTYICNVNHKPSNTKVDKKVEPKSCGGGGSGGGGSGGGGSGGGGSQVQLVQSGAEVKKPGASVKVSCKASGYTFAGFEMHWVRQAPGQGLEWMGAIDPKTGGTDYNQKFKDRVTMTRDTSISTAYMELSRLRSDDTAVYYCARDLGYFDVWGQGTLVTVSSGGGGSDKTHTCPPCPAPEAAGPSVFLFPPKPKDTLMISRTPEVTCVVVDVSHEDPEVKFNWYVDGVEVHNAKTKPREEQYNSTYRVVSVLTVLHQDWLNGKEYKCKVSNKALPAPIEKTISKAKGQPREPQVYTLPPSREEMTKNQVSLWCLVKGFYPSDIAVEWESNGQPENNYKTTPPVLDSDGSFFLYSKLTVDKSRWQQGNVFSCSVMHEALHNHYTQKSLSLSPGGGGGSGGGGSGGGGSGGGGSQVQLQESGPGLVKPSETLSLTCTVSGFSLTSYNVHWIRQPPGKGLEWIGVIWSGVRTDYNSVLKPRVTISVDTSKNQFSLKLSSVTAADTAVYYCARGTYDDNYHDVMDAWGQGTLVTVSS

SEQ ID NO: 510 - protein, 741 aa, synthetic construct
QVTLKESGPALVKPTQTLTLTCTFSGFSLSTSGTCVSWIRQPPGKALEWLATICWEDSKGYNPSLKSRLTISKDTSKNQAVLTMTNMDPVDTATYYCARREDSGYFWFPYWGQGTLVTVSSASTKGPSVFPLAPSSKSTSGGTAALGCLVKDYFPEPVTVSWNSGALTSGVHTFPAVLQSSGLYSLSSVVTVPSSSLGTQTYICNVNHKPSNTKVDKKVEPKSCGGGGSGGGGSGGGGSGGGGSQVQLVQSGAEVKKPGASVKVSCKASGYTFTGYYMHWVRQAPGQGLEWMGWINPDSGGTNYAQKFQGRVTMTRDTSISTAYMELNRLRSDDTAVYYCARDQPLGYCTNGVCSYFDYWGQGTLVTVSSGGGGSDKTHTCPPCPAPEAAGPSVFLFPPKPKDTLMISRTPEVTCVVVDVSHEDPEVKFNWYVDGVEVHNAKTKPREEQYNSTYRVVSVLTVLHQDWLNGKEYKCKVSNKALPAPIEKTISKAKGQPREPQVYTLPPSREEMTKNQVSLWCLVKGFYPSDIAVEWESNGQPENNYKTTPPVLDSDGSFFLYSKLTVDKSRWQQGNVFSCSVMHEALHNHYTQKSLSLSPGGGGGSGGGGSGGGGSGGGGSQVQLQESGPGLVKPSETLSLTCTVSGFSLTSYNVHWIRQPPGKGLEWIGVIWSGVRTDYNSVLKPRVTISVDTSKNQFSLKLSSVTAADTAVYYCARGTYDDNYHDVMDAWGQGTLVTVSS

SEQ ID NO: 511 - protein, 214 aa, synthetic construct
SYVLTQPPSVSVAPGQTARITCGGNNIGSKSVHWYQQPPGQAPVVVVYDDSDRPSGIPERFSGSNSGNTATLTISRVEAGDEAVYYCQVWDSSSDHVVFGGGTKLTVLGQPKAAPSVTLFPPSSEELQANKATLVCLISDFYPGAVTVAWKGDSSPVKAGVETTTPSKQSNNKYAASSYLSLTPEQWKSHRSYSCQVTHEGSTVEKTVAPTECS

SEQ ID NO: 512 - protein, 30 aa, synthetic construct
  MOD_RES 4..30: note = may be absent
GGSGGSGGSGGSGGSGGSGGSGGSGGSGGS

SEQ ID NO: 513 - protein, 40 aa, synthetic construct
  MOD_RES 5..40: note = may be absent
GGGSGGGSGGGSGGGSGGGSGGGSGGGSGGGSGGGSGGGS

SEQ ID NO: 514 - protein, 50 aa, synthetic construct
  MOD_RES 6..50: note = may be absent
GGGGSGGGGSGGGGSGGGGSGGGGSGGGGSGGGGSGGGGSGGGGSGGGGS

SEQ ID NO: 515 - protein, 60 aa, synthetic construct
  MOD_RES 7..60: note = may be absent
GGGGGSGGGGGSGGGGGSGGGGGSGGGGGSGGGGGSGGGGGSGGGGGSGGGGGSGGGGGS

SEQ ID NO: 516 - protein, 70 aa, synthetic construct
  MOD_RES 8..70: note = may be absent
GGGGGGSGGGGGGSGGGGGGSGGGGGGSGGGGGGSGGGGGGSGGGGGGSGGGGGGSGGGGGGSGGGGGGS